European Patent Specification EP 3 137 491 B1, published October 9, 2024. Title: Mantle Phenotype Detection in Palm. Applicant: Abdullah, Meilina Ong Eng, Ooi Siew Ti, Leslie Low Eng Singh, Rajinder Nookiah, Rajanaidu Sambanthamurthi, Ravigadevi Jiang, Nan Smith, Steven W. Lakey, Nathan D. Martienssen, Rob Ordway, Jared Hogan, Michael Malaysian Palm Oil Board. The sequence listing filed with the application follows.

SEQUENCE LISTING (161 sequences)

SEQ ID NO: 1 - DNA, 78321 bp, Elaeis guineensis
  misc_feature (14421)..(15355): n is a, c, g, or t
  misc_feature (55950)..(57363): n is a, c, g, or t
  misc_feature (64044)..(65002): n is a, c, g, or t
aatctattagtatctgacaaaagttaaattagagtcgaaacactaaatgacaattagggatcaacttgatcaagtagatagagaatattagaaaagagagaaattaacaagatagaacatgattaattaggtgacatagcccgacaatccaattggtctaagcaagttgatttaatcaaatcacggttgaactaatatatagatagctcaataaaaatcatacataattgaatctaatgatatttggatctgaccaagatggaatttgacatgctgtccgatgatcgtgaatcaagactctctttgctaattaagatcaaattagaatcattgaaagagaatcttttactggatcaagagagagaaatatataaagagagtgaaatagtctatagaaaaaaaatttagagagagaaattaagaagaaaaaataaatttttttagagaaagaaagtgggtatacaagctcagagaagggagagaggaaagagagagaaatgctctcttattttcttttttttcttttttcttcttttcttttttttttccattcttctttcccttttctgcttaatggaataggggacctcccattccccttctatttctagagttgggggctcaaaattgatgatagctatcattggggatgtaggctatggtgatgcagtagaggatcaccgaccgatgatcgatggtgatgttgcaatcaaaaaatcaagaaagatagatggaaaataaaggaaaataaggagaaatagatctcaacttgtttggatgctaacccactcactgacgactccacttcaactatggccggagcttgctatggaaaagaagccaaggccttcaaggatgaacaccaatggtgaggaagatggtcgaaaatagaagaatggctggcttttctaatcgacaaaatagggtatcgcccttcttagcaaatattcggcaataaatatctagaatccaggatcctaggactatggaagagggagaggagggcaagtcaaaggatgccagattcttatctagcttccgacaatgatggggccctattttcgataaacacaatcgaggatgttcggaaaagggttttttcgatgatgattctagtgaccaactatgagatttcaaagggggtgaggggggtttaaataagatgggagggaagtttgaatcctccttaaatctgaacctttttcgacaaagccaagagcgtgaaggagactccttcgtgaagtcaaagatggaatagactcccttcgggagtttggttcatcacccaacttccctagcatgtgcggagtatgtgctagccttttctctcttttttttttcattttttttcatcctttaagatccatgcagtttctaggttgagggattggggtatcacattctctctcctaaaaaaaaattattttcaaaatttttttacctatattttcaaaagttgggattcatggtccaaatctcatccttgaatttttttgatattctaattctcgaaaaaatttcatcgttaaatcatttcataagagaaaagtcaatacctcaagagttgatctgaatcaaaattattatctctagtaatcgaaatcaatatcttaatttcaaataagaatatccagtttattgtcaaaattattaactactcttgacttaattgatctattacataatcgtaaataaattctaacatactcttgaagtgtagaatataagattgataaacaatcctatatccgttctaatagatataaaagcataaactttaaatattttaaatccaagattaagaatcaatgatccacttatcctagactcaagatattagaaatttttttttgtacaatagatagaggatgtactggtgaaaatcatgtagcgatatccaaaataatttttaattaaaaatattatccttttcattatcaatgaattttatctataagaaagatcaaatcatatgatccatcttaaatttttaactcaaaaaattaatattgcaaactagctcaaaataattttgatcactacatttctgctgtgcattctaatttaaaccgttcacattttttagattcatgaaataattttgaccaaagtattactccatactatagtcaaaaaagattaaaatattagattctaattaaagccaaagataaacttttgattctcatccttaattttgcctaaagtataattattttgattaacccttaagcgcaataacacattcaaaaccaacagataggtttactataatccaaatgaattaaatcttaattcttttatcaattcatttagacaatttcaaatcaaaattctataagtaatatcaataaaaaaaaattttgatgctccaataagttagaacttaaatcaaaatatataagtaaaattgatttaatcatctcttctaaagtttcttctattaagatctttaatatctatcaaatacattccacaataatcatgcaaaccttttaaaaattaaattctcaatgcctttactacattttaacaccaagctcgataatagtgataaagaaacatctagatcagctttataatcaaaaattttgacttacaattttacgtgtgtctcaaaatcttgaataaatataaataagatcttttatcttgatccaaaaatagtaatcaaggatttcattagtaacttcaacaacaatggtaaaaaaattttctatccattgataaacccaaattttgaattgaagtttcatgcataccatatagcctttaataagatctattatttggatctaaagatagtaattaaaattgttaatgattccactaagatgaatactttacaatctcataattaatttcttcaataaaaatagacttcttgataatgtctccaattgtatatttttttttatttctacaagaaaacttcatacattttttacgttccaatataaatcttaaaaagttattccaatcaaatatcataaaagatcttcttagtccaaccttaaataacttttatgaatgaatctttatcttgccactaaataatgaattttaaaatcaagagcaacatcacagcattctgtcatgtcaaatttgtgttagatgtatgtcctagaaatcaattagattgacaatgtaaattttttaaggatataatttatatattttgatttattaataaaataaaatttaaattaatttttattcatatttttttatctatgaatcatctaaagaattaataagatgatgatacatattcttaagagttcaaaatttgaaatatatgtcattgatgattaatttctgaatacttttgaattcttaagagtttagaagatcttgacccaagtagtgtgaatagtgaaaaaaagttttcacatacttcacatcaaaaatttaagttgaataaattgtacatatgacaggtattatagtttgacgagtaatctataacctctatcttatcaaaattctgatagaaagattgtattgtatgataactgtacttagaggttcaccttttattttactggattaccactacatgttgctagatgtcactggtggattgtgagatctacgaagattatcttgatgatcgataattctcattgaaaagattgaaactattttaatgatgttgtgatagagatcataatatatcttattatcagacagaatagaattctatgggatcatacacaataggagattaagactgatcaaatagttgaatgatgattaagaatcattacggagttcagattatcaatataattgataattagactaacttataattgttacaagtagcaaggacttaactgctaaaggttaataggttcaaaaagaacttatgtataaatgttgtgcatcttaatttgattggatcaaattagttatggctgaattcaagatgaatcaaataggaatttggttcaattgaatttgggtcaagctttaggcttaggtcacatatacccaaaatcatttggatgcatcaggtgtgtgacacctgaatcaggcctttctaaactattttgagtaagtttgatcaagtcaaaaggatccacaccctaaggtttcttgaataaaaccttaggcaccacattgaggacctataggaaactttgaccctctctcatatggggtggcacactgaggttttataaaaaccttaggcacccattttagccataaaaaaaaagctccaagggatggggcagtagccatgaagaatccttggctgtcaggactctattcaaaagagttctcaaggttttggactcttatggagccctaggatttgtttgcctataaatagatggccaccccaaggctttagataatgttagagacttgtgaagctctcccctttctcttggttgccggcccaccctctctcctctctcttccatgccccaagacttctttcttgtctccatcatcttgctgaaatttagatttcagcaagaaaagtcaagtagaagtcaaagttctaatgtagctcacaagatgttgagaacttcctccatctggcaaaggttctgcaagagagctagcatcctgagaaacaaaaagattgctgatcagccctcatctccatatggatatttgtagagatcagatgcatgcatagctagaagagaatcttatcacgatcatcactcgtgaagatcatctacctgtgcaaaggtatgagataagaaaaatattttttttatcataattcatgaatcctttgcttatattatactgagattcttggaatggattttttctctagtaaaactctagagatcagatctcgaagtcttcttcatataaaggttttgaaagttctttatattttcgctgctttgattcaaaataaattagatctattttgcctttcaacctttctcatatttattgacatataaagctttaattaatgagattaatgaaaagcatgtgcgaaatactgagaaaatcctaacagtgatatcagagctacttttgtacataagaaaaggattcaagttaaataaaatctgtttgatttaagtaaatgaatcaatcaaaatttatcctaacataagtttgtcctggtataatggtcaagaccattatgttgaaaggttatcctaggacaaaaagtctaagtaaaatctattttatttaagtaaatgaatcaattaaagtttattctaatataagattgccttagcataatggtgaagacccttatgttgaaaggttgtcctaggatggaaagtgattgatgagacaaatatatcatgaaagtatttttcacagatggaataaaatatatatattttgtttgtgaaaatgagatttcatgaatgtgtttgtcattcaatatgtgtggtgatcatcttgaattgccacaaatcctttttggattagggttgtatcatgactcacaaatcctgatggtttgcaaaattttgcattctgtagtgatagaaaccaaaagttaatccagttttggaataagattgatcaattggtatctaaggcaagtattttataatggtggttacttaattagttataaaagtacgaagagtctcctaccaatcttacacttatctagccaatttggttgattgaattctgaatttgggttgcttaagtgttaagttcactacaaatatattgcaaccatgattccgacttagtcaaccaagcctagatctcttgaatagattcatgttaattatggatttacataggatataaataaataattaaaacttgaagagatctaaatgaaaccttctcgtacatattaaatcgaatgatcttccatcattgtagatatacggatactctactgatgttgatgattttcgactagatatagtactttggttgcatcgaaaaagtacaaccactttataacatgagatgttgcagggtagagatggggttgggcccaataattgttaggtgaggatccaaatgatggctgcacttgcgtgtgaatggcgagtctgacttaattaagaaatagagctaataactattagatgaggcttcaggacttagagacttatgaccactacaacttacttgagaagcaatggataaagagtcgtctatttatcaactgacgcatcaccaataactatcagatggagtgatgtataattagtgggactatagtatccacttgaaatcttaatcgtaaaaatttttgtttctccacctgaagagcatgggagattcgaaaaaatagtgggggtagtttatttttaaaataaagctcctaaaataaactaaaataagttaaatacaaagtctaactagaatcttcttctctctgtagaaaatatctgcttccaacctctatttcatatccttaagactaattgtttgactagacccagttataaagattgactctaaaacttaaagatagtcttgagttttgaaaagatgagctatgtcctggatcaagatatcctctctctaccagcttgtcccacccctaatcaaggggcatcctatgaaaagtggttaaacgatgataacaaggcttggtgctgtgtgctgacatctatgtccattgaactccaatgccagcataagggtacaaactgtccaaggtatattgactcatctacaagagttatatagtgagtagagccatgtatctcactaggaagtatttaagagactcttcaagatgaagaagtatgatggatagtctgttaatgatcattgtctgataatgatcaagaacttgaaagaacttgagaagctcgatatgtctatcaataagaaattgcagattgatttgatcctacaattccttactgattcatatgtgtagtttattataaactaccatatgaataaaatacagtgcaccaaggttgagttgttaaatatactgataactactgaagggacctcgaagagttcaagaggcactgttcttattatggagcagacctcatctttcaagaaaaagtctactgaaaagaagaaaaagtttgtgaagaagcagaagttagagaataggccaaagaaagaagttttcaagaagaaggccacaaaaaaggaaaagtattttcactgcaactctgatgaccattggaagagaaactattctgattatgtggcaagcttgaagaacaaaaaagatagcataccttctgaagatatgtctgatcttctcgttattgaaactaatcttacaatttcttttactttcagttaggttatagactctagctctagtgctcatctatgcacttctatacaggatctggaggaaagtagaaggctgaggaaagaagaaataatccaacaagttgaaaatgatgcaagagttgttactatggctgtggagatctatcctctacgactaccatctgatcttagtttaattcttagagactgttattttatacctactgctagcaaaaaattgatctctatttcatctctagcataggataattatgtattaaattttaataaagattattataccatttatttgaaaaataaaatggttggacgtaattttttaattgacagtctctatcatttacatgttgatgtatctatgaatgtaaccaagcagaaagtgaatgccataggatctaaaagatctaaagatgaaataaattatatgtggcacattaggctagatcatataagagaagaaaggattaacagattggagaaagatgggctcttgggcttattgactactgagttatatccgatctgtgaattctgccttcaagaaaaaatgatcaagctgccctttatgaaacaaggagaaaagaccattaagatatttgccctggtacatattgatatatgtggcccattaattcgatgcgctggtcaaagaaggttgtctctatttcatcatctttatcgataattattcacagtatggatatgtgtatcttatgagatacaaatatgaagtctttgaaaaatttaaaaaatttagaaatgaagtaaaaaaataaactaaaatttttttaaagatttttcaatcagattgaaaagttgaataccttaatggagaatttctaaattatctcaaaaaaaatagcatagtcttataatggactccatttggaatgtcttaactcaatagagtttcgaaatagagaaatcaaactttattagatatggttcggtccatgattagtttcattgaccttctcttatttctttggagatatagtttacttaccactaattatctattgaatagggtttcctctaaaatcatttctaccacattgtatgagatatggtattgtagaaaatcaagtcttgatcatatcaagatttaaggatatccgacccatatcaaaatatttcagacggacaagttagaggtcagatctatgaaagctcggttcaaaagtatcttaaggagtctttaggatattatttctacttttcagaggatcacaatatgattataagccaacatgctctcttccttaaaaaatagttcatgcaagatggaagtagtaggaggcagattgagcttgaagagagtctctgaagagcaatgagtctcagaacttacgtaaaacctatttaagttgagccaatacacacacctcttcctccatctcgtagatccagtaaaatttttcattctcctgagagatacttaggtatcatcatagagaatgtagagaaaatatttctcgtgaaaaatgagacatatgaaaatgaccccaaaacctatagcgaggcaatatcaaatatcgactataagaaatggttagaggctatgaagttagaaattaactcaatacacttaaaccaagtctgaacctttatggatccgtcagaaggtatggtacctattatgtataaatagatctacaaaagaaagattggttttgatggaaaggtagagacctttaaggtaaagcctgtgactaaaggttatagctgacacgaaagcattgactatcaatatattttttcactagtagttatgctaagtccatttgaacattacttgcgattgcagcatattatgattataagatatgacagatagatgtgaaaactatttttctaaatgaatatctttaggaagttatctatatagagtagactttgtgtttcacttccagtgatggcgatcacaaagtttacaaattgtaaagatctatttatgcactcaaacaagcatcttggagctggaatacttatttcaatgatgtaatcaaatcatttagtttcatcaaaaatgagaaagaatcgtgtgtgtttaagaaaatcagtgggagtactgttacttttcttgtattgtacgtggatgacatcctcctgatcgaaaatgatatttttatgttaattttagtcaaaatatagttgtctaagaaattctccatgaaggatcttggggaagcatcctatattttggagataaatgtctatagtgataaatctatgaggatgccaggcctttcacagaagatgtacattaaggaagtgctgaagaagttcagcatgaaaaactccaagtggagacttctatccttcaggtatgggattcatctctccaagaaggtgtgcctcaacacatcttaagagatacagtacatgagcaaaatcccttatactgcggctataggaagtctcatgtatgtcatgttatgtacatgacctgatatagcttatgttgtgagtgtcacaagtagatatcagttgaatgcaggtgaaaaacactggacatctatgaaatgtatccttaagtacttgagaaggattaaggatatgttcttgatctttagaggaggagaattaagggtgcaagaatataccgacttaaattttatgtttgatattgatgatcgaaaattgacatcagattatatttttttatgcaacggtggtactgtgagttagaaaagtttcaagttgcctatcatagcagactccattatagaagatgagtttataatcacattggaagctaccaaagaggcattctggtttaaaaaatttattacagagctggatataatgccatcagatgtcataccactctactgcgacaacaatagtgccataactctagctaaggagctgaggtctcaccaaaagtctaagcacatagagcaatgatttaatctcattcgcaattatctcgaaaaaaatatatcaaggtatagaaagtagatactatggataatatgacagacccactaactaagtagctgagtcaataaaaaatcgaagtccatcttgagaagatgggacttagatttgtggccaattgattttagtgcaaataggagattgttagatgtatactctaaaagtcaattagactgacaaatataaattttctaaggacataatttatatattttgacttattaataaaataaaatttggattaattttttattcatattttagtatccatgaattatccaagagattaatatgataatgatatatattctcaagagttgaaaatttgaaacatacgtcattgatgattaatttttgaatgctttcgattaatggatgatcataaggatagtaattaatccgatcaatgtacaaatcacttcttttttgatagacgagtctcgagtctatactatggagacactggagcaagagtgcaggtatttgttagagaacaaaggtatcgagcgtgactaatacgagaagtcaattggatggctatccactcgttaatgacttatttgatactacagtagtatgtctagtccttagatctgcaatgcctcaggtgttcataatgagactgttagagtttgactgtacataaacttgatttctagccatatggatctttatagtgcatgttggctacagtaggttcgttgtaggaataggatgtgcacatagatagaatctatcatccttgatagacaaaaaaaatgatcctatataatttatgagactgagttcaaaaaatcttgactaagacagtgtgaataatgaaaagaagtttccacatatatacttcacatcagcaattccagttaaataaatcctacatataataggtattgtagtttgatgaataatctataacctccatcttattgaaactctgatagaaggactgtatcatatggtaactgtatcaagagattcatctactattttgctgaattgtcactacaaactgctagatgtcactgatagattgtgggacctatgaagattatcttgatgatcgatgattctcatggagaagattgaaactatttcaatgatgttgtggtagaaatcacaatatatcttactactagatagaatagaacctatgaggtcacacataataaaaatttgagattgatcagattgttgaatgatgattaagaattgttacaggattcagattatcaatataattgataattggactaacttgtaattattataagtagcaaagatttaattgctaaaggttagcagattcaaggaggacttatgtgtaaataatgtacatcttaatttgattggatcaacttagttatggctaaatttaagatgaatcaaacagggatttagtttaatcgaatttgggtcaagctttgggcttaggtcacatgcactcaaaagggtttggatgcatcaagtgtgtgacacccaaaccaagcctccctaaactattttgagttggttttgaccaagtcaaaagggtccacaccctagggtttcttgaataaaaccctaggtgccacattgaggaccaattaggaaactttgacattctttcacacggagcagcacactagggtttcatgaaaaccctaggcacccattttagccataaaaggaaagctccaagggatgggatggtgccatgaagaatccctggccattgggactccattcaaaagttctctaggttttgggctcttatagagccctagggtttgtttgcctataaataggtcgctaccccaaggctttagataatgctagaggcttgtgaagctctctcctttctcttgtttgccatcccaccttctctcctctctcctccatgcctcaagacttctttcttctctccatcatcttgttgaaatttagatttcaatgagaaggatcaagtagagtcagagttctactgcagttctcaaggtgttgagaactttcttcatcaggcaaagattctgcaaaggagttagcacctcaaagaaccaagaaagttgctaatctgccctcatctccatgtggatacttatagaggccaagcatgacgagaagagccttatcacgatcatcactcgtggagatcatctacccgcgcaaaggtatgagataagaaaaaaatatttttcttatcatgattcatgaatcctttgcttatgttacattgagactcttggattagattttttctctaataaaatttcaaagattagatctcgaagtcttcttcacctaaaggtattgaaagttctttatattttcgctactttgattcaaaatagattagatttgttttgcctttcaatttttctcatatttattgagatatgaagctttaattaatgagattaataaaaagcatatgtgaaatactgagaacatcctaacaatttgagcttacaattcacttaaacaactaatgatcaaattaataatcacaatgcacaataaaaattcatgataaatctttttgttgttactttagatcaaaatccaactaatcataacatgatccacggattgcctatcatatatcaaaccctctgaattattaatcttaaacgatcttttcattcatgatcataagatttagttaaaaatcatgaagacaacttatattgtaatcatcatagatctgtatcttaacatccttagtgtttacctacctatactcatcctatgtttgattctatatatcataatttattcactaatactttgatatcatataaattatcgcatccccaatctaagatcatattggtactttaatatttcattagtgggggttatgcattagtactttgataccttatcagttgaatggttaaacactggtactttgatatcctatcagtggaggttatacgctggtactttaatatcctatcagtaagatggttaaatactgatactttgataacctcccagtgggtgttgtatgctagtactttattatcctaccaatggggcagttaaatgctactactttgatacgctaccaatgggatagttaaacgctagtaatctaatcttagcttgacataaagtaacgtcgactcgagtttagggtcgactcgagagaatgttagggttagcttgatatgaaagagggtcgctcgtcaatattttggagtcaactcttgtttatggatgatctagaaagtgtcagagtgagctcgagtactgcatatttctgatacattgtctatgctagaatgtgctagaactgattatcttctttatcaaagttgatttttgagtaacttgatgatcaatttttctaggctagacttgctttgtcaaaatgagcacttgttagtttagagaatcttcacctacacatgatctcaagcattcattagtaccaaaaatacttaagtattttgatatcatcaaaatcaattcttgggttaacacaatacttttcaaataataagcatacagatataatcctataacaatttaaattttgttcatatatcaatttctttaaaaatattatattcatcttgatagctatgaactaaatcaaaatacatactagtatacaacttttactgggagagtattagattaccagcatttaaccatcccactggcaaggtatcaaattaccaatacacaacccctatttataaagtatcaaagtaccagtgttcaactgcctcactggcaggatatcatagtactagtatttaactaccacattgacaggatatggaattatcagtatttaaccatcattagtagaattttgatgcatagtcaggctgcgagtcaaaatctatctcaaatcaaaatattgatcacatgtctaattctgtatcataattcattcccttatgctctaatattatattaattgtcatacttctagctcgagatcatgagccaaggattgcagtaactaccgcatacttatagagaactctttctataagcatacaagatattctaaatatactatcaatatatcatagagaaattaatttaaataactaaaagttaatattcaattaataaattcaactggcaaatgtatttaaaaattttacatcaaataaatcttgattaataaatattaattaataacaatagatttaaatcgaaacaaggttgatattgttagaatttgatgcctcaagattcagcccacattgagtccacagtgaggttcgcgacgaaaaatgnnnnnnnnnnnnnnnnnnnnnnnnnnnnnnnnnnnnnnnnnnnnnnnnnnnnnnnnnnnnnnnnnnnnnnnnnnnnnnnnnnnnnnnnnnnnnnnnnnnnnnnnnnnnnnnnnnnnnnnnnnnnnnnnnnnnnnnnnnnnnnnnnnnnnnnnnnnnnnnnnnnnnnnnnnnnnnnnnnnnnnnnnnnnnnnnnnnnnnnnnnnnnnnnnnnnnnnnnnnnnnnnnnnnnnnnnnnnnnnnnnnnnnnnnnnnnnnnnnnnnnnnnnnnnnnnnnnnnnnnnnnnnnnnnnnnnnnnnnnnnnnnnnnnnnnnnnnnnnnnnnnnnnnnnnnnnnnnnnnnnnnnnnnnnnnnnnnnnnnnnnnnnnnnnnnnnnnnnnnnnnnnnnnnnnnnnnnnnnnnnnnnnnnnnnnnnnnnnnnnnnnnnnnnnnnnnnnnnnnnnnnnnnnnnnnnnnnnnnnnnnnnnnnnnnnnnnnnnnnnnnnnnnnnnnnnnnnnnnnnnnnnnnnnnnnnnnnnnnnnnnnnnnnnnnnnnnnnnnnnnnnnnnnnnnnnnnnnnnnnnnnnnnnnnnnnnnnnnnnnnnnnnnnnnnnnnnnnnnnnnnnnnnnnnnnnnnnnnnnnnnnnnnnnnnnnnnnnnnnnnnnnnnnnnnnnnnnnnnnnnnnnnnnnnnnnnnnnnnnnnnnnnnnnnnnnnnnnnnnnnnnnnnnnnnnnnnnnnnnnnnnnnnnnnnnnnnnnnnnnnnnnnnnnnnnnnnnnnnnnnnnnnnnnnnnnnnnnnnnnnnnnnnnnnnnnnnnnnnnnnnnnnnnnnnnnnnnnnnnnnnnnnnnnnnnnnnnnnnnnnnnnnnnnnnnnnnnnnnnnnnnnnnnnnnnnnnnnnnnnnnnnnnnnnnnnnnnnnnnnnnnnnnnnnnnnnnnnnnnnnnnnnnnnnnnnnnnaagatattactaaattttgcttctaatctcactcttaaatagtacttacctttgaaactaggcatttgaatctgaaaaagaaagaggagattatgagcttgatagttcagtaaatcatgaataaattagctaaataaatctatgaataatagtatattaaaaataaatatgtaagatacaataattcaaaaatgaattcatatatataatactttccaaataataagtatgtggctgcaatcctttcgtaattcaaattttgttcattaattatttttttcaaaacatcacatggatagtcatgaactaaatcaaagtaccagtgcataacccctattgataaagaatcaaataacaagtgtttgactgcctcattatcaggatatcaaattattaatgcataacctccactgctagggtatcaaagtagcaacctcaatcacctcactggaagggcatctagtttcagtatttaactactccactggcaaggtgttaaattatcaatatttaacctccactgataggattttgatatatagtcagactgcgagccaaaattcatttcaaaccaaaatatttttctcaaagacatattttatgtttcacattgaaaaattcacaaaaattatgcgatattgaaatcaattggataaaatccacgtcaaatttagtatattcaatcataaatcatttactattctagaaaaggtatattaaaagtataatgcatcaatttcataaatcataaatatctcaatataaaaaatattttattatttattaataaatctaggagaagtgaagcattacttatcttgtaagtaaaactaaccaactgatcaaattaattctgagaatctttctcaaaactcatcaccactatatcaaaaacttgtgcttcttgctatgtaagagcatagaccctttcttcgatctggggttccaagtttctattttattttgttcaactatcaaattagactgacttttcatttttttgtggatattcagctattttatggcctttctaacaataaccaaagtatgtaccaatattccaacaataatcatttattgcatgattttcaccgcatcgaaatatttgatattatcaatcaatccaaacttgttattcactgacctcttattcaaacccttagtatatttaatattctacctttgtgattcattcaatcgatttctttttttttattttctttccctttctatatgctcttcattaacttttctttcaattatcaatgctttattcaatacatctgtataagtagttaactcatatagtaccatttattttctaatttctatcctcaattccaactcaaatttatctactcagtcacattcatcttcaaccaatctcgaagcaaacttgacaagctccataaatttagcttcatattctacaactattatatttctttatttcagataaataaatttttattctttctgaatcctcatactctaagaaaaatatttttatcataaaatatcttttgaaatcactcccaagcgagttgttctccatcttgttcatatttaggtttcattctctattatcaattaaatgtctcatctttcaacatgtatgatgcatataagattttttcatcatcatggtatctcttaacaataaatgctttctccatctccataagctaatttttagctcctatttcatagttttcttaaaagtcaatggagacaacttcttaaattctatgatattactttattgctcctattgctcttatgtccttgtggtgacaatatttattgttgcacttgctgtagaggcagttactgttactgcaattgctattacgattccatcaagccgactagtgtctgcattatttggataatagttgatttttgctactttatttagatgttggtggcaaaatcaatgacttctttttgctgagagatgccaccaacctactaagtatcatcatcttattggttgatacctttagcagcacctcgagtggttctttttatctgatatggaaccatcttaatcttgcatgaaaaacaaacttcgcaaaattttcttttaaaatctaatatctaatattatacttttattaaaatttaattatgattattttaagaataaaaaatttaaattttgaaatcctcacaaggctggccaagagataatgaccatcatcctagtcggtttgacgtaggacatccaaagatcaactataattcaagcatcatattgagatgctaggatataatcgatggtgaaatttaatgatgctcgactgatcaagatgggggccggcccgatggcctgttcaacaatcattgatcaaaattttttaaccaaggtctatcaagatcattaaaaagtctttctaagatctataaattgtaataaagagacacaatctagagagagacactttttacataaagaaagtagaaattttagggagagaaattagagagaaaggggaaagagagaggaagctgagaggaagaaagaaaagagaaagactctctctctttttcttttctttcttttctctcttttctttttcttttcttttttttcttccttttctttctttctttctttggctcattagaaaaataggggacctattgatccccttgtttcctaaataggggaggaatctcatcttggtagctatggccggcgatgtgagccaaagtggcaaaatcatgaatctcccaacctgcagccgacattgacttttggcactggaaaatcaaagaaatttgacaaaaaatgggaaaaaattgaaaccaaaatagggaccaaaatccggtaatagctagcaaaaatccttgatctttgctcatggaggataggaaaaaagattattcaagagattaagggaatcttatctcatttttttgctgtgcttaggccatggtggttgcagaaatcgtttgtgaaagctcgacaaactctgcaatttcttcgggcttgggcctcgatctttaataggagaagagagaagtcctctttcttttaaatagagtcggagggaaggagtttgattccctccttatggtggtttcaaactctgatcggaagtccattggaaaagaagactcccattagttttaaaatctaataagatttattgattagaaaattgataaaaaatgattattaaaaaagtagcataattatttaaatcaatgatgcttagattgttggaggtaaatagtaataaaatcaaaaaattaaaattcatgggaccaaaaaataatgaacaagatttgaaagaaatgtctataaataagaatttatgaaacaggggaacattgatcaaaggtgtgttaaatagtgtccttaaagtgttattgtccctctcacgtagactttgtgtgttgggagagaacatagtaattctctcaacctatgcaacctaaatcttttgaaaagaaatttaaaattatagaaaaattggcaaactagaattttggtcattttctttattagtaaaaaatatactaagttatatgtctttatttatactagtgaggtctatctttgcacaattcagaccaaatttatattctagttaaaagaggtatagattttttaaaatagatataactagtggaaatagtcatagaaaagttaaaaatcaatgaaaggtagatttcacttctatattggctttatttgtggtcactttatctaattcttttttttgatggagcaatataccctgttaaaatcttctcgatttttttttcactttaagcaacctatttcgatgcctaaacaatggaatttagtttaaccacttaatatgctacacttttaaaaggagcaccatattgtagggcttgaaaagttacttgatttaaaaaaagagcatcttaattggacatcatacaagtaagttatgacctccgaaaatttgatacatgatttatcatcttgatatggtaaatcttgttaagatttcctcatggtgtctaaagtggccggttcatactgagtttggtgattcttctggtcaatggttaattgctcgaatatttttaagatataactaatctccaactctgccgactccttagtagtatgagcacatggaaagcttgacctaattgatttcttaaattgcttgaaatcagtacttagaaaatatgcaaaatggatgaaatgtttattgcagcgagagctttctgatctgtacgaccgagagcttactagttttttatgagctatacgttttgcacttaagcctaatttaaatagtgaaatagttttgcaacaattcaaaacaattaaaatcaaaagacaagctgctatgcatgttcaactgactcggctttcaatcgcaatatgtcacataggctggcctagaatgcagatgcgtgcgtggtgagcatcctaaaaacctacatatccaataaattcccactagttggtgaagtattaaatgtaactcgtattaactttttaatgtaggactaaagtttattcgactaattaagaactaaatactttaataattgaacttttccaaccagaaatcagaaaatatttaagtaattaaatattacataataactagatcaaaatatcatggttcctctctcgctcgagatcaattgggatgttggtttatcttggtcatccatcgagatgactctatcttagcctttcaaaacggcgcggtaccacgggtctcaccgcttcgttacatcgaatgccaccatcccttttttttttttttttttatttatttatgctttcttgctcctagattggtgcggcctcattacaactccactgctacttgatgcttccctctagcatctcctttgcagctctctcacttccaccactcttcggcctaatgttgggaaacgacgaaggggccttacaaaaatgtcatccatgatggcagtggagaagaaaacatcgctggggctttccttcgatatccttcgcagccaaagctcttatagggttatatgggagaacgctgcattatttgggtgatctttttggatggtgttgttgactgatgctagttttgcttcatgaattgaatatttacacaagatgagaatacaatctagtacaattggtaccaattacctgggtttgactcctgctcgcatctgattgaagcttggttaatgtgcatctcaattaattcagaaagatcatcggacttcatgtgaattattttgactagcatgaatagggctaaataaggctgaaatatgtgttaaatttttaaaattataacttgatcatatgatgtccaattgagatgttttcaaatcaaaatttttttcgagatttatcacttaatgttaaactcttagaaggtcgaaacagactgaaagttttcttttcaagatgtattttgaccgagtatataacttgatgatcatatgatgcccaattgagatgttttcaaatgaaaattttttttgagatttatgacttaatgttaaactcttaaaaggtcgaaacagactgaaagttttcttttcaagatgtattttgaccaaatatatctcataatctataaagaatatatttcataatctatgaataattagatagagcgacagaagataatgctaatgtaaaaatcacgatctattttttataaaatttaatatttttatataatcacttttactatagtcatatttatttttaaaaatttagttatatttaaaatatcaaaaaaatttgacttgaattatataagaaaggatcttcctactattatagatagaagctttatatcatagtttacagtgtatggatcatcaatgaaagaaagagggatgtaaaccttacttttgaaatttttctatttgtttctaaattttttaaaggatccaagttgagaattgagagaattctttctttctgcaaatcaaatcattagtataatccacatggagacgttgtaatagaaagtagaaactatattttatgaataatagaaagggagttgatttacgccaagccttttgtttgcttgattaattatttatttttatggtgttagctggaccccatgaatagcaaccatcgttgggtcagggtcgtgtatttgttttggggtcttcattaatatacacggtggtaaattgttgggggcgcgtcagatggaaccaatcctggttccttacggtactgtagtgctctatatgtggacggctgtcattctatccgtgaaataagaggtgttgtttttctttaaaaagcagcactctcctcagcaaaaacctcagaatccaccatgtaatattactcatccttggtcttaaagctgtagcaatacattacttccaaatgccaagcaattaaataaactacatacatcgaacctctttagtacgtacgtcttttcaaaaatatttttttcgaagatccgacaaatgtgaaatgcttattaacttctttaatgtctgtttttgcttgcatatttacacagacataccatcaactccatcagttgttgtttgataattcgcttgccgagcagagaagagagagagcaagagagaaaggaggcatagagagcgtgagatgggaaaagcgaccgattcttaaactggcgagacatcacacgttacccggtacacccaaagctttcacgaatttggaaagtgaagccattatggaagcgctagctttttgctctcccttgccggaatggaaaggcccccgaccttctttacccctttctccacgccacccacccaccactcttctatacacctttatagctcccttctcctttggctttcttttaagcagagctcagaggaaaagagaccttcctgggtgcttgagaaatagagaagagagaaaagagagttggagatggggagggggaagatagagatcaagaagatagagaatcctacaaacaggcaggtgacctactccaagaggaggacggggatcatgaagaaggctaaggaactgacggtgctttgcgatgctgaggtctcgcttatcatgttctccagcaccggcaagttctccgagtattgcagccccctttccgagtgtgtacacgatattatccctcctcgtcccccttttttttttttttgataaaaatgaaactcatatagtcttcttttatgattatgtgtttgtaatgatggatgattgatggctggatggcagcaccaagaccatatttgatcgctaccagcaggtgtcagggatcaacctgtggagcgcccaatacgaggcagaaactcttcttcttcttcttctcctctctctctacaaatatgctttttttctaatttttcttttcaaagaaaaaagaaaaaaaatgatttctaatattgatgtattttcttgtgggagtagaaaatgcaaaacactttgaaccatctgagggagatcaaccagaacctccgcagagaaataaggtggagggccaaaagagaatattgtaatattagtactttctggtaaaaataagcatgtagtttctttttgcctttaaattttgttgtgctggttctgatgagcaggcagcggatgggtgaagatctcgacagtttgggcatccatgaactgcgcggtcttgagcaaaatttagatgaggctttgaaggttgttcgtcacagaaaagtaagatcccccatttattcactgcacctattttaattccttattctccatgttttgagagcttttgagataaatgatgagaagcgcatcgagatcgagttgtctatattctggaatgattaattttttaattctcaattaatgctgtttcattgctaaatattcagccatatattttgtctctgcatgggatttctatgctaaaattcctcagatttcagcatacagaatccatgagacttgccttggctttaccacaagtactccagaatcaaaattgtgaaagaaaaataggataaatctggttaagctgtaatttatttacttactttctatctatattaaaattattcagattattttgcaaatttatggatatgcttgaatcacgtatctgatactttctcttcatctggatggcagtaccatgtgatcaccacgcagacggatacctacaagaaaaaggcaaggctaacatgctttcttaccatcattctttacggtctttgatccggttttgcgtgtccacttcttacgtagtctttttcaaacattcctatctaagactgaaggtaatgatttgcaaaggaatagctttactgttttcctctaagtagatgaaatattactcacgtagaaaggagccatcataattgcagaaagaataaaactgaatggaatatgagtagaattgtcaaaatcttggtttaagggttttaatagccagatgagaaagcaacctacttttcttgaacaacttgtttgtgactgtcttgttgctcccatcttgcatctatgattagcaaaatatatgataaatagatattcagatttgatcgaaaagaaggaagattttctttaatccatttaatttgaatctcacaaaaaaaaagtagaagatttggacacgatcgctgggggcagcacgctcttaatagaatggtgtcacgttgcagatctcgaaaaattattcaattttttttaaaaaaaaaagagtcattgaaattagacgttgtatgaccatgttatgatctctgaaagtttgacttctgactcaacttcccaatatagcagattttactcctgaaccatgtttaacctcctgactcatagtggccaaagtatctacatcgagttcactggtcttcttggatcacattcataagaatacttcccataattttgctcaacgttgtttttctcatcaaccaaaggtatatgctttttaaaattgaaatgcccatgaatattatggcattcttttatttgacattttggttgatcctatattgtttgtttggcattcaacacttcttcatgggaacctttgaaatgaggtaggtgctaggatttttctttttacctatccatatcatatttccaatgtcttcttttacattaggttctttagtgacaataggggaaacgacccaatataatacccttgaaaatttgggcaatatctactaaaactaacttgaataaaatattaacataaaaagggatttagtaacataaaagcataactcaaaatcactcaccttgtgtgccacgttctcattgcccttattatttttgcattgtgaattgtgtcccccaataaagcaacgtgaatggtggaagagagttgaatggctttgttgagtaattgttttgagttactatagcattgctctactaaaattgaaatcttgctgtgaggctatgtatgagaagcaagttcatgctttttgactgttgggatggaagtatgagcaatctttttaatagaaaatggacgaatcatgaagtttttcctttttattgaaaaagatgatcgaaaaatatgtgcaagatagaaaaacactgaaaagataaaatgagaagtaaaagtggaagtctaggagaagaaaatttaagagaaatatcttcaatgagaggatgtgtgcaccaacaaagccaactttcactaaagaatgtaatgactcacctctactttcttcgaataaggggttccagttgtggaaagtatatagaatcttctgaaagactgagtaaatggagcaattccttctaagaaatattatggcatttctctcccacgaaatttcaaagcaaagagcagctagtagttgatcctctaatctcttaattgaagtttggaatttctcttgcctctatttggcccaaaggtcatgaagatctaccggccaacctcttaagttgaattagatcttaatagaagtccaaatgcttcttgtagaagaacatctaataaataaatgagtgatagattctaatccagagacaaagagcacacctcgaattcacttgccatccttttctagctagaacttctctagcatgaaacttgttccttaaggcaagccaaataaatactcacattttaggaatgactgccttccaaataattttataatatggacaaattagaccaccattattgataaacttgcaatgaacaattataaatgagttttcaggttggcacattagcaatataggatggtttgattattaaaaggatgatatgaagggtttcaaggtggtttgcctcgttcaaatcaaaggattttgaagattaatattccaagataaggttctccaactccattaggaaagtgtcttcatgtcatcttagagaagcagctcgtaccaaacttgacagatgttttatttatttagagtgacacagataccctttggcaatactctccatccttgtccgaacaacttctaatcacacctcacttatcttgcatctaactcagaggctacaagttacacctttcaacaaaccttttcggtttgaaaatttgtgatttcattatttagagttcgaagagcatatcaagtattggtcggagttggcacccaaagcaaacgaaacagttactgacatggtccaaaagctgagatttctaagatcccaacttaagcactgaataaagccattatgggaaatatcattttaacgaaagaggaatttagagtaagaattgattctcttgataccgaagaagaactaatacagctttcatcacttcaaaatgatgaacagatgcatctcaagtcagcactagaccatcttctaaaataggaagatctatggaagcaacactcccaaatgcagtggcttcaaaatggggattgcaatacgaagtttatccatgtttgggcaagtaacaggaaaaaaagaatactatcactgaactctagcaaggcgatcagaagattatcgaatagcagcaaatccaatccacattctacaactttttttctaccctactaggctcgactgaggaatgactcatccaagctgattagaagattctttatccagaaggacctctggatcttgctgacattgagtatccatttatggagaaagaaatccatgatacagtgtatgacttggctttggaaaagtcacccggatgatattttcccattctccttctatatgcacttctagtgtatcatcaaacatgacctgatgaacctactgtaaaatcagctaatgtagaccatctgaactacttgttcatcacccttatcccaaaaaaaaattggtgtgtattcagttagagacttcaggccaataagcctgattaatggagtaataaaaaatatttcaaaaactctatcgaaaaggctctcacagaaaatgaatttgttaattttatccacagagcttgctttcaacaaaggaagaaatatctctgaatattttgtaatgactatggaaactatacacttctgcaaagctgaagtacacaaggatctcaattataaagtcgacttcgagaaagcttttgacaatgtggattggagctttctattgaaattgctatccagcacggggctttgattcgaggtggtgtcaatggatagaatatctgatttatacagctaaattctcagtccttattaatggtgataaaggtaaactttttaaattgaggaaagatctcaggcaaggagatcctctattcgcctagctctttctcttagttgttgatatagaatgatcaagggagcaagtaggttcaatctttttgttggaattggatcatataatatcatgggataacttcaaagcttttagttcactgatgacacacttatattttgcagatatgatctaaaatacatcaaaactcttaaatttttactctatagttatgagctactgatgggtctcaaaattaactttgaaaaattccaattttttggcttgagaattgcaaagatgtcagtacagcaagttgcatctatcctagaaagcaaggtggctacattttccattacttatttgggtctcccactccatcattctaaactgaggaaaacttattggaatccactccttgagaaggttcagaagaaattgatcgggtagaaaggtaaacttcttaacctctagggtaggcttatactaactaatgcagtgcttacagggatcccactactctggagggatacattccttctccctcaattcattatcaaataaattgataaaatccatcgatcattcatttggagaggaaacgaggagtataactaagggcactctagaatatgttggtcgaatatttgtcgatcaaaaaaatttggaggactgggggttcctcaatctaaaaattttcaatacaattcttctttgtaaatggtggtggaagctctactctaatgctggtgacccgtggtgtagttttattgccactatccacccaacttcacactagagatctaaaggtatacacaaatcaacctcttcattttggaatggtttacagcacacatgaaatatttctactcctaatccactttcaagttagcaactagtattattttggaaagatagttggttacataatcatccactgaaggatcgatttcctcacctttacacaatagcattgaagtgcaacaactcagtggcaaaggtattaagcaatctacttgataatagctcttttagtactcctcttcctcaaagataccaagaagattttcagagtctataggaaagcattgaacaaattacattaacggaacgacctgatactatacaatggaaatggtttagtagcaatatttttttggcatgaaggatctactattttctgcaagatggaggagtttggcctctactgagtaatattatataaaaactcctaataccaaagaaagccaagttatttgcttggctaagtgctcacaacaaaatcccaatgaaagctaatcttcttaatagaggaataattggaactgattactgtacactttgcgatgacttatcagaaactaatgatcatctaatgctcatctatactttttcaaaagcaatttggaatcaagtactttcagacctgcaattgtcgaaacttttatgcatgcttaacaccctatgggatacttggagactcatcaatatgcaacacgatagaagacctaaactagctgctctattcgtaattggtcaatggtgtctttggaaggaaagaaataaaagattattcgacttctatactttttatccacgatcgattgctgaaactgtgtcactttttctttcttgggcatcacacctaacaacggagcaactaaagatgttagctcctgttcgagaagttctcttatctaagaatgaaaacacacaatctttagtgagaattacagatgctaacaggcgcagatgaatgttttatgagcatttttatagctgcagcttatatgtgatctatggtgcaaggagttaattataaccatggatattagttaggttgactatcagaaatcatctccaatacattctatgtaaccactgatcaattccatgttcaactagataggaacctgcctatatacaggtatgtccctgatgtaactatagtatactattattcataaataaataacgaaggttttaccttcttctcataaaaaaaaagtatcttcatgtcatcctatatgtcatgcatctcctttgctacttcttttatttacttcttaaacttggttctaccatatattatcagccccttttaaatttgcttttggatattgcatattccactcttcaatcacctcatgccaagcaaaacatttattcacacttgaaaaccaatataagaataccaaagaatttatccatgaaattctagaaactttggttttactcctttctccatcattcaaaaaggttcaaaatgatgataactctatatagcttatttatcaaatttacgaggttggtgttcaatgtttttgtgaaaaaaatatcttgctatccacatagtttgaatccatacttttgctatcttgagtttcaaaaattttaatttgctacaatttgttgctattagcatatgactacttttaagaagataagccaatatactattttcctaagaatttaaaaaatcaaaaataaaaatttttatttaagattttttaagggttgttttccaaatgtgcaatggggcttaatcttggcatcattttctaacttgtagaattttgacccaagtaacatttgtccaatcacttagaacttctataacttcgtacaatcatttgttaatgttgttcatctatttatctatattatctatctggaatatagttgctcttaattatttttatatatcgcctattatccaccctaagctttcatgttcatcctcatgttgttggaggtgcatgtcttattccaaactatttaccattgctgtagattttaaaaaatttgctagtttaggactttttaatcttttgatatcatgttgatgtaagctaaccctctaaggctagtcataatacattttaaggatttatgttatatgagaccaaaattttaacaaaatgaagtgttggaaattggtagaatggaagtgtaaagatgcttagagacatagaactagccctgggccatgtaaatcttccaaaagaagaagaaaataataaaattaagatcatattcaatctctacagaaaagttggtctttgttgtataataagccatcttaacatatgatggacaataaaatatataaacttatgagttttaatacttagatggaagaaaagggacagatatgtcacaccccatcctactagcatgagtaggcacatgatacacggttgcatgccctgcagagtttgactcatgaggcatgcaaggtattgaatagtagtctaggtaaaattaaaaaacttggagcattctaaaaataaatcaagttcattttataaaatcaatatttattatggactccatcaaatattatgcgcataacattttatttgcaaatagaagaagataagtcctagatcctaagtctcctactcttagtctcataattcatccaagctatccaccaaatatctaaaacgaaaaagaaaaacgatagtatgctaatagctttgtaagtcaccttttatctctaattagatcaagcatattagatataaaacaataattttcaaagtatatgatttgcaattaggaataaatatttgataaatacagaataaattttcataaagcatatttactaacattatttataaaatatataatgcttatatcaataaatcaatttctaaatcaatatatataaactatccattctgtcttagccttacaactattgctaccattccctgtagcatggttaggaagagactagctcttgaatactcatgtcatttatcaacatatgcgaatgatcattcgactaatatagtcaaaaaaaaattactctgatttatataaattaaaaattagtaaataatatatgctagtaatcaccttaccagctaagctctaaagaaaattagcttttgaatatacatcatgctattgattattatatgtcagtgcttgtctcattttgtggcatgcaagaagactagatcctaaacttatatgcatagtcagattaaagagcaaatgttgcatctgattatatgaacatctattatgatgtagagtttgtatcatgtatatttaatttaaacacaaatataattatacataaataatattcatattttaaattttaaatatttagataattattctagtgcaggtataaaaataagcaatataaaattttaaatcgatttatataacatgcataataaaaaaaattaaggatagaggtacttactgctcaactcataaaacataagaaatctctttaactaactttagtgcaacctagatagaacatattaatgattaagttttcatctaaaataaacatagatatcattttaaaatcttaggcatttaaatggtctcatgatttgtgaggctttcttcagattctacaattttgaaattttttcaaattataatttttttaccttgattgataacaaagccaataatacacctcaaatccaaatgtattcctaatagttttcaataaatctaatatcaataaatcataattaagatatcaatccattctatgaatttgaccataaatcctacttgtttctctgaccttcactataaattaatcatcaaactaaataagtgaggggatcataattcttttacgacaatccaagaattcaagtctagcatccacattagatggcttcctgtccagatatttgcgcctctccaaaattgagattatcagattaagaaaaataaaataagagagagggttaaaggacaatgccttctaggtagtgatgtccgacatcataattttgatcaaatctatggggcaaccaataatattagggaaagaggattggatttgagcaagaatagcaaagtcattgtcatcaatggcctgattcattgagttcaatgaaggattggtggttgagtggtggaggtggcatctaggaaggagagagaaagaaaaagatagagagaaagagataagaaaaatagagagaaggtggcagttaagatccctttttgtgattaatatatagcggtaagatactcaaagatctcaccttatcgacctcaaacactaagggaggtggaaggagggactactacccatgaagctagagaaagggatgatgatgattggaggaaggaagaaggaaaaatagtagactcgatgatgataagactaaaagaaaagggtttgacttagccacttggtatataatgaggtttggtatggagtcaatagcttgagtaatagcatggaaagagagaaggagctgaagagagtactaagtcttattagaataaagaaagatagaatcttagcgaaaaatagggcctcaaatctttcaggtagaggaaaaagagggatcaacgaatgaaagactaaggaaaaggtgtggagtaggatatactctcgattagtctctcaatcatggattctagtagggcttcgtcagctgctcaatcatggattctgatagctcaaatggtggtaagtagaaagagagagatctaaagagattgatagtggccttaaaaccagcacggtcaaggataggcatgccttagagagaggaaaagagagagagattaatggaaataagcgagaaaaatatattcttagagaatagattggcgataagaagaggaggtggttggggcatgcttaaagaaataaagaaaattgagtaggcggaaagtggtgatgcttggcgatgagaagatttgagagagagagcaaaaaaatgtggatgatggtcataggatagggaaaggaaagaacaaagaagggggtgctaagctaactctttctaccttcctcacaccctgaagcaaaggatttggccaaggatggacaaatgggcgagggctttggtggatccatgcctaccctttctccctctcacgatgattctagtcaagctatctatctttgatagcttgagccaagccaattgacttgatccaatctctctaaatccatacaaacttaagagagtgtattgattcacttattctcttctaagttgataagaaacataattaagtggagctcattaagtatttcaggtagttgctaacttggcaaaatggaagcaataataaattttaaaagactatagcttggtataatctcaaccatccatgatttagaaagatcttcagactcaatatagattactttggctactacaggtaagagctaaataggatccaaaagtaagatccatcacattagtaagtcaaattatatgtcaaatcttagtaggtatacttagtcctacgatgcctaattaaaatgatcatcatttgaaccttaaaatggactagtcaactaaaatttttctttttgaagaagatttagaccataaaatatcttctaatctgtgaagaattagatagagcgaggaatataaaattgatgtagaaatcaagatctatcatatatacaattttaatatttttttcataatttttaaatatttatcttctttttttataggtctagtcctatttaaactaggaagaggagtccaacttgacttatgcaataggggatgtccttctagaagataagaataatttgatcagaattatataagagcaaacctcattattataaataggggctatatacatcaatttatgagatagagaatcaatgaaacaaaagtagacttaagttttattttcataattcttctatcttctactttttttctaggagattcaagttgagtggattgaagaaaatctttcatcttctcgatcggatcatattggtattagagcgttggtcttctatatttatggagagctttaatgtattgtttaaatacgtgaacaatacaaacaatcaagagaagtgctatccatgcttcaaatacatcgaaatataaaagcaaatatggctactaattctttttcaatggacaatgagataaaaggatgtcttacacaactcaaggagaagattgtgcaactcatgaagattgtctccagattgaagataatttcaatacaagcacaaacaccagcaactcatgttgtgaaactgtttcctatgtttggagatgaagatcttctatctagtgaggagattgaattacctaaaagtatgaaaaatctttcttcaatcattgaaagttaaagcttgaattgagatccccatatataatggaaccattgatgaaaaaaagctagataattggctaaactaattacaaacctattttattatctatagatattatggcatctagaagatagcttttacttatctcaagctttctagccatgctcttatctgatgaaattcatatatgagaaataataatatttttaatatggtgcagagccaattcaaaggtttaatcaagaagtaattttatctaattggccataaggaagatcggtggatcaaatgataatacttatgatagaaacataatcaatccacttaggactataccaccaagttccacaaacaggcaatctgccttggaatctttatcaacaattatacaatttttataaagtatgttgaaagtcttcatgagagcatctaaaaaaagatgaaactctttaaggttgatgatatcagtaaagctaacatgaaagtcatagagattgaggagaaaaatcaaattagagaagataaggaaggcaaaaagcatatcaacataactcaaaaaaaaaaaattatgatcattgaaatctttgaaaatacatcaaggagaagtattgaaagtttcatcctgaattggagctaaagtagaagaagcccaaggatgataattttaagaaaaataaaaagtggtcctcaattctatagagattgaggagctatctgaacttgagtaagcaaacttcaaattgagcttgatggtgagaaaacctaatacaacaattaaaacggatctagaggtacatgacaactcacccacttaaagattcaagtgaagcagagtatcattaaggctattataaatctttgaagctagaagaacctcattttccaatatttggttcagaaatcgaggttgtagatcaagcctcatccatatccttatcctcttagttggattcagaaggatgtcaagttaaaaattatgagatagtgtaccttcaagttagccatcactgagaggtttatttgtgaggtaacttttgaaatagtttctttggatatttgtcaagttatccttagaaatgtgtacctttagaatcaagatgcaattttctatagacgatagagaaagtatcatcttataagggatgagaaaaagttcatgatcaacacctcaagaacataaggtaactttgaccttgcaactgttgcccaagtgaagtgatttgttaatgtttgtgatgagtgcatgatgatggtataaagaaccgatatcactcatgagaggtcaaggccttgtcctttggttccatcaatcgatcaatagagattgagattaaggaggagtcactatagtccttgtcgatgaggaaggatgacaacaagcattcctaccatgaagtctagatttgagagcaaatgaaagtaatccactgagacctgagagcaaaaaaaggcgagaccaaaaatcatcttcaagtaaagtcaaatggttcaaccatgagatggggaagtaagtattttcccaccttcaattctaactttgtagaaactaaatcccttaaacaggggagccctaatttaagaggatcctcagattcattgtggactactttggctattacaataagagctggataggaatcgaaagcaaaattcaccacattaggaagccaaattgtatggcaaacttcaagagaccataacttgatcacatgaaatccaattaagatgattttatttttgaatttgaatatttttttgagatctataactttagatctaaatcaagctaaaattttattgcttacgccttcaaaataggctagtcaaatcaaaacttttcttttcaaaaaagactttgactgaaagatatctttcaatctatgaagaatcaagtagagtgatgaaagataaagttgatataaaaattgagatctatctcttataaaattttagtaattttattttttttaatatttatctttatttagagatctattcctatttaaactagaaagaattgtccaacctaacttgttcaatgatcaacatcctcctaaaagataaaaagaagaatctgactcaaattataaaagggcggacctttttttttgatgaaaagggaggaaaaaaatccatcaaaatttattaagaaaaaaagagtacaagaaaagaaggatatgaaagagtaagagaagccccacaacatccatcaatatttaaaatttaaatttaaatctcccccatcattctatcaatatttgatattcaaatttaaattcttcgcagcatcccaccaacatttgaaattcaaatcctttcatacaaacaaaataatatttttcaaattctcaactttgagtttcaaaattgagaagcctacatattgtctgctcttcaccaaagaggggagattgttggcttagcttggcccaagagaagagaagaaggccaaggcccaatctgtagcctagagaaggagggtttggtagctacttaataatcggatctaaccgataaagacactatctctattagaagaaaaggtagagagaaaaagaggcaattggttaacttcagagggggaggaggtaagctgttgaggagattaatctgacgcaaggaaaaaagaagagctgacaactagccaatgatcgagaagggctggagacaatccaagcccagcaccaagaagcaagagaaagaatttggaggtcaaaggaggagtccaggaagagagagcgaaacacaatgttcggatctagccgacaacgataccaattatactaggaaagaaggtaaaaagggaaagagcaatcgatcatcttcagcaaagaaaaataaaagaggcacccgacagtcaagcccatggccaaatcagtcagcaagaggacctcacaagatctagacgatgctaaggggaagggaggaagaaaagagatccagtaactgtccaacaccaggaaaaggaggagataagaggaagggagaagtcatttttctatcttgggccgaaggagggagaaggaagaaagaggaaagaacatcctcaaagtcgaaggaaggaaggaaagagaggggggaaggggtcacagtcagatataccagaagggatagatccagtgtcaaagagagaaaagagagaggagatcagaaaataaaatttgatgactgactaattgtcatgaaaggctaatgacaactcataaaaaaagtatagtagtaaagagagggggataggcttggttagggaagagattccgacaacaaagagaaagaaagagagagagagagagaaccggctcccagccaaaaatagcttgacccaccatcgagaaggaccgacaaagagagagaaagatagaatagggagaatagcttggcttcgaatcaaaaatgatctaacacactgctgaaaaggactaggaagagagagagagggggtaggggagtatctcggctcgcaatcagaatcaactggccaatgccagaaaagagaggaagagagagatagagaagatatagcaaaagagaagagatggacaaaaggagagaggaagggagggagagagagaaaaaataggagagagaggggcttggtggctgactgtcagaagaagcctcgatgctcgaagattagatggaagaaaaaaaaatttctcaaaacttctcttttctataagagcaaacctcactattataaatagggttatgtatctcagtttatgatgtgaagaattaatgaaaaattggactttagctctatttttgtaattctttcatcttctatttttatgaaattcaagttgagccgattaaaagaaataatctttctttccgattggatcaatccattaactagatacttcaaaaatcaaaatgacctatctaaaatcctaaatcaaatacaaaaccaaaataactaaattaagatagaacaaactacaattacaaaaaactggctaaagtgtttaaatgcttttactcctaagtttcttcttgctcaccattaatgcttgatctttagctgggatcatatcagccttatgaccactataagaccaacataacaactcacttgtattgctcctttaaaattatacaaaactagtgtctaatatgtaccatgcgaatgtctgtttctcaccagaaaatggatgggcttcttgtgcaagcaccttcttcctacaaataataaaatatgcatcccttctctcatcttactaaataaaataattaaaggctttactatcaggaaatctggctttatccatataattttggaagttttatttgaacataacattacgagtactagattacatcaggaggtggttcctcttatttctattaagagaaaaatcaattttcttttaagaaagatcatttcattttcatcaggtagcgtactctactaatatacttccacaacaatatatagggattagattataggatggactttaaggcttcttttcgagagccctgatttctcaatcacattcccttttctttctcatgtaatggcatttaagagtgcatccagggcccaacaattagtcacaagtgttctttttatacatggtacatatttgctattttttagcttattttaacttgattgtgaagatatcatgagaaaattagatttaaagcctagcaatcttgaacccataatttcaagttaacaggtggaagagtccattattatgtgagaccaacttagactgcaaaactatctgatattggactatttactaacaccctttttcatgtgcaatgtttgtaaagagaagatatatgatgtagcgagataggatagtttggctctaatattgtgttaatattcaaaccaaaatcctaagctaatagatggaagagaaatgacttatatacatgtgcattattggatatatctttatgggagaaataatcacatggatgtttatatcacacatctcatatgtgcatgttgttgtaaggcttcaaaagacagacgatgagattggtcttggatcaaattggaatgtttcttagttgaatttggagaagtctgcaacaaatcctataaaagaagtcccgaaattggtggggcacctttcgatccaagacccttcgatggataagtcaaataaagccttgagaacagattgtggaaatggaagaatagaaggatgagaaaagagattgtgaacaaatggagagaggactcttgtttccttcagtggaggagttgaaaatgattcaacaaagtctccactctatctatcccgacttaccttatggagggtatgttaccctcctttatatagaggggtgaggaggcttgctcaagttgttaggccgttaatttattataatagaatggtcagctatataaagatcatgggatgtttatccatgtgatgattagctataggatagctagaaaatatctaatgcttaattagatgatagctgtcagataaccgtctgcattcttatagtacatcgatattttatcgacgtgactagcttaaatcagcaactgactgaactgaatattatgattcttttagttaacaatcatattggttagagaccgatgtaattcatagtagatcgatcacaagctgagatgagtatcatattttaagaacaatactagcaagttagatcgatcaaatgtcagatgaaaaagtagatcagtaaacgttcgatggaacctgaaagaatatttatgatttagataataatctatcatcacgtatccagataatgagatcatataacatgtaccaatatatgccctccatttttcacaccgaagtgaagttcttcacatcgggtgtggaaagtctcttcagaagatctcacctgacctgtattgtcatcataaatgctccataccacgatggttggaagtattaattttttaatcactcaaagtcatacacaatttcttgaaaatgatttgttgaacttagtaatgatgagcgcttagaaaatcgggagctcacaattatttgggtggctagtccctaatgtgtatgtgctaggtgtcatactgtaattggccacttcagctatcacatggatcctgcttgcatggcttaatcaagaagaggtgcgtcgcaacaactctctgcagaaccatcggataactgacaagtggcattgatctaatggcatatcaaatggattgagactgttagtaaattttataaataggtctatactctgttcaaaaattactttactatttttttcacatgacagtcttgctgaaattttttcagagcccctaacatcattggtatcggagtagagaccccccaaagtcattggagccggagaagaaagaagtaaagaagtcttttaaaagcttcctcaaattcctctttacatattaggcagactctttcatcttcaacttcttttccatgaacatctgagattttaggttttacaatctttatttttttttttggatagttattcccttttctctctttttttttctgtttctcttttcccattcacctttactttcttctttcctttcaaaaatatcttttgataggactaatgagataagtcaggaccaatggatatctcggtcaacccaaccactgctcaagtttgagatggaaaatctatctcggacaacagctgaagttagtacctcaggttaggatgatctagaatctcctataagagattttttagattatttcggcccaagtactgaacaatctgtcctgaccaatctcgatctttaggaacttaagaaaaaatattcgattcagcttataactccaagttgggatggtaggattattgaacctccagaaggttatgtcgtattttatgatgaggcacttcgatctggactttaatttctcttacatcctttcttcagtaatgttttagacttctataaactccatccaatctaggttactcccaatgccattaggatgatcatagttttcattatctatcgtaaattttttgctatagaactaagaatttctctctttaggatgctggtcatcctaagaaaacatccttatgaaaaagactgatggtatttcttaccttggcctcaatataaattcggtcccactcttcctttttcaatacataattgaaaaaatcattttttctttatttcttctaatgtttcgtagggttttatttgtaaatagtctaagcctaaaaccaaatggaactcaaataacaaaatattatctgaggatgaggagacttttgtagagcttttagatatgaaagtatccaagttgagcctactggtgtccaatcagtccttgtttgacaccgacatcagtcagatctctccttaagataagtctgatgttaattctttttctttattgctttatcatttttcatcatttttcttttctaacaatctttttccttatatagtagcaataatgaagttcaacctacaaaggctggctaactcaaagaagaggaagaaggatctaaccgattgctctcaagaagagtaaggagactgctcctctaagatcgattggcccccgatcatcacctgggccaatattaattgacatagatgctacatcgatctccactataccaccagcaaaatcaactcatcaacctactaaggtggcttgtccacctcctaaagagtctgcacatccaaagtaggcatcttccccaacacctccaacatcggccaagttagtttggctgagcaatcagcatctgaggtcacagactcctgatgtcaacccaccaactttctcatcaaaaaaaaattgacttggcgaaggtatcacttttggagacacccagactaggcaaggacttgctctgtacaatgatgcctcaaaaggacctagatgctgataggagggatctttctttggagcaaataataaattatggattcaacagtatcatgaacgtgagtcttcattctcttccactctcttctttctttttcttttttttttttacattggctatttgttgatctgaatatatctttctttttgcagtcggttgtgtatttcaagttgctcaatgagcacttgacatggttcttcaaaaataaaaatttttttgaaagagaggctcaaggccaagaaagaggccaaaaaagcagttgaggaggtcaagaaggcagtaaagaagaaggctgtcaaagaaagcaaaatgatggaggggctgaagaaacagctccaagaaaaaatagattccattaaggagactggacaaccaatgacagatgaatgataaagatgacaagttgtaaaaacagcctgaaaaaaatctcaaagttggaggccaagctgaaggaggtcgagtcaataattgaaaagcatgatgaagctcttgtcccatattagagacaacttgataaagacaaagagtggatgtcaaggattattgaagattataagaattccgacacttttcaagatgacgttactgaggcctcaaaaggagctttcaattatggctttttgagctacaggagtttaattatcaagctctttcctaaccttgatctcagcaaggtcataatagaagcagctctagaagtagtagccgaagtgacttctgcaacaactactgagcttgcttccacttctatcattggagtttctccgatcgaagtcccaaacagtccaatcgaggcctccatcatcgaagctatttcgaaggaatcagtcggcaaagaccttacctcaactcctccaacaaataactcccaagctaaggcctgaattatcttcttcttttttttctaaacatttgtattagcccgatgtgggcttctataaatactttttacattaatgaatgagtttttcaatgtcaatattttttctttttaactaatactaatcttggatgatccgatctgggttggatgtctcaaaaaatatcattcacgatagatagttattttctgacttcggttagatgattatgagtatatgtaattcaaccttggttaggtaagtaatcaaatattaactattctcaaaccaagtagataacgaagtcaatgtgattaactttaacaagtaagattgttatggaatgaaattgaatcagatcaactaactatagataacttaatctctcataattcactgtaaaggttctaaaagtacctttatctaagttcgaagtgacaagtcgggttcttttattcgtggatttatgacccatgctgtctttttgtgatcttcattattaatcaccttaaatcgatatagcaaaatccagtttatagatctgagtgctttcttgtcagattgagtctatcctattatctgtgaaacctgatctagagatcaagtattttaggttttttatttaaggtccaattcgaagattgagtatccaatgtcatattgttaggtccaatttggagattggatgtctcactatcatctcgtgaggtccaatccaaagatcgaatatctcactatcatctcatgaggtccaatccagagattggatgtctcacatcatcttgtgagatccaattcgaagattggatgtctcacatcatctcatcctattgtggttggaatttttgtagccttagtttgactttttctgacctcatttggacacctaaatcttattatcatcgtttgatcgatttttactaatctactttggatgaaaaagaattcttcaatggaacttttgattagaactttatcttcattgggatagaaatcgaatgctttattgaaagattttattgataatacattctgagatttttaatatttcatgttctcgaaatgatcgtaccatctaaatttttaattcgataagctcttggatggatcacctcagtaatctgataaggtccttcccaattcgggatgagtttttcttactccattggttttgagacttcagctcattggagaaccaaatctccttataaaaaattttaggctttacctgagagttgtaatatctggctactttttgtttataaactaccatatgaatctgggctttttctcgagttttctcaaataaattgagatcagtcctcagttgatctgaattattttcttcatgaaaattttctattctggttgtaggtaaactgatctcgactagtattatagcctctgttccgaaagtaagtttaaaagatatttctctagttggtctctgaggtgtagttctgtatacccataaaatattataaaattattctaccccgagacttttagcctcaatgagttttatttttaggccttgaaagatagttctataaataaatttagcttctccatttgattgtagatgtccaatcgaagtaaatatatgatctatgtagagctcagaataaatttttttaaaattttgattatcaaattattgctcattattagtaattataactcaaggcaaaccaaaatggtaaataattatttttcacataaaatctcatattttttctcagtgatttatgtcagaggttcaatttctatccattgggtaaaataatcaatagtcacaactaaaaattttctttgctccatggccattagaaaggatcccagaatatccattctccatatagcaaaaggccacagcactgtaatagaaataagttcagttgtaggctgatgttatatattggcgtacctttgacactgatcgcagtacttattaataaagtcggttgaatctttttgaatagtaggccaataataatcttactgaattatttcataagctaaaattttaccccccaaatggttactagagattcctttatgaacttctcgaaggatgtaatcagcttccgatggccttaggcataggagcagtgggagtgaatataacctctgatataattgattatcttgaacaacataccatggggcctgtcttttaattcttgttccttcgactggatcaaccggtagaggttctttagtaatatactccattaatgggtcaatggaacttagctcatattaaatttggacaattagtaaggcctcgatactagactttttaagaatatcaataagaacaccttgatttagtttgaaaaaatctgatgtggctaaatgagatagggcatcagctcagacattttgtccttggtatttgcatgatcttcagattttcaaagttttttaataattctttcatattatataaatattgaaacatcataaaatctttagcttcaaattaatctcatacctgactgacgataaattgagaatcaataaaaattttaatttttttaacattaagctccttagccattttgagtcctacaattagcgtttcatattctactccattgtttgagtgttaaaattaaatctcaaagcacgctcactaacaatgccttctagactcgttagaattaaactagttctactttctttcgaatttgaggctccatcaatgtacagtatcaaataagaatctttgatatttttcaattcttttaagattggttcttcattaggaatagagcattcaataataaaatcagctaatacttaaactttcaatgaagatcgaggcccatattgatatcaaattcatttaattcaatagcctatttgaatatccttcttaaagtatcaagctactgtaaaattaattttaaaggttgatcgatcagaattataatagaatgagcctaaaaatacgatcaaagtcatcttgctaatgcaatgagggtataaattatcttctcaattttagaatatcgagtttcaacatctctaaataatttatttgtataataaatggatctttgtatccctgcatcatttcaagctaaaatcgaactaacagcatttgctgaaatagatagatacatgaataatttttgacctttgatcggctttgatagtaatggagctgtgccgagatatttcttgagatcatcgaaggctgcttgacattcatcttatcaatcgaagtctttgatctgccttagaattttaaagaaaggaagatatttatcagctgatctgaaaataaattaactaagcaatgctactcatccagtaagttggtgtacttctttgatggagctcggatgcttcatttcacatagagcttgaattttcttaagattgactttaattcctctttgagttacaaaaaaatctaaaaaaatttttgaagttacttcaaaagcatatttgttgggattgagcttcatttgatattttcgtagtctctaaaggcttcttccagattggcaatatactgatctgactcagtattttttactaatatatcatcaacataaactttgatattaatttcaatttgttacttaaaaatcttattaatcaagtattagtatgtagcacctacatttttaagatcaaaagacatcattttataacaatgcaaatctttttcagtgatgaaggccatattttcttcatcctcaagtgccattttgatctgatataaccagaaaaagtatccataaagcttagtaatttgtgtcttgaagtagcatcaacaagctgatcaatttttgagagagaaaaactatcttttaggcaagctttattgagatcggtataatcaacatagatccttcatttttcattagcctttttaaccatgacaacatttacaatccactttggatattatgcttctctgatgaatttgtctttcaagagtttgtcgacttcctcatctattattttttatcttttcggggtgaaacttcttttcttctgttgcattggtttatgctttggatcaacattcagcttatgtacaataagatcagttaaaatctcaggcatattagagactgactaaacaaagacatcggcattcatccgaagaaaagatattaatttctccctcagatcaggcttcaatagagatccaatttggacagttttttttggatcatcacacaaaagaacagtaataagtttctcgactggttctcctcgatttttgatgatatcaactttactttcttgatcaagtattttaattggtagagcttccacagaccttttcatttttacagctatcagaaaatactacttagcaagtatctgatttcctcatatttctccaactccatacttagtttggaattggattagtaaatgataagtgaagactatagccttaagggcgttgagcctaggtcggtcaagaatagcattataagctgatggtattttgacaataaaaaaagtgagtcttacagttgactggcatggttctatccctgcagtgacggacaaagtgacctctccttccacagctacaggatttctagaaaatccaattacgggggtaccaacctatttagctaatttatcatattcattctttggaatgtatcatagaacaatatattagcagagctttcattatcaataagtattctttttatatcatatttggctattgccataaagatgacaacagcatcattacgaggagtttgaactctaacatcatcatcgaaaaatgaaattatgtgatccatgcactgatgctttggaaggctttcagtaatctcagccacctcctcagttccgtcgagatctgagatcatattgatgactgcagcagtagacttgttgtgatcattctcattgttgggcttctatcattggtcagtagcttgacttgcccgatctcgaacatatttactaaagtaacattagtggatcaatacttcaattttatcttttaattatcgatgctcctcagtatcatggccatagtctcgatggaaatgacagtattttctcttatctctctttgctggaggggctttcataggattaggttggcgaatatatcctaaatcctcgatttctatcagtatctgagctcgaggagtagatagtgaggtatagatgtcgaatcaccgaggtgggcttttgaacttcagattcttctgaggtcgttcagagttatcctgttggtttttatgatcttcttcctagggccacttttttccatctctttttttcttcacctaacgaagtatgcatgctctctttcttttcagcttgagcatacttacaaacctagatcaatatttgttcataattgtttgggtagttcttattaagagagaagatcaggcgattactcttgagtccttgcttcaaagctgccattgcaatggactcattgaagttcttcactttcagtatggcggcattaaagcatgccacatattcttgaagagattcaccttcctactatttgatagtaaaaagattgctagtatttttcaaatgaatccatttattatcaaaatacgtgatgaatatttgctaactgtgtgaaagatgaaatagatcatgtctggaggtcagagaactagattcttgcagatgttttgagagtgattggaaaagtgatgcaaaatagggcattagataccccttgtagtcttataatggctctgaagccttcaagatgatttaagggattgatggagccatcgaatgtttccactgtaggtatcttgaatcgaggaggaactgatttaccaagaattttttgagaaaaaagagatcgtaagttgaaatctcttctaccttgagaatggcttccaatctatatctccatcattttcttctcaagattttgaatcttttgtccaagaccctcctccatacatggcttcttatgtggagcagatttcacttcccaagagtgatcagtatggtcaagaagatgatcatgatgaagatcttgaggagttggttgctaagtgtgatgtgattggactacttggggggctactttttgctaccgttctgtcgtatactacagcagtaagagcttggacctgctgaaccaagagactaaactattgtggatcaataataattgaaggttaggtattctcctgaacatcttcaggagaagatgaagtaggtaaaggatgatttggtgccttcttgttcaccatttctactaaaatattttaagtgcccttcctctaacactaatctattactgcaaggcttcaaaagacaggcaacgagatgggtcttgaatcgaactagaatgtttcttggttgaatttggcgaagtctgtaacaaatcttgcaaagaaaatctcgaaacctacgggtaccttctggttcaagatcctctgatggataagttaggtaaagtcttgagaataggttgtgaaaatagaagaatagaaggatgagaagagagattgtcggtaaatggagagatgactcttatttctttcaatgggggagctgaaaataattcagcagagtttccactctatcaatcctgacttattttgtggagggtaccttggccccttcatatataggggatgaagaggcctggtaaggttgttagactattaggagagtttgttagatcgttaatttattataatagaatgaccagctatataaaaatcatggagtatttacccacatggtgattgactgtagtataactgaaagatagctaatgcttagctggatgactgctgttagataactgtctgcattcttacggtacattgatattttaccaatgtgacatagcttaaatcggcaactggctgaactaaatattatgtatccctttagttaacaatcatgtcggttagagatcaatgtaattcgcagcagatcgatcataagctgagatgagtatcatattttaagaacaacgctgggcgagttaggccgatcaaatgtcagactgaaaaagcagatcaataaacctctgatgtgatctgaaagaatatttatgatttaaataataatctatcaccacgtatccagataatgaggtcatataacatgtaccaacagtgcatttttccatctagttaagaggttggttagtggcatttgtcttcgatatgtaatgttcacataactaatgtgcttagtagcattcttttgtaaggttaaatcttcaatgatcttaagttcacataattgcctttgtgccctattagtttatagttgaccttttaattcaagagacagtcaccttagcaatcgatgtctgcttagattgggccaattaggtactcacattaatatattgaatcatgtttgaatataaaggattagattgatttataagtttccttttattgtttacatactgatacttagattgacttactacattatttgatatgttatgttctaatttttggattaaaattgttgtttctgatttctccttacatctaatactttgtataatttattattttttagcatgattgagtgtagaggattagattgatttttaagtttattttgattatttacatgccgatacttaaattgacttactacattattcaatatgttatgtttcaattattgagttaaaatttttatttctgatttctactgatgtccagtgtgtgtgtgtgtacgtatgtgtgtatatatttatttacatatatatgtatgtatgtatacagacatacatacatacatacatacatacgtacacacacacacacacacacacacacacacacacacacacatatatatatatatatatctgtgtgtgtgtgtgtctctctctctatatatgtataagtatgtatgtatgtatgtgtatatatatatatatatatatatatatatctatatgtgtgtatgcatgtatgtatatgtatgtatgtatatacatatatgtatatatatgtatatatatgtgtatatatgtatatatatgtgtgtgtgtgtatacatatgtatacatacatatctatacatacatatgtatacatacatacatatatatgtatatatacatatacatgtatacatacatgtatacacatacatgtatacatatacatgtatacatatatgtatacatatacatatatacatatatatatatatatgtatatacgtgtgtgtgtgtgtgtaagtaattaagtatgtagtgtgtgtgtgtgtgtgtatatatatttatatctgtgtgtgtgtgtatatatgtatgtatgtatgtatgtatatatatataaatacatacatacatatttatacacacatatctatacacaaatatgtatacatatagacacacacacacgcgtgcgcgcgcgcgcgcacacacacacatatatatatatatatatagatagatagatatatgtatgtatgtatatatatatgtatatatatgtatacatatgtgtatatatgtatatatatatgtgtgtgtgtgtgtgtgtgtgtacatatgtatacatacatatctatacatatatatatatatacatatatatatacatatacatatatatatatatacataaatatatatacatatacatacatacatatatatatatatatatatatatatatatatatatatatacacatacatacatacatatacatatatacatacacacacacacatacacacatgtatacgtacatgtatgcatatacatgtatacgtacatgtatacatatacatgtatacatacatatatagatatatatatacacatatatgtatatatatatatatatatacacatatataggttatttggaacctaagaaacttgcaaagttactagatgcaatgttcggaaaccatggaccgtaacaactggagtagtatttgggtcatgaattcatggctagatcatgaattgagtgggagtcaaccgaagtagggccagctcagacacttgtatttaggtcccatgcttgcgtgcattctcttccctgatatcctttggctttgctgcctcaaatcctcgagctatcttatcatcatcgcattgagctccataccttgctctttcctaactgtcactgtccccatcaaacctccggagatcctctttcttctccaatgttgagatttgttggagtcttcccaccttctcacttcaatgggtggcaatttcaagtgccagttcccttatttgtcccagctatattgacaatggggcttattctagggtttctcatggacatagtgataataataatcaagggaccaagagagaaaaatctttctagtctgtgttctttaagtttgagagataggcagcacatttttttaataagcctttttcactcatcggatcctgattttcagttgttcgacctgaacagttcaagcaattgaactgcttgggtcactattttggacgattttcagccatttttaagtattgtttgactggatccacgctgcgtagtgggcattgcgttgatcaagtagacctgtaagggtcaacaaggtctgagaacactgaatggatgctccataatcctcttgttatctgtcaaccatttggaatcttttaaaacaacatgtggtgataatatatatgataaactgtgatagattcatgtatagattatacatatgaaaatgtagagtgcttagtaaaagtgatgaagagcaatgcgttagaatgtgctagcctttgacctaaaaattggaatgcccaatgatgagttatgataaaattgtgacgtgatttatgaagtctaatgtttagttggcttgcagtttcagatgcgataaagaattttatgatttagctctttggttttttaacatgcaaacatttaattgtactgaaaaacatttatttcgaaacatgtaggagactattggatattgaaattaaaattgactttttggtgtttcacaatatttcttaataaacactacgactatgtaaataggtggtggatcaaagggaaagaaatgtttggtgattatttttagaaaagacaagaagtatttgataaatggttatttttcaaccgattaatgagagaatgactatgaacctatgaggtgcacctcttatgatgttgcatggatgaagcatctaatccatgggtacaatttactaaaatataggcccaattctgagacaggaacatttacaactcatgtacaaagaagaaacttaaagtatcatggatgccgggatatttccttcttcaaatctttcaaaagctgtagttttcattataaggaaaaatgattataactaacatcttctataggtgatgagtggacactagaaggctttcctataataacagtagagagagtagaaaagcctgtcagcatgcggtccataagtatatatacatattttcagcgcttaaagtaaattttcttgtaccaaaaaaagataaattttcaaaataagaactaaaatcaactgaaatgtttgaaatctgattcgtaggtacatggagaagagtgtaagacagcaaatatcataaaggcagaataagagctggtaatcttgtaacctggcgcaactatgttatgcatgtctatatgtgtgcatgtttatgtataacaagtaatatttcttttcttatttactcacttcagttaggaagtcaatccaatctccctttgcttgggtgtgttcagattatcaagggccataacagtagtgctggtaagcacctgtttaatggataaatggcgacaaattctctccccttctgctcactctattatcataccttccgtcttacccatctgctatatcttataaggaacataaggatcgacatagcttcatgctatcacattacaagctaagatcggaataatacctaatcttttcgatctactattaggtattactatagggttgtaaattgggtttaggttttgaactatattatattttggtgtaagaatatagtgccacactatcttgaaccagactagctgttgcacttttttgcaggcatcaatattttgttcatccaaaaaaaaatattgcacatgcacagatgaagtatgagggctgtaatcatgtgagaggaaacacagatggttgtgatcctataatgcttgaagaatgtgatccctcttttagttagtatacctttcttgtttttctccctgataggaaatatgaaatgaaggtatatctttatgaaaaagatggatgcatagaatatacaaatataaatttatacaggataagagaaaggcctccagcaatttgcacaataatagtgaaaaaagattaaataaattcccaacaatggcgccaatatgtgatatgcaactatgagtaggctttcctgttgcaacaatcaataaatatgtcatgcgaggcttttaaggtagagcactaacattctaatctgaaggcctaggtacaattttgaatttaggacttgtttggatgactgagtacaaaatcccataagaatcattgatttgggccaacacaactacctacatgaggcttaacctagtctaattttataaataccaagggaactattatagtaggccagcccaaatgccatagggaataaaagatgaagtatggaggttttttttattccttatgggatttggactagtccactgcaatgattctttaaatatttctaaataagtctaacctaacctcatttggacagttgtattagtccaaatccgtaatttccatagaattttggctacagtcatcccaggcccttaaatttaaaagatcatatttaaaacatgcttgaattctagattttaatctgggccctttaacttccatagttggtcttgaaatagacagcccagccccaagctcatggccctactgtatcttcgtttggctgtgccctttagtaggatgtcttaggtgtgtgaaaagcacctgaatatttcccacacaatgtgtttttttttcagtacaaaccggctatcacaccattctaatatgagtacagtccagagaatcagaatacaaaatatctcgtaaggcccaagggtagtcatcgccttcacaccaagtccagtctccgatatgcttcgcaacaaaagaggcagcccaatccatggtgctattcgcctcccggaatacatgttggacaaacgacatattggcgtgatgaagggacttctagatatcatagaacagtgaataggtttttaggtgtttcaccttgtcctgaatccaactaatgaccatggccgagtcatcctcgataaagatcctctccgctcgtagctcatatcttatgcagatgatgtccgcccaaacaacgtggagctctgccccatgaacggatgggtcgaagatcttctagcaaccaaaagcttgacatctggatctcaaataatatagcccgcaccacccctaccatctctgacactactatcaaagttgaccttgacaaactccaaggatggagcttctcaagaaatgaaaagagtcctcggagtcactgcaggcatagcaagggagtcccagaaactcatggtgtcaagggacgtggtggcagtactcctcagctaagcaacaagctctccaccactcgctacacaggcacaatctcgattttaaaaatcaagctgtttctgtacagccaaatctgataggcggtgtacgccatcctaataccccaaggcaacccctcaaccatattctgatggaccgcatcccgaaaaggcaaaagccatgggccactatcaaccttctagatttggccccccgccatcctccaaatcagatatgccctcgagcaatggagtaaggcatactctattgactcatcctctagttcatagatcaagcaagcagtaggaagctccgtgcttctgtctttgagaagtgtctgagtaggtagtcgatcccaggcaaccttctagaggaaaagtctgatcctagagtggactagccatgtgtatatatatatatatatatatgtatgtatgtatgtatgtatgtatgtatgtatgtacgtacatacatacatacacacacatacatacatatacatacatacatatacatacatacatannnnnnnnnnnnnnnnnnnnnnnnnnnnnnnnnnnnnnnnnnnnnnnnnnnnnnnnnnnnnnnnnnnnnnnnnnnnnnnnnnnnnnnnnnnnnnnnnnnnnnnnnnnnnnnnnnnnnnnnnnnnnnnnnnnnnnnnnnnnnnnnnnnnnnnnnnnnnnnnnnnnnnnnnnnnnnnnnnnnnnnnnnnnnnnnnnnnnnnnnnnnnnnnnnnnnnnnnnnnnnnnnnnnnnnnnnnnnnnnnnnnnnnnnnnnnnnnnnnnnnnnnnnnnnnnnnnnnnnnnnnnnnnnnnnnnnnnnnnnnnnnnnnnnnnnnnnnnnnnnnnnnnnnnnnnnnnnnnnnnnnnnnnnnnnnnnnnnnnnnnnnnnnnnnnnnnnnnnnnnnnnnnnnnnnnnnnnnnnnnnnnnnnnnnnnnnnnnnnnnnnnnnnnnnnnnnnnnnnnnnnnnnnnnnnnnnnnnnnnnnnnnnnnnnnnnnnnnnnnnnnnnnnnnnnnnnnnnnnnnnnnnnnnnnnnnnnnnnnnnnnnnnnnnnnnnnnnnnnnnnnnnnnnnnnnnnnnnnnnnnnnnnnnnnnnnnnnnnnnnnnnnnnnnnnnnnnnnnnnnnnnnnnnnnnnnnnnnnnnnnnnnnnnnnnnnnnnnnnnnnnnnnnnnnnnnnnnnnnnnnnnnnnnnnnnnnnnnnnnnnnnnnnnnnnnnnnnnnnnnnnnnnnnnnnnnnnnnnnnnnnnnnnnnnnnnnnnnnnnnnnnnnnnnnnnnnnnnnnnnnnnnnnnnnnnnnnnnnnnnnnnnnnnnnnnnnnnnnnnnnnnnnnnnnnnnnnnnnnnnnnnnnnnnnnnnnnnnnnnnnnnnnnnnnnnnnnnnnnnnnnnnnnnnnnnnnnnnnnnnnnnnnnnnnnnnnnnnnnnnnnnnnnnnnnnnnnnnnnnnnnnnnnnnnnnnnnnnnnnnnnnnnnnnnnnnnnnnnnnnnnnnnnnnnnnnnnnnnnnnnnnnnnnnnnnnnnnnnnnnnnnnnnnnnnnnnnnnnnnnnnnnnnnnnnnnnnnnnnnnnnnnnnnnnnnnnnnnnnnnnnnnnnnnnnnnnnnnnnnnnnnnnnnnnnnnnnnnnnnnnnnnnnnnnnnnnnnnnnnnnnnnnnnnnnnnnnnnnnnnnnnnnnnnnnnnnnnnnnnnnnnnnnnnnnnnnnnnnnnnnnnnnnnnnnnnnnnnnnnnnnnnnnnnnnnnnnnnnnnnnnnnnnnnnnnnnnnnnnnnnnnnnnnnnnnnnnnnnnnnnnnnnnnnnnnnnnnnnnnnnnnnnnnnnnnnnnnnnnnnnnnnnnnnnnnnnnnnnnnnnnnnnnnnnnnnnnnnnnnnnnnnnnnnnnnnnnnnnnnnnnnnnnnnnnnnnnnnnnnnnnnnnnnnnnnnnnnnnnnnnnnnnnnnnnnnntatatatatatagtatactatatagtatatatatagtatatatagtatatatatatatatatatatatagtatatatatatatatatatatatatatgtgtgtgtgtgtgtgtgcgcgtgcgcgcacgcacgtgtgtatctcgatctgtgtgtgtgtggtccatcttcacacttttccctcaaaaaaaccccccttgagattttgttcagctgaaaggggttcataaaacttgcccttgcttggtcctagggtttaagatttatatgcaatattcattaagacgtctaaatgtcataatattttgaggttacaaatattaacaaacagccttggatacaaacctttttctcaaagaatcttgtatctgttcttcctcagatgacatgtgatttatgctacggcctagttctaaggacttttctctgtcattaacataaaaaaaaaacagaaatatattccttagtaaggaaatagttgtgcactatgattgctatgtctctcaaaattataccaaactttttatgatatagagtgaaaatcaaatcagcatgtatggtctatttgccaaatagggttgagcataggtcgggttcggtcgagttgagagaaaaatttcatccgatcaaattcaatcggattgaagaaaattcaatccactgccaatcattcattatgcataaactatctaaaactgaaatgaatagtttgtagcaggatcaggtgttatgtcagtttggacttcaatgttaacccaatattgattttaaatccaacattggtccacttagacttatttatttatttttatcaatttaatataaaaaagatctaaacctcataagtcataaattttggatttatttttgaacatgtacaaaataaaacagaaaaaagaaaaaattacttatctaaaagtaactatatctgaaaactttcactttagaattgtcttaaattaatgtacttccatcaacaattcaatgttaatatttttatgaatccaaatggatgatagagtattttttagaatgaagtattgaagtctaaatgacatcgtcccaaaataaaagtgaatttatgaaatactacatctgtcggattcggtttcatacggattaaaagtgtaggaatagaatccgattataaataattatttttttataaattctaattcaattttattcgatttatattttttaaccggtcaaaattaatatttattaagtaggattggatggatttattcgtatctcgattatttgctcagcccattgccaaatctaaactcttttcagataggttccatgtgaacatgatacatgagatgcagtgtgatagtacacaccattgctaagaaaactttggagtttgcgtaacaatatctgtttaccatttaaaaaatggcagttttgaattttaacacgctctcctccagattcagcttatgaacttttcgaataaaaatacccctggactatttttccaaaaagtaccagcatcttttgaacttgaatggaaattcggccaataaaatgttttcatttattgaagaaataaacagggtaacgcagtagctctatttcctctgcttttcttttctatattaataacatgattattcatctctctcggatcacaaaaaaattaagctattcaagctttatttatatttcatttttaaattttttacttaaatacaaaatctcccatcccactactacggcagcatgttttctatgtatgattattttcattcaaatgatatcattttttataatttatattgtatgtaattaattcatttatagttcttacattttcctgtttctagtagatacaataaagcggttttggactagtagcttgttctctgtatcgaagtttaactaaagctttgacaataatatatgaatccatatcactgggtaggagaggaatatgttgggtataaaggatttaaggaattagatattttcatacaattgtattgcattgcagacagtaattagattactatgcaattattctctctctccatgtttgttgcagttgaagaactctaatgaagctcacaaaaatttactgcatgaacttgtaagtggaattagacgactccgttgtcctccattttcttttattttctttaaaatcatctgccattcaaatagacagaaaaaaaaggattgattagctattggatgcctcttgaattcaggaaatgaaggacgagcacccagtttatggttttgtggatgatgaccctagcaactacgcaggtgcactggctcttgccaatggggcttcccacatgtatgctttccgtgttcagccgagccagccgaatctccatcgaatggggtttggctcccatgacctgcgccttgcttgattttattgtagcttaaagaccttacaacttccagagtggtgttatatattagtatcttaagctatatgacagtggtaagcctctctatccgctacttgttatcctttaggtactttgcatgtggtgcaaggttataattgccttgtgtttctattgtcttcctcatggtacttactggactgatgatgtcaagtgaaatggagttgtttgaatcctgactgaaatttctcttggtccatcaagtgcaagagtaagtttagacatcacttgcaagcttttgctaggaaataagtagtttcattgcactaatgatttcgaatttttgttttcgggttagagaaacctagattaatgctgttattggatgctggcagtcagatgaagattatgtttgattgtacctcgttggacagatgctcatgcgtagatccataactctatttcatttcatttccctgtacacaattgaaacagggcatatatgaataggtatagaacagatgattcctgcaatattggaggtggctagctcagcttagactaaagttggtctagctgggatattctgaacacctgagatgttcaaataatgtgggataacttggcccaactcaactaaacattggctcaaagcatagtcaaggtaaagcttgagcaagctcttttgagcttggttcgagtccgagctgagcccgggccgcttgtttagctgatgaactgaattcaaatagccggtactcagcttggctccactcgattcatgagttcgaatcccctcaagttcaacctcgaacttgacggtgtagtcccacaaccatggccacctcataatgtgggacggccattatgcattcctctagtgcctgctccatatgacttttgttctcattataccatgcacctaaatgagtgctcatagtgacaatgtttagcctccacgtataatgtgtgccagctaactagaagcctaaactttggtgaaatttctgcaatgttgtggttgtaaaacgctcctacgttgagacatgatggtatctaagattatagacaaactatcatgctgaatcaacccaaatccaaggtgaataaaacttgatacaaagccgagctccattgcaatagtacaatggattctgcacttgaagaacattacaaaatcattttttcccaaaaagaaacattgcgaacagaccaaagcgtaaagaaattacatgattcaactaattcaagctttccatgatgtaggcactcgctagatgtagtagggtgataacttgctttgtgagggtggatcataagcttaacctcaatctatcccaatctatcctttcccttgacctatccatgccaatctaggccatttctgcataaatataacttaatcccagtggatccggcctagtttcactcactccaacacattcctactcaatggtagccaatcctttctttagccctcaaatataatcctaatctagcatagccaaccatcaatcatgcctaataaagcccgactacaccaacccgatcattcctgatcgtacacaatcaagacttatcctaattgatcctagctttttttaggcctctcttatagaacctgtgccaattctggacaagctaatccaatcttagcagccaaaaatattacatgtttaattagccaaatcgaacctatcataaacccaatatataatcggaccataccaagatcatcatcctatatttccttctcttgttataactacacctaaaaaggaatttcttcatacttatgaggggtatattatgataaaaattccttcattttagccctccatccttgtctatttttgggaccactagccaagtaacaccttaagagccctccatcttaatattccctctaactagctcgatttcttcttcattctttctttgcgatgtgtcccctccaatttaattcttacatgttgggatttgagtactgaaaaataatagataaagagaaagtaaaaactatgctaatgataataccaaaggcataaagaaatcacagcagtcgcaaaaacatcaaatttttttatggttcggcctaagcctatatctacatagggacgagagtaagaagaagcttccactataataatagtttagagtacaaaaacttctctgacaccatgtagggaacatcgcttctaatacaagaaagaagaaatccaagattaaacaaacctctagaaaaattcttctcgatggaataactctaatctgagattgaacaatcttctccaatcgatgatctccaatcttcttttcttaaatgaagcacccttcaagcctctcttcttttctctcttcctatcctcttttgtggctcacaacctcctctcctttttatgttctatgttcctcacatcacatccacagactcatttttatagataaaaaattagagtctatttcggactccttttccacacacaagatggcttcccacgccattggttccgtgcgcatgacttttttcatgccacaaaggattccgtgctgcaaaagttttccatatccatgcagtttccacacaccacaaaaactttcgcacacttctcgaaggcttttcatgctcgaccctttttggttttcaattaaattgatggatcccatatgaggagggaccacaccaataaatctcctccttctaactcatatggtaggttccatcaagcctgtagcacctttgcattttatcagttttgttcctgaagccggcttcatcaatatattagaactattttcttcagtgtcaacttttttaagcttgaaccacttcatctctagcatattgacatgcttttggaaagtatgtcaaattgctcaaaattaatcttacggttctctttttcgttagattctagtgcatattacgcactttaacataagatctaaggaaggaagaggactgaggtaaggtgaagtgatttttttttgagttggtaatggtacaaaagttatactagaccgtgggtacctaatctcggagattaccatttagatttggttcttgatcatttgtatagtgatgcatttaaaaaattatttgagcaaaacagtgaatgccattgggtctgagagatccaaaatcaaataacctaaagtatatagatggttcctttagctaggtcatgtatgagaaaaaatgatctgccgactggagaaaatagatctttgagctcattgactgttaagtcatatctagtctgtgaatcatctctttgaggattaatgatcaagctatcctttatgggttaaaagaataggatcactgaaatacttatcctagtatacatataatgtgcatggcctatttgatgagtcagactagaaggttatcactacttcatcacctttactgatgagcaatcatgatatggatatgtatgtgagatacaaatctaaaagattttgaatggttcaaagaattcagatatgaagtagaaaagataaatcaaaaaatttttaaaggtacttgatcggatctagaatgcaataccaaataaaaaatttgttgattatctaaaaaaagtgatatagtttcatgatggaattcttcttgtacacctcagctcaacggtatatatatgaggagcaatagcactatatgagatatggtccggtccatcatgaatatcactaatttaattattatttatttaagagcaagatttaatttttaaaatttaaattagattttttctaaaattggtttcaccgcaccatatgagatatgatttggtggataagttagaggatagatctgtgagaactcatttatagggtatcccaaaaggtatttaaaatattactttttctttccagtagttgacaatatgattgtgagcaatcatactgttttcttaaaaatagtggaaggatgaactcaaaaagaaagtctctaaagaacaacgagtcacaagacctatacaacctatttaagatgagccagtatatgtagtacttccttcacctcatcaatttagtaggatctcctatcttttagaaagatactcggtattcttacaaaggatttagagaaagtgtttcttgagggagattgagaatatagggatgatctcaaaacctacaatgacataatataaggaatcatgtagttacatgaaggtcagtgggagggttccatactgacatcgattatgatgtggttacatatagaatttttttttcaaagatctagatcaaacattctgaaaataaaaggtctatagagataaatccgaaaaggatgtttgannnnnnnnnnnnnnnnnnnnnnnnnnnnnnnnnnnnnnnnnnnnnnnnnnnnnnnnnnnnnnnnnnnnnnnnnnnnnnnnnnnnnnnnnnnnnnnnnnnnnnnnnnnnnnnnnnnnnnnnnnnnnnnnnnnnnnnnnnnnnnnnnnnnnnnnnnnnnnnnnnnnnnnnnnnnnnnnnnnnnnnnnnnnnnnnnnnnnnnnnnnnnnnnnnnnnnnnnnnnnnnnnnnnnnnnnnnnnnnnnnnnnnnnnnnnnnnnnnnnnnnnnnnnnnnnnnnnnnnnnnnnnnnnnnnnnnnnnnnnnnnnnnnnnnnnnnnnnnnnnnnnnnnnnnnnnnnnnnnnnnnnnnnnnnnnnnnnnnnnnnnnnnnnnnnnnnnnnnnnnnnnnnnnnnnnnnnnnnnnnnnnnnnnnnnnnnnnnnnnnnnnnnnnnnnnnnnnnnnnnnnnnnnnnnnnnnnnnnnnnnnnnnnnnnnnnnnnnnnnnnnnnnnnnnnnnnnnnnnnnnnnnnnnnnnnnnnnnnnnnnnnnnnnnnnnnnnnnnnnnnnnnnnnnnnnnnnnnnnnnnnnnnnnnnnnnnnnnnnnnnnnnnnnnnnnnnnnnnnnnnnnnnnnnnnnnnnnnnnnnnnnnnnnnnnnnnnnnnnnnnnnnnnnnnnnnnnnnnnnnnnnnnnnnnnnnnnnnnnnnnnnnnnnnnnnnnnnnnnnnnnnnnnnnnnnnnnnnnnnnnnnnnnnnnnnnnnnnnnnnnnnnnnnnnnnnnnnnnnnnnnnnnnnnnnnnnnnnnnnnnnnnnnnnnnnnnnnnnnnnnnnnnnnnnnnnnnnnnnnnnnnnnnnnnnnnnnnnnnnnnnnnnnnnnnnnnnnnnnnnnnnnnnnnnnnnnnnnnnnnnnnnnnnnnnnnnnnnnnnnnnnnnnnnnnnnnnnnnnnnnnnnnnnnnnnnnnnnnnnnnnnnnnnnnnnnnnnnnnactatgtatgttggctatgtaggttccgattcgctgtttggaatatgatatacctagatgaaatctatcgatcttgatagaaaaagagaagtcctatgtgattcgtaagactgagttcagaaaaatctctgaccagagtaagtgtgaatattgaaaaattttttttacgaaattcacaaatgaactcgagtcgagccaatgtagcatatgactgatgatagagtttgacgagttctcaatgacctccgtcaaattgggactctcgatagagggattgtatcacacgataactgcacctagggattcacttttctattttgctagcttgccactatatgttgctagacgtcactggtggatcgtgagaactcactaaaatcattttcggatcaacgatctttgctgaggtaagttggaatcgtttcagtccatcgaaaagagtttcgatgatactgtgatggagatcacgatatgtctcactatcaaacagaatagaacctgaggagtcacatacaaaaagagcttaacctgatcaatggcttggattatatttgaattatcaattagattgatagtttgaatattagaaactgctaatttgtaaccgttacagttttgacaactactaattgttagcgcaaggacttaattgcaagtattataatttttttgaggctgattaaattataaattaaattttaattaatttaattcagatttaatttaattagacttaatttaatttaatattaattggattcaattatccaaatcagatttggatttcaagcctgattggatcaggcttgacagccttttcgaatttggctcattttagactcgatttgaatccgtttgaggttctatttggatcagataaaccatgacttagagagctcaagttttttgggactctctttagaaatcatgtcaaaaggagaagtagagcnnnnnnnnnnnnnnnnnnnnnnnnnnnnnnnnnnnnnnnnnnnnnnnnnnnnnnnnnnnnnnnnnnnnnnnnnnnnnnnnnnnnnnnnnnnnnnnnnnnnnnnnnnnnnnnnnnnnnnnnnnnnnnnnnnnnnnnnnnnnnnnnnnnnnnnnnnnnnnnnnnnnnnnnnnnnnnnnnnnnnnnnnnnnnnnnnnnnnnnnnnnnnnnnnnnnnnnnnnnnnnnnnnnnnnnnnnnnnnnnnnnnnnnnnnnnnnnnnnnnnnnnnnnnnnnnnnnnnnnnnnnnnnnnnnnnnnnnnnnnnnnnnnnnnnnnnnnnnnnnnnnnnnnnnnnnnnnnnnnnnnnnnnnnnnnnnnnnnnnnnnnnnnnnnnnnnnnnnnnnnnnnnnnnnnnnnnnnnnnnnnnnnnnnnnnnnnnnnnnnnnnnnnnnnnnnnnnnnnnnnnnnnnnnnnnnnnnnnnnnnnnnnnnnnnnnnnnnnnnnnnnnnnnnnnnnnnnnnnnnnnnnnnnnnnnnnnnnnnnnnnnnnnnnnnnnnnnnnnnnnnnnnnnnnnnnnnnnnnnnnnnnnnnnnnnnnnnnnnnnnnnnnnnnnnnnnnnnnnnnnnnnnnnnnnnnnnnnnnnnnnnnnnnnnnnnnnnnnnnnnnnnnnnnnnnnnnnnnnnnnnnnnnnnnnnnnnnnccccatcgaaaagagtttcgatgatactgtgatggagatcacgatatgtctcactatcaaacagaatagaacctgaggagtcatatacaaaaggagcttaacctgatcaatggcttggattatatttgaattatcaattagattgatagtttgaatattagaaactgctaatttgtaaccgttacagttttgacaactactaattgttagcgcaaggacttaattgcaagtattgtattttttttgaggctgattaaattataaattaaattttaattaatttaattcagatttaatttaattagacttaatttaatttaatattaattaggttcaattatccaaatcagatttggatttcaagcctgattggatcaggcttgacagtcttttcgaatttggctcattttagactcgatttgaatccgtttgaggttctatttggatcagatgaaccatgacttagagagctcaagttttttgggactctctctagaaatcatgtcaaaaggagaagtagagtattatttttttcatccttctttcttcacacgcatgaaaggagagggggcaccaatagttggtgccctgccttatctggatgtctttttcatccaattttttttttaattgaatttgatttaaaatagaatagaaatatcttagattaaggtatagaagtactttttttatgtgataaaaaaaatagagaaagaggacgtgcgctaattattggcgtgagacatctttccttctttcttcccttatctcaacgcacatctatcctttgatttgtttttgaacaccttggattaaaagagatgagatctcttgggcattaagaaggagttgtgcgtgggatttgagatgtggtgcgacaaaaaattaaaagaggatgcatgaagggaggtggcgtgcgttagatgcgagaggcttctttcttacatctttctctcctccccaatgcctcttccttccttctccacttcacgtccatgcccagattcaataaagatcagatctaagaaaagaaaagagagagaaaaagagaagaagaagggttcttcttttcttcatggtgatctggtatagatcctgttggatttgtgcgaaagagtttgagcaacgatctgcttctttaagatctgaaagaaaagatcaagatccatggatgaagagtgagatctgcaaggtgctagcacaccagtgatctcggtgctccgatcaaatggctccgtgtggatatcagctgaggtcgaacgcgtgcatggctacgatcagaatctgcgatatctgcaggatccgagatatggagattcgatctccattttatttttctaacagtttatttttctatttcagatatcagatcgtgggtacatatttgtatcaagatctttactatggttttcagatctgatttgatacgtaaataaattaaaattattttaatttatttattttcactgtgtagatgtctagaaaaaattttaaactacacgtacgaaatcgaagcattttctaacaactctgactatcaccatagacgacgtatatctcttgcttcccaccaaacttctttaataagttctttagccatagcatttctttatcgacctttgttatggtgatgtattcaacctccatcgacgataatgtgacacttttatgactttgattgccacaacaccgctccctctgagaatatcatcagataatctgacgtggatttctgtatgtccacatcatcgatcatgtccgtatctgtgtaagcctgtagcataggatctccactatcatggcataaatatatcctggatatctatttaagatatcttattttccacttcattgctttccggtgctcctttccaaagtttgaaagaaaccgattgaccataccatccacttgagcaatattagacctggtgtacaccatagcatacataagactccccaccacttagtccttctcactctttctgctttgctctttaatcaatgtaaagtgtcctacaagcagacaccaccggcttcactctactcatgttgaatcaatccagcaccttctcaacataggcctcctatgacaaccataggacctggatctcctatctctagcaattcttatccttaatatcattttgacctatcccaagtcttccgtcataaatgttcgatccaactttaccttcaaatcattgattttggtaatgtggcatcccacaatcagcatgtcatcaacatatagcaaaaatttgataaaattattgtcaaaatattttttcatgaacatgcaatggtcagaacttactttcttatatccattctccattatgatggaatcaaacttcttgtactactatcatggtgcctgcttcagttcataaagatttttcttcaagcaacacactatgttctcattaacctttcatttcaaactcttctagttactctatatattctcctcctccaagtcgccatgaaggaatgccatcttcacatcaaattgttccacctcaacatctaaacagccagcgagatcgaggataactcgagtagacgtgagctttacaacgattgagaaaatctcttcaaaatcgatactttttctctgaccaaaatctttcacaactaatctcatcttgtaccttggttataaactattctcctatggcttcaatctgaacatctatttatttttgagtgcttgctttttcttaggtatattcaccaactcatatgtattatttttctataaagaattcatctcctctttcattgccttcatccactcctcactatgctggagctctatggcttcagagtaggactcaagctcttccacatctgttaatagcacataatcctatggtggatatcttatggatggcgtccactctcttgtgaatctctggacctcttatgcaggtggttcaacatgcaactcaatttgaacaccatccgcactctcctcagcctcatgactatcatatgtaccgtcatctgtagttgctctcctgttatcaagacttctcgaagaggtatctgggcataagtctatagggctgctcggggttgacttcggcttcttaggcttcttaaaatcatcgatcgtctgatcctccaaaaaaataatgtcatagttgcacacgatcttccactccatagaatcccacaatcgatagttgaactctccgtcctcactatagctcaggaatatgcactgcttcaccttgacatctagtttggatctctcatctttaggaatatgcacgaatgtcctgcatccaaagattttcaaataatcataagaaatatctttctccaacaatattctctatagtgtatcacacttaagagtataagaaaaaaaaagattaatgctatggatcacagtcatcaatgcctccctccagaatgccttcgatagtttagcataagagcgcatgctcccgatcctctcgcaaatcatcctgttcaccctctcaacaatctcattttgttgtggcatcttaggcactgtcttctctagtctgatgccatttcattgatagtattttttgaaagaacccctgtattcacccctgttgtccgtccaaatatacttcagcttttgcccagtctttctttcaacagagatgtcaaattacttgaatattatcgagcacttgatccttcatttttaaaatatatgtccaaattttttagaagtgatcatcaataaaagtcatgaagtaagaacatccataaaaaattttatcactcagagaacaaacatcactgtgaataagatctaatgcaccaatttttcttttagaaaaaaattctaaaaagaaacttggatttgcttacccatcaagcaactttcatatatcttcaatccaaaactatgaataggaagagcattcttcttagtcaaaattgacattcctttttggcttatatgtcccagtcgtcaatgccataattctaaggtagaagattcttccactacattcacctcccctttaccgagcttggcttgtatgaagtagagaaagccttgcttgatacttttggctactactagcgattttttggttagcttctatttgctgtctccaaatatattgtagtagtcctcctcatctaatacccctatcgataacaagttcagatgaatatctagtacatgtcgaatatttttcaaaaatagcctgtaccccaagctcgtgatcagcataatatctccaatatcaaggatttttaattctccatcattctccatctttattgtcccaaagttactgaaatgacaagatgagaataattttcacctcactgtaacatgatacgaagtggccaaatcgatcacccagatagagtctcaaccaatagtacttgcaagatcatcatttgttgtgccacaagcaacgatcatctctccatccgtagctactgctatcatcttattgttcgagctggagtcatcacttgattattttttgacttctccttttttagtaatcggtagtctttcttaaagtgatcctttttgccgtagttgtaatatctatcacttcgagacttggatctcttccgtaatttagtggggccatcattcaagttagattgggagtccttgtgcttgtttcttccctttctttctatgatgagagcctcatggtggctcgagacaccttgctcctttctcctagcctcctcattaagcatatagtctttcaccattgccaaggctatcgaactatctggtgaagaattgcttagagacaccaccaaagtctcctaactatcgagtaagaaacttaacaatagtaaagcctagagctcctcatctaacagcatcttcatcacagtaagctggttcaccacgttctaaaagttgcttagatgctccaccatataagctccctccttatatttcatatttatcagtttgtgaattaggaacaccttgttctataccatctctcttgtatagactttttagtttcaaccaaaggccatgagcattaacctccattgaaatatggtggaagatgctatcatcaatccactgttggataatcccaacgattttatgattcaatttctcccattctttatttgacatcttatcaaactgaataataacatcctcgattggatcatgaaaatcttagcagtaaaggaggtcttccatgtaaggattccagattgagtagttagttaatgtcagcttgatcgtagtgcccgacgaagattggttctccatctattagcatcttaatttctttttgaatactttagattttgtaaaatttggctctgataccacttattgggatttgagtactaaaagataatagaaaaagcaaaagcaaaaatcacgccaacgataataccaaaggcacaaagaatcatagcaatcgcaagagcactagaattttttatggctcgatcaaagtctatgtctgcacagggatgaaaataaaaagaaacttttactataataatagtttagagtataaaaacttctctgacactacgccgacaatactacttctaatacaagaaagaagaaattcaagattaaacaaacctccagaagaatcctttttgatggaatatgaaagaataatattctacaagtcaatcgcatgagtaatgcaataagatattgttctatattttatcttccaaattcatatatttgatattaattattaataaaattagatattttatttcattatatgctgcattttaatacttgtttaaaattataatgaactccataggttaggacaataattttaaggtcatgatgagatcataccagtgagatttaaatctttgataaccttaatctaaaatattctcaatagtaggatcattaagtcaaaaatcaatgatactgataaaactggtacatcctatatattctcgacagagagggtggttgatgtcataatcacttgtgtggagacactaatacgaagatgtggtgctcattagagaataagttcattgaatttactgatcgagagaatatatgatgcaagtgatcctttgacctaagatcaccatggtgccttgtatatatgaatctatgttttggttcattctttagcttcattttttgagccttgtgtggggtgctccggacatggtgcagtatgtatggaggttgtgagtggtcaacaaaaaatcaatcactccttgtaaaaggagcgaatatcttatgtgatcttataggttgatccaaaaaatctttgaccaaagcagaatgataattagaaagagtttttaatatatcattaactgaatcaatatcttctgatcgagatacatataaataagtatttgaatttgacatgattttatatccataactaatctgaaatattgtatgattgaagaattgaattgtacaattttttaccattgaaaaaaatttttgatattttttttcaaatttaatatctttttgatagtcatgacatgttgctagacatcaatcttgacttgtgggctcacaaaaattaaaaagattttatttgaaagttaattagaaagtattctgattaattgatgtatttggactgacctaatctaattggattgatttaggtcatgagcttgagcccactgctggctagatgatcgctgtcgtaggcagtcaagaataaaaatcaactcaaactatatagatagggtgagtagggatcatttctatggagatctaggatgattatctttttttttaagaaaaaataaaaagagaattgattgtagaagaattaaaagaaatagaatagcaagaattaaattaaaagtatgaattaatttatgaaaaaaaataagtcagagaaataactcagaaattttgaatccaccatgcaaattagatttattttcttcttttttttatgttgcaacattaattcttgtgattaaggtattagtatagcttatctctaagagatacggactgtatcagtagattacaactcgtcctgttgaagtataaactatctaaattcaattacaaaatataagattcaatctaacatactacgatctatctctccaaagcacgtatcgtatctagggatcacgatacgtcaatagagggtataagccgtgtaggctggatcaatacctcaaaaaaaaataaaaagatatgaaataaaagtataattttattacataaaaatttaatataaaaaaaaaccgtttacaggctttatcatatttctggattgaagagatttagccacgcatcaagctctctagctccataatctctcaataattgatccctaaagctctttaatttttttttttattatttttttgttttttctttaatttttttctcttcttatttttgctgccatctgctgcctctgttttctctgctcctgctgcctccttttatagagcacagcttcttcgaattataagcatctatggactttcaattcccactatcttttattttgattgggattttaaaactttatccgcatcccagcatcttgtttcacgcgagatcctagcgtccacatgtgttttgaattccttatgggccacagaccatttaaaccaccaaagaccactttactattttgatttgaatcccatggaagccggctgcctctggtctcattcacccttccagtgcttcacatgggtcccattaatttgaattcctatgagccacatccaagcttttgaatccaagccttccttattttttaaatcaattaaaactttgctttaaatgccttgtagaccctcctatttgcatgctacgtgagaacattgttaagctcctcttggcccacttaagaacttctatgggctacatgcttttggctagctttaaaatggttttgggcctaactttggatcaccattcgaagtccattttgaattcaatttatttttatttttttttttaacctacaaatcgagctcttttattggtgatcatttttcctataaaacaaaaacaaaaagcatcaagtcttaagaaataaaagttaattaatatatattttgatacttttattgggatatttaatgtacttatcactagatatgaaatccaatgggtcacacactttgaaatttgatcttagtctaatctaactaggatttattataaatcttatgggttaaatttacatgctagcacatgaattaactcaagttttcaattggatttagttctaaggtgtttgagctaaccctatcctgataccttaaacctaattagattagatttgaacctatggttttcttgatgccttatgcttattacatgaaagagtttcatgtgacttaaattcctccatgccaccacatcttcatccatgccaaattaatatggaacaccccatttaattgtgcatttaagaaggaatagtccttcttaaacactcctcttaatttcccacactttcctttgttctacacaccatcaaatggcttttggaaatatgcgggcgcagaagtggaggtgtcctatatgaaggctcttccacattataagttatcacatggtgaattaaattattgtgtgagaaaatcatgcgccaagagttggcaccccttgggagttttaggcactccttcttatcctataaataaggggcaccccatatggataaatacaagggaattcaagtttaggcatgagattgagaggagaaaaagacacaaaaatctgaaaaaaagataagaaaaaaaaagagagaaaaatagaaagaaaagacgagagaaaacgaaaggcaagggttgctaatcctagggttcaatttttcaatagttggatttctgaatcaatttggggtggtgagattttttgagaaaaagtttctgatgtggccctagtagaagattgaaggcattcagatgatggtgcaatccgtttttgaaaaagaaaagtgagtagtatacttgtgaagaaagctgcaacactacatcaaattggaaaggaccttgatcaaacccatatggatcaccgttgcaggatatctactttggtatcttgtgaaggttattttttttatcagatcatcatcttcaaaaaggtataattttctacctaatatgcatgcttgatttgtttgattaaaatctataaagtgttcataaggtttgtgttctgattgtattgttttaagtattaaaacttactttaaaaatataaaaaaatttgaaaactatcttctactgtgcaactaaaatccaacagaataaccctaatatgagattgagcgatctccgtcaaccgatgttctctgatcttcttttcttgaatgaagcctcttcaagcctttcttcttctctctctctccctatcttcttttgtggcccacggcctcctcttctttttatgttttgtatttctcatgtcacatccataaactcccttttatagataaaaaattagagtccattttggactccttttccatgcttcccacgccattggttctgtgcacacgactttttccatgctacaaaagtttttcatgtctcacgtagtttccatgcgccataaaattttgcatacttctccaagactttttatgctcgaccctttttggttttcatttaaatcagtgggtcccatatgacgagggatcacaccaacatcatatgctctcctcaccataccaaatggtatccccaactataagacaaaacattcatcaagttgctaacagggttgaagatcagcattcactatagaaattttgtttttttgctaacagacgaaaagcatcaccaaaggcatcaaaaccattggcatagaccctggggtgttttaccgacagacacaaaaagcatcaaaaaatatccctatcagcaaagagttttgctgatgctttttttttcatcaccctttatcgatacttttttactcgtcgataaatcatcgacataactctcaaaaaattgatgatccctattgaatgtcagcataactctaaagcctttagtcatgcctgactaaaccatcagcaaaaggcttatttttagtgatacctgagcagtctattacgaaaaatctgaataatatgctagcaattttattgtaaatgcacaggagtttcatgcatacatttcaaaaatttttaataaaaaaatattagattaaattatttaatctacaaatgcatgtataagatctgaccttaaaactactataaatggatcgatgacatgaatttatatacataaaaatctgaatctaaaatgacaagcatatgaaccaaaaacagcatttagtaatagatctaatctaccacttctagaattccgaatccaatacctaagtgtgggtagttgaactccatgatcaaaaatgtagatctgaaaatcttctctggtcgctcatagccgcacaagcatccgacctctacggatggttcacacgaagctcctcggacctatcagctctctgcgggagtgctagcttgtgcagtcagtttctgatggtagattgacttgatctccttcttcgattatctcgaacctttttaatgttgaagatggatcagaggaagatgttggatggtagagaaaaaatagatgaagactctcttctctttgatttttttcttacccaaaaatctgaaacagttctaggtctctcacccgagaggagaatggtctcttcttttgttcatgccaaggaagaaagaaaaccacccaaaccttacaccccaaagaaaaattttggcccctctttctctctagtatcacacaatgaaaagttctctcttgttggcacacaaaattatggtcattttatggttgtcgcacaaaccaggtaagacaggataagagccagagtttgttgcaattcaaaccattttaaatttcaatttatcttcaactttttctcactcttatctgacttaaagagagacttataagagaaaattgggtataaaaaaccatcagaaagacttccttttcttacacacaataggccccttcaaaaataaccaacgtgtggaaggatatggataaggttttaggttgaaattcaaatcattttgaattcaaatcaaaatcaatcaattcctatccttaatggatgataaaagaagggttatcttctaattttatcatacataaactaattttgtacggtgagaaaagacgtaagataatttgggtggtgcaagggagagagtcccattcatttaggactctagggtttaaccaattgaattttttttcaaacccaatccaattagatccaattaaaatatgatgaacctaatctaattaggctcctataatctttattaaatttaatcaatcaataaattaattgagccatagacctgatcaaattaggatcatttctcttttaccgattaggtcatctcataacctaatcagacttgacctgattgaatccaattcaatcaaacttgatacagacttcaatgctcaatcaaattaagctaattagtgatctattcactaattaatcttctattaatgatagtgatccagactcttctctagagtctccgtccagtgggactctccagcagagtcccaatctagtgggactcttcaccagagtctccattcattgggactcttcagattagccatgtgattggagagaaacttttaatgtgaatccatcatccacattttatgtgaatgaca

SEQ ID NO: 2 - DNA, 15569 bp, Elaeis guineensis
  misc_feature (11900)..(12834): n is a, c, g, or t
actacattttaacaccaagctcgataatagtgataaagaaacatctagatcagctttataatcaaaaattttgacttacaattttacgtgtgtctcaaaatcttgaataaatataaataagatcttttatcttgatccaaaaatagtaatcaaggatttcattagtaacttcaacaacaatggtaaaaaaattttctatccattgataaacccaaattttgaattgaagtttcatgcataccatatagcctttaataagatctattatttggatctaaagatagtaattaaaattgttaatgattccactaagatgaatactttacaatctcataattaatttcttcaataaaaatagacttcttgataatgtctccaattgtatatttttttttatttctacaagaaaacttcatacattttttacgttccaatataaatcttaaaaagttattccaatcaaatatcataaaagatcttcttagtccaaccttaaataacttttatgaatgaatctttatcttgccactaaataatgaattttaaaatcaagagcaacatcacagcattctgtcatgtcaaatttgtgttagatgtatgtcctagaaatcaattagattgacaatgtaaattttttaaggatataatttatatattttgatttattaataaaataaaatttaaattaatttttattcatatttttttatctatgaatcatctaaagaattaataagatgatgatacatattcttaagagttcaaaatttgaaatatatgtcattgatgattaatttctgaatacttttgaattcttaagagtttagaagatcttgacccaagtagtgtgaatagtgaaaaaaagttttcacatacttcacatcaaaaatttaagttgaataaattgtacatatgacaggtattatagtttgacgagtaatctataacctctatcttatcaaaattctgatagaaagattgtattgtatgataactgtacttagaggttcaccttttattttactggattaccactacatgttgctagatgtcactggtggattgtgagatctacgaagattatcttgatgatcgataattctcattgaaaagattgaaactattttaatgatgttgtgatagagatcataatatatcttattatcagacagaatagaattctatgggatcatacacaataggagattaagactgatcaaatagttgaatgatgattaagaatcattacggagttcagattatcaatataattgataattagactaacttataattgttacaagtagcaaggacttaactgctaaaggttaataggttcaaaaagaacttatgtataaatgttgtgcatcttaatttgattggatcaaattagttatggctgaattcaagatgaatcaaataggaatttggttcaattgaatttgggtcaagctttaggcttaggtcacatatacccaaaatcatttggatgcatcaggtgtgtgacacctgaatcaggcctttctaaactattttgagtaagtttgatcaagtcaaaaggatccacaccctaaggtttcttgaataaaaccttaggcaccacattgaggacctataggaaactttgaccctctctcatatggggtggcacactgaggttttataaaaaccttaggcacccattttagccataaaaaaaaagctccaagggatggggcagtagccatgaagaatccttggctgtcaggactctattcaaaagagttctcaaggttttggactcttatggagccctaggatttgtttgcctataaatagatggccaccccaaggctttagataatgttagagacttgtgaagctctcccctttctcttggttgccggcccaccctctctcctctctcttccatgccccaagacttctttcttgtctccatcatcttgctgaaatttagatttcagcaagaaaagtcaagtagaagtcaaagttctaatgtagctcacaagatgttgagaacttcctccatctggcaaaggttctgcaagagagctagcatcctgagaaacaaaaagattgctgatcagccctcatctccatatggatatttgtagagatcagatgcatgcatagctagaagagaatcttatcacgatcatcactcgtgaagatcatctacctgtgcaaaggtatgagataagaaaaatattttttttatcataattcatgaatcctttgcttatattatactgagattcttggaatggattttttctctagtaaaactctagagatcagatctcgaagtcttcttcatataaaggttttgaaagttctttatattttcgctgctttgattcaaaataaattagatctattttgcctttcaacctttctcatatttattgacatataaagctttaattaatgagattaatgaaaagcatgtgcgaaatactgagaaaatcctaacagtgatatcagagctacttttgtacataagaaaaggattcaagttaaataaaatctgtttgatttaagtaaatgaatcaatcaaaatttatcctaacataagtttgtcctggtataatggtcaagaccattatgttgaaaggttatcctaggacaaaaagtctaagtaaaatctattttatttaagtaaatgaatcaattaaagtttattctaatataagattgccttagcataatggtgaagacccttatgttgaaaggttgtcctaggatggaaagtgattgatgagacaaatatatcatgaaagtatttttcacagatggaataaaatatatatattttgtttgtgaaaatgagatttcatgaatgtgtttgtcattcaatatgtgtggtgatcatcttgaattgccacaaatcctttttggattagggttgtatcatgactcacaaatcctgatggtttgcaaaattttgcattctgtagtgatagaaaccaaaagttaatccagttttggaataagattgatcaattggtatctaaggcaagtattttataatggtggttacttaattagttataaaagtacgaagagtctcctaccaatcttacacttatctagccaatttggttgattgaattctgaatttgggttgcttaagtgttaagttcactacaaatatattgcaaccatgattccgacttagtcaaccaagcctagatctcttgaatagattcatgttaattatggatttacataggatataaataaataattaaaacttgaagagatctaaatgaaaccttctcgtacatattaaatcgaatgatcttccatcattgtagatatacggatactctactgatgttgatgattttcgactagatatagtactttggttgcatcgaaaaagtacaaccactttataacatgagatgttgcagggtagagatggggttgggcccaataattgttaggtgaggatccaaatgatggctgcacttgcgtgtgaatggcgagtctgacttaattaagaaatagagctaataactattagatgaggcttcaggacttagagacttatgaccactacaacttacttgagaagcaatggataaagagtcgtctatttatcaactgacgcatcaccaataactatcagatggagtgatgtataattagtgggactatagtatccacttgaaatcttaatcgtaaaaatttttgtttctccacctgaagagcatgggagattcgaaaaaatagtgggggtagtttatttttaaaataaagctcctaaaataaactaaaataagttaaatacaaagtctaactagaatcttcttctctctgtagaaaatatctgcttccaacctctatttcatatccttaagactaattgtttgactagacccagttataaagattgactctaaaacttaaagatagtcttgagttttgaaaagatgagctatgtcctggatcaagatatcctctctctaccagcttgtcccacccctaatcaaggggcatcctatgaaaagtggttaaacgatgataacaaggcttggtgctgtgtgctgacatctatgtccattgaactccaatgccagcataagggtacaaactgtccaaggtatattgactcatctacaagagttatatagtgagtagagccatgtatctcactaggaagtatttaagagactcttcaagatgaagaagtatgatggatagtctgttaatgatcattgtctgataatgatcaagaacttgaaagaacttgagaagctcgatatgtctatcaataagaaattgcagattgatttgatcctacaattccttactgattcatatgtgtagtttattataaactaccatatgaataaaatacagtgcaccaaggttgagttgttaaatatactgataactactgaagggacctcgaagagttcaagaggcactgttcttattatggagcagacctcatctttcaagaaaaagtctactgaaaagaagaaaaagtttgtgaagaagcagaagttagagaataggccaaagaaagaagttttcaagaagaaggccacaaaaaaggaaaagtattttcactgcaactctgatgaccattggaagagaaactattctgattatgtggcaagcttgaagaacaaaaaagatagcataccttctgaagatatgtctgatcttctcgttattgaaactaatcttacaatttcttttactttcagttaggttatagactctagctctagtgctcatctatgcacttctatacaggatctggaggaaagtagaaggctgaggaaagaagaaataatccaacaagttgaaaatgatgcaagagttgttactatggctgtggagatctatcctctacgactaccatctgatcttagtttaattcttagagactgttattttatacctactgctagcaaaaaattgatctctatttcatctctagcataggataattatgtattaaattttaataaagattattataccatttatttgaaaaataaaatggttggacgtaattttttaattgacagtctctatcatttacatgttgatgtatctatgaatgtaaccaagcagaaagtgaatgccataggatctaaaagatctaaagatgaaataaattatatgtggcacattaggctagatcatataagagaagaaaggattaacagattggagaaagatgggctcttgggcttattgactactgagttatatccgatctgtgaattctgccttcaagaaaaaatgatcaagctgccctttatgaaacaaggagaaaagaccattaagatatttgccctggtacatattgatatatgtggcccattaattcgatgcgctggtcaaagaaggttgtctctatttcatcatctttatcgataattattcacagtatggatatgtgtatcttatgagatacaaatatgaagtctttgaaaaatttaaaaaatttagaaatgaagtaaaaaaataaactaaaatttttttaaagatttttcaatcagattgaaaagttgaataccttaatggagaatttctaaattatctcaaaaaaaatagcatagtcttataatggactccatttggaatgtcttaactcaatagagtttcgaaatagagaaatcaaactttattagatatggttcggtccatgattagtttcattgaccttctcttatttctttggagatatagtttacttaccactaattatctattgaatagggtttcctctaaaatcatttctaccacattgtatgagatatggtattgtagaaaatcaagtcttgatcatatcaagatttaaggatatccgacccatatcaaaatatttcagacggacaagttagaggtcagatctatgaaagctcggttcaaaagtatcttaaggagtctttaggatattatttctacttttcagaggatcacaatatgattataagccaacatgctctcttccttaaaaaatagttcatgcaagatggaagtagtaggaggcagattgagcttgaagagagtctctgaagagcaatgagtctcagaacttacgtaaaacctatttaagttgagccaatacacacacctcttcctccatctcgtagatccagtaaaatttttcattctcctgagagatacttaggtatcatcatagagaatgtagagaaaatatttctcgtgaaaaatgagacatatgaaaatgaccccaaaacctatagcgaggcaatatcaaatatcgactataagaaatggttagaggctatgaagttagaaattaactcaatacacttaaaccaagtctgaacctttatggatccgtcagaaggtatggtacctattatgtataaatagatctacaaaagaaagattggttttgatggaaaggtagagacctttaaggtaaagcctgtgactaaaggttatagctgacacgaaagcattgactatcaatatattttttcactagtagttatgctaagtccatttgaacattacttgcgattgcagcatattatgattataagatatgacagatagatgtgaaaactatttttctaaatgaatatctttaggaagttatctatatagagtagactttgtgtttcacttccagtgatggcgatcacaaagtttacaaattgtaaagatctatttatgcactcaaacaagcatcttggagctggaatacttatttcaatgatgtaatcaaatcatttagtttcatcaaaaatgagaaagaatcgtgtgtgtttaagaaaatcagtgggagtactgttacttttcttgtattgtacgtggatgacatcctcctgatcgaaaatgatatttttatgttaattttagtcaaaatatagttgtctaagaaattctccatgaaggatcttggggaagcatcctatattttggagataaatgtctatagtgataaatctatgaggatgccaggcctttcacagaagatgtacattaaggaagtgctgaagaagttcagcatgaaaaactccaagtggagacttctatccttcaggtatgggattcatctctccaagaaggtgtgcctcaacacatcttaagagatacagtacatgagcaaaatcccttatactgcggctataggaagtctcatgtatgtcatgttatgtacatgacctgatatagcttatgttgtgagtgtcacaagtagatatcagttgaatgcaggtgaaaaacactggacatctatgaaatgtatccttaagtacttgagaaggattaaggatatgttcttgatctttagaggaggagaattaagggtgcaagaatataccgacttaaattttatgtttgatattgatgatcgaaaattgacatcagattatatttttttatgcaacggtggtactgtgagttagaaaagtttcaagttgcctatcatagcagactccattatagaagatgagtttataatcacattggaagctaccaaagaggcattctggtttaaaaaatttattacagagctggatataatgccatcagatgtcataccactctactgcgacaacaatagtgccataactctagctaaggagctgaggtctcaccaaaagtctaagcacatagagcaatgatttaatctcattcgcaattatctcgaaaaaaatatatcaaggtatagaaagtagatactatggataatatgacagacccactaactaagtagctgagtcaataaaaaatcgaagtccatcttgagaagatgggacttagatttgtggccaattgattttagtgcaaataggagattgttagatgtatactctaaaagtcaattagactgacaaatataaattttctaaggacataatttatatattttgacttattaataaaataaaatttggattaattttttattcatattttagtatccatgaattatccaagagattaatatgataatgatatatattctcaagagttgaaaatttgaaacatacgtcattgatgattaatttttgaatgctttcgattaatggatgatcataaggatagtaattaatccgatcaatgtacaaatcacttcttttttgatagacgagtctcgagtctatactatggagacactggagcaagagtgcaggtatttgttagagaacaaaggtatcgagcgtgactaatacgagaagtcaattggatggctatccactcgttaatgacttatttgatactacagtagtatgtctagtccttagatctgcaatgcctcaggtgttcataatgagactgttagagtttgactgtacataaacttgatttctagccatatggatctttatagtgcatgttggctacagtaggttcgttgtaggaataggatgtgcacatagatagaatctatcatccttgatagacaaaaaaaatgatcctatataatttatgagactgagttcaaaaaatcttgactaagacagtgtgaataatgaaaagaagtttccacatatatacttcacatcagcaattccagttaaataaatcctacatataataggtattgtagtttgatgaataatctataacctccatcttattgaaactctgatagaaggactgtatcatatggtaactgtatcaagagattcatctactattttgctgaattgtcactacaaactgctagatgtcactgatagattgtgggacctatgaagattatcttgatgatcgatgattctcatggagaagattgaaactatttcaatgatgttgtggtagaaatcacaatatatcttactactagatagaatagaacctatgaggtcacacataataaaaatttgagattgatcagattgttgaatgatgattaagaattgttacaggattcagattatcaatataattgataattggactaacttgtaattattataagtagcaaagatttaattgctaaaggttagcagattcaaggaggacttatgtgtaaataatgtacatcttaatttgattggatcaacttagttatggctaaatttaagatgaatcaaacagggatttagtttaatcgaatttgggtcaagctttgggcttaggtcacatgcactcaaaagggtttggatgcatcaagtgtgtgacacccaaaccaagcctccctaaactattttgagttggttttgaccaagtcaaaagggtccacaccctagggtttcttgaataaaaccctaggtgccacattgaggaccaattaggaaactttgacattctttcacacggagcagcacactagggtttcatgaaaaccctaggcacccattttagccataaaaggaaagctccaagggatgggatggtgccatgaagaatccctggccattgggactccattcaaaagttctctaggttttgggctcttatagagccctagggtttgtttgcctataaataggtcgctaccccaaggctttagataatgctagaggcttgtgaagctctctcctttctcttgtttgccatcccaccttctctcctctctcctccatgcctcaagacttctttcttctctccatcatcttgttgaaatttagatttcaatgagaaggatcaagtagagtcagagttctactgcagttctcaaggtgttgagaactttcttcatcaggcaaagattctgcaaaggagttagcacctcaaagaaccaagaaagttgctaatctgccctcatctccatgtggatacttatagaggccaagcatgacgagaagagccttatcacgatcatcactcgtggagatcatctacccgcgcaaaggtatgagataagaaaaaaatatttttcttatcatgattcatgaatcctttgcttatgttacattgagactcttggattagattttttctctaataaaatttcaaagattagatctcgaagtcttcttcacctaaaggtattgaaagttctttatattttcgctactttgattcaaaatagattagatttgttttgcctttcaatttttctcatatttattgagatatgaagctttaattaatgagattaataaaaagcatatgtgaaatactgagaacatcctaacaatttgagcttacaattcacttaaacaactaatgatcaaattaataatcacaatgcacaataaaaattcatgataaatctttttgttgttactttagatcaaaatccaactaatcataacatgatccacggattgcctatcatatatcaaaccctctgaattattaatcttaaacgatcttttcattcatgatcataagatttagttaaaaatcatgaagacaacttatattgtaatcatcatagatctgtatcttaacatccttagtgtttacctacctatactcatcctatgtttgattctatatatcataatttattcactaatactttgatatcatataaattatcgcatccccaatctaagatcatattggtactttaatatttcattagtgggggttatgcattagtactttgataccttatcagttgaatggttaaacactggtactttgatatcctatcagtggaggttatacgctggtactttaatatcctatcagtaagatggttaaatactgatactttgataacctcccagtgggtgttgtatgctagtactttattatcctaccaatggggcagttaaatgctactactttgatacgctaccaatgggatagttaaacgctagtaatctaatcttagcttgacataaagtaacgtcgactcgagtttagggtcgactcgagagaatgttagggttagcttgatatgaaagagggtcgctcgtcaatattttggagtcaactcttgtttatggatgatctagaaagtgtcagagtgagctcgagtactgcatatttctgatacattgtctatgctagaatgtgctagaactgattatcttctttatcaaagttgatttttgagtaacttgatgatcaatttttctaggctagacttgctttgtcaaaatgagcacttgttagtttagagaatcttcacctacacatgatctcaagcattcattagtaccaaaaatacttaagtattttgatatcatcaaaatcaattcttgggttaacacaatacttttcaaataataagcatacagatataatcctataacaatttaaattttgttcatatatcaatttctttaaaaatattatattcatcttgatagctatgaactaaatcaaaatacatactagtatacaacttttactgggagagtattagattaccagcatttaaccatcccactggcaaggtatcaaattaccaatacacaacccctatttataaagtatcaaagtaccagtgttcaactgcctcactggcaggatatcatagtactagtatttaactaccacattgacaggatatggaattatcagtatttaaccatcattagtagaattttgatgcatagtcaggctgcgagtcaaaatctatctcaaatcaaaatattgatcacatgtctaattctgtatcataattcattcccttatgctctaatattatattaattgtcatacttctagctcgagatcatgagccaaggattgcagtaactaccgcatacttatagagaactctttctataagcatacaagatattctaaatatactatcaatatatcatagagaaattaatttaaataactaaaagttaatattcaattaataaattcaactggcaaatgtatttaaaaattttacatcaaataaatcttgattaataaatattaattaataacaatagatttaaatcgaaacaaggttgatattgttagaatttgatgcctcaagattcagcccacattgagtccacagtgaggttcgcgacgaaaaatgnnnnnnnnnnnnnnnnnnnnnnnnnnnnnnnnnnnnnnnnnnnnnnnnnnnnnnnnnnnnnnnnnnnnnnnnnnnnnnnnnnnnnnnnnnnnnnnnnnnnnnnnnnnnnnnnnnnnnnnnnnnnnnnnnnnnnnnnnnnnnnnnnnnnnnnnnnnnnnnnnnnnnnnnnnnnnnnnnnnnnnnnnnnnnnnnnnnnnnnnnnnnnnnnnnnnnnnnnnnnnnnnnnnnnnnnnnnnnnnnnnnnnnnnnnnnnnnnnnnnnnnnnnnnnnnnnnnnnnnnnnnnnnnnnnnnnnnnnnnnnnnnnnnnnnnnnnnnnnnnnnnnnnnnnnnnnnnnnnnnnnnnnnnnnnnnnnnnnnnnnnnnnnnnnnnnnnnnnnnnnnnnnnnnnnnnnnnnnnnnnnnnnnnnnnnnnnnnnnnnnnnnnnnnnnnnnnnnnnnnnnnnnnnnnnnnnnnnnnnnnnnnnnnnnnnnnnnnnnnnnnnnnnnnnnnnnnnnnnnnnnnnnnnnnnnnnnnnnnnnnnnnnnnnnnnnnnnnnnnnnnnnnnnnnnnnnnnnnnnnnnnnnnnnnnnnnnnnnnnnnnnnnnnnnnnnnnnnnnnnnnnnnnnnnnnnnnnnnnnnnnnnnnnnnnnnnnnnnnnnnnnnnnnnnnnnnnnnnnnnnnnnnnnnnnnnnnnnnnnnnnnnnnnnnnnnnnnnnnnnnnnnnnnnnnnnnnnnnnnnnnnnnnnnnnnnnnnnnnnnnnnnnnnnnnnnnnnnnnnnnnnnnnnnnnnnnnnnnnnnnnnnnnnnnnnnnnnnnnnnnnnnnnnnnnnnnnnnnnnnnnnnnnnnnnnnnnnnnnnnnnnnnnnnnnnnnnnnnnnnnnnnnnnnnnnnnnnnnnnnnnnnnnnnnnnnnnnnnnnnnnnnnnnnnnnnnnnnnnnnnnnnnnnnnnnnnnnaagatattactaaattttgcttctaatctcactcttaaatagtacttacctttgaaactaggcatttgaatctgaaaaagaaagaggagattatgagcttgatagttcagtaaatcatgaataaattagctaaataaatctatgaataatagtatattaaaaataaatatgtaagatacaataattcaaaaatgaattcatatatataatactttccaaataataagtatgtggctgcaatcctttcgtaattcaaattttgttcattaattatttttttcaaaacatcacatggatagtcatgaactaaatcaaagtaccagtgcataacccctattgataaagaatcaaataacaagtgtttgactgcctcattatcaggatatcaaattattaatgcataacctccactgctagggtatcaaagtagcaacctcaatcacctcactggaagggcatctagtttcagtatttaactactccactggcaaggtgttaaattatcaatatttaacctccactgataggattttgatatatagtcagactgcgagccaaaattcatttcaaaccaaaatatttttctcaaagacatattttatgtttcacattgaaaaattcacaaaaattatgcgatattgaaatcaattggataaaatccacgtcaaatttagtatattcaatcataaatcatttactattctagaaaaggtatattaaaagtataatgcatcaatttcataaatcataaatatctcaatataaaaaatattttattatttattaataaatctaggagaagtgaagcattacttatcttgtaagtaaaactaaccaactgatcaaattaattctgagaatctttctcaaaactcatcaccactatatcaaaaacttgtgcttcttgctatgtaagagcatagaccctttcttcgatctggggttccaagtttctattttattttgttcaactatcaaattagactgacttttcatttttttgtggatattcagctattttatggcctttctaacaataaccaaagtatgtaccaatattccaacaataatcatttattgcatgattttcaccgcatcgaaatatttgatattatcaatcaatccaaacttgttattcactgacctcttattcaaacccttagtatatttaatattctacctttgtgattcattcaatcgatttctttttttttattttctttccctttctatatgctcttcattaacttttctttcaattatcaatgctttattcaatacatctgtataagtagttaactcatatagtaccatttattttctaatttctatcctcaattccaactcaaatttatctactcagtcacattcatcttcaaccaatctcgaagcaaacttgacaagctccataaatttagcttcatattctacaactattatatttctttatttcagataaataaatttttattctttctgaatcctcatactctaagaaaaatatttttatcataaaatatcttttgaaatcactcccaagcgagttgttctccatcttgttcatatttaggtttcattctctattatcaattaaatgtctcatctttcaacatgtatgatgcatataagattttttcatcatcatggtatctcttaacaataaatgctttctccatctccataagctaatttttagctcctatttcatagttttcttaaaagtcaatggagacaacttcttaaattctatgatattactttattgctcctattgctcttatgtccttgtggtgacaatatttattgttgcacttgctgtagaggcagttactgttactgcaattgctattacgattccatcaagccgactagtgtctgcattatttggataatagttgatttttgctactttatttagatgttggtggcaaaatcaatgacttctttttgctgagagatgccaccaacctactaagtatcatcatcttattggttgatacctttagcagcacctcgagtggttctttttatctgatatggaaccatcttaatcttgcatgaaaaacaaacttcgcaaaattttcttttaaaatctaatatctaatattatacttttattaaaatttaattatgattattttaagaataaaaaatttaaattttgaaatcctcacaaggctggccaagagataatgaccatcatcctagtcggtttgacgtaggacatccaaagatcaactataattcaagcatcatattgagatgctaggatataatcgatggtgaaatttaatgatgctcgactgatcaagatgggggccggcccgatggcctgttcaacaatcattgatcaaaattttttaaccaaggtctatcaagatcattaaaaagtctttctaagatctataaattgtaataaagagacacaatctagagagagacactttttacataaagaaagtagaaattttagggagagaaattagagagaaaggggaaagagagaggaagctgagaggaagaaagaaaagagaaagactctctctctttttcttttctttcttttctctcttttctttttcttttcttttttttcttccttttctttctttctttctttggctcattagaaaaataggggacctattgatccccttgtttcctaaataggggaggaatctcatcttggtagctatggccggcgatgtgagccaaagtggcaaaatcatgaatct

SEQ ID NO: 3 - DNA, 3181 bp, Elaeis guineensis
ttcaaaatgatgaacagatgcatctcaagtcagcactagaccatcttctaaaataggaagatctatggaagcaacactcccaaatgcagtggcttcaaaatggggattgcaatacgaagtttatccatgtttgggcaagtaacaggaaaaaaagaatactatcactgaactctagcaaggcgatcagaagattatcgaatagcagcaaatccaatccacattctacaactttttttctaccctactaggctcgactgaggaatgactcatccaagctgattagaagattctttatccagaaggacctctggatcttgctgacattgagtatccatttatggagaaagaaatccatgatacagtgtatgacttggctttggaaaagtcacccggatgatattttcccattctccttctatatgcacttctagtgtatcatcaaacatgacctgatgaacctactgtaaaatcagctaatgtagaccatctgaactacttgttcatcacccttatcccaaaaaaaaattggtgtgtattcagttagagacttcaggccaataagcctgattaatggagtaataaaaaatatttcaaaaactctatcgaaaaggctctcacagaaaatgaatttgttaattttatccacagagcttgctttcaacaaaggaagaaatatctctgaatattttgtaatgactatggaaactatacacttctgcaaagctgaagtacacaaggatctcaattataaagtcgacttcgagaaagcttttgacaatgtggattggagctttctattgaaattgctatccagcacggggctttgattcgaggtggtgtcaatggatagaatatctgatttatacagctaaattctcagtccttattaatggtgataaaggtaaactttttaaattgaggaaagatctcaggcaaggagatcctctattcgcctagctctttctcttagttgttgatatagaatgatcaagggagcaagtaggttcaatctttttgttggaattggatcatataatatcatgggataacttcaaagcttttagttcactgatgacacacttatattttgcagatatgatctaaaatacatcaaaactcttaaatttttactctatagttatgagctactgatgggtctcaaaattaactttgaaaaattccaattttttggcttgagaattgcaaagatgtcagtacagcaagttgcatctatcctagaaagcaaggtggctacattttccattacttatttgggtctcccactccatcattctaaactgaggaaaacttattggaatccactccttgagaaggttcagaagaaattgatcgggtagaaaggtaaacttcttaacctctagggtaggcttatactaactaatgcagtgcttacagggatcccactactctggagggatacattccttctccctcaattcattatcaaataaattgataaaatccatcgatcattcatttggagaggaaacgaggagtataactaagggcactctagaatatgttggtcgaatatttgtcgatcaaaaaaatttggaggactgggggttcctcaatctaaaaattttcaatacaattcttctttgtaaatggtggtggaagctctactctaatgctggtgacccgtggtgtagttttattgccactatccacccaacttcacactagagatctaaaggtatacacaaatcaacctcttcattttggaatggtttacagcacacatgaaatatttctactcctaatccactttcaagttagcaactagtattattttggaaagatagttggttacataatcatccactgaaggatcgatttcctcacctttacacaatagcattgaagtgcaacaactcagtggcaaaggtattaagcaatctacttgataatagctcttttagtactcctcttcctcaaagataccaagaagattttcagagtctataggaaagcattgaacaaattacattaacggaacgacctgatactatacaatggaaatggtttagtagcaatatttttttggcatgaaggatctactattttctgcaagatggaggagtttggcctctactgagtaatattatataaaaactcctaataccaaagaaagccaagttatttgcttggctaagtgctcacaacaaaatcccaatgaaagctaatcttcttaatagaggaataattggaactgattactgtacactttgcgatgacttatcagaaactaatgatcatctaatgctcatctatactttttcaaaagcaatttggaatcaagtactttcagacctgcaattgtcgaaacttttatgcatgcttaacaccctatgggatacttggagactcatcaatatgcaacacgatagaagacctaaactagctgctctattcgtaattggtcaatggtgtctttggaaggaaagaaataaaagattattcgacttctatactttttatccacgatcgattgctgaaactgtgtcactttttctttcttgggcatcacacctaacaacggagcaactaaagatgttagctcctgttcgagaagttctcttatctaagaatgaaaacacacaatctttagtgagaattacagatgctaacaggcgcagatgaatgttttatgagcatttttatagctgcagcttatatgtgatctatggtgcaaggagttaattataaccatggatattagttaggttgactatcagaaatcatctccaatacattctatgtaaccactgatcaattccatgttcaactagataggaacctgcctatatacaggtatgtccctgatgtaactatagtatactattattcataaataaataacgaaggttttaccttcttctcataaaaaaaaagtatcttcatgtcatcctatatgtcatgcatctcctttgctacttcttttatttacttcttaaacttggttctaccatatattatcagccccttttaaatttgcttttggatattgcatattccactcttcaatcacctcatgccaagcaaaacatttattcacacttgaaaaccaatataagaataccaaagaatttatccatgaaattctagaaactttggttttactcctttctccatcattcaaaaaggttcaaaatgatga

SEQ ID NO: 4 - DNA, 14184 bp, Artificial Sequence
  synthetic predicted full EgDEF1 cDNA transcript
aggagagagaggggcttggtggctgactgtcagaagaagcctcgatgctcgaagattagatggaagaaaaaaaaatttctcaaaacttctcttttctataagagcaaacctcactattataaatagggttatgtatctcagtttatgatgtgaagaattaatgaaaaattggactttagctctatttttgtaattctttcatcttctatttttatgaaattcaagttgagccgattaaaagaaataatctttctttccgattggatcaatccattaactagatacttcaaaaatcaaaatgacctatctaaaatcctaaatcaaatacaaaaccaaaataactaaattaagatagaacaaactacaattacaaaaaactggctaaagtgtttaaatgcttttactcctaagtttcttcttgctcaccattaatgcttgatctttagctgggatcatatcagccttatgaccactataagaccaacataacaactcacttgtattgctcctttaaaattatacaaaactagtgtctaatatgtaccatgcgaatgtctgtttctcaccagaaaatggatgggcttcttgtgcaagcaccttcttcctacaaataataaaatatgcatcccttctctcatcttactaaataaaataattaaaggctttactatcaggaaatctggctttatccatataattttggaagttttatttgaacataacattacgagtactagattacatcaggaggtggttcctcttatttctattaagagaaaaatcaattttcttttaagaaagatcatttcattttcatcaggtagcgtactctactaatatacttccacaacaatatatagggattagattataggatggactttaaggcttcttttcgagagccctgatttctcaatcacattcccttttctttctcatgtaatggcatttaagagtgcatccagggcccaacaattagtcacaagtgttctttttatacatggtacatatttgctattttttagcttattttaacttgattgtgaagatatcatgagaaaattagatttaaagcctagcaatcttgaacccataatttcaagttaacaggtggaagagtccattattatgtgagaccaacttagactgcaaaactatctgatattggactatttactaacaccctttttcatgtgcaatgtttgtaaagagaagatatatgatgtagcgagataggatagtttggctctaatattgtgttaatattcaaaccaaaatcctaagctaatagatggaagagaaatgacttatatacatgtgcattattggatatatctttatgggagaaataatcacatggatgtttatatcacacatctcatatgtgcatgttgttgtaaggcttcaaaagacagacgatgagattggtcttggatcaaattggaatgtttcttagttgaatttggagaagtctgcaacaaatcctataaaagaagtcccgaaattggtggggcacctttcgatccaagacccttcgatggataagtcaaataaagccttgagaacagattgtggaaatggaagaatagaaggatgagaaaagagattgtgaacaaatggagagaggactcttgtttccttcagtggaggagttgaaaatgattcaacaaagtctccactctatctatcccgacttaccttatggagggtatgttaccctcctttatatagaggggtgaggaggcttgctcaagttgttaggccgttaatttattataatagaatggtcagctatataaagatcatgggatgtttatccatgtgatgattagctataggatagctagaaaatatctaatgcttaattagatgatagctgtcagataaccgtctgcattcttatagtacatcgatattttatcgacgtgactagcttaaatcagcaactgactgaactgaatattatgattcttttagttaacaatcatattggttagagaccgatgtaattcatagtagatcgatcacaagctgagatgagtatcatattttaagaacaatactagcaagttagatcgatcaaatgtcagatgaaaaagtagatcagtaaacgttcgatggaacctgaaagaatatttatgatttagataataatctatcatcacgtatccagataatgagatcatataacatgtaccaatatatgccctccatttttcacaccgaagtgaagttcttcacatcgggtgtggaaagtctcttcagaagatctcacctgacctgtattgtcatcataaatgctccataccacgatggttggaagtattaattttttaatcactcaaagtcatacacaatttcttgaaaatgatttgttgaacttagtaatgatgagcgcttagaaaatcgggagctcacaattatttgggtggctagtccctaatgtgtatgtgctaggtgtcatactgtaattggccacttcagctatcacatggatcctgcttgcatggcttaatcaagaagaggtgcgtcgcaacaactctctgcagaaccatcggataactgacaagtggcattgatctaatggcatatcaaatggattgagactgttagtaaattttataaataggtctatactctgttcaaaaattactttactatttttttcacatgacagtcttgctgaaattttttcagagcccctaacatcattggtatcggagtagagaccccccaaagtcattggagccggagaagaaagaagtaaagaagtcttttaaaagcttcctcaaattcctctttacatattaggcagactctttcatcttcaacttcttttccatgaacatctgagattttaggttttacaatctttatttttttttttggatagttattcccttttctctctttttttttctgtttctcttttcccattcacctttactttcttctttcctttcaaaaatatcttttgataggactaatgagataagtcaggaccaatggatatctcggtcaacccaaccactgctcaagtttgagatggaaaatctatctcggacaacagctgaagttagtacctcaggttaggatgatctagaatctcctataagagattttttagattatttcggcccaagtactgaacaatctgtcctgaccaatctcgatctttaggaacttaagaaaaaatattcgattcagcttataactccaagttgggatggtaggattattgaacctccagaaggttatgtcgtattttatgatgaggcacttcgatctggactttaatttctcttacatcctttcttcagtaatgttttagacttctataaactccatccaatctaggttactcccaatgccattaggatgatcatagttttcattatctatcgtaaattttttgctatagaactaagaatttctctctttaggatgctggtcatcctaagaaaacatccttatgaaaaagactgatggtatttcttaccttggcctcaatataaattcggtcccactcttcctttttcaatacataattgaaaaaatcattttttctttatttcttctaatgtttcgtagggttttatttgtaaatagtctaagcctaaaaccaaatggaactcaaataacaaaatattatctgaggatgaggagacttttgtagagcttttagatatgaaagtatccaagttgagcctactggtgtccaatcagtccttgtttgacaccgacatcagtcagatctctccttaagataagtctgatgttaattctttttctttattgctttatcatttttcatcatttttcttttctaacaatctttttccttatatagtagcaataatgaagttcaacctacaaaggctggctaactcaaagaagaggaagaaggatctaaccgattgctctcaagaagagtaaggagactgctcctctaagatcgattggcccccgatcatcacctgggccaatattaattgacatagatgctacatcgatctccactataccaccagcaaaatcaactcatcaacctactaaggtggcttgtccacctcctaaagagtctgcacatccaaagtaggcatcttccccaacacctccaacatcggccaagttagtttggctgagcaatcagcatctgaggtcacagactcctgatgtcaacccaccaactttctcatcaaaaaaaaattgacttggcgaaggtatcacttttggagacacccagactaggcaaggacttgctctgtacaatgatgcctcaaaaggacctagatgctgataggagggatctttctttggagcaaataataaattatggattcaacagtatcatgaacgtgagtcttcattctcttccactctcttctttctttttcttttttttttttacattggctatttgttgatctgaatatatctttctttttgcagtcggttgtgtatttcaagttgctcaatgagcacttgacatggttcttcaaaaataaaaatttttttgaaagagaggctcaaggccaagaaagaggccaaaaaagcagttgaggaggtcaagaaggcagtaaagaagaaggctgtcaaagaaagcaaaatgatggaggggctgaagaaacagctccaagaaaaaatagattccattaaggagactggacaaccaatgacagatgaatgataaagatgacaagttgtaaaaacagcctgaaaaaaatctcaaagttggaggccaagctgaaggaggtcgagtcaataattgaaaagcatgatgaagctcttgtcccatattagagacaacttgataaagacaaagagtggatgtcaaggattattgaagattataagaattccgacacttttcaagatgacgttactgaggcctcaaaaggagctttcaattatggctttttgagctacaggagtttaattatcaagctctttcctaaccttgatctcagcaaggtcataatagaagcagctctagaagtagtagccgaagtgacttctgcaacaactactgagcttgcttccacttctatcattggagtttctccgatcgaagtcccaaacagtccaatcgaggcctccatcatcgaagctatttcgaaggaatcagtcggcaaagaccttacctcaactcctccaacaaataactcccaagctaaggcctgaattatcttcttcttttttttctaaacatttgtattagcccgatgtgggcttctataaatactttttacattaatgaatgagtttttcaatgtcaatattttttctttttaactaatactaatcttggatgatccgatctgggttggatgtctcaaaaaatatcattcacgatagatagttattttctgacttcggttagatgattatgagtatatgtaattcaaccttggttaggtaagtaatcaaatattaactattctcaaaccaagtagataacgaagtcaatgtgattaactttaacaagtaagattgttatggaatgaaattgaatcagatcaactaactatagataacttaatctctcataattcactgtaaaggttctaaaagtacctttatctaagttcgaagtgacaagtcgggttcttttattcgtggatttatgacccatgctgtctttttgtgatcttcattattaatcaccttaaatcgatatagcaaaatccagtttatagatctgagtgctttcttgtcagattgagtctatcctattatctgtgaaacctgatctagagatcaagtattttaggttttttatttaaggtccaattcgaagattgagtatccaatgtcatattgttaggtccaatttggagattggatgtctcactatcatctcgtgaggtccaatccaaagatcgaatatctcactatcatctcatgaggtccaatccagagattggatgtctcacatcatcttgtgagatccaattcgaagattggatgtctcacatcatctcatcctattgtggttggaatttttgtagccttagtttgactttttctgacctcatttggacacctaaatcttattatcatcgtttgatcgatttttactaatctactttggatgaaaaagaattcttcaatggaacttttgattagaactttatcttcattgggatagaaatcgaatgctttattgaaagattttattgataatacattctgagatttttaatatttcatgttctcgaaatgatcgtaccatctaaatttttaattcgataagctcttggatggatcacctcagtaatctgataaggtccttcccaattcgggatgagtttttcttactccattggttttgagacttcagctcattggagaaccaaatctccttataaaaaattttaggctttacctgagagttgtaatatctggctactttttgtttataaactaccatatgaatctgggctttttctcgagttttctcaaataaattgagatcagtcctcagttgatctgaattattttcttcatgaaaattttctattctggttgtaggtaaactgatctcgactagtattatagcctctgttccgaaagtaagtttaaaagatatttctctagttggtctctgaggtgtagttctgtatacccataaaatattataaaattattctaccccgagacttttagcctcaatgagttttatttttaggccttgaaagatagttctataaataaatttagcttctccatttgattgtagatgtccaatcgaagtaaatatatgatctatgtagagctcagaataaatttttttaaaattttgattatcaaattattgctcattattagtaattataactcaaggcaaaccaaaatggtaaataattatttttcacataaaatctcatattttttctcagtgatttatgtcagaggttcaatttctatccattgggtaaaataatcaatagtcacaactaaaaattttctttgctccatggccattagaaaggatcccagaatatccattctccatatagcaaaaggccacagcactgtaatagaaataagttcagttgtaggctgatgttatatattggcgtacctttgacactgatcgcagtacttattaataaagtcggttgaatctttttgaatagtaggccaataataatcttactgaattatttcataagctaaaattttaccccccaaatggttactagagattcctttatgaacttctcgaaggatgtaatcagcttccgatggccttaggcataggagcagtgggagtgaatataacctctgatataattgattatcttgaacaacataccatggggcctgtcttttaattcttgttccttcgactggatcaaccggtagaggttctttagtaatatactccattaatgggtcaatggaacttagctcatattaaatttggacaattagtaaggcctcgatactagactttttaagaatatcaataagaacaccttgatttagtttgaaaaaatctgatgtggctaaatgagatagggcatcagctcagacattttgtccttggtatttgcatgatcttcagattttcaaagttttttaataattctttcatattatataaatattgaaacatcataaaatctttagcttcaaattaatctcatacctgactgacgataaattgagaatcaataaaaattttaatttttttaacattaagctccttagccattttgagtcctacaattagcgtttcatattctactccattgtttgagtgttaaaattaaatctcaaagcacgctcactaacaatgccttctagactcgttagaattaaactagttctactttctttcgaatttgaggctccatcaatgtacagtatcaaataagaatctttgatatttttcaattcttttaagattggttcttcattaggaatagagcattcaataataaaatcagctaatacttaaactttcaatgaagatcgaggcccatattgatatcaaattcatttaattcaatagcctatttgaatatccttcttaaagtatcaagctactgtaaaattaattttaaaggttgatcgatcagaattataatagaatgagcctaaaaatacgatcaaagtcatcttgctaatgcaatgagggtataaattatcttctcaattttagaatatcgagtttcaacatctctaaataatttatttgtataataaatggatctttgtatccctgcatcatttcaagctaaaatcgaactaacagcatttgctgaaatagatagatacatgaataatttttgacctttgatcggctttgatagtaatggagctgtgccgagatatttcttgagatcatcgaaggctgcttgacattcatcttatcaatcgaagtctttgatctgccttagaattttaaagaaaggaagatatttatcagctgatctgaaaataaattaactaagcaatgctactcatccagtaagttggtgtacttctttgatggagctcggatgcttcatttcacatagagcttgaattttcttaagattgactttaattcctctttgagttacaaaaaaatctaaaaaaatttttgaagttacttcaaaagcatatttgttgggattgagcttcatttgatattttcgtagtctctaaaggcttcttccagattggcaatatactgatctgactcagtattttttactaatatatcatcaacataaactttgatattaatttcaatttgttacttaaaaatcttattaatcaagtattagtatgtagcacctacatttttaagatcaaaagacatcattttataacaatgcaaatctttttcagtgatgaaggccatattttcttcatcctcaagtgccattttgatctgatataaccagaaaaagtatccataaagcttagtaatttgtgtcttgaagtagcatcaacaagctgatcaatttttgagagagaaaaactatcttttaggcaagctttattgagatcggtataatcaacatagatccttcatttttcattagcctttttaaccatgacaacatttacaatccactttggatattatgcttctctgatgaatttgtctttcaagagtttgtcgacttcctcatctattattttttatcttttcggggtgaaacttcttttcttctgttgcattggtttatgctttggatcaacattcagcttatgtacaataagatcagttaaaatctcaggcatattagagactgactaaacaaagacatcggcattcatccgaagaaaagatattaatttctccctcagatcaggcttcaatagagatccaatttggacagttttttttggatcatcacacaaaagaacagtaataagtttctcgactggttctcctcgatttttgatgatatcaactttactttcttgatcaagtattttaattggtagagcttccacagaccttttcatttttacagctatcagaaaatactacttagcaagtatctgatttcctcatatttctccaactccatacttagtttggaattggattagtaaatgataagtgaagactatagccttaagggcgttgagcctaggtcggtcaagaatagcattataagctgatggtattttgacaataaaaaaagtgagtcttacagttgactggcatggttctatccctgcagtgacggacaaagtgacctctccttccacagctacaggatttctagaaaatccaattacgggggtaccaacctatttagctaatttatcatattcattctttggaatgtatcatagaacaatatattagcagagctttcattatcaataagtattctttttatatcatatttggctattgccataaagatgacaacagcatcattacgaggagtttgaactctaacatcatcatcgaaaaatgaaattatgtgatccatgcactgatgctttggaaggctttcagtaatctcagccacctcctcagttccgtcgagatctgagatcatattgatgactgcagcagtagacttgttgtgatcattctcattgttgggcttctatcattggtcagtagcttgacttgcccgatctcgaacatatttactaaagtaacattagtggatcaatacttcaattttatcttttaattatcgatgctcctcagtatcatggccatagtctcgatggaaatgacagtattttctcttatctctctttgctggaggggctttcataggattaggttggcgaatatatcctaaatcctcgatttctatcagtatctgagctcgaggagtagatagtgaggtatagatgtcgaatcaccgaggtgggcttttgaacttcagattcttctgaggtcgttcagagttatcctgttggtttttatgatcttcttcctagggccacttttttccatctctttttttcttcacctaacgaagtatgcatgctctctttcttttcagcttgagcatacttacaaacctagatcaatatttgttcataattgtttgggtagttcttattaagagagaagatcaggcgattactcttgagtccttgcttcaaagctgccattgcaatggactcattgaagttcttcactttcagtatggcggcattaaagcatgccacatattcttgaagagattcaccttcctactatttgatagtaaaaagattgctagtatttttcaaatgaatccatttattatcaaaatacgtgatgaatatttgctaactgtgtgaaagatgaaatagatcatgtctggaggtcagagaactagattcttgcagatgttttgagagtgattggaaaagtgatgcaaaatagggcattagataccccttgtagtcttataatggctctgaagccttcaagatgatttaagggattgatggagccatcgaatgtttccactgtaggtatcttgaatcgaggaggaactgatttaccaagaattttttgagaaaaaagagatcgtaagttgaaatctcttctaccttgagaatggcttccaatctatatctccatcattttcttctcaagattttgaatcttttgtccaagaccctcctccatacatggcttcttatgtggagcagatttcacttcccaagagtgatcagtatggtcaagaagatgatcatgatgaagatcttgaggagttggttgctaagtgtgatgtgattggactacttggggggctactttttgctaccgttctgtcgtatactacagcagtaagagcttggacctgctgaaccaagagactaaactattgtggatcaataataattgaaggttaggtattctcctgaacatcttcaggagaagatgaagtaggtaaaggatgatttggtgccttcttgttcaccatttctactaaaatattttaagtgcccttcctctaacactaatctattactgcaaggcttcaaaagacaggcaacgagatgggtcttgaatcgaactagaatgtttcttggttgaatttggcgaagtctgtaacaaatcttgcaaagaaaatctcgaaacctacgggtaccttctggttcaagatcctctgatggataagttaggtaaagtcttgagaataggttgtgaaaatagaagaatagaaggatgagaagagagattgtcggtaaatggagagatgactcttatttctttcaatgggggagctgaaaataattcagcagagtttccactctatcaatcctgacttattttgtggagggtaccttggccccttcatatataggggatgaagaggcctggtaaggttgttagactattaggagagtttgttagatcgttaatttattataatagaatgaccagctatataaaaatcatggagtatttacccacatggtgattgactgtagtataactgaaagatagctaatgcttagctggatgactgctgttagataactgtctgcattcttacggtacattgatattttaccaatgtgacatagcttaaatcggcaactggctgaactaaatattatgtatccctttagttaacaatcatgtcggttagagatcaatgtaattcgcagcagatcgatcataagctgagatgagtatcatattttaagaacaacgctgggcgagttaggccgatcaaatgtcagactgaaaaagcagatcaataaacctctgatgtgatctgaaagaatatttatgatttaaataataatctatcaccacgtatccagataatgaggtcatataacatgtaccaacagtgcatttttccatctagttaagaggttggttagtggcatttgtcttcgatatgtaatgttcacataactaatgtgcttagtagcattcttttgtaaggttaaatcttcaatgatcttaagttcacataattgcctttgtgccctattagtttatagttgaccttttaattcaagagacagtcaccttagcaatcgatgtctgcttagattgggccaattaggtactcacattaatatattgaatcatgtttgaatataaaggattagattgatttataagtttccttttattgtttacatactgatacttagattgacttactacattatttgatatgttatgttctaatttttggattaaaattgttgtttctgatttctccttacatctaatactttgtataatttattattttttagcatgattgagtgtagaggattagattgatttttaagtttattttgattatttacatgccgatacttaaattgacttactacattattcaatatgttatgtttcaattattgagttaaaatttttatttctgatttctactgatgtccagtgtgtgtgtgtgtacgtatgtgtgtatatatttatttacatatatatgtatgtatgtatacagacatacatacatacatacatacatacgtacacacacacacacacacacacacacacacacacacacacatatatatatatatatatctgtgtgtgtgtgtgtctctctctctatatatgtataagtatgtatgtatgtatgtgtatatatatatatatatatatatatatatctatatgtgtgtatgcatgtatgtatatgtatgtatgtatatacatatatgtatatatatgtatatatatgtgtatatatgtatatatatgtgtgtgtgtgtatacatatgtatacatacatatctatacatacatatgtatacatacatacatatatatgtatatatacatatacatgtatacatacatgtatacacatacatgtatacatatacatgtatacatatatgtatacatatacatatatacatatatatatatatatgtatatacgtgtgtgtgtgtgtgtaagtaattaagtatgtagtgtgtgtgtgtgtgtgtatatatatttatatctgtgtgtgtgtgtatatatgtatgtatgtatgtatgtatatatatataaatacatacatacatatttatacacacatatctatacacaaatatgtatacatatagacacacacacacgcgtgcgcgcgcgcgcgcacacacacacatatatatatatatatatagatagatagatatatgtatgtatgtatatatatatgtatatatatgtatacatatgtgtatatatgtatatatatatgtgtgtgtgtgtgtgtgtgtgtacatatgtatacatacatatctatacatatatatatatatacatatatatatacatatacatatatatatatatacataaatatatatacatatacatacatacatatatatatatatatatatatatatatatatatatatatacacatacatacatacatatacatatatacatacacacacacacatacacacatgtatacgtacatgtatgcatatacatgtatacgtacatgtatacatatacatgtatacatacatatatagatatatatatacacatatatgtatatatatatatatatatacacatatataggttatttggaacctaagaaacttgcaaagttactagatgcaatgttcggaaaccatggaccgtaacaactggagtagtatttgggtcatgaattcatggctagatcatgaattgagtgggagtcaaccgaagtagggccagctcagacacttgtatttaggtcccatgcttgcgtgca

SEQ ID NO: 5 - DNA, 678 bp, Elaeis guineensis
atggggagggggaagatagagatcaagaagatagagaatcctacaaacaggcaggtgacctactccaagaggaggacggggatcatgaagaaggctaaggaactgacggtgctttgcgatgctgaggtctcgcttatcatgttctccagcaccggcaagttctccgagtattgcagccccctttccgacaccaagaccatatttgatcgctaccagcaggtgtcagggatcaacctgtggagcgcccaatacgagaaaatgcaaaacactttgaaccatctgagggagatcaaccagaacctccgcagagaaataaggcagcggatgggtgaagatctcgacagtttgggcatccatgaactgcgcggtcttgagcaaaatttagatgaggctttgaaggttgttcgtcacagaaaataccatgtgatcaccacgcagacggatacctacaagaaaaagttgaagaactctaatgaagctcacaaaaatttactgcatgaacttgaaatgaaggacgagcacccagtttatggttttgtggatgatgaccctagcaactacgcaggtgcactggctcttgccaatggggcttcccacatgtatgctttccgtgttcagccgagccagccgaatctccatcgaatggggtttggctcccatgacctgcgccttgcttga

SEQ ID NO: 6 - protein, 225 aa, Artificial Sequence
  synthetic
MGRGKIEIKKIENPTNRQVTYSKRRTGIMKKAKELTVLCDAEVSLIMFSSTGKFSEYCSPLSDTKTIFDRYQQVSGINLWSAQYEKMQNTLNHLREINQNLRREIRQRMGEDLDSLGIHELRGLEQNLDEALKVVRHRKYHVITTQTDTYKKKLKNSNEAHKNLLHELEMKDEHPVYGFVDDDPSNYAGALALANGASHMYAFRVQPSQPNLHRMGFGSHDLRLA

SEQ ID NO: 7 - DNA, 61 bp, Artificial Sequence
  synthetic
aaattaatattgcaaactagctcaaaataattttgatcactacatttctgctgtgcattct

SEQ ID NO: 8 - DNA, 61 bp, Artificial Sequence
  synthetic
actacattttaacaccaagctcgataatagtgataaagaaacatctagatcagctttataa

SEQ ID NO: 9 - DNA, 61 bp, Artificial Sequence
  synthetic
tgcatgcatagctagaagagaatcttatcacgatcatcactcgtgaagatcatctacctgt

SEQ ID NO: 10 - DNA, 61 bp, Artificial Sequence
  synthetic
gctcgagtactgcatatttctgatacattgtctatgctagaatgtgctagaactgattatc

SEQ ID NO: 11 - DNA, 61 bp, Artificial Sequence
  synthetic
tatattaattgtcatacttctagctcgagatcatgagccaaggattgcagtaactaccgca

SEQ ID NO: 12 - DNA, 61 bp, Artificial Sequence
  synthetic
ggaatctcatcttggtagctatggccggcgatgtgagccaaagtggcaaaatcatgaatct

SEQ ID NO: 13 - DNA, 61 bp, Artificial Sequence
  synthetic
tataactaatctccaactctgccgactccttagtagtatgagcacatggaaagcttgacct

SEQ ID NO: 14 - DNA, 61 bp, Artificial Sequence
  synthetic
ataaatgagtgatagattctaatccagagacaaagagcacacctcgaattcacttgccatc

SEQ ID NO: 15 - DNA, 61 bp, Artificial Sequence
  synthetic
aagaagaactaatacagctttcatcacttcaaaatgatgaacagatgcatctcaagtcagc

SEQ ID NO: 16 - DNA, 61 bp, Artificial Sequence
  synthetic
ttgatatagaatgatcaagggagcaagtaggttcaatctttttgttggaattggatcatat

SEQ ID NO: 17 - DNA, 61 bp, Artificial Sequence
  synthetic
ggcgcagatgaatgttttatgagcatttttatagctgcagcttatatgtgatctatggtgc

SEQ ID NO: 18 - DNA, 61 bp, Artificial Sequence
  synthetic
atttgcttttggatattgcatattccactcttcaatcacctcatgccaagcaaaacattta

SEQ ID NO: 19 - DNA, 61 bp, Artificial Sequence
  synthetic
cggttgcatgccctgcagagtttgactcatgaggcatgcaaggtattgaatagtagtctag

SEQ ID NO: 20 - DNA, 61 bp, Artificial Sequence
  synthetic
cgtcagctgctcaatcatggattctgatagctcaaatggtggtaagtagaaagagagagat

SEQ ID NO: 21 - DNA, 61 bp, Artificial Sequence
  synthetic
aagattgtgcaactcatgaagattgtctccagattgaagataatttcaatacaagcacaaa

SEQ ID NO: 22 - DNA, 61 bp, Artificial Sequence
  synthetic
atcggtggatcaaatgataatacttatgatagaaacataatcaatccacttaggactatac

SEQ ID NO: 23 - DNA, 61 bp, Artificial Sequence
  synthetic
ttgaggagattaatctgacgcaaggaaaaaagaagagctgacaactagccaatgatcgaga

SEQ ID NO: 24 - DNA, 61 bp, Artificial Sequence
  synthetic
tgatctcagcaaggtcataatagaagcagctctagaagtagtagccgaagtgacttctgca

SEQ ID NO: 25 - DNA, 61 bp, Artificial Sequence
  synthetic
atattttcgtagtctctaaaggcttcttccagattggcaatatactgatctgactcagtat

SEQ ID NO: 26 - DNA, 61 bp, Artificial Sequence
  synthetic
atagctaatgcttagctggatgactgctgttagataactgtctgcattcttacggtacatt

SEQ ID NO: 27 - DNA, 61 bp, Artificial Sequence
  synthetic
aattattgagttaaaatttttatttctgatttctactgatgtccagtgtgtgtgtgtgtac

SEQ ID NO: 28 - DNA, 61 bp, Artificial Sequence
  synthetic
tcttcctcagatgacatgtgatttatgctacggcctagttctaaggacttttctctgtcat

SEQ ID NO: 29 - DNA, 61 bp, Artificial Sequence
  synthetic
cctagattaatgctgttattggatgctggcagtcagatgaagattatgtttgattgtacct

SEQ ID NO: 30 - DNA, 61 bp, Artificial Sequence
  synthetic
taaatgagtgctcatagtgacaatgtttagcctccacgtataatgtgtgccagctaactag

SEQ ID NO: 31 - DNA, 61 bp, Artificial Sequence
  synthetic
atcctcttttgtggctcacaacctcctctcctttttatgttctatgttcctcacatcacat

SEQ ID NO: 32 - DNA, 61 bp, Artificial Sequence
  synthetic
atcctttcaatctcataagaagttaaatgacatggatgacatgaagctttgatatgcatcg

SEQ ID NO: 33 - DNA, 61 bp, Artificial Sequence
  synthetic
accatcaaatggcttttggaaatatgcgggcgcagaagtagaggtgtcctatatgaaggct

SEQ ID NO: 34 - DNA, 61 bp, Artificial Sequence
  synthetic
gacgagggatcacaccaacatcatatgctctcctcaccataccaaatggtatccccaacta

SEQ ID NO: 35 - DNA, 4061 bp, Artificial Sequence
  synthetic
aaatctattagtatctgacaaaagttaaattagagtcgaaacactaaatgacaattagggatcaacttgatcaagtagatagagaatattagaaaagagagaaattaacaagatagaacatgattaattaggtgacatagcccgacaatccaattggtctaagcaagttgatttaatcaaatcacggttgaactaatatatagatagctcaataaaaatcatacataattgaatctaatgatatttggatctgaccaagatggaatttgacatgctgtccgatgatcgtgaatcaagactctctttgctaattaagatcaaattagaatcattgaaagagaatcttttactggatcaagagagagaaatatataaagagagtgaaatagtctatagaaaaaaattttagagagagaaattaagaagaaaaaataaattttttagagaaagaaagtgggtatacaagctcagagaagggagagaggaaagagagagaaatgctctcttattttcttttttttcttttttcttcttttcttttttttttcctattcttctttcccttttctgcttaatggaataggggacctcccattccccttctatttctagagttgggggctcaaaattgatgatagctatcattggggatgtaggctatggtgatgcagtagaggatcaccgaccgatgatcgatggtgatgttgcaatcaaaaaatcaagaaagatagatggaaaataaaggaaaataaggagaaatagatctcaacttgtttggatgctaacccactcactgacgactccacttcaactatggccggagcttgctatggaaaagaagccaaggccttcaaggatgaacaccaatggtgaggaagatggtcgaaaatagaagaatggctggcttttctaatcgacaaaatagggtatcgcccttcttagcaaatattcggcaataaatatctagaatccaggatcctaggactatggaagagggagaggagggcaagtcaaaggatgccagattcttatctagcttccgacaatgatggggccctattttcgataaacacaattgaggatgttcggaaaagggttttttcgatgatgattctagtgaccaactatgagatttcaaagggggtgaggggggtttaaataagatgggagggaagtttgaatcctccttaaatctgaacctttttcgacaaagccaagagcgtgaaggagactccttcgtgaagtcaaagatggaatagactcccttcgggagtttggttcatcacccaacttccctagcatgtgcggagtatgtgctagccttttctctctttttttttcattttttttcatcctttaagatccatgcagtttctaggttgagggattggggtatcacattctctctcctaaaaaaaaattattttcaaaatttttttacctatattttcaaaagttgggattcatggtccaaatctcatccttgaatttttttgatattctaattctcgaaaaaatttcatcgttaaatcatttcataagagaaaagtcaatacctcaagagttgatctgaatcaaaattattatctctagtaatcgaaatcaatatcttaatttcaaataagaatatccagtttattgtcaaaattattaactactcttgacttaattgatctattacataatcgtaaataaattctaacatactcttgaagtgtagaatataagattgataaacaatcctatatccgttctaatagatataaaagcataaactttaaatattttaaatccaagattaagaatcaatgatccacttatcctagactcaagatattagaaatttttttttgtacaatagatagaggatgtactggtgaaaatcatgtagcgatatccaaaataatttttaattaaaaatattatccttttcattatcaatgaattttatctataagaaagatcaaatcatatgatccatcttaaatttttaactcaaaaaattaatattgcaaactagctcaaaataattttgatcactacatttctgctgtgcattctaatttaaaccgttcacattttttagattcatgaaataattttgaccaaagtattactccatactatagtcaaaaaagattaaaatattagattctaattaaagccaaagataaacttttgattctcatccttaattttgcctaaagtataattattttgattaacccttaagcgcaataacacattcaaaaccaacagataggtttactataatccaaatgaattaaatcttaattcttttatcaattcatttagacaatttcaaatcaaaattctataagtaatatcaataaaaaaaatttttgatgctccaataagttagaacttaaatcaaaatatataagtaaaattgatttaatcatctcttctaaagtttcttctattaagatctttaatatctatcaaatacattccacaataatcatgcaaaccttttaaaaattaaattctcaatgcctttactacattttaacaccaagctcgataatagtgataaagaaacatctagatcagctttataatcaaaaattttgacttacaattttacgtgtgtctcaaaatcttgaataaatataaataagatcttttatcttgatccaaaaatagtaatcaaggatttcattagtaacttcaacaacaatggtaaaaaaattttctatccattgataaacccaaattttgaattgaagtttcatgcataccatatagcctttaataagatctattatttggatctaaagatagtaattaaaattgttaatgattccactaagatgaatactttacaatctcataattaatttcttcaataaaaatagacttcttgataatgtctccaattgtatatttttttttatttctacaagaaaacttcatacattttttacgttccaatataaatcttaaaaagttattccaatcaaatatcataaaagatcttcttagtccaaccttaaataacttttatgaatgaatctttatcttgccactaaataatgaattttaaaatcaagagcaacatcacagcattctgtcatgtcaaatttgtgttagatgtatgtcctagaaatcaattagattgacaatgtaaattttttaaggatataatttatatattttgatttattaataaaataaaatttaaattaatttttattcatatttttttatctatgaatcatctaaagaattaataagatgatgatacatattcttaagagttcaaaatttgaaatatatgtcattgatgattaatttctgaatacttttgaattcttaagagtttagaagatcttgacccaagtagtgtgaatagtgaaaaaaagttttcacatacttcacatcaaaaatttaagttgaataaattgtacatatgacaggtattatagtttgacgagtaatctataacctctatcttatcaaaattctgatagaaagattgtattgtatgataactgtacttagaggttcaccttttattttactggattaccactacatgttgctagatgtcactggtggattgtgagatctacgaagattatcttgatgatcgataattctcattgaaaagattgaaactattttaatgatgttgtgatagagatcataatatatcttattatcagacagaatagaattctatgggatcatacacaataggagattaagactgatcaaatagttgaatgatgattaagaatcattacggagttcagattatcaatataattgataattagactaacttataattgttacaagtagcaaggacttaactgctaaaggttaataggttcaaaaagaacttatgtataaatgttgtgcatcttaatttgattggatcaaattagttatggctgaattcaagatgaatcaaataggaatttggttcaattgaatttgggtcaagctttaggcttaggtcacatatacccaaaatcatttggatgcatcaggtgtgtgacacctgaatcaggcctttctaaactattttgagt

SEQ ID NO: 36 - DNA, 4061 bp, Artificial Sequence
  synthetic
cttttttcttcttttcttttttttttcctattcttctttcccttttctgcttaatggaataggggacctcccattccccttctatttctagagttgggggctcaaaattgatgatagctatcattggggatgtaggctatggtgatgcagtagaggatcaccgaccgatgatcgatggtgatgttgcaatcaaaaaatcaagaaagatagatggaaaataaaggaaaataaggagaaatagatctcaacttgtttggatgctaacccactcactgacgactccacttcaactatggccggagcttgctatggaaaagaagccaaggccttcaaggatgaacaccaatggtgaggaagatggtcgaaaatagaagaatggctggcttttctaatcgacaaaatagggtatcgcccttcttagcaaatattcggcaataaatatctagaatccaggatcctaggactatggaagagggagaggagggcaagtcaaaggatgccagattcttatctagcttccgacaatgatggggccctattttcgataaacacaattgaggatgttcggaaaagggttttttcgatgatgattctagtgaccaactatgagatttcaaagggggtgaggggggtttaaataagatgggagggaagtttgaatcctccttaaatctgaacctttttcgacaaagccaagagcgtgaaggagactccttcgtgaagtcaaagatggaatagactcccttcgggagtttggttcatcacccaacttccctagcatgtgcggagtatgtgctagccttttctctctttttttttcattttttttcatcctttaagatccatgcagtttctaggttgagggattggggtatcacattctctctcctaaaaaaaaattattttcaaaatttttttacctatattttcaaaagttgggattcatggtccaaatctcatccttgaatttttttgatattctaattctcgaaaaaatttcatcgttaaatcatttcataagagaaaagtcaatacctcaagagttgatctgaatcaaaattattatctctagtaatcgaaatcaatatcttaatttcaaataagaatatccagtttattgtcaaaattattaactactcttgacttaattgatctattacataatcgtaaataaattctaacatactcttgaagtgtagaatataagattgataaacaatcctatatccgttctaatagatataaaagcataaactttaaatattttaaatccaagattaagaatcaatgatccacttatcctagactcaagatattagaaatttttttttgtacaatagatagaggatgtactggtgaaaatcatgtagcgatatccaaaataatttttaattaaaaatattatccttttcattatcaatgaattttatctataagaaagatcaaatcatatgatccatcttaaatttttaactcaaaaaattaatattgcaaactagctcaaaataattttgatcactacatttctgctgtgcattctaatttaaaccgttcacattttttagattcatgaaataattttgaccaaagtattactccatactatagtcaaaaaagattaaaatattagattctaattaaagccaaagataaacttttgattctcatccttaattttgcctaaagtataattattttgattaacccttaagcgcaataacacattcaaaaccaacagataggtttactataatccaaatgaattaaatcttaattcttttatcaattcatttagacaatttcaaatcaaaattctataagtaatatcaataaaaaaaatttttgatgctccaataagttagaacttaaatcaaaatatataagtaaaattgatttaatcatctcttctaaagtttcttctattaagatctttaatatctatcaaatacattccacaataatcatgcaaaccttttaaaaattaaattctcaatgcctttactacattttaacaccaagctcgataatagtgataaagaaacatctagatcagctttataatcaaaaattttgacttacaattttacgtgtgtctcaaaatcttgaataaatataaataagatcttttatcttgatccaaaaatagtaatcaaggatttcattagtaacttcaacaacaatggtaaaaaaattttctatccattgataaacccaaattttgaattgaagtttcatgcataccatatagcctttaataagatctattatttggatctaaagatagtaattaaaattgttaatgattccactaagatgaatactttacaatctcataattaatttcttcaataaaaatagacttcttgataatgtctccaattgtatatttttttttatttctacaagaaaacttcatacattttttacgttccaatataaatcttaaaaagttattccaatcaaatatcataaaagatcttcttagtccaaccttaaataacttttatgaatgaatctttatcttgccactaaataatgaattttaaaatcaagagcaacatcacagcattctgtcatgtcaaatttgtgttagatgtatgtcctagaaatcaattagattgacaatgtaaattttttaaggatataatttatatattttgatttattaataaaataaaatttaaattaatttttattcatatttttttatctatgaatcatctaaagaattaataagatgatgatacatattcttaagagttcaaaatttgaaatatatgtcattgatgattaatttctgaatacttttgaattcttaagagtttagaagatcttgacccaagtagtgtgaatagtgaaaaaaagttttcacatacttcacatcaaaaatttaagttgaataaattgtacatatgacaggtattatagtttgacgagtaatctataacctctatcttatcaaaattctgatagaaagattgtattgtatgataactgtacttagaggttcaccttttattttactggattaccactacatgttgctagatgtcactggtggattgtgagatctacgaagattatcttgatgatcgataattctcattgaaaagattgaaactattttaatgatgttgtgatagagatcataatatatcttattatcagacagaatagaattctatgggatcatacacaataggagattaagactgatcaaatagttgaatgatgattaagaatcattacggagttcagattatcaatataattgataattagactaacttataattgttacaagtagcaaggacttaactgctaaaggttaataggttcaaaaagaacttatgtataaatgttgtgcatcttaatttgattggatcaaattagttatggctgaattcaagatgaatcaaataggaatttggttcaattgaatttgggtcaagctttaggcttaggtcacatatacccaaaatcatttggatgcatcaggtgtgtgacacctgaatcaggcctttctaaactattttgagtaagtttgatcaagtcaaaaggatccacaccctaaggtttcttgaataaaaccttaggcaccacattgaggacctataggaaactttgaccctctctcatatggggtggcacactgaggttttataaaaaccttaggcacccattttagccataaaaaaaaagctccaagggatggggcagtagccatgaagaatccttggctgtcaggactctattcaaaagagttctcaaggttttggactcttatggagccctaggatttgtttgcctataaatagatggccaccccaaggctttagataatgttagagacttgtgaagctctcccctttctcttggttgccggcccaccctctctcctctctcttccatgccccaagacttctttcttgtctccatcatcttgctgaaatttagatttcagcaagaaaagtcaagtagaagtcaaagttctaatgtagctcacaagatgttgagaacttcctccatctggcaaaggttctgcaagagagctagcatcc

SEQ ID NO: 37 - DNA, 4061 bp, Artificial Sequence
  synthetic
tcttttatcttgatccaaaaatagtaatcaaggatttcattagtaacttcaacaacaatggtaaaaaaattttctatccattgataaacccaaattttgaattgaagtttcatgcataccatatagcctttaataagatctattatttggatctaaagatagtaattaaaattgttaatgattccactaagatgaatactttacaatctcataattaatttcttcaataaaaatagacttcttgataatgtctccaattgtatatttttttttatttctacaagaaaacttcatacattttttacgttccaatataaatcttaaaaagttattccaatcaaatatcataaaagatcttcttagtccaaccttaaataacttttatgaatgaatctttatcttgccactaaataatgaattttaaaatcaagagcaacatcacagcattctgtcatgtcaaatttgtgttagatgtatgtcctagaaatcaattagattgacaatgtaaattttttaaggatataatttatatattttgatttattaataaaataaaatttaaattaatttttattcatatttttttatctatgaatcatctaaagaattaataagatgatgatacatattcttaagagttcaaaatttgaaatatatgtcattgatgattaatttctgaatacttttgaattcttaagagtttagaagatcttgacccaagtagtgtgaatagtgaaaaaaagttttcacatacttcacatcaaaaatttaagttgaataaattgtacatatgacaggtattatagtttgacgagtaatctataacctctatcttatcaaaattctgatagaaagattgtattgtatgataactgtacttagaggttcaccttttattttactggattaccactacatgttgctagatgtcactggtggattgtgagatctacgaagattatcttgatgatcgataattctcattgaaaagattgaaactattttaatgatgttgtgatagagatcataatatatcttattatcagacagaatagaattctatgggatcatacacaataggagattaagactgatcaaatagttgaatgatgattaagaatcattacggagttcagattatcaatataattgataattagactaacttataattgttacaagtagcaaggacttaactgctaaaggttaataggttcaaaaagaacttatgtataaatgttgtgcatcttaatttgattggatcaaattagttatggctgaattcaagatgaatcaaataggaatttggttcaattgaatttgggtcaagctttaggcttaggtcacatatacccaaaatcatttggatgcatcaggtgtgtgacacctgaatcaggcctttctaaactattttgagtaagtttgatcaagtcaaaaggatccacaccctaaggtttcttgaataaaaccttaggcaccacattgaggacctataggaaactttgaccctctctcatatggggtggcacactgaggttttataaaaaccttaggcacccattttagccataaaaaaaaagctccaagggatggggcagtagccatgaagaatccttggctgtcaggactctattcaaaagagttctcaaggttttggactcttatggagccctaggatttgtttgcctataaatagatggccaccccaaggctttagataatgttagagacttgtgaagctctcccctttctcttggttgccggcccaccctctctcctctctcttccatgccccaagacttctttcttgtctccatcatcttgctgaaatttagatttcagcaagaaaagtcaagtagaagtcaaagttctaatgtagctcacaagatgttgagaacttcctccatctggcaaaggttctgcaagagagctagcatcctgagaaacaaaaagattgctgatcagccctcatctccatatggatatttgtagagatcaaatgcatgcatagctagaagagaatcttatcacgatcatcactcgtgaagatcatctacctgtgcaaaggtatgagataagaaaaatattttttttatcataattcatgaatcctttgcttatattatactgagattcttggaatggattttttctctagtaaaactctagagatcagatctcaaagtcttcttcacataaaggttttgaaagttctttatatttccgctgctttgattcaaaataaattagatctattttgcctttcaacctttctcatatttattgacatataaagctttaattaatgagattaatgaaaagcatgtgcgaaatactgagaaaatcctaacagtgatatcagagctacttttgtacataagaaaaggattcaagttaaataaaatatgtttgatttaagtaaatgaatcaatcaaaatttatcctaacataagtttgtcctggtataatggtcaagaccattatgttgaaaggttatcctaggacaaaaagtctaagtaaaatctattttatttaagtaaatgaatcaattaaagtttattctaatataagattgccttagcataatggtgaagacccttatgttgaaaggttgtcctaggatggaaagtgattgatgagacaaatatatcatgaaagtatttttcacagatggaataaaatatatatattttgtttgtgaaaatgagatttcatgaatgtgtttgtcattcaatatgtgtggtgatcatcttgaattgccacaaatcctttttggattagggttgtatcatgactcacaaatcctgatggtttgcaaaattttgcattctgtagtgatagaaaccaaaagttaatccaattttggaataagattgatcaattggtatctaaggcaagtattttataatggtggttacttaattagttataaaagtacgaagagtctcctaccaatcttacacttatctagccaatttggttgattgaattctgaatttgggttgcttaagtgttaagttcactacaaatatattgcaaccatgattccgacttagtcaaccaagcctagatctcttgaatagattcatgttaattatggatttacataggatataaataaataattaaaacttgaagagatctaaatgaaaccttctcgtacatattaaatcgaatgatcttccatcattgtagatatacggatactctactgatgttgatgattttcgactagatatagtactttggttgcatcgaaaaagtacaaccactttataacatgagatgttgcagggtagagatggggttgggcccaataattgttaggtgaggatccaaatgatggctgcacttgcgtgtgaatggcgagtctgacttaattaagaaatagagctaataactattagatgaggcttcaggacttagagacttatgaccactacaacttacttgagaagcaatggataaagagtcgtctatttatcaactgacgcatcaccaataactatcagatggagtgatgtataattagtgggactatagtatccacttgaaatcttaatcgtaaaaatttttgtttctccacctgaagagcatgggagattcgaaaaaatagtgggggtagtttatttttaaaataaagctcctaaaataaactaaaataagttaaatacaaagtctaactagaatcttcttctctctgtagaaaatatctgcttccaacctctatttcatatccttaagactaattgtttgactagacccagttataaagattgactctaaaacttaaagatagtcttgagttttgaaaagatgagctatgtcctggatcaagatatcctctctctaccagcttgtcccacccctaatcaaggggcatcctatgaaaagtggttaaacgatgataacaaggcttggtgctgtgtgctgacatctatgtccattgaactccaatgccagcataagggtacaaactgtccaaggtatattgactcatctacaagagttatatagtgagtagagccatgtatctcactaggaagtatttaagagactct

SEQ ID NO: 38 - DNA, 4061 bp, Artificial Sequence
  synthetic
  misc_feature (3017)..(3951): n is a, c, g, or t
cagattatcaatataattgataattggactaacttgtaattattataagtagcaaagatttaattgctaaaggttagcagattcaaggaggacttatgtgtaaataatgtacatcttaatttgattggatcaacttagttatggctaaatttaagatgaatcaaacagggatttagtttaatcgaatttgggtcaagctttgggcttaggtcacatgcactcaaaagggtttggatacatcaagtgtgtgacacccaaaccaagcctccctaaactattttgagttggttttgaccaagtcaaaagggtccacaccctagggtttcttgaataaaaccctaggtgccacattgaggaccaattaggaaactttgacattctttcacacggagcagcacactagggtttcatgaaaaccctaggcacccattttagccataaaaggaaagctccaagggatgggatggtgccatgaagaatccctggccattgggactccattcaaaagttctctaggttttgggctcttatagagccctagggtttgtttgcctataaataggtcgctaccccaaggctttagataatgctagaggcttgtgaagctctctcctttctcttgtttgccatcccaccttctctcctctctcctccatgcctcaagacttctttcttctctccatcatcttgttgaaatttagatttcaatgagaaggatcaagtagagtcagagttctactgcagttctcaaggtgttgagaactttcttcatcaggcaaagattctgcaaaggagttagcacctcaaagaaccaagaaagttgctaatctgccctcatctccatgtggatacttatagaggccaagcatgacgagaagagccttatcacgatcatcactcgtggagatcatctacccgcgcaaaggtatgagataagaaaaaaatatttttcttatcatgattcatgaatcctttgcttatgttacattgagactcttggattagattttttctctaataaaatttcaaagattagatctcgaagtcttcttcacctaaaggtattgaaagttctttatattttcgctactttgattcaaaatagattagatttgttttgcctttcaatttttctcatatttattgagatatgaagctttaattaatgagattaataaaaagcatatgtgaaatactgagaacatcctaacaatttgagcttacaattcacttaaacaactaatgatcaaattaataatcacaatgcacaataaaaattcatgataaatctttttgttgttactttagatcaaaatccaactaatcataacatgatccacggattgcctatcatatatcaaaccctctgaattattaatcttaaacgatcttttcattcatgatcataagatttagttaaaaatcatgaagacaacttatattgtaatcatcatagatctgtatcttaacatccttagtgtttacctacctatactcatcctatgtttgattctatatatcataatttattcactaatactttgatatcatataaattatcgcatccccaatctaagatcatattggtactttaatatttcattagtgggggttatgcattagtactttgataccttatcagttgaatggttaaacactggtactttgatatcctatcagtggaggttatacgctggtactttaatatcctatcagtaagatggttaaatactgatactttgataacctcccagtgggtgttgtatgctagtactttattatcctaccaatggggcagttaaatgctactactttgatacgctaccaatgggatagttaaacgctagtaatctaatcttagcttgacataaagtaacgtcgactcgagtttagggtcgactcgagagaatgttagggttagcttgatatgaaagagggtcgctcgtcaatattttggagtcaactcttgtttatggacgatctagaaagtgtcagagtgagctcgagtactgcatatttctgatacattgtctatgctagaatgtgctagaactgattatcttctttatcaaagttgatttttgagtaacttgatgatcaatttttctaggctagacttgctttgtcaaaatgagcacttgttagtttagagaatcttcacctacacatgatctcaagcattcattagtaccaaaaatacttaagtattttgatatcatcaaaatcaattcttgggttaacacaatacttttcaaataataagcatacagatataatcctataacaatttaaattttgttcatatatcaatttctttaaaaatattatattcatcttgatagctatgaactaaatcaaaatacatactagtatacaacttttactgggagagtattagattaccagcatttaaccatcccactggcaaggtatcaaattaccaatacacaacccctatttataaagtatcaaagtaccagtgttcaactgcctcactggcaggatatcatagtactagtatttaactaccacattgacaggatatggaattatcagtatttaaccatcattagtagaattttgatgcatagtcaggctgcgagtcaaaatctatctcaaatcaaaatattgatcacatgtctaattctgtatcataattcattcccttatgctctaatattatattaattgtcatacttctagctcgagatcatgagccaaggattgcagtaactaccgcatacttatagagaactctttctataagcatacaagatattctaaatatactatcaatatatcatagagaaattaatttaaataactaaaagttaatattcaattaataaattcaactggcaaatgtatttaaaaattttacatcaaataaatcttgattaataaatattaattaataacaatagatttaaatcgaaacaaggttgatattgttagaatttgatgcctcaagattcagcccacattgagtccacagtgaggttcgcgacgaaaaatgnnnnnnnnnnnnnnnnnnnnnnnnnnnnnnnnnnnnnnnnnnnnnnnnnnnnnnnnnnnnnnnnnnnnnnnnnnnnnnnnnnnnnnnnnnnnnnnnnnnnnnnnnnnnnnnnnnnnnnnnnnnnnnnnnnnnnnnnnnnnnnnnnnnnnnnnnnnnnnnnnnnnnnnnnnnnnnnnnnnnnnnnnnnnnnnnnnnnnnnnnnnnnnnnnnnnnnnnnnnnnnnnnnnnnnnnnnnnnnnnnnnnnnnnnnnnnnnnnnnnnnnnnnnnnnnnnnnnnnnnnnnnnnnnnnnnnnnnnnnnnnnnnnnnnnnnnnnnnnnnnnnnnnnnnnnnnnnnnnnnnnnnnnnnnnnnnnnnnnnnnnnnnnnnnnnnnnnnnnnnnnnnnnnnnnnnnnnnnnnnnnnnnnnnnnnnnnnnnnnnnnnnnnnnnnnnnnnnnnnnnnnnnnnnnnnnnnnnnnnnnnnnnnnnnnnnnnnnnnnnnnnnnnnnnnnnnnnnnnnnnnnnnnnnnnnnnnnnnnnnnnnnnnnnnnnnnnnnnnnnnnnnnnnnnnnnnnnnnnnnnnnnnnnnnnnnnnnnnnnnnnnnnnnnnnnnnnnnnnnnnnnnnnnnnnnnnnnnnnnnnnnnnnnnnnnnnnnnnnnnnnnnnnnnnnnnnnnnnnnnnnnnnnnnnnnnnnnnnnnnnnnnnnnnnnnnnnnnnnnnnnnnnnnnnnnnnnnnnnnnnnnnnnnnnnnnnnnnnnnnnnnnnnnnnnnnnnnnnnnnnnnnnnnnnnnnnnnnnnnnnnnnnnnnnnnnnnnnnnnnnnnnnnnnnnnnnnnnnnnnnnnnnnnnnnnnnnnnnnnnnnnnnnnnnnnnnnnnnnnnnnnnnnnnnnnnnnnnnnnnnnnnnnnnnnnnnnnnnnnnnnnnnnnnnnnnnnnnnnnnnnnnnnnnnnnnnnnagatattactaaattttgcttctaatctcactcttaaatagtacttacctttgaaactaggcatttgaatctgaaaaagaaagaggagattatgagcttgatagttcagt

SEQ ID NO: 39 - DNA, 4061 bp, Artificial Sequence
  synthetic
  misc_feature (2337)..(3271): n is a, c, g, or t
catcatcttgttgaaatttagatttcaatgagaaggatcaagtagagtcagagttctactgcagttctcaaggtgttgagaactttcttcatcaggcaaagattctgcaaaggagttagcacctcaaagaaccaagaaagttgctaatctgccctcatctccatgtggatacttatagaggccaagcatgacgagaagagccttatcacgatcatcactcgtggagatcatctacccgcgcaaaggtatgagataagaaaaaaatatttttcttatcatgattcatgaatcctttgcttatgttacattgagactcttggattagattttttctctaataaaatttcaaagattagatctcgaagtcttcttcacctaaaggtattgaaagttctttatattttcgctactttgattcaaaatagattagatttgttttgcctttcaatttttctcatatttattgagatatgaagctttaattaatgagattaataaaaagcatatgtgaaatactgagaacatcctaacaatttgagcttacaattcacttaaacaactaatgatcaaattaataatcacaatgcacaataaaaattcatgataaatctttttgttgttactttagatcaaaatccaactaatcataacatgatccacggattgcctatcatatatcaaaccctctgaattattaatcttaaacgatcttttcattcatgatcataagatttagttaaaaatcatgaagacaacttatattgtaatcatcatagatctgtatcttaacatccttagtgtttacctacctatactcatcctatgtttgattctatatatcataatttattcactaatactttgatatcatataaattatcgcatccccaatctaagatcatattggtactttaatatttcattagtgggggttatgcattagtactttgataccttatcagttgaatggttaaacactggtactttgatatcctatcagtggaggttatacgctggtactttaatatcctatcagtaagatggttaaatactgatactttgataacctcccagtgggtgttgtatgctagtactttattatcctaccaatggggcagttaaatgctactactttgatacgctaccaatgggatagttaaacgctagtaatctaatcttagcttgacataaagtaacgtcgactcgagtttagggtcgactcgagagaatgttagggttagcttgatatgaaagagggtcgctcgtcaatattttggagtcaactcttgtttatggacgatctagaaagtgtcagagtgagctcgagtactgcatatttctgatacattgtctatgctagaatgtgctagaactgattatcttctttatcaaagttgatttttgagtaacttgatgatcaatttttctaggctagacttgctttgtcaaaatgagcacttgttagtttagagaatcttcacctacacatgatctcaagcattcattagtaccaaaaatacttaagtattttgatatcatcaaaatcaattcttgggttaacacaatacttttcaaataataagcatacagatataatcctataacaatttaaattttgttcatatatcaatttctttaaaaatattatattcatcttgatagctatgaactaaatcaaaatacatactagtatacaacttttactgggagagtattagattaccagcatttaaccatcccactggcaaggtatcaaattaccaatacacaacccctatttataaagtatcaaagtaccagtgttcaactgcctcactggcaggatatcatagtactagtatttaactaccacattgacaggatatggaattatcagtatttaaccatcattagtagaattttgatgcatagtcaggctgcgagtcaaaatctatctcaaatcaaaatattgatcacatgtctaattctgtatcataattcattcccttatgctctaatattatattaattgtcatacttctagctcgagatcatgagccaaggattgcagtaactaccgcatacttatagagaactctttctataagcatacaagatattctaaatatactatcaatatatcatagagaaattaatttaaataactaaaagttaatattcaattaataaattcaactggcaaatgtatttaaaaattttacatcaaataaatcttgattaataaatattaattaataacaatagatttaaatcgaaacaaggttgatattgttagaatttgatgcctcaagattcagcccacattgagtccacagtgaggttcgcgacgaaaaatgnnnnnnnnnnnnnnnnnnnnnnnnnnnnnnnnnnnnnnnnnnnnnnnnnnnnnnnnnnnnnnnnnnnnnnnnnnnnnnnnnnnnnnnnnnnnnnnnnnnnnnnnnnnnnnnnnnnnnnnnnnnnnnnnnnnnnnnnnnnnnnnnnnnnnnnnnnnnnnnnnnnnnnnnnnnnnnnnnnnnnnnnnnnnnnnnnnnnnnnnnnnnnnnnnnnnnnnnnnnnnnnnnnnnnnnnnnnnnnnnnnnnnnnnnnnnnnnnnnnnnnnnnnnnnnnnnnnnnnnnnnnnnnnnnnnnnnnnnnnnnnnnnnnnnnnnnnnnnnnnnnnnnnnnnnnnnnnnnnnnnnnnnnnnnnnnnnnnnnnnnnnnnnnnnnnnnnnnnnnnnnnnnnnnnnnnnnnnnnnnnnnnnnnnnnnnnnnnnnnnnnnnnnnnnnnnnnnnnnnnnnnnnnnnnnnnnnnnnnnnnnnnnnnnnnnnnnnnnnnnnnnnnnnnnnnnnnnnnnnnnnnnnnnnnnnnnnnnnnnnnnnnnnnnnnnnnnnnnnnnnnnnnnnnnnnnnnnnnnnnnnnnnnnnnnnnnnnnnnnnnnnnnnnnnnnnnnnnnnnnnnnnnnnnnnnnnnnnnnnnnnnnnnnnnnnnnnnnnnnnnnnnnnnnnnnnnnnnnnnnnnnnnnnnnnnnnnnnnnnnnnnnnnnnnnnnnnnnnnnnnnnnnnnnnnnnnnnnnnnnnnnnnnnnnnnnnnnnnnnnnnnnnnnnnnnnnnnnnnnnnnnnnnnnnnnnnnnnnnnnnnnnnnnnnnnnnnnnnnnnnnnnnnnnnnnnnnnnnnnnnnnnnnnnnnnnnnnnnnnnnnnnnnnnnnnnnnnnnnnnnnnnnnnnnnnnnnnnnnnnnnnnnnnnnnnnnnnnnnnnnnnnnnnnnnnnnnnnnnnnnnnnnnnnnnnnnnnagatattactaaattttgcttctaatctcactcttaaatagtacttacctttgaaactaggcatttgaatctgaaaaagaaagaggagattatgagcttgatagttcagtaaatcatgaataaattagctaaataaatctatgaataatagtatattaaaaataaatatgtaagatacaataattcaaaaatgaattcatatatataatactttccaaataataagtatgtggctgcaatcctttcgtaattcaaattttgttcattaattatttttttcaaaacatcacatggatagtcatgaactaaatcaaagtaccagtgcataacccctattgataaagaatcaaataacaagtgtttgactgcctcattatcaggatatcaaattattaatgcataacctccactgctagggtatcaaagtagcaacctcaatcacctcactggaagggcatctagtttcagtatttaactactccactggcaaggtgttaaattatcaatatttaacctccactgataggattttgatatatagtcagactgcgagccaaaattcatttcaaaccaaaatatttttctcaaagacatattttatgtttcacattgaaaaattcacaaaaattatgcgatattgaaatcaattggataaaatccacgtcaaatttagtatattcaatcataaatcatttactattctagaaaaggtatattaaaagtataatgcatcaatttcataaatcataaatatctcaatataaaaaatattttattatttattaataaa

SEQ ID NO: 40 - DNA, 4061 bp, Artificial Sequence
  synthetic
agtatattcaatcataaatcatttactattctagaaaaggtatattaaaagtataatgcatcaatttcataaatcataaatatctcaatataaaaaatattttattatttattaataaatctaggagaagtgaagcattacttatcttgtaagtaaaactaaccaactgatcaaattaattctgagaatctttctcaaaactcatcaccactatatcaaaaacttgtgcttcttgctatgtaagagcatagaccctttcttcgatctggggttccaagtttctattttattttgttcaactatcaaattagactgacttttcatttttttgtggatattcagctattttatggcctttctaacaataaccaaagtatgtaccaatattccaacaataatcatttattgcatgattttcaccgcatcgaaatatttgatattatcaatcaatccaaacttgttattcactgacctcttattcaaacccttagtatatttaatattctacctttgtgattcattcaatcgatttcttttttttattttctttccctttctatatgctcttcattaacttttctttcaattatcaatgctttattcaatacatctgtataagtagttaactcatatagtaccatttattttctaatttctatcctcaattccaactcaaatttatctactcagtcacattcatcttcaaccaatctcgaagcaaacttgacaagctccataaatttagcttcatattctacaactattatatttctttatttcagataaataaatttttattctttctgaatcctcatactctaagaaaaatatttttatcataaaatatcttttgaaatcactcccaagcgagttgttctccatcttgttcatatttaggtttcattctctattatcaattaaatgtctcatctttcaacatgtatgatgcatataagattttttcatcatcatggtatctcttaacaataaatgctttctccatctccataagctaatttttagctcctatttcatagttttcttaaaagtcaatggagacaacttcttaaattctatgatattactttattgctcctattgctcttatgtccttgtggtgacaatatttattgttgcacttgctgtagaggcagttactgttactgcaattgctattacgattccatcaagccgactagtgtctgcattatttggataatagttgatttttgctactttatttagatgttggtggcaaaatcaatgacttctttttgctgagagatgccaccaacctactaagtatcatcatcttattggttgatacctttagcagcacctcgagtggttctttttatctgatatggaaccatcttaatcttgcatgaaaaacaaacttcgcaaaattttcttttaaaatctaatatctaatattatacttttattaaaatttaattatgattattttaagaataaaaaatttaaattttgaaatcctcacaaggctggccaagagataatgaccatcatcctagtcggtttgacgtaggacatccaaagatcaactataattcaagcatcatattgagatgctaggatataatcgatggtgaaatttaatgatgctcgactgatcaagatgggggccggcccgatggcctgttcaacaatcattgatcaaaattttttaaccaaggtctatcaagatcattaaaaagtctttctaagatctataaattgtaataaagagacacaatctagagagagacactttttacataaagaaagtagaaattttagggagagaaattagagagaaaggggaaagagagaggaagctgagaggaagaaagaaaagagaaagactctctctctttttcttttctttcttttctttcttttctttttcttttctttttttcttccttttctttctttctttctttggctcattagaaaaataggggacctattgatccccttgtttcctaaataggggaggaatctcatcttggtagctatggccggcgatgtgagccaaagtggcaaaatcatgaatctcccaacttgcagccgacattgacttttggcactggaaaatcaaagaaatttgacaaaaaatgggaaaaaattgaaaccaaaatagggaccaaaatccggtaatagctagccaaaaatccttgatctttgctcatggaggataggaaaaaagattattcaagagattaagggaatcttatctcatttttttgctgtgcttcggccatggtggttgcagaaatcgtttgtgaaagctcgacaaactctgcaatttcctcgggcttgggcctcgatctttaataggagaagagagaagtcctctttcttttaaatagagtcggagggaaggagtttgatttcctccttatggtggtttcaaactctgatcggaagtccattggaaaagaagactcccattagttttaaaatctaataagatttattgattagaaaattgataaaaaatgattattaaaaaagtagcataattatttaaatcaatgatgcttagattgttggaggtaaatagtaataaaatcaaaaaattaaaattcatgggaccaaaaaataatgaacaagatttgaaagaaatgtctataaataagaatttatgaaacaggggaacattgatcaaaggtgtgttaaatagtgtccttaaagtgttattgtccctctcacgtagactttgtgtgttgggagagaacatagtaattctctcaacctatgcaacctaaatcttttgaaaagaaatttaaaattatagaaaaattggcaaactagaattttggtcattttctttattagtaaaaaatatactaagttatatgtctttatttatactagtgaggtctatctttgcacaattcagaccaaatttatattctagttaaaagaggtatagattttttaaaatagatataactagtggaaatagtcatagaaaagttaaaaatcaatgaaaggtagatttcacttctatattggctttatttgtggtcactttatctaattcttttttttgatggagcaatataccctgttaaaatcttctcgatttttttttcactttaagcaacctatttcgatgcctaaacaatggaatttagtttaaccacttaatatgctacacttttaaaaggagcaccatattgtagggcttgaaaagttacttgatttaaaaaaagagcatcttaattggacatcatacaagtaagttatgacctctgaaaatttgatacatgatttatcatcttgatatggtaaatcttgttaagatttcctcatggtgtctaaagtggccggttcatactgagtttggtgattcttctggtcaatggttaattgctcgaatatttttaagatataactaatctccaactctgccgactccttagtagtatgagcacatggaaagcttgacctaattgatttcttaaattgcttgaaatcagtacttagaaaatatgcaaaatggatgaaatgtttattgcagcgagagctttctgatctgtacgaccgagagcttactagttttttatgagctatacgttttgcacttaagcctaatttaaatagtgaaatagttttgcaacaattcaaaacaattaaaatcaaaagacaagctgctatgcatgttcaactgactcggctttcaatcgcaatatgtcacataggctggcctagaatgcagatgcgtgcgtggtgagcatcctaaaaacctacatatccaataaattcccactagttggtgaagtattaaatgtaactcgtattaactttttaatgtaggactaaagtttattcgactaattaagaactaaatactttaataattgaacttttccaaccagaaatcagaaaatatttaagtaattaaatattacataataactagatcaaaatatcatggttcctctctcgctcgagatcaattgggatgttggtttatcttggtcatccatcgagatgactctatcttagcctttcaaaacggcgcggtaccacgggtctcaccgcttcgt

SEQ ID NO: 41 - DNA, 4061 bp, Artificial Sequence
  synthetic
caaaattttcttttaaaatctaatatctaatattatacttttattaaaatttaattatgattattttaagaataaaaaatttaaattttgaaatcctcacaaggctggccaagagataatgaccatcatcctagtcggtttgacgtaggacatccaaagatcaactataattcaagcatcatattgagatgctaggatataatcgatggtgaaatttaatgatgctcgactgatcaagatgggggccggcccgatggcctgttcaacaatcattgatcaaaattttttaaccaaggtctatcaagatcattaaaaagtctttctaagatctataaattgtaataaagagacacaatctagagagagacactttttacataaagaaagtagaaattttagggagagaaattagagagaaaggggaaagagagaggaagctgagaggaagaaagaaaagagaaagactctctctctttttcttttctttcttttctttcttttctttttcttttctttttttcttccttttctttctttctttctttggctcattagaaaaataggggacctattgatccccttgtttcctaaataggggaggaatctcatcttggtagctatggccggcgatgtgagccaaagtggcaaaatcatgaatctcccaacttgcagccgacattgacttttggcactggaaaatcaaagaaatttgacaaaaaatgggaaaaaattgaaaccaaaatagggaccaaaatccggtaatagctagccaaaaatccttgatctttgctcatggaggataggaaaaaagattattcaagagattaagggaatcttatctcatttttttgctgtgcttcggccatggtggttgcagaaatcgtttgtgaaagctcgacaaactctgcaatttcctcgggcttgggcctcgatctttaataggagaagagagaagtcctctttcttttaaatagagtcggagggaaggagtttgatttcctccttatggtggtttcaaactctgatcggaagtccattggaaaagaagactcccattagttttaaaatctaataagatttattgattagaaaattgataaaaaatgattattaaaaaagtagcataattatttaaatcaatgatgcttagattgttggaggtaaatagtaataaaatcaaaaaattaaaattcatgggaccaaaaaataatgaacaagatttgaaagaaatgtctataaataagaatttatgaaacaggggaacattgatcaaaggtgtgttaaatagtgtccttaaagtgttattgtccctctcacgtagactttgtgtgttgggagagaacatagtaattctctcaacctatgcaacctaaatcttttgaaaagaaatttaaaattatagaaaaattggcaaactagaattttggtcattttctttattagtaaaaaatatactaagttatatgtctttatttatactagtgaggtctatctttgcacaattcagaccaaatttatattctagttaaaagaggtatagattttttaaaatagatataactagtggaaatagtcatagaaaagttaaaaatcaatgaaaggtagatttcacttctatattggctttatttgtggtcactttatctaattcttttttttgatggagcaatataccctgttaaaatcttctcgatttttttttcactttaagcaacctatttcgatgcctaaacaatggaatttagtttaaccacttaatatgctacacttttaaaaggagcaccatattgtagggcttgaaaagttacttgatttaaaaaaagagcatcttaattggacatcatacaagtaagttatgacctctgaaaatttgatacatgatttatcatcttgatatggtaaatcttgttaagatttcctcatggtgtctaaagtggccggttcatactgagtttggtgattcttctggtcaatggttaattgctcgaatatttttaagatataactaatctccaactctgccgactccttagtagtatgagcacatggaaagcttgacctaattgatttcttaaattgcttgaaatcagtacttagaaaatatgcaaaatggatgaaatgtttattgcagcgagagctttctgatctgtacgaccgagagcttactagttttttatgagctatacgttttgcacttaagcctaatttaaatagtgaaatagttttgcaacaattcaaaacaattaaaatcaaaagacaagctgctatgcatgttcaactgactcggctttcaatcgcaatatgtcacataggctggcctagaatgcagatgcgtgcgtggtgagcatcctaaaaacctacatatccaataaattcccactagttggtgaagtattaaatgtaactcgtattaactttttaatgtaggactaaagtttattcgactaattaagaactaaatactttaataattgaacttttccaaccagaaatcagaaaatatttaagtaattaaatattacataataactagatcaaaatatcatggttcctctctcgctcgagatcaattgggatgttggtttatcttggtcatccatcgagatgactctatcttagcctttcaaaacggcgcggtaccacgggtctcaccgcttcgttacatcgaatgccaccatcccttttttttttttttttatttatttatgctttcttgctcctagattggtgcggcctcattacaactccactgctacttgatgcttccctctagcatctcctttgcagctctctcacttccaccactcttcggcctaatgttgggaaacgacgaaggggccttacaaaaatgtcatccatgatggcagtggagaagaaaacatcgctggggctttccttcgatatccttcgcagccaaagctcttatagggttatatgggagaacgctgcattatttgggtgatctttttggatggtgttgttgactgatgctagttttgcttcatgaattgaatatttacacaagatgagaatacaatctagtacaattggtaccaattacctgggtttgactcctgctcgcatctgattgaagcttggttaatgtgcatctcaattaattcagaaagatcatcggacttcatgtgaattattttgactagcatgaatagggctaaataaggctgaaatatgtgttaaatttttaaaattataacttgatcatatgatgtccaattgagatgttttcaaatcaaaaatttttttcgagatttatcacttaatgttaaactcttagaaggtcgaaacagactgaaagttttcttttcaagatgtattttgaccgagtatataacttgatgatcatatgatgcccaattgagatgttttcaaatgaaaattttttttgagatttatgacttaatgttaaactcttaaaaggtcgaaacagactgaaagttttcttttcaagatgtattttgaccaaatatatctcataatctataaagaatatatttcataatctatgaataattagatagagcgacagaagataatgctaatgtaaaaatcacgatctattttttataaaatttaatatttttatataatcacttttactatagtcatatttattttaaaaaatttagttatatttaaaatatcaaaaaaatttgacttgaattatataagaaaggatcttcctactattatagatagaagctttatatcatagtttacagtgtatggatcatcaatgaaagaaagagggatgtaaaccttacttttgaaatttttctatttgtttctaaattttttaaaggatccaagttgagaattgagagaattctttctttctgcaaatcaaatcattagtataatccacatggagacgttgtaatagaaagtagaaactatattttatgaataatagaaagggagttgatttacgccaagccttttgtttgcttgattaattatttatttttatggtgttagctggaccccatgaatagcaaccatcgttgggtcagggtcgtgtatttgttttggggtcttcatta

SEQ ID NO: 42 - DNA, 4061 bp, Artificial Sequence
  synthetic
caagtactccagaatcaaaattgtgaaagaaaaataggataaatctggttaagctgtaatttatttacttactttctatctatattaaaattattcagattattttgcaaatttatggatatgcttgaatcacgtatctgatactttctcttcatctggatggcagtaccatgtgatcaccacgcagacggatacctacaagaaaaaggcaaggctaacatgctttcttaccatcattctttacggtctttgatccggttttgcgtgtccacttcttacgtagtctttttcaaacattcctatctaagactgaaggtaatgatttgcaaaggaatagctttactgttttcctctaagtagatgaaatattactcacgtagaaaggagccatcataattgcagaaagaataaaactgaatggaatatgagtagaattgtcaaaatcttggtttaagggttttaatagccagatgagaaagcaacctacttttcttgaacaacttgtttgtgactgtcttgttgctcccatcttgcatctatgattagcaaaatatatgataaatagatattcagatttgatcgaaaagaaggaagattttctttaatccatttaatttgaatctcacaaaaaaaaagtagaagatttggacacgatcgctgggggcagcacgctcttaatagaatggtgtcacgttgcagatctcgaaaaattattcaattttttttaaaaaaaaagagtcattgaaattagacgttgtatgaccatgttatgatctctgaaagtttgacttctgactcaacttcccaatgtagcagattttactcctgaaccatgtttaacctcctgactcatagtggccaaagtatctacatcgagttcactggtcttcttggatcacattcataagaatacttcccataattttgctcaacgttgtttttctcatcaaccaaaggtatatgctttttaaaattgaaatgcccatgaatattatggcattcttttatttgacattttggttgatcctatattgtttgtttggcattcaacacttcttcatgggaacctttgaaatgaggtaggtgctaggatttttctttttacctatccatatcatatttccaatgtcttcttttacattaggttctttagtgacaataggggaaacgacccaatataatacccttgaaaatttgggcaatatctactaaaactaacttgaataaaatattaacataaaaagggatttagtaacataaaagcataactcaaaatcactcaccttgtgtgccacgttctcattgcccttattatttttgcattgtgaattgtgtcccccaataaagcaacgtgaatggtggaagagagttgaatggctttgttgagtaattgttttgagttactatagcattgctctactaaaattgaaatcttgctgtgaggctatgtatgagaagcaagttcatgctttttgactgttgggatggaagtatgagcaatctttttaatagaaaatggacgaatcatgaagtttttcctttttattgaaaaagatgatcgaaaaatatgtgcaagatagaaaaacactgaaaagataaaatgagaagtaaaagtggaagtctaggagaagaaaatttaagagaaatatcttcaatgagaggatgtgtgcaccaacaaagccaactttcactaaagaatgtaatgactcacctctactttcttcgaataaggggttcccagttgtggaaagtatatagaatcttctgaaagactgagtaaatggagcaattccttctaagaaatattatggcatttctctcccacgaaatttcaaagcaaagagcagctagtagttgatcctctaatctcttaattgaagtttggaatttctcttgcctctatttggcccaaaggtcatgaagatctaccggccaacctcttaagttgaattagatcttaatagaagtccaaatgcttcttgtagaagaacatctaataaataaatgagtgatagattctaatccagagacaaagagcacacctcgaattcacttgccatccttttctagctagaacttctctagcatgaaacttgttccttaaggcaagccaaataaatactcacattttaggaatgactgccttccaaataattttataatatggacaaattagaccaccattattgataaacttgcaatgaacaattataaatgagttttcaggttggcacattagcaatataggatggtttgattattaaaaggatgatatgaagggtttcaaggtggtttgcctcgttcaaatcaaaggattttgaagattaatattccaagataaggttctccaactccattaggaaagtgtcttcatgtcatcttagagaagcagctcgtaccaaacttgacagatgttttatttatttagagtgacacagataccctttggcaatactctccatccttgtccgaacaacttctaatcacacctcacttatcttgcatctaactcagaggctacaagttacacctttcaacaaaccttttcggtttgaaaatttgtgatttcattatttagagttcgaagagcatatcaagtattggtcggagttggcacccaaagcaaacgaaacagttactgacatggtccaaaagctgagatttctaagatcccaacttaagcactgaataaagccattatgggaaatatcattttaacgaaagaggaatttagagtaagaattgattctcttgataccgaagaagaactaatacagctttcatcacttcaaaatgatgaacagatgcatctcaagtcagcactagaccatcttctaaaataggaagatctatggaagcaacactcccaaatgcagtggcttcaaaatggggattgcaatacgaagtttatccatgtttgggcaagtaacaggaaaaaaagaatactatcactgaactctagcaaggcgatcagaagattatcgaatagcagcaaatccaatccacattctacaactttttttctaccctactaggctcgactgaggaatgactcatccaagctgattggaagattctttatccagaaggacctctggatcttgctgacattgagtatccatttatggagaaagaaatccatgatacagtgtatgacttggctttggaaaagtcacccggatgatattttcccattctccttctataagcacttctagtgtatcatcaaacatgacctgatgaacctactgtaaaatcagctaatgtagaccatctgaactacttgttcatcacccttatcccaaaaaaaaattggtgtgtattcagttagagacttcaggccaataagcctgattaatggagtaataaaaaatatttcaaaaactctatcgaaaaggctcccacagaaaatgaatttgttaattttatccacagagcttgctttcaacagaggaagaaatatctctgaatattttgtaatgactatggaaactatacacttctgcaaagctgaagtacacaaggatctcaattataaagtcgacttcgagaaagcttttgacaatgtggattggagctttctattgaaattgctatccagcacggggctttgattcgaggtggtgtcaatggatagaatatctgatttatacagctaaattctcagtccttattaatggtgataaaggtaaactttttaaattgaggaaagatctcaggcaaggagatcctctattcgcctagctctttctcttagttgttgatatagaatgatcaagggagcaagtaggttcaatctttttgttggaattggatcatataatatcatgggataacttcaaagcttttagttcactgatgacacacttatattttgcagatatgatctaaaatacatcaaaactcttaaatttttactctatagttatgagctactgatgggtctcaaaattaactttgaaaaattccaattttttggcttgagaattgcaaagatgtcagtacagcaagttgcatctatcctagaaagcaaggtggctacattttccattacttatttg

SEQ ID NO: 43 - DNA, 4061 bp, Artificial Sequence
  synthetic
gaccatgttatgatctctgaaagtttgacttctgactcaacttcccaatgtagcagattttactcctgaaccatgtttaacctcctgactcatagtggccaaagtatctacatcgagttcactggtcttcttggatcacattcataagaatacttcccataattttgctcaacgttgtttttctcatcaaccaaaggtatatgctttttaaaattgaaatgcccatgaatattatggcattcttttatttgacattttggttgatcctatattgtttgtttggcattcaacacttcttcatgggaacctttgaaatgaggtaggtgctaggatttttctttttacctatccatatcatatttccaatgtcttcttttacattaggttctttagtgacaataggggaaacgacccaatataatacccttgaaaatttgggcaatatctactaaaactaacttgaataaaatattaacataaaaagggatttagtaacataaaagcataactcaaaatcactcaccttgtgtgccacgttctcattgcccttattatttttgcattgtgaattgtgtcccccaataaagcaacgtgaatggtggaagagagttgaatggctttgttgagtaattgttttgagttactatagcattgctctactaaaattgaaatcttgctgtgaggctatgtatgagaagcaagttcatgctttttgactgttgggatggaagtatgagcaatctttttaatagaaaatggacgaatcatgaagtttttcctttttattgaaaaagatgatcgaaaaatatgtgcaagatagaaaaacactgaaaagataaaatgagaagtaaaagtggaagtctaggagaagaaaatttaagagaaatatcttcaatgagaggatgtgtgcaccaacaaagccaactttcactaaagaatgtaatgactcacctctactttcttcgaataaggggttcccagttgtggaaagtatatagaatcttctgaaagactgagtaaatggagcaattccttctaagaaatattatggcatttctctcccacgaaatttcaaagcaaagagcagctagtagttgatcctctaatctcttaattgaagtttggaatttctcttgcctctatttggcccaaaggtcatgaagatctaccggccaacctcttaagttgaattagatcttaatagaagtccaaatgcttcttgtagaagaacatctaataaataaatgagtgatagattctaatccagagacaaagagcacacctcgaattcacttgccatccttttctagctagaacttctctagcatgaaacttgttccttaaggcaagccaaataaatactcacattttaggaatgactgccttccaaataattttataatatggacaaattagaccaccattattgataaacttgcaatgaacaattataaatgagttttcaggttggcacattagcaatataggatggtttgattattaaaaggatgatatgaagggtttcaaggtggtttgcctcgttcaaatcaaaggattttgaagattaatattccaagataaggttctccaactccattaggaaagtgtcttcatgtcatcttagagaagcagctcgtaccaaacttgacagatgttttatttatttagagtgacacagataccctttggcaatactctccatccttgtccgaacaacttctaatcacacctcacttatcttgcatctaactcagaggctacaagttacacctttcaacaaaccttttcggtttgaaaatttgtgatttcattatttagagttcgaagagcatatcaagtattggtcggagttggcacccaaagcaaacgaaacagttactgacatggtccaaaagctgagatttctaagatcccaacttaagcactgaataaagccattatgggaaatatcattttaacgaaagaggaatttagagtaagaattgattctcttgataccgaagaagaactaatacagctttcatcacttcaaaatgatgaacagatgcatctcaagtcagcactagaccatcttctaaaataggaagatctatggaagcaacactcccaaatgcagtggcttcaaaatggggattgcaatacgaagtttatccatgtttgggcaagtaacaggaaaaaaagaatactatcactgaactctagcaaggcgatcagaagattatcgaatagcagcaaatccaatccacattctacaactttttttctaccctactaggctcgactgaggaatgactcatccaagctgattggaagattctttatccagaaggacctctggatcttgctgacattgagtatccatttatggagaaagaaatccatgatacagtgtatgacttggctttggaaaagtcacccggatgatattttcccattctccttctataagcacttctagtgtatcatcaaacatgacctgatgaacctactgtaaaatcagctaatgtagaccatctgaactacttgttcatcacccttatcccaaaaaaaaattggtgtgtattcagttagagacttcaggccaataagcctgattaatggagtaataaaaaatatttcaaaaactctatcgaaaaggctcccacagaaaatgaatttgttaattttatccacagagcttgctttcaacagaggaagaaatatctctgaatattttgtaatgactatggaaactatacacttctgcaaagctgaagtacacaaggatctcaattataaagtcgacttcgagaaagcttttgacaatgtggattggagctttctattgaaattgctatccagcacggggctttgattcgaggtggtgtcaatggatagaatatctgatttatacagctaaattctcagtccttattaatggtgataaaggtaaactttttaaattgaggaaagatctcaggcaaggagatcctctattcgcctagctctttctcttagttgttgatatagaatgatcaagggagcaagtaggttcaatctttttgttggaattggatcatataatatcatgggataacttcaaagcttttagttcactgatgacacacttatattttgcagatatgatctaaaatacatcaaaactcttaaatttttactctatagttatgagctactgatgggtctcaaaattaactttgaaaaattccaattttttggcttgagaattgcaaagatgtcagtacagcaagttgcatctatcctagaaagcaaggtggctacattttccattacttatttgggtctcccactccatcattctaaactgaggaaaacttattggaatccactccttgagaaggttcagaagaaattgatcgggtagaaaggtaaacttcttaacctctagggtaggcttatactaactaatgcagtgcttacagggatcccactactctggagggatacattccttctccctcaattcattatcaaataaattgataaaatccatcgatcattcatttggagaggaaacgaggagtataactaagggcactctagaatatgttggtcgaatatttgtcgatcaaaaaaatttggaggactgggggttcctcaatctaaaaattttcaatacaattcttctttgtaaatggtggtggaagctctactctaatgctggtgacccgtggtgtagttttattgccactgtccacccaacttcacactagagatctaaaggtatacacaaatcaacctcttcattttggaatggtttacagcacacatgaaatatttctactcctaatccactttcaagttagcaactagtattattttggaaagatagttggttacataatcatccactgaaggatcgatttcctcacctttacacaatagcattgaagtgcaacaactcagtggcaaaggtattaagcaatctacttgataatagctcttttagtactcctcttcctcaaagataccaagaagattttcagagtctataggaaagcattgaacaaattacattaacggaacgacctgatactata

SEQ ID NO: 44 - DNA, 4061 bp, Artificial Sequence
  synthetic
tcttctgaaagactgagtaaatggagcaattccttctaagaaatattatggcatttctctcccacgaaatttcaaagcaaagagcagctagtagttgatcctctaatctcttaattgaagtttggaatttctcttgcctctatttggcccaaaggtcatgaagatctaccggccaacctcttaagttgaattagatcttaatagaagtccaaatgcttcttgtagaagaacatctaataaataaatgagtgatagattctaatccagagacaaagagcacacctcgaattcacttgccatccttttctagctagaacttctctagcatgaaacttgttccttaaggcaagccaaataaatactcacattttaggaatgactgccttccaaataattttataatatggacaaattagaccaccattattgataaacttgcaatgaacaattataaatgagttttcaggttggcacattagcaatataggatggtttgattattaaaaggatgatatgaagggtttcaaggtggtttgcctcgttcaaatcaaaggattttgaagattaatattccaagataaggttctccaactccattaggaaagtgtcttcatgtcatcttagagaagcagctcgtaccaaacttgacagatgttttatttatttagagtgacacagataccctttggcaatactctccatccttgtccgaacaacttctaatcacacctcacttatcttgcatctaactcagaggctacaagttacacctttcaacaaaccttttcggtttgaaaatttgtgatttcattatttagagttcgaagagcatatcaagtattggtcggagttggcacccaaagcaaacgaaacagttactgacatggtccaaaagctgagatttctaagatcccaacttaagcactgaataaagccattatgggaaatatcattttaacgaaagaggaatttagagtaagaattgattctcttgataccgaagaagaactaatacagctttcatcacttcaaaatgatgaacagatgcatctcaagtcagcactagaccatcttctaaaataggaagatctatggaagcaacactcccaaatgcagtggcttcaaaatggggattgcaatacgaagtttatccatgtttgggcaagtaacaggaaaaaaagaatactatcactgaactctagcaaggcgatcagaagattatcgaatagcagcaaatccaatccacattctacaactttttttctaccctactaggctcgactgaggaatgactcatccaagctgattggaagattctttatccagaaggacctctggatcttgctgacattgagtatccatttatggagaaagaaatccatgatacagtgtatgacttggctttggaaaagtcacccggatgatattttcccattctccttctataagcacttctagtgtatcatcaaacatgacctgatgaacctactgtaaaatcagctaatgtagaccatctgaactacttgttcatcacccttatcccaaaaaaaaattggtgtgtattcagttagagacttcaggccaataagcctgattaatggagtaataaaaaatatttcaaaaactctatcgaaaaggctcccacagaaaatgaatttgttaattttatccacagagcttgctttcaacagaggaagaaatatctctgaatattttgtaatgactatggaaactatacacttctgcaaagctgaagtacacaaggatctcaattataaagtcgacttcgagaaagcttttgacaatgtggattggagctttctattgaaattgctatccagcacggggctttgattcgaggtggtgtcaatggatagaatatctgatttatacagctaaattctcagtccttattaatggtgataaaggtaaactttttaaattgaggaaagatctcaggcaaggagatcctctattcgcctagctctttctcttagttgttgatatagaatgatcaagggagcaagtaggttcaatctttttgttggaattggatcatataatatcatgggataacttcaaagcttttagttcactgatgacacacttatattttgcagatatgatctaaaatacatcaaaactcttaaatttttactctatagttatgagctactgatgggtctcaaaattaactttgaaaaattccaattttttggcttgagaattgcaaagatgtcagtacagcaagttgcatctatcctagaaagcaaggtggctacattttccattacttatttgggtctcccactccatcattctaaactgaggaaaacttattggaatccactccttgagaaggttcagaagaaattgatcgggtagaaaggtaaacttcttaacctctagggtaggcttatactaactaatgcagtgcttacagggatcccactactctggagggatacattccttctccctcaattcattatcaaataaattgataaaatccatcgatcattcatttggagaggaaacgaggagtataactaagggcactctagaatatgttggtcgaatatttgtcgatcaaaaaaatttggaggactgggggttcctcaatctaaaaattttcaatacaattcttctttgtaaatggtggtggaagctctactctaatgctggtgacccgtggtgtagttttattgccactgtccacccaacttcacactagagatctaaaggtatacacaaatcaacctcttcattttggaatggtttacagcacacatgaaatatttctactcctaatccactttcaagttagcaactagtattattttggaaagatagttggttacataatcatccactgaaggatcgatttcctcacctttacacaatagcattgaagtgcaacaactcagtggcaaaggtattaagcaatctacttgataatagctcttttagtactcctcttcctcaaagataccaagaagattttcagagtctataggaaagcattgaacaaattacattaacggaacgacctgatactatacaatggaaatggtttagtagcaatatttttttggcatgaaggatctactattttctgcaagatggaggagtttggcctctactgagtaatattatataaaaactcctaataccaaagaaagccaagttatttgcttggctaagtgctcacaacaaaatcccaatgaaagctaatcttcttaatagaggaataattggaactgattactgtacactttgcgatgacttatcagaaactaatgatcatctaatgctcatctatactttttcaaaagcaatttggaatcaagtactttcagacctgcaattgtcgaaacttttatgcatgcttaacaccctatgggatacttggagactcatcaatatgcaacacgatagaagacctaaactagctgctctattcgtaattggtcaatggtgtctttggaaggaaagaaataaaagattattcgacttctatactttttatccacgatcgattgctgaaactgtgtcactttttctttcttgggcatcacacctaacaacggagcaactaaagatgttagctcctgttcgagaagttctcttatctaagaatgaaaacacacaatctttagtgagaattacagatgctaacaggcgcagatgaatgttttatgagcatttttatagctgcagcttatatgtgatctatggtgcaaggagttaattataaccatggatattagttaggttgactatcagaaatcatctccaatacattctatgtaaccactgatcaattccatgttcaactagataggaacctgcctatatacaggtatgtccctgatgtaactatagtatactattattcataaataaataacgaaggttttaccttcttctcataaaaaaaaagtatcttcatgtcatcctatatgtcatgcatctcctttgctacttcttttatttacttcttaaacttggttctaccatatattatcagccccttttaaatttgcttttggatattgcat

SEQ ID NO: 45 - DNA, 4061 bp, Artificial Sequence
  synthetic
gctttcaacagaggaagaaatatctctgaatattttgtaatgactatggaaactatacacttctgcaaagctgaagtacacaaggatctcaattataaagtcgacttcgagaaagcttttgacaatgtggattggagctttctattgaaattgctatccagcacggggctttgattcgaggtggtgtcaatggatagaatatctgatttatacagctaaattctcagtccttattaatggtgataaaggtaaactttttaaattgaggaaagatctcaggcaaggagatcctctattcgcctagctctttctcttagttgttgatatagaatgatcaagggagcaagtaggttcaatctttttgttggaattggatcatataatatcatgggataacttcaaagcttttagttcactgatgacacacttatattttgcagatatgatctaaaatacatcaaaactcttaaatttttactctatagttatgagctactgatgggtctcaaaattaactttgaaaaattccaattttttggcttgagaattgcaaagatgtcagtacagcaagttgcatctatcctagaaagcaaggtggctacattttccattacttatttgggtctcccactccatcattctaaactgaggaaaacttattggaatccactccttgagaaggttcagaagaaattgatcgggtagaaaggtaaacttcttaacctctagggtaggcttatactaactaatgcagtgcttacagggatcccactactctggagggatacattccttctccctcaattcattatcaaataaattgataaaatccatcgatcattcatttggagaggaaacgaggagtataactaagggcactctagaatatgttggtcgaatatttgtcgatcaaaaaaatttggaggactgggggttcctcaatctaaaaattttcaatacaattcttctttgtaaatggtggtggaagctctactctaatgctggtgacccgtggtgtagttttattgccactgtccacccaacttcacactagagatctaaaggtatacacaaatcaacctcttcattttggaatggtttacagcacacatgaaatatttctactcctaatccactttcaagttagcaactagtattattttggaaagatagttggttacataatcatccactgaaggatcgatttcctcacctttacacaatagcattgaagtgcaacaactcagtggcaaaggtattaagcaatctacttgataatagctcttttagtactcctcttcctcaaagataccaagaagattttcagagtctataggaaagcattgaacaaattacattaacggaacgacctgatactatacaatggaaatggtttagtagcaatatttttttggcatgaaggatctactattttctgcaagatggaggagtttggcctctactgagtaatattatataaaaactcctaataccaaagaaagccaagttatttgcttggctaagtgctcacaacaaaatcccaatgaaagctaatcttcttaatagaggaataattggaactgattactgtacactttgcgatgacttatcagaaactaatgatcatctaatgctcatctatactttttcaaaagcaatttggaatcaagtactttcagacctgcaattgtcgaaacttttatgcatgcttaacaccctatgggatacttggagactcatcaatatgcaacacgatagaagacctaaactagctgctctattcgtaattggtcaatggtgtctttggaaggaaagaaataaaagattattcgacttctatactttttatccacgatcgattgctgaaactgtgtcactttttctttcttgggcatcacacctaacaacggagcaactaaagatgttagctcctgttcgagaagttctcttatctaagaatgaaaacacacaatctttagtgagaattacagatgctaacaggcgcagatgaatgttttatgagcatttttatagctgcagcttatatgtgatctatggtgcaaggagttaattataaccatggatattagttaggttgactatcagaaatcatctccaatacattctatgtaaccactgatcaattccatgttcaactagataggaacctgcctatatacaggtatgtccctgatgtaactatagtatactattattcataaataaataacgaaggttttaccttcttctcataaaaaaaaagtatcttcatgtcatcctatatgtcatgcatctcctttgctacttcttttatttacttcttaaacttggttctaccatatattatcagccccttttaaatttgcttttggatattgcatattccactcttcaatcacctcatgccaagcaaaacatttattcacacttgaaaaccaatataagaataccaaagaatttatccatgaaattctagaaactttggttttactcctttctccatcattcaaaaaggttcaaaatgatgataactctatatagcttatttatcaaatttacgaggttggtgttcaatgtttttgtgaaaaaaatatcttgctatccacatagtttgaatccatacttttgctatcttgagtttcaaaaattttaatttgctacaatttgttgctattagcatatgactacttttaagaagataagccaatatactattttcctaagaatttaaaaaatcaaaaataaaaatttttatttaagattttttaagggttgttttccaaatgtgcaatggggcttaatcttggcatcattttctaacttgtagaattttgacccaagtaacatttgtccaatcacttagaacttctataacttcgtacaatcatttgttaatgttgttcatctatttatctatattatctatctggaatatagttgctcttaattatttttatatatcgcctattatccaccctaagctttcatgttcatcctcatgttgttggaggtgcatgtcttattccaaactatttaccattgctgtagattttaaaaaatttgctagtttaggactttttaatcttttgatatcatgttgatgtaagctaaccctctaaggctagtcataatacattttaaggatttatgttatatgagaccaaaattttaacaaaatgaagtgttggaaattggtagaatggaagtgtaaagatgcttagagacatagaactagccctgggccatgtaaatcttccaaaagaagaagaaaataataaaattaagatcatattcaatctctacagaaaagttggtctttgttgtataataagccatcttaacatatgatggacaataaaatatataaacttatgagttttaatacttagatggaagaaaagggacagatatgtcacaccccatcctactagcatgagtaggcacatgatacacggttgcatgccctgcagagtttgactcatgaggcatgcaaggtattgaatagtagtctaggtaaaattaaaaaacttggagcattctaaaaataaatcaagttcattttataaaatcaatatttattatggactccatcaaatattatgcgcataacattttatttgcaaatagaagaagataagtcctagatcctaagtctcctactcttagtctcataattcatccaagctatccaccaaatatctaaaacgaaaaagaaaaacgatagtatgctaatagctttgtaagtcaccttttatctctaattagatcaagcatattagatataaaacaataattttcaaagtatatgatttgcaattaggaataaatatttgataaatacagaataaattttcataaagcatatttactaacattatttataaaatatataatgcttatatcaataaattaatttctaaatcaatatatataaactatccattctgtcttagccttacaactattgctaccattccctgtagcatggttaggaagagactagctcttgaatactcatgtcatttatcaacatatgcgaatgatcattcgactaatatagt

SEQ ID NO: 46 - DNA, 4061 bp, Artificial Sequence
  synthetic
tttgttggaattggatcatataatatcatgggataacttcaaagcttttagttcactgatgacacacttatattttgcagatatgatctaaaatacatcaaaactcttaaatttttactctatagttatgagctactgatgggtctcaaaattaactttgaaaaattccaattttttggcttgagaattgcaaagatgtcagtacagcaagttgcatctatcctagaaagcaaggtggctacattttccattacttatttgggtctcccactccatcattctaaactgaggaaaacttattggaatccactccttgagaaggttcagaagaaattgatcgggtagaaaggtaaacttcttaacctctagggtaggcttatactaactaatgcagtgcttacagggatcccactactctggagggatacattccttctccctcaattcattatcaaataaattgataaaatccatcgatcattcatttggagaggaaacgaggagtataactaagggcactctagaatatgttggtcgaatatttgtcgatcaaaaaaatttggaggactgggggttcctcaatctaaaaattttcaatacaattcttctttgtaaatggtggtggaagctctactctaatgctggtgacccgtggtgtagttttattgccactgtccacccaacttcacactagagatctaaaggtatacacaaatcaacctcttcattttggaatggtttacagcacacatgaaatatttctactcctaatccactttcaagttagcaactagtattattttggaaagatagttggttacataatcatccactgaaggatcgatttcctcacctttacacaatagcattgaagtgcaacaactcagtggcaaaggtattaagcaatctacttgataatagctcttttagtactcctcttcctcaaagataccaagaagattttcagagtctataggaaagcattgaacaaattacattaacggaacgacctgatactatacaatggaaatggtttagtagcaatatttttttggcatgaaggatctactattttctgcaagatggaggagtttggcctctactgagtaatattatataaaaactcctaataccaaagaaagccaagttatttgcttggctaagtgctcacaacaaaatcccaatgaaagctaatcttcttaatagaggaataattggaactgattactgtacactttgcgatgacttatcagaaactaatgatcatctaatgctcatctatactttttcaaaagcaatttggaatcaagtactttcagacctgcaattgtcgaaacttttatgcatgcttaacaccctatgggatacttggagactcatcaatatgcaacacgatagaagacctaaactagctgctctattcgtaattggtcaatggtgtctttggaaggaaagaaataaaagattattcgacttctatactttttatccacgatcgattgctgaaactgtgtcactttttctttcttgggcatcacacctaacaacggagcaactaaagatgttagctcctgttcgagaagttctcttatctaagaatgaaaacacacaatctttagtgagaattacagatgctaacaggcgcagatgaatgttttatgagcatttttatagctgcagcttatatgtgatctatggtgcaaggagttaattataaccatggatattagttaggttgactatcagaaatcatctccaatacattctatgtaaccactgatcaattccatgttcaactagataggaacctgcctatatacaggtatgtccctgatgtaactatagtatactattattcataaataaataacgaaggttttaccttcttctcataaaaaaaaagtatcttcatgtcatcctatatgtcatgcatctcctttgctacttcttttatttacttcttaaacttggttctaccatatattatcagccccttttaaatttgcttttggatattgcatattccactcttcaatcacctcatgccaagcaaaacatttattcacacttgaaaaccaatataagaataccaaagaatttatccatgaaattctagaaactttggttttactcctttctccatcattcaaaaaggttcaaaatgatgataactctatatagcttatttatcaaatttacgaggttggtgttcaatgtttttgtgaaaaaaatatcttgctatccacatagtttgaatccatacttttgctatcttgagtttcaaaaattttaatttgctacaatttgttgctattagcatatgactacttttaagaagataagccaatatactattttcctaagaatttaaaaaatcaaaaataaaaatttttatttaagattttttaagggttgttttccaaatgtgcaatggggcttaatcttggcatcattttctaacttgtagaattttgacccaagtaacatttgtccaatcacttagaacttctataacttcgtacaatcatttgttaatgttgttcatctatttatctatattatctatctggaatatagttgctcttaattatttttatatatcgcctattatccaccctaagctttcatgttcatcctcatgttgttggaggtgcatgtcttattccaaactatttaccattgctgtagattttaaaaaatttgctagtttaggactttttaatcttttgatatcatgttgatgtaagctaaccctctaaggctagtcataatacattttaaggatttatgttatatgagaccaaaattttaacaaaatgaagtgttggaaattggtagaatggaagtgtaaagatgcttagagacatagaactagccctgggccatgtaaatcttccaaaagaagaagaaaataataaaattaagatcatattcaatctctacagaaaagttggtctttgttgtataataagccatcttaacatatgatggacaataaaatatataaacttatgagttttaatacttagatggaagaaaagggacagatatgtcacaccccatcctactagcatgagtaggcacatgatacacggttgcatgccctgcagagtttgactcatgaggcatgcaaggtattgaatagtagtctaggtaaaattaaaaaacttggagcattctaaaaataaatcaagttcattttataaaatcaatatttattatggactccatcaaatattatgcgcataacattttatttgcaaatagaagaagataagtcctagatcctaagtctcctactcttagtctcataattcatccaagctatccaccaaatatctaaaacgaaaaagaaaaacgatagtatgctaatagctttgtaagtcaccttttatctctaattagatcaagcatattagatataaaacaataattttcaaagtatatgatttgcaattaggaataaatatttgataaatacagaataaattttcataaagcatatttactaacattatttataaaatatataatgcttatatcaataaattaatttctaaatcaatatatataaactatccattctgtcttagccttacaactattgctaccattccctgtagcatggttaggaagagactagctcttgaatactcatgtcatttatcaacatatgcgaatgatcattcgactaatatagtcaaaaaaaaattactctgatttatataaattaaaaattagtaaataatatatgctagtaatcaccttaccagctaagctctaaagaaaattagcttttgaatatacatcatgctattgattattatatgtcagtgcttgtctcattttgtggcatgcaagaagactagatcctaaacttatatgcatagtcagattaaagagcaaatgttgcatctgattatatgaacatctattatgatgtagagtttgtatcatgtatatttaatttaaacacaaatataattatacataaataatattcatattttaaattttaaatatttagataattattctagtgcaggtataaaaataagcaa

SEQ ID NO: 47 - DNA, 4061 bp, Artificial Sequence
  synthetic
ttggcctctactgagtaatattatataaaaactcctaataccaaagaaagccaagttatttgcttggctaagtgctcacaacaaaatcccaatgaaagctaatcttcttaatagaggaataattggaactgattactgtacactttgcgatgacttatcagaaactaatgatcatctaatgctcatctatactttttcaaaagcaatttggaatcaagtactttcagacctgcaattgtcgaaacttttatgcatgcttaacaccctatgggatacttggagactcatcaatatgcaacacgatagaagacctaaactagctgctctattcgtaattggtcaatggtgtctttggaaggaaagaaataaaagattattcgacttctatactttttatccacgatcgattgctgaaactgtgtcactttttctttcttgggcatcacacctaacaacggagcaactaaagatgttagctcctgttcgagaagttctcttatctaagaatgaaaacacacaatctttagtgagaattacagatgctaacaggcgcagatgaatgttttatgagcatttttatagctgcagcttatatgtgatctatggtgcaaggagttaattataaccatggatattagttaggttgactatcagaaatcatctccaatacattctatgtaaccactgatcaattccatgttcaactagataggaacctgcctatatacaggtatgtccctgatgtaactatagtatactattattcataaataaataacgaaggttttaccttcttctcataaaaaaaaagtatcttcatgtcatcctatatgtcatgcatctcctttgctacttcttttatttacttcttaaacttggttctaccatatattatcagccccttttaaatttgcttttggatattgcatattccactcttcaatcacctcatgccaagcaaaacatttattcacacttgaaaaccaatataagaataccaaagaatttatccatgaaattctagaaactttggttttactcctttctccatcattcaaaaaggttcaaaatgatgataactctatatagcttatttatcaaatttacgaggttggtgttcaatgtttttgtgaaaaaaatatcttgctatccacatagtttgaatccatacttttgctatcttgagtttcaaaaattttaatttgctacaatttgttgctattagcatatgactacttttaagaagataagccaatatactattttcctaagaatttaaaaaatcaaaaataaaaatttttatttaagattttttaagggttgttttccaaatgtgcaatggggcttaatcttggcatcattttctaacttgtagaattttgacccaagtaacatttgtccaatcacttagaacttctataacttcgtacaatcatttgttaatgttgttcatctatttatctatattatctatctggaatatagttgctcttaattatttttatatatcgcctattatccaccctaagctttcatgttcatcctcatgttgttggaggtgcatgtcttattccaaactatttaccattgctgtagattttaaaaaatttgctagtttaggactttttaatcttttgatatcatgttgatgtaagctaaccctctaaggctagtcataatacattttaaggatttatgttatatgagaccaaaattttaacaaaatgaagtgttggaaattggtagaatggaagtgtaaagatgcttagagacatagaactagccctgggccatgtaaatcttccaaaagaagaagaaaataataaaattaagatcatattcaatctctacagaaaagttggtctttgttgtataataagccatcttaacatatgatggacaataaaatatataaacttatgagttttaatacttagatggaagaaaagggacagatatgtcacaccccatcctactagcatgagtaggcacatgatacacggttgcatgccctgcagagtttgactcatgaggcatgcaaggtattgaatagtagtctaggtaaaattaaaaaacttggagcattctaaaaataaatcaagttcattttataaaatcaatatttattatggactccatcaaatattatgcgcataacattttatttgcaaatagaagaagataagtcctagatcctaagtctcctactcttagtctcataattcatccaagctatccaccaaatatctaaaacgaaaaagaaaaacgatagtatgctaatagctttgtaagtcaccttttatctctaattagatcaagcatattagatataaaacaataattttcaaagtatatgatttgcaattaggaataaatatttgataaatacagaataaattttcataaagcatatttactaacattatttataaaatatataatgcttatatcaataaattaatttctaaatcaatatatataaactatccattctgtcttagccttacaactattgctaccattccctgtagcatggttaggaagagactagctcttgaatactcatgtcatttatcaacatatgcgaatgatcattcgactaatatagtcaaaaaaaaattactctgatttatataaattaaaaattagtaaataatatatgctagtaatcaccttaccagctaagctctaaagaaaattagcttttgaatatacatcatgctattgattattatatgtcagtgcttgtctcattttgtggcatgcaagaagactagatcctaaacttatatgcatagtcagattaaagagcaaatgttgcatctgattatatgaacatctattatgatgtagagtttgtatcatgtatatttaatttaaacacaaatataattatacataaataatattcatattttaaattttaaatatttagataattattctagtgcaggtataaaaataagcaatataaaattttaaatcgatttatataacatgcataataaaaaaaattaaggatagaggtacttactgctcaactcataaaacataagaaatctctttaactaactttagtgcaacctagatagaacatattaatgattaagttttcatctaaaataaacatagatatcattttaaaatcttaggcatttaaatggtctcatgatttgtgaggctttcttcagattctacaattttgaaattttttcaaattataatttttttaccttgattgataacaaagccaataatacacctcaaatccaaatgtattcctaatagttttcaataaatctaatatcaataaatcataattaagatatcaatccattctatgaatttgaccataaatcctacttgtttctctgaccttcactataaattaatcatcaaactaaataagtgaggggatcataattcttttacgacaatccaagaattcaagtctagcatccacattagatggcttcctgtccagatatttgcgcctctccaaaattgagattatcagattaagaaaaataaaataagagagagggttaaaggacaatgccttctaggtagtgatgtccgacatcataattttgatcaaatctatggggcaaccaataatattagggaaagaggattggatttgagcaagaatagcaaagtcattgtcatcaatggcctgattcattgagttcaatgaaggattggtggttgagtggtggaggtggcatctaggaaggagagagaaagaaaaagatagagagaaagagataagaaaaatagagagaaggtggcagttaagatccctttttgtgattaatatatagccgtaagatactcaaagatctcaccttatcgacctcaaacactaagggaggtggaaggagggactactacccatgaagctagagaaagggatgatgatgattggaggaaggaagaaggaaaaatagtagactcgatgatgataagactaaaagaaaagggtttgacttagccacttggtatataatgaggtttggtatggagtcaatagcttgagtaatagcatggaaagagagaag

SEQ ID NO: 48 - DNA, 4061 bp, Artificial Sequence
  synthetic
aaatatctaaaacgaaaaagaaaaacgatagtatgctaatagctttgtaagtcaccttttatctctaattagatcaagcatattagatataaaacaataattttcaaagtatatgatttgcaattaggaataaatatttgataaatacagaataaattttcataaagcatatttactaacattatttataaaatatataatgcttatatcaataaattaatttctaaatcaatatatataaactatccattctgtcttagccttacaactattgctaccattccctgtagcatggttaggaagagactagctcttgaatactcatgtcatttatcaacatatgcgaatgatcattcgactaatatagtcaaaaaaaaattactctgatttatataaattaaaaattagtaaataatatatgctagtaatcaccttaccagctaagctctaaagaaaattagcttttgaatatacatcatgctattgattattatatgtcagtgcttgtctcattttgtggcatgcaagaagactagatcctaaacttatatgcatagtcagattaaagagcaaatgttgcatctgattatatgaacatctattatgatgtagagtttgtatcatgtatatttaatttaaacacaaatataattatacataaataatattcatattttaaattttaaatatttagataattattctagtgcaggtataaaaataagcaatataaaattttaaatcgatttatataacatgcataataaaaaaaattaaggatagaggtacttactgctcaactcataaaacataagaaatctctttaactaactttagtgcaacctagatagaacatattaatgattaagttttcatctaaaataaacatagatatcattttaaaatcttaggcatttaaatggtctcatgatttgtgaggctttcttcagattctacaattttgaaattttttcaaattataatttttttaccttgattgataacaaagccaataatacacctcaaatccaaatgtattcctaatagttttcaataaatctaatatcaataaatcataattaagatatcaatccattctatgaatttgaccataaatcctacttgtttctctgaccttcactataaattaatcatcaaactaaataagtgaggggatcataattcttttacgacaatccaagaattcaagtctagcatccacattagatggcttcctgtccagatatttgcgcctctccaaaattgagattatcagattaagaaaaataaaataagagagagggttaaaggacaatgccttctaggtagtgatgtccgacatcataattttgatcaaatctatggggcaaccaataatattagggaaagaggattggatttgagcaagaatagcaaagtcattgtcatcaatggcctgattcattgagttcaatgaaggattggtggttgagtggtggaggtggcatctaggaaggagagagaaagaaaaagatagagagaaagagataagaaaaatagagagaaggtggcagttaagatccctttttgtgattaatatatagccgtaagatactcaaagatctcaccttatcgacctcaaacactaagggaggtggaaggagggactactacccatgaagctagagaaagggatgatgatgattggaggaaggaagaaggaaaaatagtagactcgatgatgataagactaaaagaaaagggtttgacttagccacttggtatataatgaggtttggtatggagtcaatagcttgagtaatagcatggaaagagagaaggagctgaagagagtactaagtcttattagaataaagaaagatagaatcttagcgaaaaatagggcctcaaatctttcaggtagaggaaaaagagggatcaacgaatgaaagactaaggaaaaggtgtggagtaggatatactctcgattagtctctcaatcatggattctagtagggcttcgtcagctgctcaatcatggattctgatagctcaaatggtggtaagtagaaagagagagatctaaagagattgatagtggccttaaaaccagcacggtcaaggataggcatgccttagagagaggaaaagagagagagattaatggaaataagcgagaaaaatatattcttagagaatagattggcgataagaagaggaggtggttggggcatgcttaaagaaataaagaaaattgagtaggcggaaagtggtgatgcttggcgatgagaagatttgagagagagagcaaaaaaatgtggatgatggtcataggatagggaaaggaaagaacaaagaagggggtgctaagctaactctttctaccttcctcacaccctgaagcaaaggatttggccaaggatggacaaatgggcgagggctttggtggatccatgcctaccctttctccctctcacgatgattctagtcaagctatctatctttgatagcttgagccaagccaattgacttgatccaatctctctaaatccatacaaacttaagagagtgtattgattcacttattctcttctaagttgataagaaacataattaagtggagctcattaagtatttcaggtagttgctaacttggcaaaatggaagcaataataaatcttaaaagactatagcttggtataatctcaaccatccatgatttagaaagatcttcagactcaatatagattactttggctactacaggtaagagctaaataggatccaaaagtaagatccatcacattagtaagtcaaattatatgtcaaattttagtaggtatacttagtcctacgatgcctaattaaaatgatcatcatttgaaccttaaaatggactagtcaactaaaatttttctttttgaagaagatttagaccataaaatatcttctaatctgtgaagaattagatagagcgaggaatataaaattgatgtagaaatcaagatctatcatatatacaattttaatatttttttcataatttttaaatatttatcttctttttttataggtctagtcctatttaaactaggaagaggagtccaacttgacttatgcaataggggatgtccttctagaagataagaataatttgatcagaattatataagagcaaacctcattattataaataggggctatatacatcaatttatgagatagagaatcaatgaaacaaaagtagacttaagttttattttcataattcttctatcttctactttttttctaggagattcaagttgagtggattgaagaaaatctttcatcttctcgatcggatcatattggtattagagcgttggtcttctatatttatggagagctttaatgtattgtttaaatacgtgaacaatacaaacaatcaagagaagtgctatccatgcttcaaatacatcgaaatataaaagcaaatatggctactaattctttttcaatggacaatgagataaaaggatgtcttacacaactcaaggagaagattgtgcaactcatgaagattgtctccagattgaagataatttcaatacaagcacaaacaccagcaactcatgttgtgaaactgtttcctatgtttggagatgaagatcttctatctagtgaggagattgaattacctaaaagtatgaaaaatctttcttcaatcattgaaagttaaagcttgaattgagatccccatatataatggaaccattgatgaaaaaaagctagataattggctaaactaattacaaacctattttattatctatagatattatggcatctagaagatagcttttacttatctcaagctttctagccatgctcttatctgatgaaattcatatatgagaaataataatatttttaatatggtgcagagccaattcaaaggtttaatcaagaagtaattttatctaattggccataaggaagatcggtggatcaaatgataatacttatgatagaaacataatcaatccacttaggactataccaccaagttccacaaacaggcaatctgccttggaatcttt

SEQ ID NO: 49 - DNA, 4061 bp, Artificial Sequence
  synthetic
aaagagataagaaaaatagagagaaggtggcagttaagatccctttttgtgattaatatatagccgtaagatactcaaagatctcaccttatcgacctcaaacactaagggaggtggaaggagggactactacccatgaagctagagaaagggatgatgatgattggaggaaggaagaaggaaaaatagtagactcgatgatgataagactaaaagaaaagggtttgacttagccacttggtatataatgaggtttggtatggagtcaatagcttgagtaatagcatggaaagagagaaggagctgaagagagtactaagtcttattagaataaagaaagatagaatcttagcgaaaaatagggcctcaaatctttcaggtagaggaaaaagagggatcaacgaatgaaagactaaggaaaaggtgtggagtaggatatactctcgattagtctctcaatcatggattctagtagggcttcgtcagctgctcaatcatggattctgatagctcaaatggtggtaagtagaaagagagagatctaaagagattgatagtggccttaaaaccagcacggtcaaggataggcatgccttagagagaggaaaagagagagagattaatggaaataagcgagaaaaatatattcttagagaatagattggcgataagaagaggaggtggttggggcatgcttaaagaaataaagaaaattgagtaggcggaaagtggtgatgcttggcgatgagaagatttgagagagagagcaaaaaaatgtggatgatggtcataggatagggaaaggaaagaacaaagaagggggtgctaagctaactctttctaccttcctcacaccctgaagcaaaggatttggccaaggatggacaaatgggcgagggctttggtggatccatgcctaccctttctccctctcacgatgattctagtcaagctatctatctttgatagcttgagccaagccaattgacttgatccaatctctctaaatccatacaaacttaagagagtgtattgattcacttattctcttctaagttgataagaaacataattaagtggagctcattaagtatttcaggtagttgctaacttggcaaaatggaagcaataataaatcttaaaagactatagcttggtataatctcaaccatccatgatttagaaagatcttcagactcaatatagattactttggctactacaggtaagagctaaataggatccaaaagtaagatccatcacattagtaagtcaaattatatgtcaaattttagtaggtatacttagtcctacgatgcctaattaaaatgatcatcatttgaaccttaaaatggactagtcaactaaaatttttctttttgaagaagatttagaccataaaatatcttctaatctgtgaagaattagatagagcgaggaatataaaattgatgtagaaatcaagatctatcatatatacaattttaatatttttttcataatttttaaatatttatcttctttttttataggtctagtcctatttaaactaggaagaggagtccaacttgacttatgcaataggggatgtccttctagaagataagaataatttgatcagaattatataagagcaaacctcattattataaataggggctatatacatcaatttatgagatagagaatcaatgaaacaaaagtagacttaagttttattttcataattcttctatcttctactttttttctaggagattcaagttgagtggattgaagaaaatctttcatcttctcgatcggatcatattggtattagagcgttggtcttctatatttatggagagctttaatgtattgtttaaatacgtgaacaatacaaacaatcaagagaagtgctatccatgcttcaaatacatcgaaatataaaagcaaatatggctactaattctttttcaatggacaatgagataaaaggatgtcttacacaactcaaggagaagattgtgcaactcatgaagattgtctccagattgaagataatttcaatacaagcacaaacaccagcaactcatgttgtgaaactgtttcctatgtttggagatgaagatcttctatctagtgaggagattgaattacctaaaagtatgaaaaatctttcttcaatcattgaaagttaaagcttgaattgagatccccatatataatggaaccattgatgaaaaaaagctagataattggctaaactaattacaaacctattttattatctatagatattatggcatctagaagatagcttttacttatctcaagctttctagccatgctcttatctgatgaaattcatatatgagaaataataatatttttaatatggtgcagagccaattcaaaggtttaatcaagaagtaattttatctaattggccataaggaagatcggtggatcaaatgataatacttatgatagaaacataatcaatccacttaggactataccaccaagttccacaaacaggcaatctgccttggaatctttatcaacaattatacaatttttataaagtatgttgaaagtcttcatgagagcatctaaaaaaagatgaaactctttaaggttgatgatatcagtaaagctaacatgaaagtcatagagattgaggagaaaaatcaaattagagaagataaggaaggcaaaaagcatatcaacataactcaaaaaaaaaaattatgatcattgaaatctttgaaaatacatcaaggagaagtattgaaagtttcatcctgaattggagctaaagtagaagaagcccaaggatgataattttaagaaaaataaaaagtggtcctcaattctatagagattgaggagctatctgaacttgagtaagcaaacttcaaattgagcttgatggtgagaaaacctaatacaacaattaaaacggatctagaggtacatgacaactcacccacttaaagattcaagtgaagcagagtatcattaaggctattataaatctttgaagctagaagaacctcattttccaatatttggttcagaaatcgaggttgtagatcaagcctcatccatatccttatcctcttagttggattcagaaggatgtcaagttaaaaattatgagatagtgtaccttcaagttagccatcactgagaggtttatttgtgaggtaacttttgaaatagtttctttggatatttgtcaagttatccttagaaatgtgtacctttagaatcaagatgcaattttctatagacgatagagaaagtatcatcttataagggatgagaaaaagttcatgatcaacacctcaagaacataaggtaactttgaccttgcaactgttgcccaagtgaagtgatttgttaatgtttgtgatgagtgcatgatgatggtataaagaaccgatatcactcatgagaggtcaaggccttgtcctttggttccatcaatcgatcaatagagattgagattaaggaggagtcactatagtccttgtcgatgaggaaggatgacaacaagcattcctaccatgaagtctagatttgagagcaaatgaaagtaatccactgagacctgagagcaaaaaaaggcgagaccaaaaatcatcttcaagtaaagtcaaatggttcaaccatgagatggggaagtaagtattttcccaccttcaattctaactttgtagaaactaaatcccttaaacaggggagccctaatttaagaggatcctcagattcattgtggactactttggctattacaataagagctggataggaatcgaaagcaaaattcaccacattaggaagccaaattgtatggcaaacttcaagagaccataacttgatcacatgaaatccaattaagatgattttatttttgaatttgaatatttttttgagatctataactttagatctaaatcaagctaaaattttattgcttatgccttcaaaataggctagtcaaatcaaaacttttcttttcaaaaaagactttgactgaaagatatctttcaatctatgaagaatcaagtaga

SEQ ID NO: 50 - DNA, 4061 bp, Artificial Sequence
  synthetic
ctctcgattagtctctcaatcatggattctagtagggcttcgtcagctgctcaatcatggattctgatagctcaaatggtggtaagtagaaagagagagatctaaagagattgatagtggccttaaaaccagcacggtcaaggataggcatgccttagagagaggaaaagagagagagattaatggaaataagcgagaaaaatatattcttagagaatagattggcgataagaagaggaggtggttggggcatgcttaaagaaataaagaaaattgagtaggcggaaagtggtgatgcttggcgatgagaagatttgagagagagagcaaaaaaatgtggatgatggtcataggatagggaaaggaaagaacaaagaagggggtgctaagctaactctttctaccttcctcacaccctgaagcaaaggatttggccaaggatggacaaatgggcgagggctttggtggatccatgcctaccctttctccctctcacgatgattctagtcaagctatctatctttgatagcttgagccaagccaattgacttgatccaatctctctaaatccatacaaacttaagagagtgtattgattcacttattctcttctaagttgataagaaacataattaagtggagctcattaagtatttcaggtagttgctaacttggcaaaatggaagcaataataaatcttaaaagactatagcttggtataatctcaaccatccatgatttagaaagatcttcagactcaatatagattactttggctactacaggtaagagctaaataggatccaaaagtaagatccatcacattagtaagtcaaattatatgtcaaattttagtaggtatacttagtcctacgatgcctaattaaaatgatcatcatttgaaccttaaaatggactagtcaactaaaatttttctttttgaagaagatttagaccataaaatatcttctaatctgtgaagaattagatagagcgaggaatataaaattgatgtagaaatcaagatctatcatatatacaattttaatatttttttcataatttttaaatatttatcttctttttttataggtctagtcctatttaaactaggaagaggagtccaacttgacttatgcaataggggatgtccttctagaagataagaataatttgatcagaattatataagagcaaacctcattattataaataggggctatatacatcaatttatgagatagagaatcaatgaaacaaaagtagacttaagttttattttcataattcttctatcttctactttttttctaggagattcaagttgagtggattgaagaaaatctttcatcttctcgatcggatcatattggtattagagcgttggtcttctatatttatggagagctttaatgtattgtttaaatacgtgaacaatacaaacaatcaagagaagtgctatccatgcttcaaatacatcgaaatataaaagcaaatatggctactaattctttttcaatggacaatgagataaaaggatgtcttacacaactcaaggagaagattgtgcaactcatgaagattgtctccagattgaagataatttcaatacaagcacaaacaccagcaactcatgttgtgaaactgtttcctatgtttggagatgaagatcttctatctagtgaggagattgaattacctaaaagtatgaaaaatctttcttcaatcattgaaagttaaagcttgaattgagatccccatatataatggaaccattgatgaaaaaaagctagataattggctaaactaattacaaacctattttattatctatagatattatggcatctagaagatagcttttacttatctcaagctttctagccatgctcttatctgatgaaattcatatatgagaaataataatatttttaatatggtgcagagccaattcaaaggtttaatcaagaagtaattttatctaattggccataaggaagatcggtggatcaaatgataatacttatgatagaaacataatcaatccacttaggactataccaccaagttccacaaacaggcaatctgccttggaatctttatcaacaattatacaatttttataaagtatgttgaaagtcttcatgagagcatctaaaaaaagatgaaactctttaaggttgatgatatcagtaaagctaacatgaaagtcatagagattgaggagaaaaatcaaattagagaagataaggaaggcaaaaagcatatcaacataactcaaaaaaaaaaattatgatcattgaaatctttgaaaatacatcaaggagaagtattgaaagtttcatcctgaattggagctaaagtagaagaagcccaaggatgataattttaagaaaaataaaaagtggtcctcaattctatagagattgaggagctatctgaacttgagtaagcaaacttcaaattgagcttgatggtgagaaaacctaatacaacaattaaaacggatctagaggtacatgacaactcacccacttaaagattcaagtgaagcagagtatcattaaggctattataaatctttgaagctagaagaacctcattttccaatatttggttcagaaatcgaggttgtagatcaagcctcatccatatccttatcctcttagttggattcagaaggatgtcaagttaaaaattatgagatagtgtaccttcaagttagccatcactgagaggtttatttgtgaggtaacttttgaaatagtttctttggatatttgtcaagttatccttagaaatgtgtacctttagaatcaagatgcaattttctatagacgatagagaaagtatcatcttataagggatgagaaaaagttcatgatcaacacctcaagaacataaggtaactttgaccttgcaactgttgcccaagtgaagtgatttgttaatgtttgtgatgagtgcatgatgatggtataaagaaccgatatcactcatgagaggtcaaggccttgtcctttggttccatcaatcgatcaatagagattgagattaaggaggagtcactatagtccttgtcgatgaggaaggatgacaacaagcattcctaccatgaagtctagatttgagagcaaatgaaagtaatccactgagacctgagagcaaaaaaaggcgagaccaaaaatcatcttcaagtaaagtcaaatggttcaaccatgagatggggaagtaagtattttcccaccttcaattctaactttgtagaaactaaatcccttaaacaggggagccctaatttaagaggatcctcagattcattgtggactactttggctattacaataagagctggataggaatcgaaagcaaaattcaccacattaggaagccaaattgtatggcaaacttcaagagaccataacttgatcacatgaaatccaattaagatgattttatttttgaatttgaatatttttttgagatctataactttagatctaaatcaagctaaaattttattgcttatgccttcaaaataggctagtcaaatcaaaacttttcttttcaaaaaagactttgactgaaagatatctttcaatctatgaagaatcaagtagagtgatgaaagataaagttgatataaaaattgagatctatctcttataaaattttagtaattttattttttttaatatttatctttatttagagatctattcctatttaaactagaaagaattgtccaacctaacttgttcaatgatcaacatcctcctaaaagataaaaagaagaatctgactcaaattataaaagggcggacctttttttttgatgaaaagggaggaaaaaaatccatcaaaatttattaagaaaaaaagagtacaagaaaagaaggatatgaaagagtaagagaagccccacaacatccatcaatatttaaaatttaaatttaaatctcccccatcattctatcaatatttgatattcaaatttaaattcttcgcagcatcccaccaacatttgaaattcaaatcctttcatacaaacaaaataatat

SEQ ID NO: 51 - DNA, 4061 bp, Artificial Sequence
  synthetic
caaggagaagtattgaaagtttcatcctgaattggagctaaagtagaagaagcccaaggatgataattttaagaaaaataaaaagtggtcctcaattctatagagattgaggagctatctgaacttgagtaagcaaacttcaaattgagcttgatggtgagaaaacctaatacaacaattaaaacggatctagaggtacatgacaactcacccacttaaagattcaagtgaagcagagtatcattaaggctattataaatctttgaagctagaagaacctcattttccaatatttggttcagaaatcgaggttgtagatcaagcctcatccatatccttatcctcttagttggattcagaaggatgtcaagttaaaaattatgagatagtgtaccttcaagttagccatcactgagaggtttatttgtgaggtaacttttgaaatagtttctttggatatttgtcaagttatccttagaaatgtgtacctttagaatcaagatgcaattttctatagacgatagagaaagtatcatcttataagggatgagaaaaagttcatgatcaacacctcaagaacataaggtaactttgaccttgcaactgttgcccaagtgaagtgatttgttaatgtttgtgatgagtgcatgatgatggtataaagaaccgatatcactcatgagaggtcaaggccttgtcctttggttccatcaatcgatcaatagagattgagattaaggaggagtcactatagtccttgtcgatgaggaaggatgacaacaagcattcctaccatgaagtctagatttgagagcaaatgaaagtaatccactgagacctgagagcaaaaaaaggcgagaccaaaaatcatcttcaagtaaagtcaaatggttcaaccatgagatggggaagtaagtattttcccaccttcaattctaactttgtagaaactaaatcccttaaacaggggagccctaatttaagaggatcctcagattcattgtggactactttggctattacaataagagctggataggaatcgaaagcaaaattcaccacattaggaagccaaattgtatggcaaacttcaagagaccataacttgatcacatgaaatccaattaagatgattttatttttgaatttgaatatttttttgagatctataactttagatctaaatcaagctaaaattttattgcttatgccttcaaaataggctagtcaaatcaaaacttttcttttcaaaaaagactttgactgaaagatatctttcaatctatgaagaatcaagtagagtgatgaaagataaagttgatataaaaattgagatctatctcttataaaattttagtaattttattttttttaatatttatctttatttagagatctattcctatttaaactagaaagaattgtccaacctaacttgttcaatgatcaacatcctcctaaaagataaaaagaagaatctgactcaaattataaaagggcggacctttttttttgatgaaaagggaggaaaaaaatccatcaaaatttattaagaaaaaaagagtacaagaaaagaaggatatgaaagagtaagagaagccccacaacatccatcaatatttaaaatttaaatttaaatctcccccatcattctatcaatatttgatattcaaatttaaattcttcgcagcatcccaccaacatttgaaattcaaatcctttcatacaaacaaaataatatttttcaaattctcaactttgagtttcaaaattgagaagcctacatattgtctgctcttcaccaaagaggggagattgttggcttagcttggcccaagagaagagaagaaggccaaggcccaatctgtagcctagagaaggagggtttggtagctacttaataatcggatctaaccgataaagacactatctctattagaagaaaaggtagagagaaaaagaggcaattggttaacttcagagggggaggaggtaagctgttgaggagattaatctgacgcaaggaaaaaagaagagctgacaactagccaatgatcgagaagggctggagacaatccaagcccagcaccaagaagcaagagaaagaatttggaggtcaaaggaggagtccaggaagagagagcgaaacacaatgttcggatctagccgacaacgataccaattatactaggaaagaaggtaaaaagggaaagagcaatcgatcatcttcagcaaagaaaaataaaagaggcacccgacagtcaagcccatggccaaatcagtcagcaagaggacctcacaagatctagacggtgctaaggggaagggaggaagaaaagagatccagtaactgtccaacaccaggaaaaggaggagataagaggaagggagaagtcatttttctatcttgggccgaaggagggagaaggaagaaagaggaaagaacatcctcaaagtcgaaggaaggaaggaaagagaggggggaaggggtcacagtcagatataccagaagggatagatccagtgtcaaagagagaaaagagagaggagatcagaaaataaaatttgatgactgactaattgtcatgaaaggctaatgacaactcataaaaaaagtatagtagtaaagagagggggataggcttggttagggaagagattccgacaacaaagagaaagaaagagagagagagagagaaccggctcccagccaaaaatagcttgacccaccatcgagaaggaccgacaaagagagagaaagatagaatagggagaatagcttggcttcgaatcaaaaatgatctaacacactgctgaaaaggactaggaagagagagagagggggtaggggagtatctcggctcgcaatcagaatcaactggccaatgccagaaaagagaggaagagagagatagagaagatatagcaaaagagaagagatggacaaaaggagagaggaagggagggagagagagaaaaaataggagagagaggggcttggtggctgactgtcagaagaagcctcgatgctcgaagattagatggaagaaaaaaaaatttctcaaaacttctcttttctataagagcaaacctcactattataaatagggttatgtatctcagtttatgatgtgaagaattaatgaaaaattggactttagctctatttttgtaattctttcatcttctatttttatgaaattcaagttgagccgattaaaagaaataatctttctttccgattggatcaatccattaactagatacttcaaaaatcaaaatgacctatctaaaatcctaaatcaaatacaaaaccaaaataactaaattaagatagaacaaactacaattacaaaaaactggctaaagtgtttaaatgcttttactcctaagtttcttcttgctcaccattaatgcttgatctttagctgggatcatatcagccttatgaccactataagaccaacataacaactcacttgtattgctcctttaaaattatacaaaactagtgtctaatatgtaccatgcgaatgtctgtttctcaccagaaaatggatgggcttcttgtgcaagcaccttcttcctacaaataataaaatatgcatcccttctctcatcttactaaataaaataattaaaggctttactatcaggaaatctggctttatccatataattttggaagttttatttgaacataacattacgagtactagattacatcaggaggtggttcctcttatttctattaagagaaaaatcaattttcttttaagaaagatcatttcattttcatcaggtagcgtactctactaatatacttccacaacaatatatagggattagattataggatggactttaaggcttcttttcgagagccctgatttctcaatcacattcccttttctttctcatgtaatggcatttaagagtgcatccagggcccaacaattagtcacaagtgttctttttatacatggtacatatttgctattttttagcttattttaacttgattgtgaagatatcatgagaaaattagatttaaagcctag

SEQ ID NO: 52 - DNA, 4061 bp, Artificial Sequence
  synthetic
ctttcaaaaatatcttttgataggactaatgagataagtcaggaccaatggatatctcggtcaacccaaccactgctcaagtttgagatggaaaatctatctcggacaacagctgaagttagtacctcaggttaggatgatctagaatctcctataagagattttttagattatttcggcccaagtactgaacaatctgtcctgaccaatctcgatctttaggaacttaagaaaaaatattcgattcagcttataactccaagttgggatggtaggattattgaacctccagaaggttatgtcgtattttatgatgaggcacttcgatctggactttaatttctcttacatcctttcttcagtaatgttttagacttctataaactccatccaatctaggttactcccaatgccattaggatgatcatagttttcattatctatcgtaaattttttgctatagaactaagaatttctctctttaggatgctggtcatcctaagaaaacatccttatgaaaaagactgatggtatttcttaccttggcctcaatataaattcggtcccactcttcctttttcaatacataattgaaaaaatcattttttctttatttcttctaatgtttcgtagggttttatttgtaaatagtctaagcctaaaaccaaatggaactcaaataacaaaatattatctgaggatgaggagacttttgtagagcttttagatatgaaagtatccaagttgagcctactggtgtccaatcagtccttgtttgacaccgacatcagtcagatctctccttaagataagtctgatgttaattctttttctttattgctttatcatttttcatcatttttcttttctaacaatctttttccttatatagtagcaataatgaagttcaacctacaaaggctggctaactcaaagaagaggaagaaggatctaaccgattgctctcaagaagagtaaggagactgctcctctaagatcgattggcccccgatcatcacctgggccaatattaattgacatagatgctacatcgatctccactataccaccagcaaaatcaactcatcaacctactaaggtggcttgtccacctcctaaagagtctgcacatccaaagtaggcatcttccccaacacctccaacatcggccaagttagtttggctgagcaatcagcatctgaggtcacagactcctgatgtcaacccaccaactttctcatcaaaaaaaattgacttggcgaaggtatcacttttggagacacccagactaggcaaggacttgctctgtacaatgatgcctcaaaaggacctagatgctgataggagggatctttctttggagcaaataataaattatggattcaacagtatcatgaacgtgagtcttcattctcttccactctcttctttctttttctttttttttttacattggctatttgttgatctgaatatatctttctttttgcagtcggttgtgtatttcaagttgctcaatgagcacttgacatggttcttcaaaaataaaatttttttgaaagagaggctcaaggccaagaaagaggccaaaaaagcagttgaggaggtcaagaaggcagtaaagaagaaggctgtcaaagaaagcaaaatgatggcggggctgaagaaacagctccaagaaaaaatagattccattaaggagactggacaaccaatgacagatgaatgataaagatgacaagttgtaaaaacagcctgaaaaaaatctcaaagttggaggccaagctgaaggaggtcgagtcaataattgaaaagcatgatgaagctcttgtcccatattagagacaacttgataaagacaaagagtggatgtcaaggattattgaagattataagaattccgacacttttcaagatgacgttactgaggcctcaaaaggagctttcaattatggctttttgagctacaggagtttaattatcaagctctttcctaaccttgatctcagcaaggtcataatagaagcagctctagaagtagtagccgaagtgacttctgcaacaactactgagcttgcttccacttctatcattggagtttctccgatcgaagtcccaaacagtccaatcgaggcctccatcatcgaagctatttcgaaggaatcagtcggcaaagaccttacctcaactcctccaacaaataactcccaagctaaggcctgaattatcttcttctttttttctaaacatttgtattagcccgatgtgggcttctataaatactttttacattaatgaatgagtttttcaatgtcaatattttttctttttaactaatactaatcttggatgatccgatctgggttggatgtctcaaaaaatatcattcacgatagatagttattttctgacttcggttagatgattatgagtatatgtaattcaaccttggttaggtaagtaatcaaatattaactattctcaaaccaagtagataacgaagtcaatgtgattaactttaacaagtaagattgttatggaatgaaattgaatcagatcaactaactatagataacttaatctctcataattcactgtaaaggttctaaaagtacctttatctaagttcgaagtgacaagtcgggttcttttattcgtggatttatgacccatgctgtctttttgtgatcttcattattaatcaccttaaatcgatatagcaaaatccagtttatagatctgagtgctttcttgtcagattgagtctatcctattatctgtgaaacctgatctagagatcaagtattttaggttttttatttaaggtccaattcgaagattgagtatccaatgtcatattgttaggtccaatttggagattggatgtctcactatcatctcgtgaggtccaatccaaagatcgaatatctcactatcatctcatgaggtccaatccagagattggatgtctcacatcatcttgtgagatccaattcgaagattggatgtctcacatcatctcatcctattgtggttggaatttttgtagccttagtttgactttttctgacctcatttggacacctaaatcttattatcatcgtttgatcgatttttactaatctactttggatgaaaaagaattcttcaatggaacttttgattagaactttatcttcattgggatagaaatcgaatgctttattgaaagattttattgataatacattctgagatttttaatatttcatgttctcgaaatgatcgtaccatctaaatttttaattcgataagctcttggatggatcacctcagtaatctgataaggtccttcccaattcgggatgagtttttcttactccattggttttgagacttcagctcattggagaaccaaatctccttataaaaaattttaggctttacctgagagttgtaatatctggctactttttgtttataaactaccatatgaatctgggctttttctcgagttttctcaaataaattgagatcagtcctcagttgatctgaattattttcttcatgaaaattttctattctggttgtaggtaaactgatctcgactagtattatagcctctgttccgaaagtaagtttaaaagatatttctctagttggtctctgaggtgtagttctgtatacccataaaatattataaaattattctaccccgagacttttagcctcaatgagttttatttttaggccttgaaagatagttctataaataaatttagcttctccatttgattgtagatgtccaatcgaagtaaatatatgatctatgtagagctcagaataaatttttttaaaattttgattatcaaattattgctcattattagtaattataactcaaggcaaaccaaaatggtaaataattatttttcacataaaatctcatattttttctcagtgatttatgtcagaggttcaatttctatccattgggtaaaataatcaatagtcacaactaaaaattttctttgctccatggccattagaaaggatcccagaatatccattctccatatagc

SEQ ID NO: 53 - DNA, 4061 bp, Artificial Sequence
  synthetic
aaaattattctaccccgagacttttagcctcaatgagttttatttttaggccttgaaagatagttctataaataaatttagcttctccatttgattgtagatgtccaatcgaagtaaatatatgatctatgtagagctcagaataaatttttttaaaattttgattatcaaattattgctcattattagtaattataactcaaggcaaaccaaaatggtaaataattatttttcacataaaatctcatattttttctcagtgatttatgtcagaggttcaatttctatccattgggtaaaataatcaatagtcacaactaaaaattttctttgctccatggccattagaaaggatcccagaatatccattctccatatagcaaaaggccacagcactgtaatagaaataagttcagttgtaggctgatgttatatattggcgtacctttgacactgatcgcagtacttattaataaagtcggttgaatctttttgaatagtaggccaataataatcttactgaattatttcataagctaaaattttaccccccaaatggttactagagattcctttatgaacttctcgaaggatgtaatcagcttccgatggccttaggcataggagcagtgggagtgaatataacctctgatataattgattatcttgaacaacataccatggggcctgtcttttaattcttgttccttcgactggatcaaccggtagaggttctttagtaatatactccattaatgggtcaatggaacttagctcatattaaatttggacaattagtaaggcctcgatactagactttttaagaatatcaataagaacaccttgatttagtttgaaaaaatctgatgtggctaaatgagatagggcatcagctcagacattttgtccttggtatttgcatgatcttcagattttcaaagttttttaataattctttcatattatataaatattgaaacatcataaaatctttagcttcaaattaatctcatacctgactgacgataaattgagaatcaataaaaattttaatttttttaacattaagctccttagccattttgagtcctacaattagcgtttcatattctactccattgtttgagtgttaaaattaaatctcaaagcacgctcactaacaatgccttctagactcgttagaattaaactagttctactttctttcgaatttgaggctccatcaatgtacagtatcaaataagaatctttgatatttttcaattcttttaagattggttcttcattaggaatagagcattcaataataaaatcagctaatacttaaactttcaatgaagatcgaggcccatattgatatcaaattcatttaattcaatagcctatttgaatatccttcttaaagtatcaagctactgtaaaattaattttaaaggttgatcgatcagaattataatagaatgagcctaaaaatacgatcaaagtcatcttgctaatgcaatgagggtataaattatcttctcaattttagaatatcgagtttcaacatctctaaataatttatttgtataataaatggatctttgtatccctgcatcatttcaagctaaaatcgaactaacagcatttgctgaaatagatagatacatgaataatttttgacctttgatcggctttgatagtaatggagctgtgccgagatatttcttgagatcatcgaaggctgcttgacattcatcttatcaatcgaagtctttgatctgccttagaattttaaagaaaggaagatatttatcagctgatctgaaaataaattaactaagcaatgctactcatccagtaagttggtgtacttctttgatggagctcggatgcttcatttcacatagagcttgaattttcttaagattgactttaattcctctttgagttacaaaaaaatctaaaaaaatttttgaagttacttcaaaagcatatttgttgggattgagcttcatttgatattttcgtagtctctaaaggcttcttccagattggcaatatactgatctgactcagtattttttactaatatatcatcaacataaactttgatattaatttcaatttgttacttaaaaatcttattaatcaagtattagtatgtagcacctacatttttaagatcaaaagacatcattttataacaatgcaaatctttttcagtgatgaaggccatattttcttcatcctcaagtgccattttgatctgatataaccagaaaaagtatccataaagcttagtaatttgtgtcttgaagtagcatcaacaagctgatcaatttttgagagagaaaaactatcttttaggcaagctttattgagatcggtataatcaacatagatccttcatttttcattagcctttttaaccatgacaacatttacaatccactttggatattatgcttctctgatgaatttgtctttcaagagtttgtcgacttcctcatctattattttttatcttttcggggtgaaacttcttttcttctgttgcattggtttatgctttggatcaacattcagcttatgtacaataagatcagttaaaatctcaggcatattagagactgactaaacaaagacatcggcattcatccgaagaaaagatattaatttctccctcagatcaggcttcaatagagatccaatttggacagttttttttggatcatcacacaaaagaacaataataagtttctcgactggttctcctcgatttttgatgatatcaactttactttcttgatcaagtattttaattggtagagcttccacagaccttttcatttttacagctatcagaaaatactacttagcaagtatctgatttcctcatatttctccaactccatacttagtttggaattggattagtaaatgataagtgaagactatagccttaagggcgttgagcctaggtcggtcaagaatagcattataagctgatggtattttgacaataaaaaaagtgagtcttacagttgactggcatggttctatccctgcagtgacggacaaagtgacctctccttccacagctacaggatttctagaaaatccaattacgggggtaccaacctatttagctaatttatcatattcattctttggaatgtatcatagaacaatatattagcagagctttcattatcaataagtattctttttatatcatatttggctattgccataaagatgacaacagcatcattacgaggagtttgaactctaacatcatcatcgaaaaatgaaattatgtgatccatgcactgatgctttggaaggctttcagtaatctcagccacctcctcagttccgtcgagatctgagatcatattgatgactgcagcagtagacttgttgtgatcattctcattgttgggcttctatcattggtcagtagcttgacttgcccgatctcgaacatatttactaaagtaacattagtggatcaatacttcaattttatcttttaattatcgatgctcctcagtatcatggccatagtctcgatggaaatgacagtattttctcttatctctctttgctggaggggctttcataggattaggttggcgaatatatcctaaatcctcgatttctatcagtatctgagctcgaggagtagatagtgaggtatagatgtcgaatcaccgaggtgggcttttgaacttcagattcttctgaggtcgttcagagttatcctgttggtttttatgatcttcttcctagggccacttttttccatctctttttttcttcacctaacgaagtatgcatgctctctttcttttcagcttgagcatacttacaaacctagatcaatatttgttcataattgtttgggtagttcttattaagagagaagatcaggcgattactcttgagtccttgcttcaaagctgccattgcaatggactcattgaagttcttcactttcagtatggcggcattaaagcatgccacatattcttgaagagattcaccttcctactatttgatagtaaaaagattgc

SEQ ID NO: 54 - DNA, 4061 bp, Artificial Sequence
  synthetic
  misc_feature (2978)..(3705): n is a, c, g, or t
catcatcgaaaaatgaaattatgtgatccatgcactgatgctttggaaggctttcagtaatctcagccacctcctcagttccgtcgagatctgagatcatattgatgactgcagcagtagacttgttgtgatcattctcattgttgggcttctatcattggtcagtagcttgacttgcccgatctcgaacatatttactaaagtaacattagtggatcaatacttcaattttatcttttaattatcgatgctcctcagtatcatggccatagtctcgatggaaatgacagtattttctcttatctctctttgctggaggggctttcataggattaggttggcgaatatatcctaaatcctcgatttctatcagtatctgagctcgaggagtagatagtgaggtatagatgtcgaatcaccgaggtgggcttttgaacttcagattcttctgaggtcgttcagagttatcctgttggtttttatgatcttcttcctagggccacttttttccatctctttttttcttcacctaacgaagtatgcatgctctctttcttttcagcttgagcatacttacaaacctagatcaatatttgttcataattgtttgggtagttcttattaagagagaagatcaggcgattactcttgagtccttgcttcaaagctgccattgcaatggactcattgaagttcttcactttcagtatggcggcattaaagcatgccacatattcttgaagagattcaccttcctactatttgatagtaaaaagattgctagtatttttcaaatgaatccatttattatcaaaatacgtgatgaatatttgctaactgtgtgaaagatgaaatagatcatgtctggaggtcagagaactagattcttgcagatgttttgagagtgattggaaaagtgatgcaaaatagggcattagataccccttgtagtcttataatggctctgaagccttcaagatgatttaagggattgatggagccatcgaatgtttccaatgtaggtatcttgaatcgaggaggaactgatttaccaagaattttttgagaaaaaagagatcgtaagttgaaatctcttctaccttgagaatggcttccaatctatatctccatcattttcttctcaagattttgaatcttttgtccaagaccctcctccatacatggcttcttatgtggagcagatttcacttcccaagagtgatcagtatggtcaagaagatgatcatgatgaagatcttgaggagttggttgctaagtgtgatgtgattggactacttggggggctactttttgctaccgttctgtcgtatactacagcagtaagagcttggacctgctgaaccaagagactaaactattgtggatcaataataattgaaggttaggtattctcctgaacatcttcaggagaagatgaagtaggtaaaggatgatttggtgccttcttgttcaccatttctactaaaatattttaagtgcccttcctctaacactaatctattactgcaaggcttcaaaagacaggcaacgagatgggtcttgaatcgaactagaatgtttcttggttgaatttggcgaagtctgtaacaaatcttgcaaagaaaatctcgaaacctacgggtaccttctggttcaagatcctctgatggataagttaggtaaagtcttgagaataggttgtgaaaatagaagaatagaaggatgagaagagagattgtcggtaaatggagagatgactcttatttctttcaatgggggagctgaaaataattcagcagagtttccactctatcaatcctgacttattttgtggagggtaccttggccccttcatatataggggatgaagaggcctggtaaggttgttagactattaggagagtttgttagatcgttaatttattataatagaatgaccagctatataaaaatcatggagtatttacccacatggtgattgactgtagtataactgaaagatagctaatgcttagctggatgactgctgttagataactgtctgcattcttacggtacattgatattttaccaatgtgacatagcttaaatcggcaactggctgaactaaatattatgtatccctttagttaacaatcatgtcggttagagatcaatgtaattcgcagcagatcgatcataagctgagatgagtatcatattttaagaacaacgctgggcgagttaggccgatcaaatgtcagactgaaaaagcagatcaataaacctctgatgtgatctgaaagaatatttatgatttaaataataatctatcaccacgtatccagataatgaggtcatataacatgtaccaacagtgcatttttccatctagttaagaggttggttagtggcatttgtcttcgatatgtaatgttcacataactaatgtgcttagtagcattcttttgtaaggttaaatcttcaatgatcttaagttcacataattgcctttgtgccctattagtttatagttgaccttttaattcaagagacagtcaccttagcaatcgatgtctgcttagattgggccaattaggtactcacattaatatattgaatcatgtttgaatataaaggattagattgatttataagtttccttttattgtttacatactgatacttagattgacttactacattatttgatatgttatgttctaatttttggattaaaattgttgtttctgatttctccttacatctaatactttgtataatttattattttttagcatgattgagtgtagaggattagattgatttttaagtttattttgattatttacatgcccatacttaaattgacttactacattattcaatatgttatgtttcaattattgagttaaaatttttatttctgatttctactgatgtccagtgtgtgtgtgtgtacgtatgtgtgtatatatttatttacatatatatgtatnnnnnnnnnnnnnnnnnnnnnnnnnnnnnnnnnnnnnnnnnnnnnnnnnnnnnnnnnnnnnnnnnnnnnnnnnnnnnnnnnnnnnnnnnnnnnnnnnnnnnnnnnnnnnnnnnnnnnnnnnnnnnnnnnnnnnnnnnnnnnnnnnnnnnnnnnnnnnnnnnnnnnnnnnnnnnnnnnnnnnnnnnnnnnnnnnnnnnnnnnnnnnnnnnnnnnnnnnnnnnnnnnnnnnnnnnnnnnnnnnnnnnnnnnnnnnnnnnnnnnnnnnnnnnnnnnnnnnnnnnnnnnnnnnnnnnnnnnnnnnnnnnnnnnnnnnnnnnnnnnnnnnnnnnnnnnnnnnnnnnnnnnnnnnnnnnnnnnnnnnnnnnnnnnnnnnnnnnnnnnnnnnnnnnnnnnnnnnnnnnnnnnnnnnnnnnnnnnnnnnnnnnnnnnnnnnnnnnnnnnnnnnnnnnnnnnnnnnnnnnnnnnnnnnnnnnnnnnnnnnnnnnnnnnnnnnnnnnnnnnnnnnnnnnnnnnnnnnnnnnnnnnnnnnnnnnnnnnnnnnnnnnnnnnnnnnnnnnnnnnnnnnnnnnnnnnnnnnnnnnnnnnnnnnnnnnnnnnnnnnnnnnnnnnnnnnnnnnnnnnnnnnnnnnnnnnnnnnnnnnnnnnnnnnnnnnnnnnnnnnnnnnnnnnnnnnnnnnnnnnnnnnnnnnnnnnnnnnnnnnnnnnnnnnnnnnnnnnnnnnnnnnnnnatgtatacatatacatgtatacatacatatatagatatatatatatacatatatgtatatatatatatatatatacacatatataggttatttggaacctaagaaacttgcaaagttactagatgcaatgttcggaaaccatggaccgtaacaactggagtagtatttgggtcatgaattcatggctagatcatgaattgagtgggagtcaaccgaagtagggccagctcagacacttgtatttaggtcccatgcttgcgtgcattctcttccctgatatcctttggctttgctgcctcaaatcctcgagctatcttatcatcatcgcattgagctccataccttgctctttccta

SEQ ID NO: 55 - DNA, 4061 bp, Artificial Sequence
  synthetic
  misc_feature (2098)..(2825): n is a, c, g, or t
tagattcttgcagatgttttgagagtgattggaaaagtgatgcaaaatagggcattagataccccttgtagtcttataatggctctgaagccttcaagatgatttaagggattgatggagccatcgaatgtttccaatgtaggtatcttgaatcgaggaggaactgatttaccaagaattttttgagaaaaaagagatcgtaagttgaaatctcttctaccttgagaatggcttccaatctatatctccatcattttcttctcaagattttgaatcttttgtccaagaccctcctccatacatggcttcttatgtggagcagatttcacttcccaagagtgatcagtatggtcaagaagatgatcatgatgaagatcttgaggagttggttgctaagtgtgatgtgattggactacttggggggctactttttgctaccgttctgtcgtatactacagcagtaagagcttggacctgctgaaccaagagactaaactattgtggatcaataataattgaaggttaggtattctcctgaacatcttcaggagaagatgaagtaggtaaaggatgatttggtgccttcttgttcaccatttctactaaaatattttaagtgcccttcctctaacactaatctattactgcaaggcttcaaaagacaggcaacgagatgggtcttgaatcgaactagaatgtttcttggttgaatttggcgaagtctgtaacaaatcttgcaaagaaaatctcgaaacctacgggtaccttctggttcaagatcctctgatggataagttaggtaaagtcttgagaataggttgtgaaaatagaagaatagaaggatgagaagagagattgtcggtaaatggagagatgactcttatttctttcaatgggggagctgaaaataattcagcagagtttccactctatcaatcctgacttattttgtggagggtaccttggccccttcatatataggggatgaagaggcctggtaaggttgttagactattaggagagtttgttagatcgttaatttattataatagaatgaccagctatataaaaatcatggagtatttacccacatggtgattgactgtagtataactgaaagatagctaatgcttagctggatgactgctgttagataactgtctgcattcttacggtacattgatattttaccaatgtgacatagcttaaatcggcaactggctgaactaaatattatgtatccctttagttaacaatcatgtcggttagagatcaatgtaattcgcagcagatcgatcataagctgagatgagtatcatattttaagaacaacgctgggcgagttaggccgatcaaatgtcagactgaaaaagcagatcaataaacctctgatgtgatctgaaagaatatttatgatttaaataataatctatcaccacgtatccagataatgaggtcatataacatgtaccaacagtgcatttttccatctagttaagaggttggttagtggcatttgtcttcgatatgtaatgttcacataactaatgtgcttagtagcattcttttgtaaggttaaatcttcaatgatcttaagttcacataattgcctttgtgccctattagtttatagttgaccttttaattcaagagacagtcaccttagcaatcgatgtctgcttagattgggccaattaggtactcacattaatatattgaatcatgtttgaatataaaggattagattgatttataagtttccttttattgtttacatactgatacttagattgacttactacattatttgatatgttatgttctaatttttggattaaaattgttgtttctgatttctccttacatctaatactttgtataatttattattttttagcatgattgagtgtagaggattagattgatttttaagtttattttgattatttacatgcccatacttaaattgacttactacattattcaatatgttatgtttcaattattgagttaaaatttttatttctgatttctactgatgtccagtgtgtgtgtgtgtacgtatgtgtgtatatatttatttacatatatatgtatnnnnnnnnnnnnnnnnnnnnnnnnnnnnnnnnnnnnnnnnnnnnnnnnnnnnnnnnnnnnnnnnnnnnnnnnnnnnnnnnnnnnnnnnnnnnnnnnnnnnnnnnnnnnnnnnnnnnnnnnnnnnnnnnnnnnnnnnnnnnnnnnnnnnnnnnnnnnnnnnnnnnnnnnnnnnnnnnnnnnnnnnnnnnnnnnnnnnnnnnnnnnnnnnnnnnnnnnnnnnnnnnnnnnnnnnnnnnnnnnnnnnnnnnnnnnnnnnnnnnnnnnnnnnnnnnnnnnnnnnnnnnnnnnnnnnnnnnnnnnnnnnnnnnnnnnnnnnnnnnnnnnnnnnnnnnnnnnnnnnnnnnnnnnnnnnnnnnnnnnnnnnnnnnnnnnnnnnnnnnnnnnnnnnnnnnnnnnnnnnnnnnnnnnnnnnnnnnnnnnnnnnnnnnnnnnnnnnnnnnnnnnnnnnnnnnnnnnnnnnnnnnnnnnnnnnnnnnnnnnnnnnnnnnnnnnnnnnnnnnnnnnnnnnnnnnnnnnnnnnnnnnnnnnnnnnnnnnnnnnnnnnnnnnnnnnnnnnnnnnnnnnnnnnnnnnnnnnnnnnnnnnnnnnnnnnnnnnnnnnnnnnnnnnnnnnnnnnnnnnnnnnnnnnnnnnnnnnnnnnnnnnnnnnnnnnnnnnnnnnnnnnnnnnnnnnnnnnnnnnnnnnnnnnnnnnnnnnnnnnnnnnnnnnnnnnnnnnnnnnnnnnnnnnatgtatacatatacatgtatacatacatatatagatatatatatatacatatatgtatatatatatatatatatacacatatataggttatttggaacctaagaaacttgcaaagttactagatgcaatgttcggaaaccatggaccgtaacaactggagtagtatttgggtcatgaattcatggctagatcatgaattgagtgggagtcaaccgaagtagggccagctcagacacttgtatttaggtcccatgcttgcgtgcattctcttccctgatatcctttggctttgctgcctcaaatcctcgagctatcttatcatcatcgcattgagctccataccttgctctttcctaactgcccccatcaaacctccggagatcctctttcttctccaatgttgagatttgttggagtcttcccaccttctcacttcaatgggtggcaatttcaagtgccagttcccttatttgtcccagctatattgacaatggggcttattctagggtttctcatggacatagtgataataataatcaagggaccaagagagaaaaatctttctagtctgtgttctttaagtttgagagataggcagcacatttttttaataagcctttttcactcatcggatcctgattttcagttgttcgacctgaacagttcaagcaattgaactgcttgggtcactattttggacgattttcagccatttttaagtattgtttgactggatccacgctgcgtagtgggcattgcgttgatcaagtagacctgtaagggtcaacaaggtctgagaacactgaatggatgctccataatcctcttgttatctgtcaaccatttggaatcttttaaaacaacatgtggtgataatatatatgataaactgtgatagattcatgtatagattatacatatgaaaatgtagagtgcttagtaaaagtgatgaagagcaatgcgttagaatgtgctagcctttgacctaaaaattggaatgcccaatgatgagttatgataaaattgtgacgtgatttatgaagtctaatgtttagttggcttgcagtttcagatgcgataaagaattttatgatttagctctttggttttttaacatgcaaacatttaattgtactgaaaaacatttatttcgaaacatgtaggagactattggatattgaaattaaaattgactttttggtgtttcacaatatttcttaataaacactacgacta

SEQ ID NO: 56 - DNA, 4061 bp, Artificial Sequence
  synthetic
  misc_feature (218)..(1631): n is a, c, g, or t
aagctccgtgcttctgtctttgagaagtgtctgagtaggtagtcgatcccaggcaaccttctagaggaaaagtctgatcctagagtggatagccatgtgtatatatatatatatatatatgtatgtatgtatgtatgtatgtatgtatgtatgtacgtacatacatacatacacacacatacatacatatacatacatacatatacatacatacatannnnnnnnnnnnnnnnnnnnnnnnnnnnnnnnnnnnnnnnnnnnnnnnnnnnnnnnnnnnnnnnnnnnnnnnnnnnnnnnnnnnnnnnnnnnnnnnnnnnnnnnnnnnnnnnnnnnnnnnnnnnnnnnnnnnnnnnnnnnnnnnnnnnnnnnnnnnnnnnnnnnnnnnnnnnnnnnnnnnnnnnnnnnnnnnnnnnnnnnnnnnnnnnnnnnnnnnnnnnnnnnnnnnnnnnnnnnnnnnnnnnnnnnnnnnnnnnnnnnnnnnnnnnnnnnnnnnnnnnnnnnnnnnnnnnnnnnnnnnnnnnnnnnnnnnnnnnnnnnnnnnnnnnnnnnnnnnnnnnnnnnnnnnnnnnnnnnnnnnnnnnnnnnnnnnnnnnnnnnnnnnnnnnnnnnnnnnnnnnnnnnnnnnnnnnnnnnnnnnnnnnnnnnnnnnnnnnnnnnnnnnnnnnnnnnnnnnnnnnnnnnnnnnnnnnnnnnnnnnnnnnnnnnnnnnnnnnnnnnnnnnnnnnnnnnnnnnnnnnnnnnnnnnnnnnnnnnnnnnnnnnnnnnnnnnnnnnnnnnnnnnnnnnnnnnnnnnnnnnnnnnnnnnnnnnnnnnnnnnnnnnnnnnnnnnnnnnnnnnnnnnnnnnnnnnnnnnnnnnnnnnnnnnnnnnnnnnnnnnnnnnnnnnnnnnnnnnnnnnnnnnnnnnnnnnnnnnnnnnnnnnnnnnnnnnnnnnnnnnnnnnnnnnnnnnnnnnnnnnnnnnnnnnnnnnnnnnnnnnnnnnnnnnnnnnnnnnnnnnnnnnnnnnnnnnnnnnnnnnnnnnnnnnnnnnnnnnnnnnnnnnnnnnnnnnnnnnnnnnnnnnnnnnnnnnnnnnnnnnnnnnnnnnnnnnnnnnnnnnnnnnnnnnnnnnnnnnnnnnnnnnnnnnnnnnnnnnnnnnnnnnnnnnnnnnnnnnnnnnnnnnnnnnnnnnnnnnnnnnnnnnnnnnnnnnnnnnnnnnnnnnnnnnnnnnnnnnnnnnnnnnnnnnnnnnnnnnnnnnnnnnnnnnnnnnnnnnnnnnnnnnnnnnnnnnnnnnnnnnnnnnnnnnnnnnnnnnnnnnnnnnnnnnnnnnnnnnnnnnnnnnnnnnnnnnnnnnnnnnnnnnnnnnnnnnnnnnnnnnnnnnnnnnnnnnnnnnnnnnnnnnnnnnnnnnnnnnnnnnnnnnnnnnnnnnnnnnnnnnnnnnnnnnnnnnnnnnnnnnnnnnnnnnnnnnnnnnnnnnnnnnnnnnnnnnnnnnnnnnnnnnnnnnnnnnnnnnnnnnnnnnnnnnnnnnnnnnnnnnnnnnnnnnnnnnnnnnnnnnnnnnnnnnnnnnnnnnnnnnnnnnnnnnnnnnnnnnnnnnnnnnnnnnnnnnnnnnnnnnnnnnnnnnnnnnnnnnnnnnnnnnnnnnnnnnnntatatatatatagtatactatatagtatatatatagtatatatagtatatatatatatatatatatatagtatatatatatatatatatatatatatgtgtgtgtgtgtgtgtgcgcgtgcgcgcacgcacgtgtgtatctcgatctgtgtgtgtgtggtccatcttcacacttttccctcaaaaaaaccccccttgagattttgttcagctgaaaggggttcataaaacttgcccttgcttggtcctagggtttaagatttatatgcaatattcattaagacgtctaaatgtcataatattttgaggttacaaatattaacaaacagccttggatacaaacctttttctcgaagaatcttgtatctgttcttcctcagatgacatgtgatttatgctacggcctagttctaaggacttttctctgtcattaacataaaaaaaaacagaaatatattccttagtaaggaaatagttgtgcactatgattgctatgtctctcaaaattataccaaactttttatgatatagagtgaaaatcaaatcagcatgtctggtctatttgccaaatagggttgagcataggtcgggttcggtcgagttgagagaaaaatttcatccgatcaaattcaatcggattgaagaaaattcaatccactgccaatcattcattatgcataaactatctaaaactgaaatgaatagtttgtagcaggatcaggtgttatgtcagtttggacttcaatgttaacccaatattgattttaaatccaacattggtccacttagacttatttatttatttttatcaatttaatataaaaaagatctaaacctcataagtcataaattttggatttatttttgaacatgtacaaaataaaacagaaaaaagaaaaaattacttatctaaaagtaactatatctgaaaactttcactttagaattgtcttaaattaatgtacttccatcaacaattcaatgttaatatttttatgaatccaaatggatgatagagtattttttagaatgaagtattgaagtctaaatgacatcgtcccaaaataaaagtgaatttatgaaatactacatctgtcggattcggtttcatacggattaaaagtgtaggaatagaatccgattataaataattatttttttataaattctaattcaattttattcgatttatattttttaaccggtcaaaattaatatttattaagtaggattggatggatttattcgtatctcgattatttgctcagcccattgccaaatctaaactcttttcagataggttccatgtgaacatgatacatgagatgcagtgtgatagtacacaccattgctaagaaaactttggagtttgcgtaacaatatctgtttaccatttaaaaaatggcagttttgaattttaacacgctctcctccagattcagcttatgaacttttcgaataaaaatacccctggactatttttccaaaaagtaccagcatcttttgaacttgaatggaaattcggccaataaaatgttttcatttattgaagaaataaacagggtaacgcagtagctctatttcctctgcttttcttttctatattaataacatgattattcatctctctcggatcacaaaaaaattaagctattcaagctttatttatatttcatttttaaattttttacttaaatacaaaatctcccatcccactactacggcagcatgttttctatgtatgattattttcattcaaatgatatcattttttataatttatattgtatgtaattaattcatttatagttcttacattttcctgtttctagtagatacaataaagcggttttggactagtagcttgttctctgtatcgaagtttaactaaagctttgacaataatatatgaatccatatcactgggtaggagaggaatatgttgggtataaaggatttaaggaattagatattttcatacaattgtattgcattgcagacagtaattagattactatgcaattattctctctctccatgtttgttgcagttgaagaactctaatgaagctcacaaaaatttactgcatgaacttgtaagtggaattagacgactccgttgtcctccattttcttttattttctttaaaatcatctgccattcaaatagacagaaaaaaaaggattgattagctattggatgcctcttgaattcaggaaatgaaggacgagcacccagtttatggttttgtggatgatgaccctagcaactacgcaggtgcactagctcttgccaatggggcttcccacatgtatgctttccgtgttcagccgagccagccgaatctccatcgaatggggtttggctcccatgacctgcgccttgcttgattttattgtagcttaaagaccttacaacttccagagtggtg

SEQ ID NO: 57 - DNA, 4061 bp, Artificial Sequence
  synthetic
cagtttggacttcaatgttaacccaatattgattttaaatccaacattggtccacttagacttatttatttatttttatcaatttaatataaaaaagatctaaacctcataagtcataaattttggatttatttttgaacatgtacaaaataaaacagaaaaaagaaaaaattacttatctaaaagtaactatatctgaaaactttcactttagaattgtcttaaattaatgtacttccatcaacaattcaatgttaatatttttatgaatccaaatggatgatagagtattttttagaatgaagtattgaagtctaaatgacatcgtcccaaaataaaagtgaatttatgaaatactacatctgtcggattcggtttcatacggattaaaagtgtaggaatagaatccgattataaataattatttttttataaattctaattcaattttattcgatttatattttttaaccggtcaaaattaatatttattaagtaggattggatggatttattcgtatctcgattatttgctcagcccattgccaaatctaaactcttttcagataggttccatgtgaacatgatacatgagatgcagtgtgatagtacacaccattgctaagaaaactttggagtttgcgtaacaatatctgtttaccatttaaaaaatggcagttttgaattttaacacgctctcctccagattcagcttatgaacttttcgaataaaaatacccctggactatttttccaaaaagtaccagcatcttttgaacttgaatggaaattcggccaataaaatgttttcatttattgaagaaataaacagggtaacgcagtagctctatttcctctgcttttcttttctatattaataacatgattattcatctctctcggatcacaaaaaaattaagctattcaagctttatttatatttcatttttaaattttttacttaaatacaaaatctcccatcccactactacggcagcatgttttctatgtatgattattttcattcaaatgatatcattttttataatttatattgtatgtaattaattcatttatagttcttacattttcctgtttctagtagatacaataaagcggttttggactagtagcttgttctctgtatcgaagtttaactaaagctttgacaataatatatgaatccatatcactgggtaggagaggaatatgttgggtataaaggatttaaggaattagatattttcatacaattgtattgcattgcagacagtaattagattactatgcaattattctctctctccatgtttgttgcagttgaagaactctaatgaagctcacaaaaatttactgcatgaacttgtaagtggaattagacgactccgttgtcctccattttcttttattttctttaaaatcatctgccattcaaatagacagaaaaaaaaggattgattagctattggatgcctcttgaattcaggaaatgaaggacgagcacccagtttatggttttgtggatgatgaccctagcaactacgcaggtgcactagctcttgccaatggggcttcccacatgtatgctttccgtgttcagccgagccagccgaatctccatcgaatggggtttggctcccatgacctgcgccttgcttgattttattgtagcttaaagaccttacaacttccagagtggtgttatatattagtatcttaagctatgacagtggtaagcctctctatccgctacttgttatcctttaggtactttgcatgtggtgcaaggttataattgccttgtgtttctattgtcttcctcatggtacttactggactgatgatgtcaagtgaaatggagttgtttgaatcctgactgaaatttctcttggtccatcaagtgcaagagtaagtttagacatcactcgcaagcttttgctaggaaataagtagtttcattgcactaatgatttcgaatttttgttttcgggttagagaaacctagattaatgctgttattggatgctggcagtcagatgaagattatgtttgattgtacctcgttggacagatgctcatgcgtagatccataactctatttcatttcatttccctgtacacaattgaaacagggcatatatgaataggtatagaacagatgattcctgcaatattggaggtggctagctcagcttagactaaagttggtctagctgggatattctgaacacctgagatgttcaaataatgtgggataacttggcccaactcaactaaacattggctcaaagcatagtcaaggtaaagcttgagcaagctcttttgagcttggttcgagtccgagctgagcccgggccgcttgtttagctgatgaactgaattcaaatagccggtactcagcttggctccactcgattcatgagttcgaatcccctcaagttcaacctcgaacttgacggtgtagtcccacaaccatggccaccttataatgtgggacggccattatgcattcctctagtgcctgctccatatgacttttgttctcattataccatgcacctaaatgagtgctcatagtgacaatgtttagcctccacgtataatgtgtgccagctaactagaagcctaaactttggtgaaatttctgcaatgttgtggttgtaaaacgctcctacgttgagacatgatggtatctaagattatagacaaactatcatgctgaatcaacccaaatccaaggtgaataaaacttgatacaaagccgagctccattgaaatagtacaatggattctgcacttgaagaacattacaaaatcattttttcccaaaaagaaacattgcgaacagaccaaagcgtaaagaaattacatgattcaactaattcaagctttccatgatgtaggcactcgctagatgtagtagggtgataacttgctttgtgagggtggatcataagcttaacctcaatctatcccaatctatcctttcccttgacctatccatgccaatctaggccatttctgcataaatataacttaatcccagtggatccggcctagtttcactcactccaacacattcctactcaatggtagccaatcctttctttagccctcaaatataatcctaatctagcatagccaaccatcaatcatgcctaataaagcccgactacaccaacccgatcattcctgatcgtacacaatcaagacttatcctaattgatcctagctttttttaggcctctcttatagaacctgtgccaattctggacaagctaatccaatcttagcagccaaaaatattacatgtttaattagccaaatcgaacctatcataaacccaatatataatcggaccataccaagatcatcatcctatatttccttctcttgttataactacacctaaaaaggaatttcttcatacttatgaggggtatattatgataaaaattccttcattttagccctccatccttgtctatttttgggaccactagccaagtaacaccttaagagccctccatcttaatattccctctaactagctcgatttcttcttcattctttctttgcgatgtgtcccctccaatttaattcttacatgttgggatttgagtactgaaaaataatagataaagagaaagtaaaaactatgctaatgataataccaaaggcataaagaaatcacagcagtcgcaaaaacatcaaatttttttatggttcggcctaagcctatatctacatagggacgagagtaagaagaagcttccactataataatagtttagagtacaaaaacttctctgacaccatgtagggaacatcgcttctaatacaagaaagaagaaatccaagattaaacaaacctctagaaaaattcttctcgatggaataactctaatctgagattgaacaatcttctccaatcgatgatctccaatcttcttttcttaaatgaagcacccttcaagcctctcttcttttctctcttcctatcctcttttgtggctcacaacctcctctcctttttatgttctatgttcctcacatcacat

SEQ ID NO: 58 - DNA, 4061 bp, Artificial Sequence
  synthetic
tttcagataggttccatgtgaacatgatacatgagatgcagtgtgatagtacacaccattgctaagaaaactttggagtttgcgtaacaatatctgtttaccatttaaaaaatggcagttttgaattttaacacgctctcctccagattcagcttatgaacttttcgaataaaaatacccctggactatttttccaaaaagtaccagcatcttttgaacttgaatggaaattcggccaataaaatgttttcatttattgaagaaataaacagggtaacgcagtagctctatttcctctgcttttcttttctatattaataacatgattattcatctctctcggatcacaaaaaaattaagctattcaagctttatttatatttcatttttaaattttttacttaaatacaaaatctcccatcccactactacggcagcatgttttctatgtatgattattttcattcaaatgatatcattttttataatttatattgtatgtaattaattcatttatagttcttacattttcctgtttctagtagatacaataaagcggttttggactagtagcttgttctctgtatcgaagtttaactaaagctttgacaataatatatgaatccatatcactgggtaggagaggaatatgttgggtataaaggatttaaggaattagatattttcatacaattgtattgcattgcagacagtaattagattactatgcaattattctctctctccatgtttgttgcagttgaagaactctaatgaagctcacaaaaatttactgcatgaacttgtaagtggaattagacgactccgttgtcctccattttcttttattttctttaaaatcatctgccattcaaatagacagaaaaaaaaggattgattagctattggatgcctcttgaattcaggaaatgaaggacgagcacccagtttatggttttgtggatgatgaccctagcaactacgcaggtgcactagctcttgccaatggggcttcccacatgtatgctttccgtgttcagccgagccagccgaatctccatcgaatggggtttggctcccatgacctgcgccttgcttgattttattgtagcttaaagaccttacaacttccagagtggtgttatatattagtatcttaagctatgacagtggtaagcctctctatccgctacttgttatcctttaggtactttgcatgtggtgcaaggttataattgccttgtgtttctattgtcttcctcatggtacttactggactgatgatgtcaagtgaaatggagttgtttgaatcctgactgaaatttctcttggtccatcaagtgcaagagtaagtttagacatcactcgcaagcttttgctaggaaataagtagtttcattgcactaatgatttcgaatttttgttttcgggttagagaaacctagattaatgctgttattggatgctggcagtcagatgaagattatgtttgattgtacctcgttggacagatgctcatgcgtagatccataactctatttcatttcatttccctgtacacaattgaaacagggcatatatgaataggtatagaacagatgattcctgcaatattggaggtggctagctcagcttagactaaagttggtctagctgggatattctgaacacctgagatgttcaaataatgtgggataacttggcccaactcaactaaacattggctcaaagcatagtcaaggtaaagcttgagcaagctcttttgagcttggttcgagtccgagctgagcccgggccgcttgtttagctgatgaactgaattcaaatagccggtactcagcttggctccactcgattcatgagttcgaatcccctcaagttcaacctcgaacttgacggtgtagtcccacaaccatggccaccttataatgtgggacggccattatgcattcctctagtgcctgctccatatgacttttgttctcattataccatgcacctaaatgagtgctcatagtgacaatgtttagcctccacgtataatgtgtgccagctaactagaagcctaaactttggtgaaatttctgcaatgttgtggttgtaaaacgctcctacgttgagacatgatggtatctaagattatagacaaactatcatgctgaatcaacccaaatccaaggtgaataaaacttgatacaaagccgagctccattgaaatagtacaatggattctgcacttgaagaacattacaaaatcattttttcccaaaaagaaacattgcgaacagaccaaagcgtaaagaaattacatgattcaactaattcaagctttccatgatgtaggcactcgctagatgtagtagggtgataacttgctttgtgagggtggatcataagcttaacctcaatctatcccaatctatcctttcccttgacctatccatgccaatctaggccatttctgcataaatataacttaatcccagtggatccggcctagtttcactcactccaacacattcctactcaatggtagccaatcctttctttagccctcaaatataatcctaatctagcatagccaaccatcaatcatgcctaataaagcccgactacaccaacccgatcattcctgatcgtacacaatcaagacttatcctaattgatcctagctttttttaggcctctcttatagaacctgtgccaattctggacaagctaatccaatcttagcagccaaaaatattacatgtttaattagccaaatcgaacctatcataaacccaatatataatcggaccataccaagatcatcatcctatatttccttctcttgttataactacacctaaaaaggaatttcttcatacttatgaggggtatattatgataaaaattccttcattttagccctccatccttgtctatttttgggaccactagccaagtaacaccttaagagccctccatcttaatattccctctaactagctcgatttcttcttcattctttctttgcgatgtgtcccctccaatttaattcttacatgttgggatttgagtactgaaaaataatagataaagagaaagtaaaaactatgctaatgataataccaaaggcataaagaaatcacagcagtcgcaaaaacatcaaatttttttatggttcggcctaagcctatatctacatagggacgagagtaagaagaagcttccactataataatagtttagagtacaaaaacttctctgacaccatgtagggaacatcgcttctaatacaagaaagaagaaatccaagattaaacaaacctctagaaaaattcttctcgatggaataactctaatctgagattgaacaatcttctccaatcgatgatctccaatcttcttttcttaaatgaagcacccttcaagcctctcttcttttctctcttcctatcctcttttgtggctcacaacctcctctcctttttatgttctatgttcctcacatcacatccacagactcatttttatagataaaaaattagagtctatttcggactccttttccacacacaagatggcttcccacgccattggttccgtgcgcatgacttttttcatgccacaaaggattccgtgctgcaaaagttttccatatccatgcagtttccacacaccacaaaaactttcgcacacttctcgaaggcttttcatgctcgaccctttttggttttcaattaaattgatggatcccatatgaggagggaccacaccaataaatctcctccttctaactcatatggtaggttccatcaagcctgtagcacctttgcattttatcagttttgttcctgaagccggcttcatcaatatattagaactattttcttcagtgtcaacttttttaagcttgaaccacttcatctctagcatattgacatgcttttggaaagtatgtcaaattgctcaaaattaatcttacggttctctttttcgttagattctagtgcatattacgcactttaacataagatctaaggaaggaagaggactgaggtaaggtgaagtgattt

SEQ ID NO: 59 - DNA, 4061 bp, Artificial Sequence
  synthetic
  misc_feature (3947)..(4061): n is a, c, g, or t
cctagattaatgctgttattggatgctggcagtcagatgaagattatgtttgattgtacctcgttggacagatgctcatgcgtagatccataactctatttcatttcatttccctgtacacaattgaaacagggcatatatgaataggtatagaacagatgattcctgcaatattggaggtggctagctcagcttagactaaagttggtctagctgggatattctgaacacctgagatgttcaaataatgtgggataacttggcccaactcaactaaacattggctcaaagcatagtcaaggtaaagcttgagcaagctcttttgagcttggttcgagtccgagctgagcccgggccgcttgtttagctgatgaactgaattcaaatagccggtactcagcttggctccactcgattcatgagttcgaatcccctcaagttcaacctcgaacttgacggtgtagtcccacaaccatggccaccttataatgtgggacggccattatgcattcctctagtgcctgctccatatgacttttgttctcattataccatgcacctaaatgagtgctcatagtgacaatgtttagcctccacgtataatgtgtgccagctaactagaagcctaaactttggtgaaatttctgcaatgttgtggttgtaaaacgctcctacgttgagacatgatggtatctaagattatagacaaactatcatgctgaatcaacccaaatccaaggtgaataaaacttgatacaaagccgagctccattgaaatagtacaatggattctgcacttgaagaacattacaaaatcattttttcccaaaaagaaacattgcgaacagaccaaagcgtaaagaaattacatgattcaactaattcaagctttccatgatgtaggcactcgctagatgtagtagggtgataacttgctttgtgagggtggatcataagcttaacctcaatctatcccaatctatcctttcccttgacctatccatgccaatctaggccatttctgcataaatataacttaatcccagtggatccggcctagtttcactcactccaacacattcctactcaatggtagccaatcctttctttagccctcaaatataatcctaatctagcatagccaaccatcaatcatgcctaataaagcccgactacaccaacccgatcattcctgatcgtacacaatcaagacttatcctaattgatcctagctttttttaggcctctcttatagaacctgtgccaattctggacaagctaatccaatcttagcagccaaaaatattacatgtttaattagccaaatcgaacctatcataaacccaatatataatcggaccataccaagatcatcatcctatatttccttctcttgttataactacacctaaaaaggaatttcttcatacttatgaggggtatattatgataaaaattccttcattttagccctccatccttgtctatttttgggaccactagccaagtaacaccttaagagccctccatcttaatattccctctaactagctcgatttcttcttcattctttctttgcgatgtgtcccctccaatttaattcttacatgttgggatttgagtactgaaaaataatagataaagagaaagtaaaaactatgctaatgataataccaaaggcataaagaaatcacagcagtcgcaaaaacatcaaatttttttatggttcggcctaagcctatatctacatagggacgagagtaagaagaagcttccactataataatagtttagagtacaaaaacttctctgacaccatgtagggaacatcgcttctaatacaagaaagaagaaatccaagattaaacaaacctctagaaaaattcttctcgatggaataactctaatctgagattgaacaatcttctccaatcgatgatctccaatcttcttttcttaaatgaagcacccttcaagcctctcttcttttctctcttcctatcctcttttgtggctcacaacctcctctcctttttatgttctatgttcctcacatcacatccacagactcatttttatagataaaaaattagagtctatttcggactccttttccacacacaagatggcttcccacgccattggttccgtgcgcatgacttttttcatgccacaaaggattccgtgctgcaaaagttttccatatccatgcagtttccacacaccacaaaaactttcgcacacttctcgaaggcttttcatgctcgaccctttttggttttcaattaaattgatggatcccatatgaggagggaccacaccaataaatctcctccttctaactcatatggtaggttccatcaagcctgtagcacctttgcattttatcagttttgttcctgaagccggcttcatcaatatattagaactattttcttcagtgtcaacttttttaagcttgaaccacttcatctctagcatattgacatgcttttggaaagtatgtcaaattgctcaaaattaatcttacggttctctttttcgttagattctagtgcatattacgcactttaacataagatctaaggaaggaagaggactgaggtaaggtgaagtgattttttttgagttggtaatggtacaaaagttatactagaccgtgggtacctaatctcggagattaccatttagatttggttcttgatcatttgtatagtgatgcatttaaaaaattatttgagcaaaacagtgaatgccattgggtctgagagatccaaaaccaaataacctaaagtatatagatggttcctttagctagatcatgtatgagaaaaaatgatctgccgactggaaaaaatagatctttgagctcattgattgttaagtcatatctagtctgtgaatcatctctttgaggattaatgatcaagctatcttttatgggttaaaagaataggatcactgaaatacttatcctagtatacatataatgtgcatggcctatttgatgagtcagactagaaggttatcactacttcatcacctttactgatgagcaatcatgatatagatatgtatgtgagatacaaatctaaaagattttgaatggttcaaagaattcagatatgaagtagaaaagataaatcaaaaaatttttaaaggtacttgatcggatctagaatgcaataccaaataaaaaatttgttgattatctaaaaaaagtgatatagtttcatgatggaattcttcttgtacacctcagctcaacggtatatatatgaggagcaatagcactatatgagatatggtccggtccatcatgaatatcactaatttaattattatttatttaagagcaagatttaatttttaaaatttaaattagattttttctaaaattggtttcaccgcaccatatgagatatgatttggtggataagttagaggataggtctgtgagaactcatttatagggtatcccaaaaggtatttaaaatattactttttctttctagtagttgacaatatgattgtgagcaatcatactgttttcttaaaaacagtggaaggatgaactcaaaaagaaagtctctaaagaacaacgagtcacaagacctatacaacctatttaagatgagccagtatatgtagtacttccttcacctcatcaatttagtaggatctcctatcctttagaaagatactcggtattcttacaaaggatttagagaaagtgtttcttgagggagattgagaatatagggatgatctcaaaacctacaatgacataatataaggaatcatgtagttacatgaaggtcagtgggagggttccatactgacatcgattatgatgtggttacatatagaatttttttttcaaagatctagatcaaacattctgaaaataaaaggtctatagagataaatccgaaaaggatgtttgnnnnnnnnnnnnnnnnnnnnnnnnnnnnnnnnnnnnnnnnnnnnnnnnnnnnnnnnnnnnnnnnnnnnnnnnnnnnnnnnnnnnnnnnnnnnnnnnnnnnnnnnnnnnnnnnnnn

SEQ ID NO: 60 - DNA, 4061 bp, Artificial Sequence
  synthetic
tataccatagatttttctgttaaccacatgtcaattcttctcctccattgattttcattacaatattcaggaacagctgctttcatcttctcaacaaataagtcaacattaaaatggttagactttagatcattcttccaatgcctccacatagcccctattttttccagtagagactttcttatggcatccatgtacttagataaaaatataaatatatcctacacctagaaactgacttttagaaaaagtgtatatatacctaaataaaatgatttaagatgaaaatattcactatacctctagttcagctatcatcttttccttgaagcctgatggcacatcatgccaagagtcataatcgattggagcattatcaaattgtcttaccattgactgtatataatttgacaaattagtagcttccacccggattgattgtccaagttcacttaggttggcaacaacatgctctccctcttttagatcacgtaactcagacatacgtatgtatcctctccttctaggccagctagtcgaacctacaaatatgtatacacaattaaaaaaatacataaaatgtaagaaaatgatccctcaaaattaataattatcatatgcaccatcctttatttggttattagtgatctatttatgcaattcattcgaagaagattatatatgtatacctagttgactttcattggtagctaagggaggtagctcttaggcaactgattcagttttctcataattttgggcttcaagtgactgctcctattgattatgagatggaggctcaccttgattctgactttaagagttttctgtaccactaatattgacaattgtctgcttgtgttttgccattattaatgtaatttgaaagaaaaaaatagaattcatatatctgaatgttagtgaccaaaaaaacttgcaagtatctccccaaccatctaaagattatacgctattttatttttcaaatcttaaaaggctaacaaggcacatagcaattacatgaagcaaaaaaagaaaataaataaagcaccaaggaaaccattacactgtcattactgaaattacattcaatagtattatgcattaaaacaaaaactacattgataaaataaaattgaaaataagaaactacaagctcgtgggtgttccctcttgatcaaaacatatcctcaaactctaaatcttcatcgtgttggtgcacttcttgaacaaccacttctttaaatggctcttcacctcgaatcaaatctgaaggttgaagctgatcctcatacatttgttgtggcacatgatcactaacaatagagttcacatctcccaaatcataattgtctctaactttaaccgacttaacaataaccacatctttatgtctaggagtattaatatagaacatctttgcttgagatgcaaatacgaaaggatcgtcaagcacaccttcaccagtatgtgctaagtaagaaaaattcacaagtacaataaaatttatctttcttgcatcctttattgatatcaacccaatcgcacttgaataaatcaatcttgattttgcaatgataatttaattgaataatgtcctttaatataccataatactctattttttctttcaacaggctacctatctctagtcctagtgtaacccattgattcaactatcaccacaaccccactattttgagttctcaacttcctctcaagtgcttttgtgtggaatctaaagccattcataacgtaaccggtatatcatcgtgcaacatcaagtggctttcgagcaaggcacctaatttgtttagtaatatagacatcaccttgttgattcatgcatgcaacctaaattaacatggatttcaaatagtatattacaagatagaacattatgaggtaaatatatggtgtttatatattcaaattataaattataaaggagcatataaaacactcatttatgaaaccactcgaaaaattcctgactatgaatcctttcaatctcataagaagttaaatgacatggatgacatgaagctttgatatgcatcgaaacatattcacatggttattaatgagatgagtgatagtttggtagacttgccaacttaataactaacttaataacaaaatctccttactctcgaaatacggtaattgcatcgtagttaaataggatatatctgtgcgcttgcatcaactctttctcatcaagatggacccttggcactcgacttcacctttctggcctccatgacttttgctacttcctttctaaagatttttctggcctaaacattcttgaatcgacatcaagttggtcttcaccatcatcgcctacaagttggtcttcaccatcatctcctacaagtagatcttcgctattatcattccttcatggccaattgaaccttatttgaatcccacttaagtgtcgtaagcagaatgtacattatacattcatttgcaagatatgcttctgctattgagccctctggaggagctctattgcacacatatatcttaaggtaaccaagaagcctaaataaaaaattgaaagaaatgataacataaattaatcatcaaaaaatatcataacacataatgaaccaaattttaactataacacatccaaaattatacctctcaataggatacattcatctatgatgaactggatcagtcatcttagcctcgctcgctagatgaaccactaagtgaaccataactgtgaaaaaagatggtggaaaaatcttcctatttgacaaaaggtaagagcagctcaagattgaagccgctcaagattatccacatccaaaaccttgctataaagttctatgaaaaaattgcatagatcaataacagctaaagaaacatggtcaggaaaagacccaggggtagcaattggaaggatttcttcaatcaggacatgacagtcatacgacttaaggtgagcaagcttgtgttgtctcaactacacacacctctaaatgttggatgaacactcttctggaaatttcaattccttaatcacattgcaaaaatcatccttttcttttgcattcatttgaggcataaacttcaaataagtattgttgggtataaaataccccccggctgaagtctgtaaaagaccgacccttccaggactctttcggcttccgaccttgtgtgtggcatcactccaaacccccatgaccgtccggacttctccgatagagaacttctgcattcgtctaccgagccgccccaaaatgctctctgggcctcaccaccagccgaccttctacagtgatcaactattctccgaactccttccgaactctgccaatatccaagcttcttcgacaacgagatttctacagtaatcagactccatccaagtttctacgacggtcgaccgccttcaggattccaactgggctcctgtgagagccaaacttctactacggacagtctactccgaactcatacagtgagcggtctactctggatatccactataagcaaactccattcgagcctctgctgtaaacaaatttcttccaaactttcgttacaggtagacttcgatcgagcttcttcgtagccggatcccatacgagcttctacgatggggcaggatccaccggccaggtcgttactccgagctcccacgacaaccgatcttcgatcgagctccaacaataagtggcttcctttcggcctcccacaagaaccagactccgtccgagcttccacagtggatggattctggatgagctttcgcaatggacgagctctagcagctggatttctacaatgactgatcacctccgacgtctgtcgaacctccccagcgccatccgaagtccatcaccagctgacctcctgccagatccttcatgaaatcaaagttctccaatggatcatcttcagatgagcttccacatcaggtaaatctcagacggactcctctagcaatcgaacttctgttgggcttcaccaacgaaaagtctccatccgagcttctacaacagatgactcccacctgtggtatcagcgcctaaggt

SEQ ID NO: 61 - DNA, 4061 bp, Artificial Sequence
  synthetic
attttaaaatttttaataggataaaaaattttagttagctttgtgataggcctagcgaatccacgagctaccattctttgcttttggacaaattgcagatgcacgaagccaatcatgatatagttagcaaaactccttcaataggacaggaatgacaaactggctggccaaagcctcagtcggtgctttcaaagtgtatcgtcacctaacaataaagtagatattagaatcaccacaaggtaaaaaatttttaacgataaaattatttgtgatagataaaatttttattataaataataatgtcaatgatggtaaaaaattttcatcgataataaaaaaatatttacgatgaataaattttttcattataaataaaagtaattaacgacgaaaatattgcttacgtcgtaacaaacagaatatttgcgatgaaaattttaatcataaataagaaaatattttttaaataaaaatatagagatattaccgatgaaattatttttgttagaaatattaaaagttttttcgatgaaatcaggttttgcatcatcaataacattatttacgataaattttttttgtcactaataaatcaaaaaaaattaaaaattagatattttcaattatttgtgatgtaaattttagtcgtaaataatttgactatttgaaaactgagacatacctttaaaaaaaataaataaataaaaattgatccagctcgagatgatgatatatatttaatatattaattatatctatctatataacaataataaaatgatatacaggtattaggggtagcattctttattgacacataaagattataagatgatccctaaagtcttctttaattttttttttatttattttttgtttttctttaattttttctcttcttatttttgctgccatctgctgcctctgttttctctgctcctgctgcctccttttatagagcacagcttcttcgaattataagcatctatggactttcaattcccactatcttttattttgattgggattttaaaactttatccgcatcccagcatcttgtttcacgcgagatcctagcgtccacatgtgttttgaattccttatgggccacagaccatttaaaccaccaaagaccactttactattttgatttgaatcccatggaagccggctgcctctggtctcattcacccttccagtgcttcacatgggtcccattaatttgaattcctatgagccacatccaagcttttgaatccaagccttccttattttttaaatcaattaaaactttgctttaaatgccttgtagaccctcctatttgcatgctacgtgagaacattgttaagctcctcttggcccacttaagaacttctatgggctacatgcttttggctagctttaaaatggttttgggcctaactttggatcaccattcgaagtccattttgaattcaatttatttttatttttttttttaaccttacaaatcgagctcttttattggtgatcatttttcctataaaacaaaaacaaaaagcatcaagtcttaagaaataaaagttaattaatatatattttgatacttttattgggatatttaatgtacttatcactagatatgaaatccaatgggtcacacactttgaaatttgatcttagtctaatctaactaggatttattataaatcttatgggttaaatttacatgctagcacatgaattaactcaagttttcaattggatttagttctaaggtgtttgagctaaccctatcctgataccttaaacctaattagattagatttgaacctatggttttcttgatgccttatgcttattacatgaaagagtttcatgtgacttaaattcctccatgccaccacatcttcatccatgccaaattaatatggaacgccccatttaattgtgcatttaagaaggaatagtccttcttaaacactcctcttaatttcccacactttcctttgttctacacaccatcaaatggcttttggaaatatgcgggcgcagaagtagaggtgtcctatatgaaggctcttccacattataagttatcacatggtgaattaaatcattgtgtgagaaaatcatgcgccaagagttggcaccccttgggagttttaggcactccttatcctataaataaggggcaccccatatggataaatacaagggaattcaagtttaggcatgagattgagaggagaaaaagacacaaaaatctgagaaaaagataagaaaaaaaaagagagaaaaatagaaagaaaagacgagagaaaatgaaaggcaagggttgctaatcctagggttcaatttttcaatagttggatttctgaatcaatttggggtggtgagattttttgagaaaaagtttctgatgtggccctagtagaagattgaaggcattcagatgatggtgcaatccgtttttgaaaaagaaaagtgagtagtatacttatgaagaaagctgcaacactacatcaaattggaaaggaccttgatcaaacccatatggatcaccgttgcaggatatctactttggtatcttgtgaaggttattttttttatcagatcatcatcttcaaaaaggtataattttctacctaatatgcatgcttgatttgtttgattaaaatctataaagtgttcataaggtttgtgttctgattgtattgttttaagtattaaaacttactttaaaaatataaaaaaatttgaaaactatcttctactgtgcaactaaaatccaacagaataaccctaatatgagattgagcgatctccgccaatgttctcgatcttcttttcttgaatgaagccttttcaagcctctcttcttctctctctctccctatcttcttttgtggcccacggcctcctcttctttttatgttttgtgtttctcatgtcacatccataaactcccttttatagataaaaaattagagtccattttggactccttttccatgcataagaaggcttcccacgccattggttctgtgcacacgactttttccatgctacaaaagtttttcatgtctcacgtagtttccatgcgccataaaattttgcatacttctccaagactttttatgctcgaccctttttggttttcatttaaatcagtgggtcccatatgacgagggatcacaccaacatcatatgctctcctcaccataccaaatggtatccccaactataagacaaaacattcatcaaattgctaacagggttgaggatcagcattcactatagaaattttgtttttcaatctgtaacccctcccaccatcctggcctcttggatatcggacccatcaagtgggtcccgcgagcccgcacggcactgtcagtccccaaactcaattttttttttaggaaaaatgttacctgcagtagaagaaagagacctccaaaaaaattatgaaaaaaaagccttaaaataaaaatgaaaaggatgaagattaaaaggggtgcaacaggaggagttcccagggggtcatccatccctgtacgactctcgcccaagcacgctcgactgtggagttctgatgggatccggtgcattagtgctggtatgatcgcacccatcatgatctcttcgaaattcatagatataacatagcttccgttgcacgccatccataaccctcccaccgtccgggcctgcagggtaccagactcatcaagtgggctcgcgagcccgcacgtcactataggtctccagacttagttttttttgatagagaacattaaccatggtagaagaaagagatctccataaaaattatgaaaaaaaatattgaaataaaaataaaaggcttaaaaattatggaaaaaaaggcttgaaatagaaataaaaaggacgaagattaaaagggatgcaacatgaggtcctcccaggggttcatccatcttagaactactctcgcccaagcatgcttaactacgaagttctgatgggatctgacgtattggtgctggcatgatctcctcgaaattcttagatataacgtagcgaccgtcgcacccca

SEQ ID NO: 62 - DNA, 4061 bp, Artificial Sequence
  synthetic
gccggctgcctctggtctcattcacccttccagtgcttcacatgggtcccattaatttgaattcctatgagccacatccaagcttttgaatccaagccttccttattttttaaatcaattaaaactttgctttaaatgccttgtagaccctcctatttgcatgctacgtgagaacattgttaagctcctcttggcccacttaagaacttctatgggctacatgcttttggctagctttaaaatggttttgggcctaactttggatcaccattcgaagtccattttgaattcaatttatttttatttttttttttaaccttacaaatcgagctcttttattggtgatcatttttcctataaaacaaaaacaaaaagcatcaagtcttaagaaataaaagttaattaatatatattttgatacttttattgggatatttaatgtacttatcactagatatgaaatccaatgggtcacacactttgaaatttgatcttagtctaatctaactaggatttattataaatcttatgggttaaatttacatgctagcacatgaattaactcaagttttcaattggatttagttctaaggtgtttgagctaaccctatcctgataccttaaacctaattagattagatttgaacctatggttttcttgatgccttatgcttattacatgaaagagtttcatgtgacttaaattcctccatgccaccacatcttcatccatgccaaattaatatggaacgccccatttaattgtgcatttaagaaggaatagtccttcttaaacactcctcttaatttcccacactttcctttgttctacacaccatcaaatggcttttggaaatatgcgggcgcagaagtagaggtgtcctatatgaaggctcttccacattataagttatcacatggtgaattaaatcattgtgtgagaaaatcatgcgccaagagttggcaccccttgggagttttaggcactccttatcctataaataaggggcaccccatatggataaatacaagggaattcaagtttaggcatgagattgagaggagaaaaagacacaaaaatctgagaaaaagataagaaaaaaaaagagagaaaaatagaaagaaaagacgagagaaaatgaaaggcaagggttgctaatcctagggttcaatttttcaatagttggatttctgaatcaatttggggtggtgagattttttgagaaaaagtttctgatgtggccctagtagaagattgaaggcattcagatgatggtgcaatccgtttttgaaaaagaaaagtgagtagtatacttatgaagaaagctgcaacactacatcaaattggaaaggaccttgatcaaacccatatggatcaccgttgcaggatatctactttggtatcttgtgaaggttattttttttatcagatcatcatcttcaaaaaggtataattttctacctaatatgcatgcttgatttgtttgattaaaatctataaagtgttcataaggtttgtgttctgattgtattgttttaagtattaaaacttactttaaaaatataaaaaaatttgaaaactatcttctactgtgcaactaaaatccaacagaataaccctaatatgagattgagcgatctccgccaatgttctcgatcttcttttcttgaatgaagccttttcaagcctctcttcttctctctctctccctatcttcttttgtggcccacggcctcctcttctttttatgttttgtgtttctcatgtcacatccataaactcccttttatagataaaaaattagagtccattttggactccttttccatgcataagaaggcttcccacgccattggttctgtgcacacgactttttccatgctacaaaagtttttcatgtctcacgtagtttccatgcgccataaaattttgcatacttctccaagactttttatgctcgaccctttttggttttcatttaaatcagtgggtcccatatgacgagggatcacaccaacatcatatgctctcctcaccataccaaatggtatccccaactataagacaaaacattcatcaaattgctaacagggttgaggatcagcattcactatagaaattttgtttttcaatctgtaacccctcccaccatcctggcctcttggatatcggacccatcaagtgggtcccgcgagcccgcacggcactgtcagtccccaaactcaattttttttttaggaaaaatgttacctgcagtagaagaaagagacctccaaaaaaattatgaaaaaaaagccttaaaataaaaatgaaaaggatgaagattaaaaggggtgcaacaggaggagttcccagggggtcatccatccctgtacgactctcgcccaagcacgctcgactgtggagttctgatgggatccggtgcattagtgctggtatgatcgcacccatcatgatctcttcgaaattcatagatataacatagcttccgttgcacgccatccataaccctcccaccgtccgggcctgcagggtaccagactcatcaagtgggctcgcgagcccgcacgtcactataggtctccagacttagttttttttgatagagaacattaaccatggtagaagaaagagatctccataaaaattatgaaaaaaaatattgaaataaaaataaaaggcttaaaaattatggaaaaaaaggcttgaaatagaaataaaaaggacgaagattaaaagggatgcaacatgaggtcctcccaggggttcatccatcttagaactactctcgcccaagcatgcttaactacgaagttctgatgggatctgacgtattggtgctggcatgatctcctcgaaattcttagatataacgtagcgaccgtcgcaccccatcaataaccctcccacgtccaggcctgtagggcaccggacctttcatgtgcatccccataaaaattgtggaaaaaagtattgaattaaaaataaaatagacaaagattaaaaaaaatgcaacacgcccatcccagtacaactctcacccaagctcgttcgactgcggagttttgatgggatccggtgcattagtgctggtatgatcacacccatcacgatctcttcgaaattcatgtatataacgtagcttcaattgcacgccatctgtaaccctcccaccattcgggcctgtagggtatcggacccttcatgcgagctcgtacggcactgtaggtctccagacccagtttttttttgagagaaaacgttaaccttggcagaagaaagagatctctataaaaattgtagaagaaagtgtttgaataaaaataaaaagcataaaaattacaaaaaaaatcttgaaatagaaataaaaaggatgaagattaaaagggatgcaacatgtggacctcgctgggggttacccttcctagttctactctcgatcaagcatgcttaactacggagttctgatgggatccaatgtattagtgctggcatgatcgcacccatcatgatctcttagaaattcttagatataacgtagcggccgttgcatgccatcagtaaacctcccacgtccaggcctgtagggcactagacctatcaagtggatccggtgaggccgcacggcactgcctgtctccagactcaatttatttttttaagaattgtggaaagtgatccccataaaaattatgaaaaaaagtgttgaattaaaaataaaatagatgaagattaaaaaagatgcaacacgaggacttcccaggggtagatataacgtagcggccgttgcatgccatcagtaaacctcccacgtccaggcctgtagggcactagacctatcaagtggatcccgcgaggccgcacggcactgcctgtctccagactcaatttatttttttaagaattgtggaaagtgatccccataaaaattatggaaaaaagtgttgaattaaaaataaaatagatgaagattaaaaaagatgcaacaagaggacttcccaggggttcacccatcctaatattactctcgtccaagcacgcttaactatagagttctgaa

SEQ ID NO: 63 - DNA, 6704 bp, Artificial Sequence
  synthetic
aaatctattagtatctgacaaaagttaaattagagtcgaaacactaaatgacaattagggatcaacttgatcaagtagatagagaatattagaaaagagagaaattaacaagatagaacatgattaattaggtgacatagcccgacaatccaattggtctaagcaagttgatttaatcaaatcacggttgaactaatatatagatagctcaataaaaatcatacataattgaatctaatgatatttggatctgaccaagatggaatttgacatgctgtccgatgatcgtgaatcaagactctctttgctaattaagatcaaattagaatcattgaaagagaatcttttactggatcaagagagagaaatatataaagagagtgaaatagtctatagaaaaaaattttagagagagaaattaagaagaaaaaataaattttttagagaaagaaagtgggtatacaagctcagagaagggagagaggaaagagagagaaatgctctcttattttcttttttttcttttttcttcttttcttttttttttcctattcttctttcccttttctgcttaatggaataggggacctcccattccccttctatttctagagttgggggctcaaaattgatgatagctatcattggggatgtaggctatggtgatgcagtagaggatcaccgaccgatgatcgatggtgatgttgcaatcaaaaaatcaagaaagatagatggaaaataaaggaaaataaggagaaatagatctcaacttgtttggatgctaacccactcactgacgactccacttcaactatggccggagcttgctatggaaaagaagccaaggccttcaaggatgaacaccaatggtgaggaagatggtcgaaaatagaagaatggctggcttttctaatcgacaaaatagggtatcgcccttcttagcaaatattcggcaataaatatctagaatccaggatcctaggactatggaagagggagaggagggcaagtcaaaggatgccagattcttatctagcttccgacaatgatggggccctattttcgataaacacaattgaggatgttcggaaaagggttttttcgatgatgattctagtgaccaactatgagatttcaaagggggtgaggggggtttaaataagatgggagggaagtttgaatcctccttaaatctgaacctttttcgacaaagccaagagcgtgaaggagactccttcgtgaagtcaaagatggaatagactcccttcgggagtttggttcatcacccaacttccctagcatgtgcggagtatgtgctagccttttctctctttttttttcattttttttcatcctttaagatccatgcagtttctaggttgagggattggggtatcacattctctctcctaaaaaaaaattattttcaaaatttttttacctatattttcaaaagttgggattcatggtccaaatctcatccttgaatttttttgatattctaattctcgaaaaaatttcatcgttaaatcatttcataagagaaaagtcaatacctcaagagttgatctgaatcaaaattattatctctagtaatcgaaatcaatatcttaatttcaaataagaatatccagtttattgtcaaaattattaactactcttgacttaattgatctattacataatcgtaaataaattctaacatactcttgaagtgtagaatataagattgataaacaatcctatatccgttctaatagatataaaagcataaactttaaatattttaaatccaagattaagaatcaatgatccacttatcctagactcaagatattagaaatttttttttgtacaatagatagaggatgtactggtgaaaatcatgtagcgatatccaaaataatttttaattaaaaatattatccttttcattatcaatgaattttatctataagaaagatcaaatcatatgatccatcttaaatttttaactcaaaaaattaatattgcaaactagctcaaaataattttgatcactacatttctgctgtgcattctaatttaaaccgttcacattttttagattcatgaaataattttgaccaaagtattactccatactatagtcaaaaaagattaaaatattagattctaattaaagccaaagataaacttttgattctcatccttaattttgcctaaagtataattattttgattaacccttaagcgcaataacacattcaaaaccaacagataggtttactataatccaaatgaattaaatcttaattcttttatcaattcatttagacaatttcaaatcaaaattctataagtaatatcaataaaaaaaatttttgatgctccaataagttagaacttaaatcaaaatatataagtaaaattgatttaatcatctcttctaaagtttcttctattaagatctttaatatctatcaaatacattccacaataatcatgcaaaccttttaaaaattaaattctcaatgcctttactacattttaacaccaagctcgataatagtgataaagaaacatctagatcagctttataatcaaaaattttgacttacaattttacgtgtgtctcaaaatcttgaataaatataaataagatcttttatcttgatccaaaaatagtaatcaaggatttcattagtaacttcaacaacaatggtaaaaaaattttctatccattgataaacccaaattttgaattgaagtttcatgcataccatatagcctttaataagatctattatttggatctaaagatagtaattaaaattgttaatgattccactaagatgaatactttacaatctcataattaatttcttcaataaaaatagacttcttgataatgtctccaattgtatatttttttttatttctacaagaaaacttcatacattttttacgttccaatataaatcttaaaaagttattccaatcaaatatcataaaagatcttcttagtccaaccttaaataacttttatgaatgaatctttatcttgccactaaataatgaattttaaaatcaagagcaacatcacagcattctgtcatgtcaaatttgtgttagatgtatgtcctagaaatcaattagattgacaatgtaaattttttaaggatataatttatatattttgatttattaataaaataaaatttaaattaatttttattcatatttttttatctatgaatcatctaaagaattaataagatgatgatacatattcttaagagttcaaaatttgaaatatatgtcattgatgattaatttctgaatacttttgaattcttaagagtttagaagatcttgacccaagtagtgtgaatagtgaaaaaaagttttcacatacttcacatcaaaaatttaagttgaataaattgtacatatgacaggtattatagtttgacgagtaatctataacctctatcttatcaaaattctgatagaaagattgtattgtatgataactgtacttagaggttcaccttttattttactggattaccactacatgttgctagatgtcactggtggattgtgagatctacgaagattatcttgatgatcgataattctcattgaaaagattgaaactattttaatgatgttgtgatagagatcataatatatcttattatcagacagaatagaattctatgggatcatacacaataggagattaagactgatcaaatagttgaatgatgattaagaatcattacggagttcagattatcaatataattgataattagactaacttataattgttacaagtagcaaggacttaactgctaaaggttaataggttcaaaaagaacttatgtataaatgttgtgcatcttaatttgattggatcaaattagttatggctgaattcaagatgaatcaaataggaatttggttcaattgaatttgggtcaagctttaggcttaggtcacatatacccaaaatcatttggatgcatcaggtgtgtgacacctgaatcaggcctttctaaactattttgagtaagtttgatcaagtcaaaaggatccacaccctaaggtttcttgaataaaaccttaggcaccacattgaggacctataggaaactttgaccctctctcatatggggtggcacactgaggttttataaaaaccttaggcacccattttagccataaaaaaaaagctccaagggatggggcagtagccatgaagaatccttggctgtcaggactctattcaaaagagttctcaaggttttggactcttatggagccctaggatttgtttgcctataaatagatggccaccccaaggctttagataatgttagagacttgtgaagctctcccctttctcttggttgccggcccaccctctctcctctctcttccatgccccaagacttctttcttgtctccatcatcttgctgaaatttagatttcagcaagaaaagtcaagtagaagtcaaagttctaatgtagctcacaagatgttgagaacttcctccatctggcaaaggttctgcaagagagctagcatcctgagaaacaaaaagattgctgatcagccctcatctccatatggatatttgtagagatcaaatgcatgcatagctagaagagaatcttatcacgatcatcactcgtgaagatcatctacctgtgcaaaggtatgagataagaaaaatattttttttatcataattcatgaatcctttgcttatattatactgagattcttggaatggattttttctctagtaaaactctagagatcagatctcaaagtcttcttcacataaaggttttgaaagttctttatatttccgctgctttgattcaaaataaattagatctattttgcctttcaacctttctcatatttattgacatataaagctttaattaatgagattaatgaaaagcatgtgcgaaatactgagaaaatcctaacagtgatatcagagctacttttgtacataagaaaaggattcaagttaaataaaatatgtttgatttaagtaaatgaatcaatcaaaatttatcctaacataagtttgtcctggtataatggtcaagaccattatgttgaaaggttatcctaggacaaaaagtctaagtaaaatctattttatttaagtaaatgaatcaattaaagtttattctaatataagattgccttagcataatggtgaagacccttatgttgaaaggttgtcctaggatggaaagtgattgatgagacaaatatatcatgaaagtatttttcacagatggaataaaatatatatattttgtttgtgaaaatgagatttcatgaatgtgtttgtcattcaatatgtgtggtgatcatcttgaattgccacaaatcctttttggattagggttgtatcatgactcacaaatcctgatggtttgcaaaattttgcattctgtagtgatagaaaccaaaagttaatccaattttggaataagattgatcaattggtatctaaggcaagtattttataatggtggttacttaattagttataaaagtacgaagagtctcctaccaatcttacacttatctagccaatttggttgattgaattctgaatttgggttgcttaagtgttaagttcactacaaatatattgcaaccatgattccgacttagtcaaccaagcctagatctcttgaatagattcatgttaattatggatttacataggatataaataaataattaaaacttgaagagatctaaatgaaaccttctcgtacatattaaatcgaatgatcttccatcattgtagatatacggatactctactgatgttgatgattttcgactagatatagtactttggttgcatcgaaaaagtacaaccactttataacatgagatgttgcagggtagagatggggttgggcccaataattgttaggtgaggatccaaatgatggctgcacttgcgtgtgaatggcgagtctgacttaattaagaaatagagctaataactattagatgaggcttcaggacttagagacttatgaccactacaacttacttgagaagcaatggataaagagtcgtctatttatcaactgacgcatcaccaataactatcagatggagtgatgtataattagtgggactatagtatccacttgaaatcttaatcgtaaaaatttttgtttctccacctgaagagcatgggagattcgaaaaaatagtgggggtagtttatttttaaaataaagctcctaaaataaactaaaataagttaaatacaaagtctaactagaatcttcttctctctgtagaaaatatctgcttccaacctctatttcatatccttaagactaattgtttgactagacccagttataaagattgactctaaaacttaaagatagtcttgagttttgaaaagatgagctatgtcctggatcaagatatcctctctctaccagcttgtcccacccctaatcaaggggcatcctatgaaaagtggttaaacgatgataacaaggcttggtgctgtgtgctgacatctatgtccattgaactccaatgccagcataagggtacaaactgtccaaggtatattgactcatctacaagagttatatagtgagtagagccatgtatctcactaggaagtatttaagagactct

SEQ ID NO: 64 - DNA, 4741 bp, Artificial Sequence
  synthetic
  misc_feature (3017)..(3951): n is a, c, g, or t
cagattatcaatataattgataattggactaacttgtaattattataagtagcaaagatttaattgctaaaggttagcagattcaaggaggacttatgtgtaaataatgtacatcttaatttgattggatcaacttagttatggctaaatttaagatgaatcaaacagggatttagtttaatcgaatttgggtcaagctttgggcttaggtcacatgcactcaaaagggtttggatacatcaagtgtgtgacacccaaaccaagcctccctaaactattttgagttggttttgaccaagtcaaaagggtccacaccctagggtttcttgaataaaaccctaggtgccacattgaggaccaattaggaaactttgacattctttcacacggagcagcacactagggtttcatgaaaaccctaggcacccattttagccataaaaggaaagctccaagggatgggatggtgccatgaagaatccctggccattgggactccattcaaaagttctctaggttttgggctcttatagagccctagggtttgtttgcctataaataggtcgctaccccaaggctttagataatgctagaggcttgtgaagctctctcctttctcttgtttgccatcccaccttctctcctctctcctccatgcctcaagacttctttcttctctccatcatcttgttgaaatttagatttcaatgagaaggatcaagtagagtcagagttctactgcagttctcaaggtgttgagaactttcttcatcaggcaaagattctgcaaaggagttagcacctcaaagaaccaagaaagttgctaatctgccctcatctccatgtggatacttatagaggccaagcatgacgagaagagccttatcacgatcatcactcgtggagatcatctacccgcgcaaaggtatgagataagaaaaaaatatttttcttatcatgattcatgaatcctttgcttatgttacattgagactcttggattagattttttctctaataaaatttcaaagattagatctcgaagtcttcttcacctaaaggtattgaaagttctttatattttcgctactttgattcaaaatagattagatttgttttgcctttcaatttttctcatatttattgagatatgaagctttaattaatgagattaataaaaagcatatgtgaaatactgagaacatcctaacaatttgagcttacaattcacttaaacaactaatgatcaaattaataatcacaatgcacaataaaaattcatgataaatctttttgttgttactttagatcaaaatccaactaatcataacatgatccacggattgcctatcatatatcaaaccctctgaattattaatcttaaacgatcttttcattcatgatcataagatttagttaaaaatcatgaagacaacttatattgtaatcatcatagatctgtatcttaacatccttagtgtttacctacctatactcatcctatgtttgattctatatatcataatttattcactaatactttgatatcatataaattatcgcatccccaatctaagatcatattggtactttaatatttcattagtgggggttatgcattagtactttgataccttatcagttgaatggttaaacactggtactttgatatcctatcagtggaggttatacgctggtactttaatatcctatcagtaagatggttaaatactgatactttgataacctcccagtgggtgttgtatgctagtactttattatcctaccaatggggcagttaaatgctactactttgatacgctaccaatgggatagttaaacgctagtaatctaatcttagcttgacataaagtaacgtcgactcgagtttagggtcgactcgagagaatgttagggttagcttgatatgaaagagggtcgctcgtcaatattttggagtcaactcttgtttatggacgatctagaaagtgtcagagtgagctcgagtactgcatatttctgatacattgtctatgctagaatgtgctagaactgattatcttctttatcaaagttgatttttgagtaacttgatgatcaatttttctaggctagacttgctttgtcaaaatgagcacttgttagtttagagaatcttcacctacacatgatctcaagcattcattagtaccaaaaatacttaagtattttgatatcatcaaaatcaattcttgggttaacacaatacttttcaaataataagcatacagatataatcctataacaatttaaattttgttcatatatcaatttctttaaaaatattatattcatcttgatagctatgaactaaatcaaaatacatactagtatacaacttttactgggagagtattagattaccagcatttaaccatcccactggcaaggtatcaaattaccaatacacaacccctatttataaagtatcaaagtaccagtgttcaactgcctcactggcaggatatcatagtactagtatttaactaccacattgacaggatatggaattatcagtatttaaccatcattagtagaattttgatgcatagtcaggctgcgagtcaaaatctatctcaaatcaaaatattgatcacatgtctaattctgtatcataattcattcccttatgctctaatattatattaattgtcatacttctagctcgagatcatgagccaaggattgcagtaactaccgcatacttatagagaactctttctataagcatacaagatattctaaatatactatcaatatatcatagagaaattaatttaaataactaaaagttaatattcaattaataaattcaactggcaaatgtatttaaaaattttacatcaaataaatcttgattaataaatattaattaataacaatagatttaaatcgaaacaaggttgatattgttagaatttgatgcctcaagattcagcccacattgagtccacagtgaggttcgcgacgaaaaatgnnnnnnnnnnnnnnnnnnnnnnnnnnnnnnnnnnnnnnnnnnnnnnnnnnnnnnnnnnnnnnnnnnnnnnnnnnnnnnnnnnnnnnnnnnnnnnnnnnnnnnnnnnnnnnnnnnnnnnnnnnnnnnnnnnnnnnnnnnnnnnnnnnnnnnnnnnnnnnnnnnnnnnnnnnnnnnnnnnnnnnnnnnnnnnnnnnnnnnnnnnnnnnnnnnnnnnnnnnnnnnnnnnnnnnnnnnnnnnnnnnnnnnnnnnnnnnnnnnnnnnnnnnnnnnnnnnnnnnnnnnnnnnnnnnnnnnnnnnnnnnnnnnnnnnnnnnnnnnnnnnnnnnnnnnnnnnnnnnnnnnnnnnnnnnnnnnnnnnnnnnnnnnnnnnnnnnnnnnnnnnnnnnnnnnnnnnnnnnnnnnnnnnnnnnnnnnnnnnnnnnnnnnnnnnnnnnnnnnnnnnnnnnnnnnnnnnnnnnnnnnnnnnnnnnnnnnnnnnnnnnnnnnnnnnnnnnnnnnnnnnnnnnnnnnnnnnnnnnnnnnnnnnnnnnnnnnnnnnnnnnnnnnnnnnnnnnnnnnnnnnnnnnnnnnnnnnnnnnnnnnnnnnnnnnnnnnnnnnnnnnnnnnnnnnnnnnnnnnnnnnnnnnnnnnnnnnnnnnnnnnnnnnnnnnnnnnnnnnnnnnnnnnnnnnnnnnnnnnnnnnnnnnnnnnnnnnnnnnnnnnnnnnnnnnnnnnnnnnnnnnnnnnnnnnnnnnnnnnnnnnnnnnnnnnnnnnnnnnnnnnnnnnnnnnnnnnnnnnnnnnnnnnnnnnnnnnnnnnnnnnnnnnnnnnnnnnnnnnnnnnnnnnnnnnnnnnnnnnnnnnnnnnnnnnnnnnnnnnnnnnnnnnnnnnnnnnnnnnnnnnnnnnnnnnnnnnnnnnnnnnnnnnnnnnnnnnnnnnnnnnnnnnnnnnnnnnnagatattactaaattttgcttctaatctcactcttaaatagtacttacctttgaaactaggcatttgaatctgaaaaagaaagaggagattatgagcttgatagttcagtaaatcatgaataaattagctaaataaatctatgaataatagtatattaaaaataaatatgtaagatacaataattcaaaaatgaattcatatatataatactttccaaataataagtatgtggctgcaatcctttcgtaattcaaattttgttcattaattatttttttcaaaacatcacatggatagtcatgaactaaatcaaagtaccagtgcataacccctattgataaagaatcaaataacaagtgtttgactgcctcattatcaggatatcaaattattaatgcataacctccactgctagggtatcaaagtagcaacctcaatcacctcactggaagggcatctagtttcagtatttaactactccactggcaaggtgttaaattatcaatatttaacctccactgataggattttgatatatagtcagactgcgagccaaaattcatttcaaaccaaaatatttttctcaaagacatattttatgtttcacattgaaaaattcacaaaaattatgcgatattgaaatcaattggataaaatccacgtcaaatttagtatattcaatcataaatcatttactattctagaaaaggtatattaaaagtataatgcatcaatttcataaatcataaatatctcaatataaaaaatattttattatttattaataaa

SEQ ID NO: 65 - DNA, 5462 bp, Artificial Sequence
  synthetic
agtatattcaatcataaatcatttactattctagaaaaggtatattaaaagtataatgcatcaatttcataaatcataaatatctcaatataaaaaatattttattatttattaataaatctaggagaagtgaagcattacttatcttgtaagtaaaactaaccaactgatcaaattaattctgagaatctttctcaaaactcatcaccactatatcaaaaacttgtgcttcttgctatgtaagagcatagaccctttcttcgatctggggttccaagtttctattttattttgttcaactatcaaattagactgacttttcatttttttgtggatattcagctattttatggcctttctaacaataaccaaagtatgtaccaatattccaacaataatcatttattgcatgattttcaccgcatcgaaatatttgatattatcaatcaatccaaacttgttattcactgacctcttattcaaacccttagtatatttaatattctacctttgtgattcattcaatcgatttcttttttttattttctttccctttctatatgctcttcattaacttttctttcaattatcaatgctttattcaatacatctgtataagtagttaactcatatagtaccatttattttctaatttctatcctcaattccaactcaaatttatctactcagtcacattcatcttcaaccaatctcgaagcaaacttgacaagctccataaatttagcttcatattctacaactattatatttctttatttcagataaataaatttttattctttctgaatcctcatactctaagaaaaatatttttatcataaaatatcttttgaaatcactcccaagcgagttgttctccatcttgttcatatttaggtttcattctctattatcaattaaatgtctcatctttcaacatgtatgatgcatataagattttttcatcatcatggtatctcttaacaataaatgctttctccatctccataagctaatttttagctcctatttcatagttttcttaaaagtcaatggagacaacttcttaaattctatgatattactttattgctcctattgctcttatgtccttgtggtgacaatatttattgttgcacttgctgtagaggcagttactgttactgcaattgctattacgattccatcaagccgactagtgtctgcattatttggataatagttgatttttgctactttatttagatgttggtggcaaaatcaatgacttctttttgctgagagatgccaccaacctactaagtatcatcatcttattggttgatacctttagcagcacctcgagtggttctttttatctgatatggaaccatcttaatcttgcatgaaaaacaaacttcgcaaaattttcttttaaaatctaatatctaatattatacttttattaaaatttaattatgattattttaagaataaaaaatttaaattttgaaatcctcacaaggctggccaagagataatgaccatcatcctagtcggtttgacgtaggacatccaaagatcaactataattcaagcatcatattgagatgctaggatataatcgatggtgaaatttaatgatgctcgactgatcaagatgggggccggcccgatggcctgttcaacaatcattgatcaaaattttttaaccaaggtctatcaagatcattaaaaagtctttctaagatctataaattgtaataaagagacacaatctagagagagacactttttacataaagaaagtagaaattttagggagagaaattagagagaaaggggaaagagagaggaagctgagaggaagaaagaaaagagaaagactctctctctttttcttttctttcttttctttcttttctttttcttttctttttttcttccttttctttctttctttctttggctcattagaaaaataggggacctattgatccccttgtttcctaaataggggaggaatctcatcttggtagctatggccggcgatgtgagccaaagtggcaaaatcatgaatctcccaacttgcagccgacattgacttttggcactggaaaatcaaagaaatttgacaaaaaatgggaaaaaattgaaaccaaaatagggaccaaaatccggtaatagctagccaaaaatccttgatctttgctcatggaggataggaaaaaagattattcaagagattaagggaatcttatctcatttttttgctgtgcttcggccatggtggttgcagaaatcgtttgtgaaagctcgacaaactctgcaatttcctcgggcttgggcctcgatctttaataggagaagagagaagtcctctttcttttaaatagagtcggagggaaggagtttgatttcctccttatggtggtttcaaactctgatcggaagtccattggaaaagaagactcccattagttttaaaatctaataagatttattgattagaaaattgataaaaaatgattattaaaaaagtagcataattatttaaatcaatgatgcttagattgttggaggtaaatagtaataaaatcaaaaaattaaaattcatgggaccaaaaaataatgaacaagatttgaaagaaatgtctataaataagaatttatgaaacaggggaacattgatcaaaggtgtgttaaatagtgtccttaaagtgttattgtccctctcacgtagactttgtgtgttgggagagaacatagtaattctctcaacctatgcaacctaaatcttttgaaaagaaatttaaaattatagaaaaattggcaaactagaattttggtcattttctttattagtaaaaaatatactaagttatatgtctttatttatactagtgaggtctatctttgcacaattcagaccaaatttatattctagttaaaagaggtatagattttttaaaatagatataactagtggaaatagtcatagaaaagttaaaaatcaatgaaaggtagatttcacttctatattggctttatttgtggtcactttatctaattcttttttttgatggagcaatataccctgttaaaatcttctcgatttttttttcactttaagcaacctatttcgatgcctaaacaatggaatttagtttaaccacttaatatgctacacttttaaaaggagcaccatattgtagggcttgaaaagttacttgatttaaaaaaagagcatcttaattggacatcatacaagtaagttatgacctctgaaaatttgatacatgatttatcatcttgatatggtaaatcttgttaagatttcctcatggtgtctaaagtggccggttcatactgagtttggtgattcttctggtcaatggttaattgctcgaatatttttaagatataactaatctccaactctgccgactccttagtagtatgagcacatggaaagcttgacctaattgatttcttaaattgcttgaaatcagtacttagaaaatatgcaaaatggatgaaatgtttattgcagcgagagctttctgatctgtacgaccgagagcttactagttttttatgagctatacgttttgcacttaagcctaatttaaatagtgaaatagttttgcaacaattcaaaacaattaaaatcaaaagacaagctgctatgcatgttcaactgactcggctttcaatcgcaatatgtcacataggctggcctagaatgcagatgcgtgcgtggtgagcatcctaaaaacctacatatccaataaattcccactagttggtgaagtattaaatgtaactcgtattaactttttaatgtaggactaaagtttattcgactaattaagaactaaatactttaataattgaacttttccaaccagaaatcagaaaatatttaagtaattaaatattacataataactagatcaaaatatcatggttcctctctcgctcgagatcaattgggatgttggtttatcttggtcatccatcgagatgactctatcttagcctttcaaaacggcgcggtaccacgggtctcaccgcttcgttacatcgaatgccaccatcccttttttttttttttttatttatttatgctttcttgctcctagattggtgcggcctcattacaactccactgctacttgatgcttccctctagcatctcctttgcagctctctcacttccaccactcttcggcctaatgttgggaaacgacgaaggggccttacaaaaatgtcatccatgatggcagtggagaagaaaacatcgctggggctttccttcgatatccttcgcagccaaagctcttatagggttatatgggagaacgctgcattatttgggtgatctttttggatggtgttgttgactgatgctagttttgcttcatgaattgaatatttacacaagatgagaatacaatctagtacaattggtaccaattacctgggtttgactcctgctcgcatctgattgaagcttggttaatgtgcatctcaattaattcagaaagatcatcggacttcatgtgaattattttgactagcatgaatagggctaaataaggctgaaatatgtgttaaatttttaaaattataacttgatcatatgatgtccaattgagatgttttcaaatcaaaaatttttttcgagatttatcacttaatgttaaactcttagaaggtcgaaacagactgaaagttttcttttcaagatgtattttgaccgagtatataacttgatgatcatatgatgcccaattgagatgttttcaaatgaaaattttttttgagatttatgacttaatgttaaactcttaaaaggtcgaaacagactgaaagttttcttttcaagatgtattttgaccaaatatatctcataatctataaagaatatatttcataatctatgaataattagatagagcgacagaagataatgctaatgtaaaaatcacgatctattttttataaaatttaatatttttatataatcacttttactatagtcatatttattttaaaaaatttagttatatttaaaatatcaaaaaaatttgacttgaattatataagaaaggatcttcctactattatagatagaagctttatatcatagtttacagtgtatggatcatcaatgaaagaaagagggatgtaaaccttacttttgaaatttttctatttgtttctaaattttttaaaggatccaagttgagaattgagagaattctttctttctgcaaatcaaatcattagtataatccacatggagacgttgtaatagaaagtagaaactatattttatgaataatagaaagggagttgatttacgccaagccttttgtttgcttgattaattatttatttttatggtgttagctggaccccatgaatagcaaccatcgttgggtcagggtcgtgtatttgttttggggtcttcatta

SEQ ID NO: 66 - DNA, 8953 bp, Artificial Sequence
  synthetic
caagtactccagaatcaaaattgtgaaagaaaaataggataaatctggttaagctgtaatttatttacttactttctatctatattaaaattattcagattattttgcaaatttatggatatgcttgaatcacgtatctgatactttctcttcatctggatggcagtaccatgtgatcaccacgcagacggatacctacaagaaaaaggcaaggctaacatgctttcttaccatcattctttacggtctttgatccggttttgcgtgtccacttcttacgtagtctttttcaaacattcctatctaagactgaaggtaatgatttgcaaaggaatagctttactgttttcctctaagtagatgaaatattactcacgtagaaaggagccatcataattgcagaaagaataaaactgaatggaatatgagtagaattgtcaaaatcttggtttaagggttttaatagccagatgagaaagcaacctacttttcttgaacaacttgtttgtgactgtcttgttgctcccatcttgcatctatgattagcaaaatatatgataaatagatattcagatttgatcgaaaagaaggaagattttctttaatccatttaatttgaatctcacaaaaaaaaagtagaagatttggacacgatcgctgggggcagcacgctcttaatagaatggtgtcacgttgcagatctcgaaaaattattcaattttttttaaaaaaaaagagtcattgaaattagacgttgtatgaccatgttatgatctctgaaagtttgacttctgactcaacttcccaatgtagcagattttactcctgaaccatgtttaacctcctgactcatagtggccaaagtatctacatcgagttcactggtcttcttggatcacattcataagaatacttcccataattttgctcaacgttgtttttctcatcaaccaaaggtatatgctttttaaaattgaaatgcccatgaatattatggcattcttttatttgacattttggttgatcctatattgtttgtttggcattcaacacttcttcatgggaacctttgaaatgaggtaggtgctaggatttttctttttacctatccatatcatatttccaatgtcttcttttacattaggttctttagtgacaataggggaaacgacccaatataatacccttgaaaatttgggcaatatctactaaaactaacttgaataaaatattaacataaaaagggatttagtaacataaaagcataactcaaaatcactcaccttgtgtgccacgttctcattgcccttattatttttgcattgtgaattgtgtcccccaataaagcaacgtgaatggtggaagagagttgaatggctttgttgagtaattgttttgagttactatagcattgctctactaaaattgaaatcttgctgtgaggctatgtatgagaagcaagttcatgctttttgactgttgggatggaagtatgagcaatctttttaatagaaaatggacgaatcatgaagtttttcctttttattgaaaaagatgatcgaaaaatatgtgcaagatagaaaaacactgaaaagataaaatgagaagtaaaagtggaagtctaggagaagaaaatttaagagaaatatcttcaatgagaggatgtgtgcaccaacaaagccaactttcactaaagaatgtaatgactcacctctactttcttcgaataaggggttcccagttgtggaaagtatatagaatcttctgaaagactgagtaaatggagcaattccttctaagaaatattatggcatttctctcccacgaaatttcaaagcaaagagcagctagtagttgatcctctaatctcttaattgaagtttggaatttctcttgcctctatttggcccaaaggtcatgaagatctaccggccaacctcttaagttgaattagatcttaatagaagtccaaatgcttcttgtagaagaacatctaataaataaatgagtgatagattctaatccagagacaaagagcacacctcgaattcacttgccatccttttctagctagaacttctctagcatgaaacttgttccttaaggcaagccaaataaatactcacattttaggaatgactgccttccaaataattttataatatggacaaattagaccaccattattgataaacttgcaatgaacaattataaatgagttttcaggttggcacattagcaatataggatggtttgattattaaaaggatgatatgaagggtttcaaggtggtttgcctcgttcaaatcaaaggattttgaagattaatattccaagataaggttctccaactccattaggaaagtgtcttcatgtcatcttagagaagcagctcgtaccaaacttgacagatgttttatttatttagagtgacacagataccctttggcaatactctccatccttgtccgaacaacttctaatcacacctcacttatcttgcatctaactcagaggctacaagttacacctttcaacaaaccttttcggtttgaaaatttgtgatttcattatttagagttcgaagagcatatcaagtattggtcggagttggcacccaaagcaaacgaaacagttactgacatggtccaaaagctgagatttctaagatcccaacttaagcactgaataaagccattatgggaaatatcattttaacgaaagaggaatttagagtaagaattgattctcttgataccgaagaagaactaatacagctttcatcacttcaaaatgatgaacagatgcatctcaagtcagcactagaccatcttctaaaataggaagatctatggaagcaacactcccaaatgcagtggcttcaaaatggggattgcaatacgaagtttatccatgtttgggcaagtaacaggaaaaaaagaatactatcactgaactctagcaaggcgatcagaagattatcgaatagcagcaaatccaatccacattctacaactttttttctaccctactaggctcgactgaggaatgactcatccaagctgattggaagattctttatccagaaggacctctggatcttgctgacattgagtatccatttatggagaaagaaatccatgatacagtgtatgacttggctttggaaaagtcacccggatgatattttcccattctccttctataagcacttctagtgtatcatcaaacatgacctgatgaacctactgtaaaatcagctaatgtagaccatctgaactacttgttcatcacccttatcccaaaaaaaaattggtgtgtattcagttagagacttcaggccaataagcctgattaatggagtaataaaaaatatttcaaaaactctatcgaaaaggctcccacagaaaatgaatttgttaattttatccacagagcttgctttcaacagaggaagaaatatctctgaatattttgtaatgactatggaaactatacacttctgcaaagctgaagtacacaaggatctcaattataaagtcgacttcgagaaagcttttgacaatgtggattggagctttctattgaaattgctatccagcacggggctttgattcgaggtggtgtcaatggatagaatatctgatttatacagctaaattctcagtccttattaatggtgataaaggtaaactttttaaattgaggaaagatctcaggcaaggagatcctctattcgcctagctctttctcttagttgttgatatagaatgatcaagggagcaagtaggttcaatctttttgttggaattggatcatataatatcatgggataacttcaaagcttttagttcactgatgacacacttatattttgcagatatgatctaaaatacatcaaaactcttaaatttttactctatagttatgagctactgatgggtctcaaaattaactttgaaaaattccaattttttggcttgagaattgcaaagatgtcagtacagcaagttgcatctatcctagaaagcaaggtggctacattttccattacttatttgggtctcccactccatcattctaaactgaggaaaacttattggaatccactccttgagaaggttcagaagaaattgatcgggtagaaaggtaaacttcttaacctctagggtaggcttatactaactaatgcagtgcttacagggatcccactactctggagggatacattccttctccctcaattcattatcaaataaattgataaaatccatcgatcattcatttggagaggaaacgaggagtataactaagggcactctagaatatgttggtcgaatatttgtcgatcaaaaaaatttggaggactgggggttcctcaatctaaaaattttcaatacaattcttctttgtaaatggtggtggaagctctactctaatgctggtgacccgtggtgtagttttattgccactgtccacccaacttcacactagagatctaaaggtatacacaaatcaacctcttcattttggaatggtttacagcacacatgaaatatttctactcctaatccactttcaagttagcaactagtattattttggaaagatagttggttacataatcatccactgaaggatcgatttcctcacctttacacaatagcattgaagtgcaacaactcagtggcaaaggtattaagcaatctacttgataatagctcttttagtactcctcttcctcaaagataccaagaagattttcagagtctataggaaagcattgaacaaattacattaacggaacgacctgatactatacaatggaaatggtttagtagcaatatttttttggcatgaaggatctactattttctgcaagatggaggagtttggcctctactgagtaatattatataaaaactcctaataccaaagaaagccaagttatttgcttggctaagtgctcacaacaaaatcccaatgaaagctaatcttcttaatagaggaataattggaactgattactgtacactttgcgatgacttatcagaaactaatgatcatctaatgctcatctatactttttcaaaagcaatttggaatcaagtactttcagacctgcaattgtcgaaacttttatgcatgcttaacaccctatgggatacttggagactcatcaatatgcaacacgatagaagacctaaactagctgctctattcgtaattggtcaatggtgtctttggaaggaaagaaataaaagattattcgacttctatactttttatccacgatcgattgctgaaactgtgtcactttttctttcttgggcatcacacctaacaacggagcaactaaagatgttagctcctgttcgagaagttctcttatctaagaatgaaaacacacaatctttagtgagaattacagatgctaacaggcgcagatgaatgttttatgagcatttttatagctgcagcttatatgtgatctatggtgcaaggagttaattataaccatggatattagttaggttgactatcagaaatcatctccaatacattctatgtaaccactgatcaattccatgttcaactagataggaacctgcctatatacaggtatgtccctgatgtaactatagtatactattattcataaataaataacgaaggttttaccttcttctcataaaaaaaaagtatcttcatgtcatcctatatgtcatgcatctcctttgctacttcttttatttacttcttaaacttggttctaccatatattatcagccccttttaaatttgcttttggatattgcatattccactcttcaatcacctcatgccaagcaaaacatttattcacacttgaaaaccaatataagaataccaaagaatttatccatgaaattctagaaactttggttttactcctttctccatcattcaaaaaggttcaaaatgatgataactctatatagcttatttatcaaatttacgaggttggtgttcaatgtttttgtgaaaaaaatatcttgctatccacatagtttgaatccatacttttgctatcttgagtttcaaaaattttaatttgctacaatttgttgctattagcatatgactacttttaagaagataagccaatatactattttcctaagaatttaaaaaatcaaaaataaaaatttttatttaagattttttaagggttgttttccaaatgtgcaatggggcttaatcttggcatcattttctaacttgtagaattttgacccaagtaacatttgtccaatcacttagaacttctataacttcgtacaatcatttgttaatgttgttcatctatttatctatattatctatctggaatatagttgctcttaattatttttatatatcgcctattatccaccctaagctttcatgttcatcctcatgttgttggaggtgcatgtcttattccaaactatttaccattgctgtagattttaaaaaatttgctagtttaggactttttaatcttttgatatcatgttgatgtaagctaaccctctaaggctagtcataatacattttaaggatttatgttatatgagaccaaaattttaacaaaatgaagtgttggaaattggtagaatggaagtgtaaagatgcttagagacatagaactagccctgggccatgtaaatcttccaaaagaagaagaaaataataaaattaagatcatattcaatctctacagaaaagttggtctttgttgtataataagccatcttaacatatgatggacaataaaatatataaacttatgagttttaatacttagatggaagaaaagggacagatatgtcacaccccatcctactagcatgagtaggcacatgatacacggttgcatgccctgcagagtttgactcatgaggcatgcaaggtattgaatagtagtctaggtaaaattaaaaaacttggagcattctaaaaataaatcaagttcattttataaaatcaatatttattatggactccatcaaatattatgcgcataacattttatttgcaaatagaagaagataagtcctagatcctaagtctcctactcttagtctcataattcatccaagctatccaccaaatatctaaaacgaaaaagaaaaacgatagtatgctaatagctttgtaagtcaccttttatctctaattagatcaagcatattagatataaaacaataattttcaaagtatatgatttgcaattaggaataaatatttgataaatacagaataaattttcataaagcatatttactaacattatttataaaatatataatgcttatatcaataaattaatttctaaatcaatatatataaactatccattctgtcttagccttacaactattgctaccattccctgtagcatggttaggaagagactagctcttgaatactcatgtcatttatcaacatatgcgaatgatcattcgactaatatagtcaaaaaaaaattactctgatttatataaattaaaaattagtaaataatatatgctagtaatcaccttaccagctaagctctaaagaaaattagcttttgaatatacatcatgctattgattattatatgtcagtgcttgtctcattttgtggcatgcaagaagactagatcctaaacttatatgcatagtcagattaaagagcaaatgttgcatctgattatatgaacatctattatgatgtagagtttgtatcatgtatatttaatttaaacacaaatataattatacataaataatattcatattttaaattttaaatatttagataattattctagtgcaggtataaaaataagcaatataaaattttaaatcgatttatataacatgcataataaaaaaaattaaggatagaggtacttactgctcaactcataaaacataagaaatctctttaactaactttagtgcaacctagatagaacatattaatgattaagttttcatctaaaataaacatagatatcattttaaaatcttaggcatttaaatggtctcatgatttgtgaggctttcttcagattctacaattttgaaattttttcaaattataatttttttaccttgattgataacaaagccaataatacacctcaaatccaaatgtattcctaatagttttcaataaatctaatatcaataaatcataattaagatatcaatccattctatgaatttgaccataaatcctacttgtttctctgaccttcactataaattaatcatcaaactaaataagtgaggggatcataattcttttacgacaatccaagaattcaagtctagcatccacattagatggcttcctgtccagatatttgcgcctctccaaaattgagattatcagattaagaaaaataaaataagagagagggttaaaggacaatgccttctaggtagtgatgtccgacatcataattttgatcaaatctatggggcaaccaataatattagggaaagaggattggatttgagcaagaatagcaaagtcattgtcatcaatggcctgattcattgagttcaatgaaggattggtggttgagtggtggaggtggcatctaggaaggagagagaaagaaaaagatagagagaaagagataagaaaaatagagagaaggtggcagttaagatccctttttgtgattaatatatagccgtaagatactcaaagatctcaccttatcgacctcaaacactaagggaggtggaaggagggactactacccatgaagctagagaaagggatgatgatgattggaggaaggaagaaggaaaaatagtagactcgatgatgataagactaaaagaaaagggtttgacttagccacttggtatataatgaggtttggtatggagtcaatagcttgagtaatagcatggaaagagagaag

SEQ ID NO: 67 - DNA, 6021 bp, Artificial Sequence
  synthetic
aaatatctaaaacgaaaaagaaaaacgatagtatgctaatagctttgtaagtcaccttttatctctaattagatcaagcatattagatataaaacaataattttcaaagtatatgatttgcaattaggaataaatatttgataaatacagaataaattttcataaagcatatttactaacattatttataaaatatataatgcttatatcaataaattaatttctaaatcaatatatataaactatccattctgtcttagccttacaactattgctaccattccctgtagcatggttaggaagagactagctcttgaatactcatgtcatttatcaacatatgcgaatgatcattcgactaatatagtcaaaaaaaaattactctgatttatataaattaaaaattagtaaataatatatgctagtaatcaccttaccagctaagctctaaagaaaattagcttttgaatatacatcatgctattgattattatatgtcagtgcttgtctcattttgtggcatgcaagaagactagatcctaaacttatatgcatagtcagattaaagagcaaatgttgcatctgattatatgaacatctattatgatgtagagtttgtatcatgtatatttaatttaaacacaaatataattatacataaataatattcatattttaaattttaaatatttagataattattctagtgcaggtataaaaataagcaatataaaattttaaatcgatttatataacatgcataataaaaaaaattaaggatagaggtacttactgctcaactcataaaacataagaaatctctttaactaactttagtgcaacctagatagaacatattaatgattaagttttcatctaaaataaacatagatatcattttaaaatcttaggcatttaaatggtctcatgatttgtgaggctttcttcagattctacaattttgaaattttttcaaattataatttttttaccttgattgataacaaagccaataatacacctcaaatccaaatgtattcctaatagttttcaataaatctaatatcaataaatcataattaagatatcaatccattctatgaatttgaccataaatcctacttgtttctctgaccttcactataaattaatcatcaaactaaataagtgaggggatcataattcttttacgacaatccaagaattcaagtctagcatccacattagatggcttcctgtccagatatttgcgcctctccaaaattgagattatcagattaagaaaaataaaataagagagagggttaaaggacaatgccttctaggtagtgatgtccgacatcataattttgatcaaatctatggggcaaccaataatattagggaaagaggattggatttgagcaagaatagcaaagtcattgtcatcaatggcctgattcattgagttcaatgaaggattggtggttgagtggtggaggtggcatctaggaaggagagagaaagaaaaagatagagagaaagagataagaaaaatagagagaaggtggcagttaagatccctttttgtgattaatatatagccgtaagatactcaaagatctcaccttatcgacctcaaacactaagggaggtggaaggagggactactacccatgaagctagagaaagggatgatgatgattggaggaaggaagaaggaaaaatagtagactcgatgatgataagactaaaagaaaagggtttgacttagccacttggtatataatgaggtttggtatggagtcaatagcttgagtaatagcatggaaagagagaaggagctgaagagagtactaagtcttattagaataaagaaagatagaatcttagcgaaaaatagggcctcaaatctttcaggtagaggaaaaagagggatcaacgaatgaaagactaaggaaaaggtgtggagtaggatatactctcgattagtctctcaatcatggattctagtagggcttcgtcagctgctcaatcatggattctgatagctcaaatggtggtaagtagaaagagagagatctaaagagattgatagtggccttaaaaccagcacggtcaaggataggcatgccttagagagaggaaaagagagagagattaatggaaataagcgagaaaaatatattcttagagaatagattggcgataagaagaggaggtggttggggcatgcttaaagaaataaagaaaattgagtaggcggaaagtggtgatgcttggcgatgagaagatttgagagagagagcaaaaaaatgtggatgatggtcataggatagggaaaggaaagaacaaagaagggggtgctaagctaactctttctaccttcctcacaccctgaagcaaaggatttggccaaggatggacaaatgggcgagggctttggtggatccatgcctaccctttctccctctcacgatgattctagtcaagctatctatctttgatagcttgagccaagccaattgacttgatccaatctctctaaatccatacaaacttaagagagtgtattgattcacttattctcttctaagttgataagaaacataattaagtggagctcattaagtatttcaggtagttgctaacttggcaaaatggaagcaataataaatcttaaaagactatagcttggtataatctcaaccatccatgatttagaaagatcttcagactcaatatagattactttggctactacaggtaagagctaaataggatccaaaagtaagatccatcacattagtaagtcaaattatatgtcaaattttagtaggtatacttagtcctacgatgcctaattaaaatgatcatcatttgaaccttaaaatggactagtcaactaaaatttttctttttgaagaagatttagaccataaaatatcttctaatctgtgaagaattagatagagcgaggaatataaaattgatgtagaaatcaagatctatcatatatacaattttaatatttttttcataatttttaaatatttatcttctttttttataggtctagtcctatttaaactaggaagaggagtccaacttgacttatgcaataggggatgtccttctagaagataagaataatttgatcagaattatataagagcaaacctcattattataaataggggctatatacatcaatttatgagatagagaatcaatgaaacaaaagtagacttaagttttattttcataattcttctatcttctactttttttctaggagattcaagttgagtggattgaagaaaatctttcatcttctcgatcggatcatattggtattagagcgttggtcttctatatttatggagagctttaatgtattgtttaaatacgtgaacaatacaaacaatcaagagaagtgctatccatgcttcaaatacatcgaaatataaaagcaaatatggctactaattctttttcaatggacaatgagataaaaggatgtcttacacaactcaaggagaagattgtgcaactcatgaagattgtctccagattgaagataatttcaatacaagcacaaacaccagcaactcatgttgtgaaactgtttcctatgtttggagatgaagatcttctatctagtgaggagattgaattacctaaaagtatgaaaaatctttcttcaatcattgaaagttaaagcttgaattgagatccccatatataatggaaccattgatgaaaaaaagctagataattggctaaactaattacaaacctattttattatctatagatattatggcatctagaagatagcttttacttatctcaagctttctagccatgctcttatctgatgaaattcatatatgagaaataataatatttttaatatggtgcagagccaattcaaaggtttaatcaagaagtaattttatctaattggccataaggaagatcggtggatcaaatgataatacttatgatagaaacataatcaatccacttaggactataccaccaagttccacaaacaggcaatctgccttggaatctttatcaacaattatacaatttttataaagtatgttgaaagtcttcatgagagcatctaaaaaaagatgaaactctttaaggttgatgatatcagtaaagctaacatgaaagtcatagagattgaggagaaaaatcaaattagagaagataaggaaggcaaaaagcatatcaacataactcaaaaaaaaaaattatgatcattgaaatctttgaaaatacatcaaggagaagtattgaaagtttcatcctgaattggagctaaagtagaagaagcccaaggatgataattttaagaaaaataaaaagtggtcctcaattctatagagattgaggagctatctgaacttgagtaagcaaacttcaaattgagcttgatggtgagaaaacctaatacaacaattaaaacggatctagaggtacatgacaactcacccacttaaagattcaagtgaagcagagtatcattaaggctattataaatctttgaagctagaagaacctcattttccaatatttggttcagaaatcgaggttgtagatcaagcctcatccatatccttatcctcttagttggattcagaaggatgtcaagttaaaaattatgagatagtgtaccttcaagttagccatcactgagaggtttatttgtgaggtaacttttgaaatagtttctttggatatttgtcaagttatccttagaaatgtgtacctttagaatcaagatgcaattttctatagacgatagagaaagtatcatcttataagggatgagaaaaagttcatgatcaacacctcaagaacataaggtaactttgaccttgcaactgttgcccaagtgaagtgatttgttaatgtttgtgatgagtgcatgatgatggtataaagaaccgatatcactcatgagaggtcaaggccttgtcctttggttccatcaatcgatcaatagagattgagattaaggaggagtcactatagtccttgtcgatgaggaaggatgacaacaagcattcctaccatgaagtctagatttgagagcaaatgaaagtaatccactgagacctgagagcaaaaaaaggcgagaccaaaaatcatcttcaagtaaagtcaaatggttcaaccatgagatggggaagtaagtattttcccaccttcaattctaactttgtagaaactaaatcccttaaacaggggagccctaatttaagaggatcctcagattcattgtggactactttggctattacaataagagctggataggaatcgaaagcaaaattcaccacattaggaagccaaattgtatggcaaacttcaagagaccataacttgatcacatgaaatccaattaagatgattttatttttgaatttgaatatttttttgagatctataactttagatctaaatcaagctaaaattttattgcttatgccttcaaaataggctagtcaaatcaaaacttttcttttcaaaaaagactttgactgaaagatatctttcaatctatgaagaatcaagtagagtgatgaaagataaagttgatataaaaattgagatctatctcttataaaattttagtaattttattttttttaatatttatctttatttagagatctattcctatttaaactagaaagaattgtccaacctaacttgttcaatgatcaacatcctcctaaaagataaaaagaagaatctgactcaaattataaaagggcggacctttttttttgatgaaaagggaggaaaaaaatccatcaaaatttattaagaaaaaaagagtacaagaaaagaaggatatgaaagagtaagagaagccccacaacatccatcaatatttaaaatttaaatttaaatctcccccatcattctatcaatatttgatattcaaatttaaattcttcgcagcatcccaccaacatttgaaattcaaatcctttcatacaaacaaaataatat

SEQ ID NO: 68 - DNA, 5329 bp, Artificial Sequence
  synthetic
  misc_feature (4258)..(4985): n is a, c, g, or t
atattttcgtagtctctaaaggcttcttccagattggcaatatactgatctgactcagtattttttactaatatatcatcaacataaactttgatattaatttcaatttgttacttaaaaatcttattaatcaagtattagtatgtagcacctacatttttaagatcaaaagacatcattttataacaatgcaaatctttttcagtgatgaaggccatattttcttcatcctcaagtgccattttgatctgatataaccagaaaaagtatccataaagcttagtaatttgtgtcttgaagtagcatcaacaagctgatcaatttttgagagagaaaaactatcttttaggcaagctttattgagatcggtataatcaacatagatccttcatttttcattagcctttttaaccatgacaacatttacaatccactttggatattatgcttctctgatgaatttgtctttcaagagtttgtcgacttcctcatctattattttttatcttttcggggtgaaacttcttttcttctgttgcattggtttatgctttggatcaacattcagcttatgtacaataagatcagttaaaatctcaggcatattagagactgactaaacaaagacatcggcattcatccgaagaaaagatattaatttctccctcagatcaggcttcaatagagatccaatttggacagttttttttggatcatcacacaaaagaacaataataagtttctcgactggttctcctcgatttttgatgatatcaactttactttcttgatcaagtattttaattggtagagcttccacagaccttttcatttttacagctatcagaaaatactacttagcaagtatctgatttcctcatatttctccaactccatacttagtttggaattggattagtaaatgataagtgaagactatagccttaagggcgttgagcctaggtcggtcaagaatagcattataagctgatggtattttgacaataaaaaaagtgagtcttacagttgactggcatggttctatccctgcagtgacggacaaagtgacctctccttccacagctacaggatttctagaaaatccaattacgggggtaccaacctatttagctaatttatcatattcattctttggaatgtatcatagaacaatatattagcagagctttcattatcaataagtattctttttatatcatatttggctattgccataaagatgacaacagcatcattacgaggagtttgaactctaacatcatcatcgaaaaatgaaattatgtgatccatgcactgatgctttggaaggctttcagtaatctcagccacctcctcagttccgtcgagatctgagatcatattgatgactgcagcagtagacttgttgtgatcattctcattgttgggcttctatcattggtcagtagcttgacttgcccgatctcgaacatatttactaaagtaacattagtggatcaatacttcaattttatcttttaattatcgatgctcctcagtatcatggccatagtctcgatggaaatgacagtattttctcttatctctctttgctggaggggctttcataggattaggttggcgaatatatcctaaatcctcgatttctatcagtatctgagctcgaggagtagatagtgaggtatagatgtcgaatcaccgaggtgggcttttgaacttcagattcttctgaggtcgttcagagttatcctgttggtttttatgatcttcttcctagggccacttttttccatctctttttttcttcacctaacgaagtatgcatgctctctttcttttcagcttgagcatacttacaaacctagatcaatatttgttcataattgtttgggtagttcttattaagagagaagatcaggcgattactcttgagtccttgcttcaaagctgccattgcaatggactcattgaagttcttcactttcagtatggcggcattaaagcatgccacatattcttgaagagattcaccttcctactatttgatagtaaaaagattgctagtatttttcaaatgaatccatttattatcaaaatacgtgatgaatatttgctaactgtgtgaaagatgaaatagatcatgtctggaggtcagagaactagattcttgcagatgttttgagagtgattggaaaagtgatgcaaaatagggcattagataccccttgtagtcttataatggctctgaagccttcaagatgatttaagggattgatggagccatcgaatgtttccaatgtaggtatcttgaatcgaggaggaactgatttaccaagaattttttgagaaaaaagagatcgtaagttgaaatctcttctaccttgagaatggcttccaatctatatctccatcattttcttctcaagattttgaatcttttgtccaagaccctcctccatacatggcttcttatgtggagcagatttcacttcccaagagtgatcagtatggtcaagaagatgatcatgatgaagatcttgaggagttggttgctaagtgtgatgtgattggactacttggggggctactttttgctaccgttctgtcgtatactacagcagtaagagcttggacctgctgaaccaagagactaaactattgtggatcaataataattgaaggttaggtattctcctgaacatcttcaggagaagatgaagtaggtaaaggatgatttggtgccttcttgttcaccatttctactaaaatattttaagtgcccttcctctaacactaatctattactgcaaggcttcaaaagacaggcaacgagatgggtcttgaatcgaactagaatgtttcttggttgaatttggcgaagtctgtaacaaatcttgcaaagaaaatctcgaaacctacgggtaccttctggttcaagatcctctgatggataagttaggtaaagtcttgagaataggttgtgaaaatagaagaatagaaggatgagaagagagattgtcggtaaatggagagatgactcttatttctttcaatgggggagctgaaaataattcagcagagtttccactctatcaatcctgacttattttgtggagggtaccttggccccttcatatataggggatgaagaggcctggtaaggttgttagactattaggagagtttgttagatcgttaatttattataatagaatgaccagctatataaaaatcatggagtatttacccacatggtgattgactgtagtataactgaaagatagctaatgcttagctggatgactgctgttagataactgtctgcattcttacggtacattgatattttaccaatgtgacatagcttaaatcggcaactggctgaactaaatattatgtatccctttagttaacaatcatgtcggttagagatcaatgtaattcgcagcagatcgatcataagctgagatgagtatcatattttaagaacaacgctgggcgagttaggccgatcaaatgtcagactgaaaaagcagatcaataaacctctgatgtgatctgaaagaatatttatgatttaaataataatctatcaccacgtatccagataatgaggtcatataacatgtaccaacagtgcatttttccatctagttaagaggttggttagtggcatttgtcttcgatatgtaatgttcacataactaatgtgcttagtagcattcttttgtaaggttaaatcttcaatgatcttaagttcacataattgcctttgtgccctattagtttatagttgaccttttaattcaagagacagtcaccttagcaatcgatgtctgcttagattgggccaattaggtactcacattaatatattgaatcatgtttgaatataaaggattagattgatttataagtttccttttattgtttacatactgatacttagattgacttactacattatttgatatgttatgttctaatttttggattaaaattgttgtttctgatttctccttacatctaatactttgtataatttattattttttagcatgattgagtgtagaggattagattgatttttaagtttattttgattatttacatgcccatacttaaattgacttactacattattcaatatgttatgtttcaattattgagttaaaatttttatttctgatttctactgatgtccagtgtgtgtgtgtgtacgtatgtgtgtatatatttatttacatatatatgtatnnnnnnnnnnnnnnnnnnnnnnnnnnnnnnnnnnnnnnnnnnnnnnnnnnnnnnnnnnnnnnnnnnnnnnnnnnnnnnnnnnnnnnnnnnnnnnnnnnnnnnnnnnnnnnnnnnnnnnnnnnnnnnnnnnnnnnnnnnnnnnnnnnnnnnnnnnnnnnnnnnnnnnnnnnnnnnnnnnnnnnnnnnnnnnnnnnnnnnnnnnnnnnnnnnnnnnnnnnnnnnnnnnnnnnnnnnnnnnnnnnnnnnnnnnnnnnnnnnnnnnnnnnnnnnnnnnnnnnnnnnnnnnnnnnnnnnnnnnnnnnnnnnnnnnnnnnnnnnnnnnnnnnnnnnnnnnnnnnnnnnnnnnnnnnnnnnnnnnnnnnnnnnnnnnnnnnnnnnnnnnnnnnnnnnnnnnnnnnnnnnnnnnnnnnnnnnnnnnnnnnnnnnnnnnnnnnnnnnnnnnnnnnnnnnnnnnnnnnnnnnnnnnnnnnnnnnnnnnnnnnnnnnnnnnnnnnnnnnnnnnnnnnnnnnnnnnnnnnnnnnnnnnnnnnnnnnnnnnnnnnnnnnnnnnnnnnnnnnnnnnnnnnnnnnnnnnnnnnnnnnnnnnnnnnnnnnnnnnnnnnnnnnnnnnnnnnnnnnnnnnnnnnnnnnnnnnnnnnnnnnnnnnnnnnnnnnnnnnnnnnnnnnnnnnnnnnnnnnnnnnnnnnnnnnnnnnnnnnnnnnnnnnnnnnnnnnnnnnnnnnnnnnnnatgtatacatatacatgtatacatacatatatagatatatatatatacatatatgtatatatatatatatatatacacatatataggttatttggaacctaagaaacttgcaaagttactagatgcaatgttcggaaaccatggaccgtaacaactggagtagtatttgggtcatgaattcatggctagatcatgaattgagtgggagtcaaccgaagtagggccagctcagacacttgtatttaggtcccatgcttgcgtgcattctcttccctgatatcctttggctttgctgcctcaaatcctcgagctatcttatcatcatcgcattgagctccatacct

SEQ ID NO: 69 - DNA, 6061 bp, Artificial Sequence
  synthetic
  misc_feature (5947)..(6061): n is a, c, g, or t
cagtttggacttcaatgttaacccaatattgattttaaatccaacattggtccacttagacttatttatttatttttatcaatttaatataaaaaagatctaaacctcataagtcataaattttggatttatttttgaacatgtacaaaataaaacagaaaaaagaaaaaattacttatctaaaagtaactatatctgaaaactttcactttagaattgtcttaaattaatgtacttccatcaacaattcaatgttaatatttttatgaatccaaatggatgatagagtattttttagaatgaagtattgaagtctaaatgacatcgtcccaaaataaaagtgaatttatgaaatactacatctgtcggattcggtttcatacggattaaaagtgtaggaatagaatccgattataaataattatttttttataaattctaattcaattttattcgatttatattttttaaccggtcaaaattaatatttattaagtaggattggatggatttattcgtatctcgattatttgctcagcccattgccaaatctaaactcttttcagataggttccatgtgaacatgatacatgagatgcagtgtgatagtacacaccattgctaagaaaactttggagtttgcgtaacaatatctgtttaccatttaaaaaatggcagttttgaattttaacacgctctcctccagattcagcttatgaacttttcgaataaaaatacccctggactatttttccaaaaagtaccagcatcttttgaacttgaatggaaattcggccaataaaatgttttcatttattgaagaaataaacagggtaacgcagtagctctatttcctctgcttttcttttctatattaataacatgattattcatctctctcggatcacaaaaaaattaagctattcaagctttatttatatttcatttttaaattttttacttaaatacaaaatctcccatcccactactacggcagcatgttttctatgtatgattattttcattcaaatgatatcattttttataatttatattgtatgtaattaattcatttatagttcttacattttcctgtttctagtagatacaataaagcggttttggactagtagcttgttctctgtatcgaagtttaactaaagctttgacaataatatatgaatccatatcactgggtaggagaggaatatgttgggtataaaggatttaaggaattagatattttcatacaattgtattgcattgcagacagtaattagattactatgcaattattctctctctccatgtttgttgcagttgaagaactctaatgaagctcacaaaaatttactgcatgaacttgtaagtggaattagacgactccgttgtcctccattttcttttattttctttaaaatcatctgccattcaaatagacagaaaaaaaaggattgattagctattggatgcctcttgaattcaggaaatgaaggacgagcacccagtttatggttttgtggatgatgaccctagcaactacgcaggtgcactagctcttgccaatggggcttcccacatgtatgctttccgtgttcagccgagccagccgaatctccatcgaatggggtttggctcccatgacctgcgccttgcttgattttattgtagcttaaagaccttacaacttccagagtggtgttatatattagtatcttaagctatgacagtggtaagcctctctatccgctacttgttatcctttaggtactttgcatgtggtgcaaggttataattgccttgtgtttctattgtcttcctcatggtacttactggactgatgatgtcaagtgaaatggagttgtttgaatcctgactgaaatttctcttggtccatcaagtgcaagagtaagtttagacatcactcgcaagcttttgctaggaaataagtagtttcattgcactaatgatttcgaatttttgttttcgggttagagaaacctagattaatgctgttattggatgctggcagtcagatgaagattatgtttgattgtacctcgttggacagatgctcatgcgtagatccataactctatttcatttcatttccctgtacacaattgaaacagggcatatatgaataggtatagaacagatgattcctgcaatattggaggtggctagctcagcttagactaaagttggtctagctgggatattctgaacacctgagatgttcaaataatgtgggataacttggcccaactcaactaaacattggctcaaagcatagtcaaggtaaagcttgagcaagctcttttgagcttggttcgagtccgagctgagcccgggccgcttgtttagctgatgaactgaattcaaatagccggtactcagcttggctccactcgattcatgagttcgaatcccctcaagttcaacctcgaacttgacggtgtagtcccacaaccatggccaccttataatgtgggacggccattatgcattcctctagtgcctgctccatatgacttttgttctcattataccatgcacctaaatgagtgctcatagtgacaatgtttagcctccacgtataatgtgtgccagctaactagaagcctaaactttggtgaaatttctgcaatgttgtggttgtaaaacgctcctacgttgagacatgatggtatctaagattatagacaaactatcatgctgaatcaacccaaatccaaggtgaataaaacttgatacaaagccgagctccattgaaatagtacaatggattctgcacttgaagaacattacaaaatcattttttcccaaaaagaaacattgcgaacagaccaaagcgtaaagaaattacatgattcaactaattcaagctttccatgatgtaggcactcgctagatgtagtagggtgataacttgctttgtgagggtggatcataagcttaacctcaatctatcccaatctatcctttcccttgacctatccatgccaatctaggccatttctgcataaatataacttaatcccagtggatccggcctagtttcactcactccaacacattcctactcaatggtagccaatcctttctttagccctcaaatataatcctaatctagcatagccaaccatcaatcatgcctaataaagcccgactacaccaacccgatcattcctgatcgtacacaatcaagacttatcctaattgatcctagctttttttaggcctctcttatagaacctgtgccaattctggacaagctaatccaatcttagcagccaaaaatattacatgtttaattagccaaatcgaacctatcataaacccaatatataatcggaccataccaagatcatcatcctatatttccttctcttgttataactacacctaaaaaggaatttcttcatacttatgaggggtatattatgataaaaattccttcattttagccctccatccttgtctatttttgggaccactagccaagtaacaccttaagagccctccatcttaatattccctctaactagctcgatttcttcttcattctttctttgcgatgtgtcccctccaatttaattcttacatgttgggatttgagtactgaaaaataatagataaagagaaagtaaaaactatgctaatgataataccaaaggcataaagaaatcacagcagtcgcaaaaacatcaaatttttttatggttcggcctaagcctatatctacatagggacgagagtaagaagaagcttccactataataatagtttagagtacaaaaacttctctgacaccatgtagggaacatcgcttctaatacaagaaagaagaaatccaagattaaacaaacctctagaaaaattcttctcgatggaataactctaatctgagattgaacaatcttctccaatcgatgatctccaatcttcttttcttaaatgaagcacccttcaagcctctcttcttttctctcttcctatcctcttttgtggctcacaacctcctctcctttttatgttctatgttcctcacatcacatccacagactcatttttatagataaaaaattagagtctatttcggactccttttccacacacaagatggcttcccacgccattggttccgtgcgcatgacttttttcatgccacaaaggattccgtgctgcaaaagttttccatatccatgcagtttccacacaccacaaaaactttcgcacacttctcgaaggcttttcatgctcgaccctttttggttttcaattaaattgatggatcccatatgaggagggaccacaccaataaatctcctccttctaactcatatggtaggttccatcaagcctgtagcacctttgcattttatcagttttgttcctgaagccggcttcatcaatatattagaactattttcttcagtgtcaacttttttaagcttgaaccacttcatctctagcatattgacatgcttttggaaagtatgtcaaattgctcaaaattaatcttacggttctctttttcgttagattctagtgcatattacgcactttaacataagatctaaggaaggaagaggactgaggtaaggtgaagtgattttttttgagttggtaatggtacaaaagttatactagaccgtgggtacctaatctcggagattaccatttagatttggttcttgatcatttgtatagtgatgcatttaaaaaattatttgagcaaaacagtgaatgccattgggtctgagagatccaaaaccaaataacctaaagtatatagatggttcctttagctagatcatgtatgagaaaaaatgatctgccgactggaaaaaatagatctttgagctcattgattgttaagtcatatctagtctgtgaatcatctctttgaggattaatgatcaagctatcttttatgggttaaaagaataggatcactgaaatacttatcctagtatacatataatgtgcatggcctatttgatgagtcagactagaaggttatcactacttcatcacctttactgatgagcaatcatgatatagatatgtatgtgagatacaaatctaaaagattttgaatggttcaaagaattcagatatgaagtagaaaagataaatcaaaaaatttttaaaggtacttgatcggatctagaatgcaataccaaataaaaaatttgttgattatctaaaaaaagtgatatagtttcatgatggaattcttcttgtacacctcagctcaacggtatatatatgaggagcaatagcactatatgagatatggtccggtccatcatgaatatcactaatttaattattatttatttaagagcaagatttaatttttaaaatttaaattagattttttctaaaattggtttcaccgcaccatatgagatatgatttggtggataagttagaggataggtctgtgagaactcatttatagggtatcccaaaaggtatttaaaatattactttttctttctagtagttgacaatatgattgtgagcaatcatactgttttcttaaaaacagtggaaggatgaactcaaaaagaaagtctctaaagaacaacgagtcacaagacctatacaacctatttaagatgagccagtatatgtagtacttccttcacctcatcaatttagtaggatctcctatcctttagaaagatactcggtattcttacaaaggatttagagaaagtgtttcttgagggagattgagaatatagggatgatctcaaaacctacaatgacataatataaggaatcatgtagttacatgaaggtcagtgggagggttccatactgacatcgattatgatgtggttacatatagaatttttttttcaaagatctagatcaaacattctgaaaataaaaggtctatagagataaatccgaaaaggatgtttgnnnnnnnnnnnnnnnnnnnnnnnnnnnnnnnnnnnnnnnnnnnnnnnnnnnnnnnnnnnnnnnnnnnnnnnnnnnnnnnnnnnnnnnnnnnnnnnnnnnnnnnnnnnnnnnnnnn

SEQ ID NO: 70 - DNA, 14226 bp, Artificial Sequence
  synthetic
  misc_feature (1949)..(2907): n is a, c, g, or t
  misc_feature (3857)..(4532): n is a, c, g, or t
atcctcttttgtggctcacaacctcctctcctttttatgttctatgttcctcacatcacatccacagactcatttttatagataaaaaattagagtctatttcggactccttttccacacacaagatggcttcccacgccattggttccgtgcgcatgacttttttcatgccacaaaggattccgtgctgcaaaagttttccatatccatgcagtttccacacaccacaaaaactttcgcacacttctcgaaggcttttcatgctcgaccctttttggttttcaattaaattgatggatcccatatgaggagggaccacaccaataaatctcctccttctaactcatatggtaggttccatcaagcctgtagcacctttgcattttatcagttttgttcctgaagccggcttcatcaatatattagaactattttcttcagtgtcaacttttttaagcttgaaccacttcatctctagcatattgacatgcttttggaaagtatgtcaaattgctcaaaattaatcttacggttctctttttcgttagattctagtgcatattacgcactttaacataagatctaaggaaggaagaggactgaggtaaggtgaagtgatttttttttgagttggtaatggtacaaaagttatactagaccgtgggtacctaatctcggagattaccatttagatttggttcttgatcatttgtatagtgatgcatttaaaaaattatttgagcaaaacagtgaatgccattgggtctgagagatccaaaatcaaataacctaaagtatatagatggttcctttagctaggtcatgtatgagaaaaaatgatctgccgactggagaaaatagatctttgagctcattgactgttaagtcatatctagtctgtgaatcatctctttgaggattaatgatcaagctatcctttatgggttaaaagaataggatcactgaaatacttatcctagtatacatataatgtgcatggcctatttgatgagtcagactagaaggttatcactacttcatcacctttactgatgagcaatcatgatatggatatgtatgtgagatacaaatctaaaagattttgaatggttcaaagaattcagatatgaagtagaaaagataaatcaaaaaatttttaaaggtacttgatcggatctagaatgcaataccaaataaaaaatttgttgattatctaaaaaaagtgatatagtttcatgatggaattcttcttgtacacctcagctcaacggtatatatatgaggagcaatagcactatatgagatatggtccggtccatcatgaatatcactaatttaattattatttatttaagagcaagatttaatttttaaaatttaaattagattttttctaaaattggtttcaccgcaccatatgagatatgatttggtggataagttagaggatagatctgtgagaactcatttatagggtatcccaaaaggtatttaaaatattactttttctttccagtagttgacaatatgattgtgagcaatcatactgttttcttaaaaatagtggaaggatgaactcaaaaagaaagtctctaaagaacaacgagtcacaagacctatacaacctatttaagatgagccagtatatgtagtacttccttcacctcatcaatttagtaggatctcctatcttttagaaagatactcggtattcttacaaaggatttagagaaagtgtttcttgagggagattgagaatatagggatgatctcaaaacctacaatgacataatataaggaatcatgtagttacatgaaggtcagtgggagggttccatactgacatcgattatgatgtggttacatatagaatttttttttcaaagatctagatcaaacattctgaaaataaaaggtctatagagataaatccgaaaaggatgtttgannnnnnnnnnnnnnnnnnnnnnnnnnnnnnnnnnnnnnnnnnnnnnnnnnnnnnnnnnnnnnnnnnnnnnnnnnnnnnnnnnnnnnnnnnnnnnnnnnnnnnnnnnnnnnnnnnnnnnnnnnnnnnnnnnnnnnnnnnnnnnnnnnnnnnnnnnnnnnnnnnnnnnnnnnnnnnnnnnnnnnnnnnnnnnnnnnnnnnnnnnnnnnnnnnnnnnnnnnnnnnnnnnnnnnnnnnnnnnnnnnnnnnnnnnnnnnnnnnnnnnnnnnnnnnnnnnnnnnnnnnnnnnnnnnnnnnnnnnnnnnnnnnnnnnnnnnnnnnnnnnnnnnnnnnnnnnnnnnnnnnnnnnnnnnnnnnnnnnnnnnnnnnnnnnnnnnnnnnnnnnnnnnnnnnnnnnnnnnnnnnnnnnnnnnnnnnnnnnnnnnnnnnnnnnnnnnnnnnnnnnnnnnnnnnnnnnnnnnnnnnnnnnnnnnnnnnnnnnnnnnnnnnnnnnnnnnnnnnnnnnnnnnnnnnnnnnnnnnnnnnnnnnnnnnnnnnnnnnnnnnnnnnnnnnnnnnnnnnnnnnnnnnnnnnnnnnnnnnnnnnnnnnnnnnnnnnnnnnnnnnnnnnnnnnnnnnnnnnnnnnnnnnnnnnnnnnnnnnnnnnnnnnnnnnnnnnnnnnnnnnnnnnnnnnnnnnnnnnnnnnnnnnnnnnnnnnnnnnnnnnnnnnnnnnnnnnnnnnnnnnnnnnnnnnnnnnnnnnnnnnnnnnnnnnnnnnnnnnnnnnnnnnnnnnnnnnnnnnnnnnnnnnnnnnnnnnnnnnnnnnnnnnnnnnnnnnnnnnnnnnnnnnnnnnnnnnnnnnnnnnnnnnnnnnnnnnnnnnnnnnnnnnnnnnnnnnnnnnnnnnnnnnnnnnnnnnnnnnnnnnnnnnnnnnnnnnnnnnnnnnnnnnnnnnnnnnnnnnnnnnnnnnnnnnnnnnnnnnnactatgtatgttggctatgtaggttccgattcgctgtttggaatatgatatacctagatgaaatctatcgatcttgatagaaaaagagaagtcctatgtgattcgtaagactgagttcagaaaaatctctgaccagagtaagtgtgaatattgaaaaattttttttacgaaattcacaaatgaactcgagtcgagccaatgtagcatatgactgatgatagagtttgacgagttctcaatgacctccgtcaaattgggactctcgatagagggattgtatcacacgataactgcacctagggattcacttttctattttgctagcttgccactatatgttgctagacgtcactggtggatcgtgagaactcactaaaatcattttcggatcaacgatctttgctgaggtaagttggaatcgtttcagtccatcgaaaagagtttcgatgatactgtgatggagatcacgatatgtctcactatcaaacagaatagaacctgaggagtcacatacaaaaagagcttaacctgatcaatggcttggattatatttgaattatcaattagattgatagtttgaatattagaaactgctaatttgtaaccgttacagttttgacaactactaattgttagcgcaaggacttaattgcaagtattataatttttttgaggctgattaaattataaattaaattttaattaatttaattcagatttaatttaattagacttaatttaatttaatattaattggattcaattatccaaatcagatttggatttcaagcctgattggatcaggcttgacagccttttcgaatttggctcattttagactcgatttgaatccgtttgaggttctatttggatcagataaaccatgacttagagagctcaagttttttgggactctctttagaaatcatgtcaaaaggagaagtagagcnnnnnnnnnnnnnnnnnnnnnnnnnnnnnnnnnnnnnnnnnnnnnnnnnnnnnnnnnnnnnnnnnnnnnnnnnnnnnnnnnnnnnnnnnnnnnnnnnnnnnnnnnnnnnnnnnnnnnnnnnnnnnnnnnnnnnnnnnnnnnnnnnnnnnnnnnnnnnnnnnnnnnnnnnnnnnnnnnnnnnnnnnnnnnnnnnnnnnnnnnnnnnnnnnnnnnnnnnnnnnnnnnnnnnnnnnnnnnnnnnnnnnnnnnnnnnnnnnnnnnnnnnnnnnnnnnnnnnnnnnnnnnnnnnnnnnnnnnnnnnnnnnnnnnnnnnnnnnnnnnnnnnnnnnnnnnnnnnnnnnnnnnnnnnnnnnnnnnnnnnnnnnnnnnnnnnnnnnnnnnnnnnnnnnnnnnnnnnnnnnnnnnnnnnnnnnnnnnnnnnnnnnnnnnnnnnnnnnnnnnnnnnnnnnnnnnnnnnnnnnnnnnnnnnnnnnnnnnnnnnnnnnnnnnnnnnnnnnnnnnnnnnnnnnnnnnnnnnnnnnnnnnnnnnnnnnnnnnnnnnnnnnnnnnnnnnnnnnnnnnnnnnnnnnnnnnnnnnnnnnnnnnnnnnnnnnnnnnnnnnnnnnnnnnnnnnnnnnnnnnnnnnnnnnnnnnnnnnnnnnnnnnnnnnnnnnnnnnnnnnnnnnnnnnnnnnnnnccccatcgaaaagagtttcgatgatactgtgatggagatcacgatatgtctcactatcaaacagaatagaacctgaggagtcatatacaaaaggagcttaacctgatcaatggcttggattatatttgaattatcaattagattgatagtttgaatattagaaactgctaatttgtaaccgttacagttttgacaactactaattgttagcgcaaggacttaattgcaagtattgtattttttttgaggctgattaaattataaattaaattttaattaatttaattcagatttaatttaattagacttaatttaatttaatattaattaggttcaattatccaaatcagatttggatttcaagcctgattggatcaggcttgacagtcttttcgaatttggctcattttagactcgatttgaatccgtttgaggttctatttggatcagatgaaccatgacttagagagctcaagttttttgggactctctctagaaatcatgtcaaaaggagaagtagagtattatttttttcatccttctttcttcacacgcatgaaaggagagggggcaccaatagttggtgccctgccttatctggatgtctttttcatccaattttttttttaattgaatttgatttaaaatagaatagaaatatcttagattaaggtatagaagtactttttttatgtgataaaaaaaatagagaaagaggacgtgcgctaattattggcgtgagacatctttccttctttcttcccttatctcaacgcacatctatcctttgatttgtttttgaacaccttggattaaaagagatgagatctcttgggcattaagaaggagttgtgcgtgggatttgagatgtggtgcgacaaaaaattaaaagaggatgcatgaagggaggtggcgtgcgttagatgcgagaggcttctttcttacatctttctctcctccccaatgcctcttccttccttctccacttcacgtccatgcccagattcaataaagatcagatctaagaaaagaaaagagagagaaaaagagaagaagaagggttcttcttttcttcatggtgatctggtatagatcctgttggatttgtgcgaaagagtttgagcaacgatctgcttctttaagatctgaaagaaaagatcaagatccatggatgaagagtgagatctgcaaggtgctagcacaccagtgatctcggtgctccgatcaaatggctccgtgtggatatcagctgaggtcgaacgcgtgcatggctacgatcagaatctgcgatatctgcaggatccgagatatggagattcgatctccattttatttttctaacagtttatttttctatttcagatatcagatcgtgggtacatatttgtatcaagatctttactatggttttcagatctgatttgatacgtaaataaattaaaattattttaatttatttattttcactgtgtagatgtctagaaaaaattttaaactacacgtacgaaatcgaagcattttctaacaactctgactatcaccatagacgacgtatatctcttgcttcccaccaaacttctttaataagttctttagccatagcatttctttatcgacctttgttatggtgatgtattcaacctccatcgacgataatgtgacacttttatgactttgattgccacaacaccgctccctctgagaatatcatcagataatctgacgtggatttctgtatgtccacatcatcgatcatgtccgtatctgtgtaagcctgtagcataggatctccactatcatggcataaatatatcctggatatctatttaagatatcttattttccacttcattgctttccggtgctcctttccaaagtttgaaagaaaccgattgaccataccatccacttgagcaatattagacctggtgtacaccatagcatacataagactccccaccacttagtccttctcactctttctgctttgctctttaatcaatgtaaagtgtcctacaagcagacaccaccggcttcactctactcatgttgaatcaatccagcaccttctcaacataggcctcctatgacaaccataggacctggatctcctatctctagcaattcttatccttaatatcattttgacctatcccaagtcttccgtcataaatgttcgatccaactttaccttcaaatcattgattttggtaatgtggcatcccacaatcagcatgtcatcaacatatagcaaaaatttgataaaattattgtcaaaatattttttcatgaacatgcaatggtcagaacttactttcttatatccattctccattatgatggaatcaaacttcttgtactactatcatggtgcctgcttcagttcataaagatttttcttcaagcaacacactatgttctcattaacctttcatttcaaactcttctagttactctatatattctcctcctccaagtcgccatgaaggaatgccatcttcacatcaaattgttccacctcaacatctaaacagccagcgagatcgaggataactcgagtagacgtgagctttacaacgattgagaaaatctcttcaaaatcgatactttttctctgaccaaaatctttcacaactaatctcatcttgtaccttggttataaactattctcctatggcttcaatctgaacatctatttatttttgagtgcttgctttttcttaggtatattcaccaactcatatgtattatttttctataaagaattcatctcctctttcattgccttcatccactcctcactatgctggagctctatggcttcagagtaggactcaagctcttccacatctgttaatagcacataatcctatggtggatatcttatggatggcgtccactctcttgtgaatctctggacctcttatgcaggtggttcaacatgcaactcaatttgaacaccatccgcactctcctcagcctcatgactatcatatgtaccgtcatctgtagttgctctcctgttatcaagacttctcgaagaggtatctgggcataagtctatagggctgctcggggttgacttcggcttcttaggcttcttaaaatcatcgatcgtctgatcctccaaaaaaataatgtcatagttgcacacgatcttccactccatagaatcccacaatcgatagttgaactctccgtcctcactatagctcaggaatatgcactgcttcaccttgacatctagtttggatctctcatctttaggaatatgcacgaatgtcctgcatccaaagattttcaaataatcataagaaatatctttctccaacaatattctctatagtgtatcacacttaagagtataagaaaaaaaaagattaatgctatggatcacagtcatcaatgcctccctccagaatgccttcgatagtttagcataagagcgcatgctcccgatcctctcgcaaatcatcctgttcaccctctcaacaatctcattttgttgtggcatcttaggcactgtcttctctagtctgatgccatttcattgatagtattttttgaaagaacccctgtattcacccctgttgtccgtccaaatatacttcagcttttgcccagtctttctttcaacagagatgtcaaattacttgaatattatcgagcacttgatccttcatttttaaaatatatgtccaaattttttagaagtgatcatcaataaaagtcatgaagtaagaacatccataaaaaattttatcactcagagaacaaacatcactgtgaataagatctaatgcaccaatttttcttttagaaaaaaattctaaaaagaaacttggatttgcttacccatcaagcaactttcatatatcttcaatccaaaactatgaataggaagagcattcttcttagtcaaaattgacattcctttttggcttatatgtcccagtcgtcaatgccataattctaaggtagaagattcttccactacattcacctcccctttaccgagcttggcttgtatgaagtagagaaagccttgcttgatacttttggctactactagcgattttttggttagcttctatttgctgtctccaaatatattgtagtagtcctcctcatctaatacccctatcgataacaagttcagatgaatatctagtacatgtcgaatatttttcaaaaatagcctgtaccccaagctcgtgatcagcataatatctccaatatcaaggatttttaattctccatcattctccatctttattgtcccaaagttactgaaatgacaagatgagaataattttcacctcactgtaacatgatacgaagtggccaaatcgatcacccagatagagtctcaaccaatagtacttgcaagatcatcatttgttgtgccacaagcaacgatcatctctccatccgtagctactgctatcatcttattgttcgagctggagtcatcacttgattattttttgacttctccttttttagtaatcggtagtctttcttaaagtgatcctttttgccgtagttgtaatatctatcacttcgagacttggatctcttccgtaatttagtggggccatcattcaagttagattgggagtccttgtgcttgtttcttccctttctttctatgatgagagcctcatggtggctcgagacaccttgctcctttctcctagcctcctcattaagcatatagtctttcaccattgccaaggctatcgaactatctggtgaagaattgcttagagacaccaccaaagtctcctaactatcgagtaagaaacttaacaatagtaaagcctagagctcctcatctaacagcatcttcatcacagtaagctggttcaccacgttctaaaagttgcttagatgctccaccatataagctccctccttatatttcatatttatcagtttgtgaattaggaacaccttgttctataccatctctcttgtatagactttttagtttcaaccaaaggccatgagcattaacctccattgaaatatggtggaagatgctatcatcaatccactgttggataatcccaacgattttatgattcaatttctcccattctttatttgacatcttatcaaactgaataataacatcctcgattggatcatgaaaatcttagcagtaaaggaggtcttccatgtaaggattccagattgagtagttagttaatgtcagcttgatcgtagtgcccgacgaagattggttctccatctattagcatcttaatttctttttgaatactttagattttgtaaaatttggctctgataccacttattgggatttgagtactaaaagataatagaaaaagcaaaagcaaaaatcacgccaacgataataccaaaggcacaaagaatcatagcaatcgcaagagcactagaattttttatggctcgatcaaagtctatgtctgcacagggatgaaaataaaaagaaacttttactataataatagtttagagtataaaaacttctctgacactacgccgacaatactacttctaatacaagaaagaagaaattcaagattaaacaaacctccagaagaatcctttttgatggaatatgaaagaataatattctacaagtcaatcgcatgagtaatgcaataagatattgttctatattttatcttccaaattcatatatttgatattaattattaataaaattagatattttatttcattatatgctgcattttaatacttgtttaaaattataatgaactccataggttaggacaataattttaaggtcatgatgagatcataccagtgagatttaaatctttgataaccttaatctaaaatattctcaatagtaggatcattaagtcaaaaatcaatgatactgataaaactggtacatcctatatattctcgacagagagggtggttgatgtcataatcacttgtgtggagacactaatacgaagatgtggtgctcattagagaataagttcattgaatttactgatcgagagaatatatgatgcaagtgatcctttgacctaagatcaccatggtgccttgtatatatgaatctatgttttggttcattctttagcttcattttttgagccttgtgtggggtgctccggacatggtgcagtatgtatggaggttgtgagtggtcaacaaaaaatcaatcactccttgtaaaaggagcgaatatcttatgtgatcttataggttgatccaaaaaatctttgaccaaagcagaatgataattagaaagagtttttaatatatcattaactgaatcaatatcttctgatcgagatacatataaataagtatttgaatttgacatgattttatatccataactaatctgaaatattgtatgattgaagaattgaattgtacaattttttaccattgaaaaaaatttttgatattttttttcaaatttaatatctttttgatagtcatgacatgttgctagacatcaatcttgacttgtgggctcacaaaaattaaaaagattttatttgaaagttaattagaaagtattctgattaattgatgtatttggactgacctaatctaattggattgatttaggtcatgagcttgagcccactgctggctagatgatcgctgtcgtaggcagtcaagaataaaaatcaactcaaactatatagatagggtgagtagggatcatttctatggagatctaggatgattatctttttttttaagaaaaaataaaaagagaattgattgtagaagaattaaaagaaatagaatagcaagaattaaattaaaagtatgaattaatttatgaaaaaaaataagtcagagaaataactcagaaattttgaatccaccatgcaaattagatttattttcttcttttttttatgttgcaacattaattcttgtgattaaggtattagtatagcttatctctaagagatacggactgtatcagtagattacaactcgtcctgttgaagtataaactatctaaattcaattacaaaatataagattcaatctaacatactacgatctatctctccaaagcacgtatcgtatctagggatcacgatacgtcaatagagggtataagccgtgtaggctggatcaatacctcaaaaaaaaataaaaagatatgaaataaaagtataattttattacataaaaatttaatataaaaaaaaaccgtttacaggctttatcatatttctggattgaagagatttagccacgcatcaagctctctagctccataatctctcaataattgatccctaaagctctttaatttttttttttattatttttttgttttttctttaatttttttctcttcttatttttgctgccatctgctgcctctgttttctctgctcctgctgcctccttttatagagcacagcttcttcgaattataagcatctatggactttcaattcccactatcttttattttgattgggattttaaaactttatccgcatcccagcatcttgtttcacgcgagatcctagcgtccacatgtgttttgaattccttatgggccacagaccatttaaaccaccaaagaccactttactattttgatttgaatcccatggaagccggctgcctctggtctcattcacccttccagtgcttcacatgggtcccattaatttgaattcctatgagccacatccaagcttttgaatccaagccttccttattttttaaatcaattaaaactttgctttaaatgccttgtagaccctcctatttgcatgctacgtgagaacattgttaagctcctcttggcccacttaagaacttctatgggctacatgcttttggctagctttaaaatggttttgggcctaactttggatcaccattcgaagtccattttgaattcaatttatttttatttttttttttaacctacaaatcgagctcttttattggtgatcatttttcctataaaacaaaaacaaaaagcatcaagtcttaagaaataaaagttaattaatatatattttgatacttttattgggatatttaatgtacttatcactagatatgaaatccaatgggtcacacactttgaaatttgatcttagtctaatctaactaggatttattataaatcttatgggttaaatttacatgctagcacatgaattaactcaagttttcaattggatttagttctaaggtgtttgagctaaccctatcctgataccttaaacctaattagattagatttgaacctatggttttcttgatgccttatgcttattacatgaaagagtttcatgtgacttaaattcctccatgccaccacatcttcatccatgccaaattaatatggaacaccccatttaattgtgcatttaagaaggaatagtccttcttaaacactcctcttaatttcccacactttcctttgttctacacaccatcaaatggcttttggaaatatgcgggcgcagaagtggaggtgtcctatatgaaggctcttccacattataagttatcacatggtgaattaaattattgtgtgagaaaatcatgcgccaagagttggcaccccttgggagttttaggcactccttcttatcctataaataaggggcaccccatatggataaatacaagggaattcaagtttaggcatgagattgagaggagaaaaagacacaaaaatctgaaaaaaagataagaaaaaaaaagagagaaaaatagaaagaaaagacgagagaaaacgaaaggcaagggttgctaatcctagggttcaatttttcaatagttggatttctgaatcaatttggggtggtgagattttttgagaaaaagtttctgatgtggccctagtagaagattgaaggcattcagatgatggtgcaatccgtttttgaaaaagaaaagtgagtagtatacttgtgaagaaagctgcaacactacatcaaattggaaaggaccttgatcaaacccatatggatcaccgttgcaggatatctactttggtatcttgtgaaggttattttttttatcagatcatcatcttcaaaaaggtataattttctacctaatatgcatgcttgatttgtttgattaaaatctataaagtgttcataaggtttgtgttctgattgtattgttttaagtattaaaacttactttaaaaatataaaaaaatttgaaaactatcttctactgtgcaactaaaatccaacagaataaccctaatatgagattgagcgatctccgtcaaccgatgttctctgatcttcttttcttgaatgaagcctcttcaagcctttcttcttctctctctctccctatcttcttttgtggcccacggcctcctcttctttttatgttttgtatttctcatgtcacatccataaactcccttttatagataaaaaattagagtccattttggactccttttccatgcttcccacgccattggttctgtgcacacgactttttccatgctacaaaagtttttcatgtctcacgtagtttccatgcgccataaaattttgcatacttctccaagactttttatgctcgaccctttttggttttcatttaaatcagtgggtcccatatgacgagggatcacaccaacatcatatgctctcctcaccataccaaatggtatccccaacta

SEQ ID NO: 71 - DNA, 61 bp, Artificial Sequence
  synthetic
tttgggtcaagctttaggcttaggtcacatatacccaaaatcatttggatgcatcaggtgt

SEQ ID NO: 72 - DNA, 61 bp, Artificial Sequence
  synthetic
ttggctttgctgcctcaaatcctcgagctatcttatcatcatcgcattgagctccatacct

SEQ ID NO: 73 - DNA, 4061 bp, Artificial Sequence
  synthetic
atcaaatcatatgatccatcttaaatttttaactcaaaaaattaatattgcaaactagctcaaaataattttgatcactacatttctgctgtgcattctaatttaaaccgttcacattttttagattcatgaaataattttgaccaaagtattactccatactatagtcaaaaaagattaaaatattagattctaattaaagccaaagataaacttttgattctcatccttaattttgcctaaagtataattattttgattaacccttaagcgcaataacacattcaaaaccaacagataggtttactataatccaaatgaattaaatcttaattcttttatcaattcatttagacaatttcaaatcaaaattctataagtaatatcaataaaaaaaatttttgatgctccaataagttagaacttaaatcaaaatatataagtaaaattgatttaatcatctcttctaaagtttcttctattaagatctttaatatctatcaaatacattccacaataatcatgcaaaccttttaaaaattaaattctcaatgcctttactacattttaacaccaagctcgataatagtgataaagaaacatctagatcagctttataatcaaaaattttgacttacaattttacgtgtgtctcaaaatcttgaataaatataaataagatcttttatcttgatccaaaaatagtaatcaaggatttcattagtaacttcaacaacaatggtaaaaaaattttctatccattgataaacccaaattttgaattgaagtttcatgcataccatatagcctttaataagatctattatttggatctaaagatagtaattaaaattgttaatgattccactaagatgaatactttacaatctcataattaatttcttcaataaaaatagacttcttgataatgtctccaattgtatatttttttttatttctacaagaaaacttcatacattttttacgttccaatataaatcttaaaaagttattccaatcaaatatcataaaagatcttcttagtccaaccttaaataacttttatgaatgaatctttatcttgccactaaataatgaattttaaaatcaagagcaacatcacagcattctgtcatgtcaaatttgtgttagatgtatgtcctagaaatcaattagattgacaatgtaaattttttaaggatataatttatatattttgatttattaataaaataaaatttaaattaatttttattcatatttttttatctatgaatcatctaaagaattaataagatgatgatacatattcttaagagttcaaaatttgaaatatatgtcattgatgattaatttctgaatacttttgaattcttaagagtttagaagatcttgacccaagtagtgtgaatagtgaaaaaaagttttcacatacttcacatcaaaaatttaagttgaataaattgtacatatgacaggtattatagtttgacgagtaatctataacctctatcttatcaaaattctgatagaaagattgtattgtatgataactgtacttagaggttcaccttttattttactggattaccactacatgttgctagatgtcactggtggattgtgagatctacgaagattatcttgatgatcgataattctcattgaaaagattgaaactattttaatgatgttgtgatagagatcataatatatcttattatcagacagaatagaattctatgggatcatacacaataggagattaagactgatcaaatagttgaatgatgattaagaatcattacggagttcagattatcaatataattgataattagactaacttataattgttacaagtagcaaggacttaactgctaaaggttaataggttcaaaaagaacttatgtataaatgttgtgcatcttaatttgattggatcaaattagttatggctgaattcaagatgaatcaaataggaatttggttcaattgaatttgggtcaagctttaggcttaggtcacatatacccaaaatcatttggatgcatcaggtgtgtgacacctgaatcaggcctttctaaactattttgagtaagtttgatcaagtcaaaaggatccacaccctaaggtttcttgaataaaaccttaggcaccacattgaggacctataggaaactttgaccctctctcatatggggtggcacactgaggttttataaaaaccttaggcacccattttagccataaaaaaaaagctccaagggatggggcagtagccatgaagaatccttggctgtcaggactctattcaaaagagttctcaaggttttggactcttatggagccctaggatttgtttgcctataaatagatggccaccccaaggctttagataatgttagagacttgtgaagctctcccctttctcttggttgccggcccaccctctctcctctctcttccatgccccaagacttctttcttgtctccatcatcttgctgaaatttagatttcagcaagaaaagtcaagtagaagtcaaagttctaatgtagctcacaagatgttgagaacttcctccatctggcaaaggttctgcaagagagctagcatcctgagaaacaaaaagattgctgatcagccctcatctccatatggatatttgtagagatcaaatgcatgcatagctagaagagaatcttatcacgatcatcactcgtgaagatcatctacctgtgcaaaggtatgagataagaaaaatattttttttatcataattcatgaatcctttgcttatattatactgagattcttggaatggattttttctctagtaaaactctagagatcagatctcaaagtcttcttcacataaaggttttgaaagttctttatatttccgctgctttgattcaaaataaattagatctattttgcctttcaacctttctcatatttattgacatataaagctttaattaatgagattaatgaaaagcatgtgcgaaatactgagaaaatcctaacagtgatatcagagctacttttgtacataagaaaaggattcaagttaaataaaatatgtttgatttaagtaaatgaatcaatcaaaatttatcctaacataagtttgtcctggtataatggtcaagaccattatgttgaaaggttatcctaggacaaaaagtctaagtaaaatctattttatttaagtaaatgaatcaattaaagtttattctaatataagattgccttagcataatggtgaagacccttatgttgaaaggttgtcctaggatggaaagtgattgatgagacaaatatatcatgaaagtatttttcacagatggaataaaatatatatattttgtttgtgaaaatgagatttcatgaatgtgtttgtcattcaatatgtgtggtgatcatcttgaattgccacaaatcctttttggattagggttgtatcatgactcacaaatcctgatggtttgcaaaattttgcattctgtagtgatagaaaccaaaagttaatccaattttggaataagattgatcaattggtatctaaggcaagtattttataatggtggttacttaattagttataaaagtacgaagagtctcctaccaatcttacacttatctagccaatttggttgattgaattctgaatttgggttgcttaagtgttaagttcactacaaatatattgcaaccatgattccgacttagtcaaccaagcctagatctcttgaatagattcatgttaattatggatttacataggatataaataaataattaaaacttgaagagatctaaatgaaaccttctcgtacatattaaatcgaatgatcttccatcattgtagatatacggatactctactgatgttgatgattttcgactagatatagtactttggttgcatcgaaaaagtacaaccactttataacatgagatgttgcagggtagagatggggttgggcccaataattgttaggtgaggatccaaatgatggctgcacttgcgtgtgaatggcgagtctgacttaa

SEQ ID NO: 74 - DNA, 4061 bp, Artificial Sequence
  synthetic
  misc_feature (990)..(1717): n is a, c, g, or t
tataactgaaagatagctaatgcttagctggatgactgctgttagataactgtctgcattcttacggtacattgatattttaccaatgtgacatagcttaaatcggcaactggctgaactaaatattatgtatccctttagttaacaatcatgtcggttagagatcaatgtaattcgcagcagatcgatcataagctgagatgagtatcatattttaagaacaacgctgggcgagttaggccgatcaaatgtcagactgaaaaagcagatcaataaacctctgatgtgatctgaaagaatatttatgatttaaataataatctatcaccacgtatccagataatgaggtcatataacatgtaccaacagtgcatttttccatctagttaagaggttggttagtggcatttgtcttcgatatgtaatgttcacataactaatgtgcttagtagcattcttttgtaaggttaaatcttcaatgatcttaagttcacataattgcctttgtgccctattagtttatagttgaccttttaattcaagagacagtcaccttagcaatcgatgtctgcttagattgggccaattaggtactcacattaatatattgaatcatgtttgaatataaaggattagattgatttataagtttccttttattgtttacatactgatacttagattgacttactacattatttgatatgttatgttctaatttttggattaaaattgttgtttctgatttctccttacatctaatactttgtataatttattattttttagcatgattgagtgtagaggattagattgatttttaagtttattttgattatttacatgcccatacttaaattgacttactacattattcaatatgttatgtttcaattattgagttaaaatttttatttctgatttctactgatgtccagtgtgtgtgtgtgtacgtatgtgtgtatatatttatttacatatatatgtatnnnnnnnnnnnnnnnnnnnnnnnnnnnnnnnnnnnnnnnnnnnnnnnnnnnnnnnnnnnnnnnnnnnnnnnnnnnnnnnnnnnnnnnnnnnnnnnnnnnnnnnnnnnnnnnnnnnnnnnnnnnnnnnnnnnnnnnnnnnnnnnnnnnnnnnnnnnnnnnnnnnnnnnnnnnnnnnnnnnnnnnnnnnnnnnnnnnnnnnnnnnnnnnnnnnnnnnnnnnnnnnnnnnnnnnnnnnnnnnnnnnnnnnnnnnnnnnnnnnnnnnnnnnnnnnnnnnnnnnnnnnnnnnnnnnnnnnnnnnnnnnnnnnnnnnnnnnnnnnnnnnnnnnnnnnnnnnnnnnnnnnnnnnnnnnnnnnnnnnnnnnnnnnnnnnnnnnnnnnnnnnnnnnnnnnnnnnnnnnnnnnnnnnnnnnnnnnnnnnnnnnnnnnnnnnnnnnnnnnnnnnnnnnnnnnnnnnnnnnnnnnnnnnnnnnnnnnnnnnnnnnnnnnnnnnnnnnnnnnnnnnnnnnnnnnnnnnnnnnnnnnnnnnnnnnnnnnnnnnnnnnnnnnnnnnnnnnnnnnnnnnnnnnnnnnnnnnnnnnnnnnnnnnnnnnnnnnnnnnnnnnnnnnnnnnnnnnnnnnnnnnnnnnnnnnnnnnnnnnnnnnnnnnnnnnnnnnnnnnnnnnnnnnnnnnnnnnnnnnnnnnnnnnnnnnnnnnnnnnnnnnnnnnnnnnnnnnnnnnnnnnnnnnnatgtatacatatacatgtatacatacatatatagatatatatatatacatatatgtatatatatatatatatatacacatatataggttatttggaacctaagaaacttgcaaagttactagatgcaatgttcggaaaccatggaccgtaacaactggagtagtatttgggtcatgaattcatggctagatcatgaattgagtgggagtcaaccgaagtagggccagctcagacacttgtatttaggtcccatgcttgcgtgcattctcttccctgatatcctttggctttgctgcctcaaatcctcgagctatcttatcatcatcgcattgagctccataccttgctctttcctaactgcccccatcaaacctccggagatcctctttcttctccaatgttgagatttgttggagtcttcccaccttctcacttcaatgggtggcaatttcaagtgccagttcccttatttgtcccagctatattgacaatggggcttattctagggtttctcatggacatagtgataataataatcaagggaccaagagagaaaaatctttctagtctgtgttctttaagtttgagagataggcagcacatttttttaataagcctttttcactcatcggatcctgattttcagttgttcgacctgaacagttcaagcaattgaactgcttgggtcactattttggacgattttcagccatttttaagtattgtttgactggatccacgctgcgtagtgggcattgcgttgatcaagtagacctgtaagggtcaacaaggtctgagaacactgaatggatgctccataatcctcttgttatctgtcaaccatttggaatcttttaaaacaacatgtggtgataatatatatgataaactgtgatagattcatgtatagattatacatatgaaaatgtagagtgcttagtaaaagtgatgaagagcaatgcgttagaatgtgctagcctttgacctaaaaattggaatgcccaatgatgagttatgataaaattgtgacgtgatttatgaagtctaatgtttagttggcttgcagtttcagatgcgataaagaattttatgatttagctctttggttttttaacatgcaaacatttaattgtactgaaaaacatttatttcgaaacatgtaggagactattggatattgaaattaaaattgactttttggtgtttcacaatatttcttaataaacactacgactatgtaaataggtggtggatcaaagggaaagaaatgtttggtgattatttttagaaaagacaagaagtatttgataaatggttatttttcaaccgattaatgagagaatgactatgaacctatgaggtgcacctcttatgatgttgcatggatgaagcatctaatccatgggtacaatttactaaaatataggcccaattctgagacaggaacatttacaactcatgtacaaagaagaaacttaaagtatcatggatgccgggatatttccttcttcaaatctttcaaaagctgtagttttcattataaggaaaaatgattataactaacatcttctataggtgatgagtggacactagaaggctttcctataataacagtagagagagtagaaaagcctgtcagcatgcggtccataagtatatatacatattttcagcgcttaaagtaaattttcttgtaccaaaaaaagataaattttcaaaataaaaactaaaatcaactgaaatgtttgaaatctgattcgtaggtacatggagaagagtgtaagacagcaaatatcataaaggcagaataagagctggtaatcttgtaacctggcgcaactatgttatgcatgtctatatgtgtgcatgtttatgtataacaagtaatatttcttttcttatttactcacttcagttaggaagtcaatccaatctccctttgcttgggtgtgttcagattatcaagggccataacagtagtgctggtaagcacctgtttaatggataaatggcgacaaattctctccccttctgctcactctattatcataccttccgtcttacccatctgctatatcttataaggaacataaggatcgacatagcttcatgctatcacattacaagctaagatcggaataatacctaatcttttcgatctactattaggtattactatagggttgtaaattgggtttaggttttgaactatattatattttggtgtaagaatatagtgccacactatcttgaaccagactagctgttgcactttttttgcaggcatcaatattttgttcatccaaaaaaaaatattgcacatgcacagatgaagtatgagggc

SEQ ID NO: 75 - DNA, 680 bp, Artificial Sequence
  synthetic
atggggagggggaagatagagatcaagaagatagagaatcctacaaacaggcaggtgacctactccaagaggaggacggggatcatgaagaaggctaaggaactgacggtgctttgcgatgctgaggtctcgcttatcatgttctccagcaccggcaagttctccgagtattgcagccccctttccgacaccaagaccatatttgatcgctaccagcaggtgtcagggatcaacctgtggagcgcccaatacgagaaaatgcaaaacactttgaaccatctgagggagatcaaccagaacctccgcagagaaataaggcagcggatgggtgaagatctcgacagtttgggcatccatgaactgcgcggtcttgagcaaaatttagatgaggctttgaaggttgttcgtcacagaaaataccatgtgatcaccacgcagacggatacctacaagaaaaaggcaaggctaacatgctttcttaccatcattctttacggtctttgatccggttttgcgtgtccacttcttacgtagtctttttcaaacattcctatctaagactgaaggtaatgatttgcaaaggaatagctttactgttttcctctaagtagatgaaatattactcacgtagaaaggagccatcataattgcagaaagaataaaactgaatggaatatgag

SEQ ID NO: 76 - protein, 167 aa, Artificial Sequence
  synthetic predicted sequence of tDEF1
MGRGKIEIKKIENPTNRQVTYSKRRTGIMKKAKELTVLCDAEVSLIMFSSTGKFSEYCSPLSDTKTIFDRYQQVSGINLWSAQYEKMQNTLNHLREINQNLRREIRQRMGEDLDSLGIHELRGLEQNLDEALKVVRHRKYHVITTQTDTYKKKARLTCFLTIILYGL

SEQ ID NO: 77 - DNA, 1850 bp, Elaeis guineensis
aaatcagctaatgtagaccatctgaactacttgttcatcacccttatcccaaaaaaaaattggtgtgtattcagttagagacttcaggccaataagcctgattaatggagtaataaaaaatatttcaaaaactctatcgaaaaggctctcacagaaaatgaatttgttaattttatccacagagcttgctttcaacaaaggaagaaatatctctgaatattttgtaatgactatggaaactatacacttctgcaaagctgaagtacacaaggatctcaattataaagtcgacttcgagaaagcttttgacaatgtggattggagctttctattgaaattgctatccagcacggggctttgattcgaggtggtgtcaatggatagaatatctgatttatacagctaaattctcagtccttattaatggtgataaaggtaaactttttaaattgaggaaagatctcaggcaaggagatcctctattcgcctagctctttctcttagttgttgatatagaatgatcaagggagcaagtaggttcaatctttttgttggaattggatcatataatatcatgggataacttcaaagcttttagttcactgatgacacacttatattttgcagatatgatctaaaatacatcaaaactcttaaatttttactctatagttatgagctactgatgggtctcaaaattaactttgaaaaattccaattttttggcttgagaattgcaaagatgtcagtacagcaagttgcatctatcctagaaagcaaggtggctacattttccattacttatttgggtctcccactccatcattctaaactgaggaaaacttattggaatccactccttgagaaggttcagaagaaattgatcgggtagaaaggtaaacttcttaacctctagggtaggcttatactaactaatgcagtgcttacagggatcccactactctggagggatacattccttctccctcaattcattatcaaataaattgataaaatccatcgatcattcatttggagaggaaacgaggagtataactaagggcactctagaatatgttggtcgaatatttgtcgatcaaaaaaatttggaggactgggggttcctcaatctaaaaattttcaatacaattcttctttgtaaatggtggtggaagctctactctaatgctggtgacccgtggtgtagttttattgccactatccacccaacttcacactagagatctaaaggtatacacaaatcaacctcttcattttggaatggtttacagcacacatgaaatatttctactcctaatccactttcaagttagcaactagtattattttggaaagatagttggttacataatcatccactgaaggatcgatttcctcacctttacacaatagcattgaagtgcaacaactcagtggcaaaggtattaagcaatctacttgataatagctcttttagtactcctcttcctcaaagataccaagaagattttcagagtctataggaaagcattgaacaaattacattaacggaacgacctgatactatacaatggaaatggtttagtagcaatatttttttggcatgaaggatctactattttctgcaagatggaggagtttggcctctactgagtaatattatataaaaactcctaataccaaagaaagccaagttatttgcttggctaagtgctcacaacaaaatcccaatgaaagctaatcttcttaatagaggaataattggaactgattactgtacactttgcgatgacttatcagaaactaatgatcatctaatgctcatctatactttttcaaaagcaatttgg

SEQ ID NO: 78 - DNA, 498 bp, Artificial Sequence
  synthetic
atggggagggggaagatagagatcaagaagatagagaatcctaccaacaggcaggtgacctactccaagaggaggacggggatcatgaagaaggctaaggagctgacggtgctttgcgatgctgaggtctcgcttatcatgttctccagcaccggcaagttctccgagtattgcagccccctttccgacaccaagaccatatttgatcgctaccagcaggtgtcagggatcaacctgtggagcgcccaatacgagaaaatgcaaaacactttgaaccatctgagggagatcaaccagaacctccgcagagaaataaggcagcggatgggtgaagatctcgacagtttgggcatccatgaactgcgcggtcttgagcaaaatttagatgaggctttgaaggttgttcgtcacagaaaataccatgtgatcaccacgcagacggatacctacaagaaaaagatgcatctcaagtcagcactagaccatcttctaaaatag

SEQ ID NO: 79 - protein, 165 aa, Artificial Sequence
  synthetic
MGRGKIEIKKIENPTNRQVTYSKRRTGIMKKAKELTVLCDAEVSLIMFSSTGKFSEYCSPLSDTKTIFDRYQQVSGINLWSAQYEKMQNTLNHLREINQNLRREIRQRMGEDLDSLGIHELRGLEQNLDEALKVVRHRKYHVITTQTDTYKKKMHLKSALDHLLK

SEQ ID NO: 80 - DNA, 459 bp, Artificial Sequence
  synthetic
atggggagggggaagatagagatcaagaagatagagaatcctacaaacaggcaggtgacctactccaagaggaggacggggatcatgaagaaggctaaggaactgacggtgctttgcgatgctgaggtctcgcttatcatgttctccagcaccggcaagttctccgagtattgcagccccctttccgacaccaagaccatatttgatcgctaccagcaggtgtcagggatcaacctgtggagcgcccaatacgagaaaatgcaaaacactttgaaccatctgagggagatcaaccagaacctccgcagagaaataaggcagcggatgggtgaagatctcgacagtttgggcatccatgaactgcgcggtcttgagcaaaatttagatgaggctttgaaggttgttcgtcacagaaaataccatgtgatcaccacgcagacggatacctacaagaaaaag

SEQ ID NO: 81 - protein, 153 aa, Artificial Sequence
  synthetic
MGRGKIEIKKIENPTNRQVTYSKRRTGIMKKAKELTVLCDAEVSLIMFSSTGKFSEYCSPLSDTKTIFDRYQQVSGINLWSAQYEKMQNTLNHLREINQNLRREIRQRMGEDLDSLGIHELRGLEQNLDEALKVVRHRKYHVITTQTDTYKKK

SEQ ID NO: 82 - DNA, 21 bp, Artificial Sequence
  synthetic
tgatatgaagggtttcaaggt

SEQ ID NO: 83 - DNA, 25 bp, Artificial Sequence
  synthetic
tcctattttagaagatggtctagtg

SEQ ID NO: 84 - DNA, 576 bp, Artificial Sequence
  synthetic
tgatatgaagggtttcaaggtggtttgcctcgttcaaatcaaaggattttgaagattaatattccaagataaggttctccaactccattaggaaagtgtcttcatgtcatcttagagaagcagctcgtaccaaacttgacagatgttttatttatttagagtgacacagataccctttggcaatactctccatccttgtccgaacaacttctaatcacacctcacttatcttgcatctaactcagaggctacaagttacacctttcaacaaaccttttcggtttgaaaatttgtgatttcattatttagagttcgaagagcatatcaagtattggtcggagttggcacccaaagcaaacgaaacagttactgacatggtccaaaagctgagatttctaagatcccaacttaagcactgaataaagccattatgggaaatatcattttaacgaaagaggaatttagagtaagaattgattctcttgataccgaagaagaactaatacagctttcatcacttcaaaatgatgaacagatgcatctcaagtcagcactagaccatcttctaaaatagga

SEQ ID NO: 85 - DNA, 22 bp, Artificial Sequence
  synthetic
agaattgattctcttgataccg

SEQ ID NO: 86 - DNA, 24 bp, Artificial Sequence
  synthetic
ttttattactccattaatcaggct

SEQ ID NO: 87 - DNA, 633 bp, Artificial Sequence
  synthetic
agaattgattctcttgataccgaagaagaactaatacagctttcatcacttcaaaatgatgaacagatgcatctcaagtcagcactagaccatcttctaaaataggaagatctatggaagcaacactcccaaatgcagtggcttcaaaatggggattgcaatacgaagtttatccatgtttgggcaagtaacaggaaaaaaagaatactatcactgaactctagcaaggcgatcagaagattatcgaatagcagcaaatccaatccacattctacaactttttttctaccctactaggctcgactgaggaatgactcatccaagctgattggaagattctttatccagaaggacctctggatcttgctgacattgagtatccatttatggagaaagaaatccatgatacagtgtatgacttggctttggaaaagtcacccggatgatattttcccattctccttctataagcacttctagtgtatcatcaaacatgacctgatgaacctactgtaaaatcagctaatgtagaccatctgaactacttgttcatcacccttatcccaaaaaaaaattggtgtgtattcagttagagacttcaggccaataagcctgattaatggagtaataaaa

SEQ ID NO: 88 - DNA, 20 bp, Artificial Sequence
  synthetic
gcaaggagatcctctattcg

SEQ ID NO: 89 - DNA, 20 bp, Artificial Sequence
  synthetic
gatcgacaaatattcgacca

SEQ ID NO: 90 - DNA, 632 bp, Artificial Sequence
  synthetic
gcaaggagatcctctattcgcctagctctttctcttagttgttgatatagaatgatcaagggagcaagtaggttcaatctttttgttggaattggatcatataatatcatgggataacttcaaagcttttagttcactgatgacacacttatattttgcagatatgatctaaaatacatcaaaactcttaaatttttactctatagttatgagctactgatgggtctcaaaattaactttgaaaaattccaattttttggcttgagaattgcaaagatgtcagtacagcaagttgcatctatcctagaaagcaaggtggctacattttccattacttatttgggtctcccactccatcattctaaactgaggaaaacttattggaatccactccttgagaaggttcagaagaaattgatcgggtagaaaggtaaacttcttaacctctagggtaggcttatactaactaatgcagtgcttacagggatcccactactctggagggatacattccttctccctcaattcattatcaaataaattgataaaatccatcgatcattcatttggagaggaaacgaggagtataactaagggcactctagaatatgttggtcgaatatttgtcgatc

SEQ ID NO: 91 - DNA, 24 bp, Elaeis guineensis
ctctagcaaggcgatcagaagatt

SEQ ID NO: 92 - DNA, 24 bp, Elaeis guineensis
tcaggtgttatgtcagtttggact

SEQ ID NO: 93 - DNA, 24 bp, Elaeis guineensis
aagtctccactctatctatcccga

SEQ ID NO: 94 - DNA, 24 bp, Elaeis guineensis
gggtcaacaaggtctgagaacact

SEQ ID NO: 95 - DNA, 24 bp, Elaeis guineensis
cgcaatcagaatcaactggccaat

SEQ ID NO: 96 - DNA, 24 bp, Elaeis guineensis
atgatacacggttgcatgccctgc

SEQ ID NO: 97 - DNA, 24 bp, Elaeis guineensis
gatctatggtgcaaggagttaatt

SEQ ID NO: 98 - DNA, 24 bp, Elaeis guineensis
agagagagggttaaaggacaatgc

SEQ ID NO: 99 - DNA, 24 bp, Elaeis guineensis
atagggagaatagcttggcttcga

SEQ ID NO: 100 - DNA, 24 bp, Elaeis guineensis
tcgggttcttttattcgtggattt

SEQ ID NO: 101 - DNA, 24 bp, Elaeis guineensis
aggggagattgttggcttagcttg

SEQ ID NO: 102 - DNA, 24 bp, Elaeis guineensis
agtagactcgatgatgataagact

SEQ ID NO: 103 - DNA, 24 bp, Elaeis guineensis
accagcacggtcaaggataggcat

SEQ ID NO: 104 - DNA, 24 bp, Elaeis guineensis
atagtagactcgatgatgataaga

SEQ ID NO: 105 - DNA, 24 bp, Elaeis guineensis
cctccaacatcggccaagttagtt

SEQ ID NO: 106 - DNA, 24 bp, Elaeis guineensis
aaatcctacttgtttctctgacct

SEQ ID NO: 107 - DNA, 24 bp, Elaeis guineensis
catgaggcatgcaaggtattgaat

SEQ ID NO: 108 - DNA, 24 bp, Elaeis guineensis
aaggctggctaactcaaagaagag

SEQ ID NO: 109 - DNA, 24 bp, Elaeis guineensis
aatgatcgagaagggctggagaca

SEQ ID NO: 110 - DNA, 24 bp, Elaeis guineensis
tgacccaccatcgagaaggaccga

SEQ ID NO: 111 - DNA, 24 bp, Elaeis guineensis
ataactgacaagtggcattgatct

SEQ ID NO: 112 - DNA, 24 bp, Elaeis guineensis
agaaggatgagaagagagattgtc

SEQ ID NO: 113 - DNA, 24 bp, Elaeis guineensis
aaagatgttagctcctgttcgaga

SEQ ID NO: 114 - DNA, 24 bp, Elaeis guineensis
aaaggctggctaactcaaagaaga

SEQ ID NO: 115 - DNA, 24 bp, Elaeis guineensis
agagattgtgaacaaatggagaga

SEQ ID NO: 116 - DNA, 24 bp, Elaeis guineensis
atattgtctgctcttcaccaaaga

SEQ ID NO: 117 - DNA, 24 bp, Elaeis guineensis
ctcgtaaggcccaagggtagtcat

SEQ ID NO: 118 - DNA, 24 bp, Elaeis guineensis
aaaatagcttgacccaccatcgag

SEQ ID NO: 119 - DNA, 24 bp, Elaeis guineensis
atagaatagggagaatagcttggc

SEQ ID NO: 120 - DNA, 24 bp, Elaeis guineensis
tcctgtccagatatttgcgcctct

SEQ ID NO: 121 - DNA, 24 bp, Elaeis guineensis
acaactagccaatgatcgagaagg

SEQ ID NO: 122 - DNA, 24 bp, Elaeis guineensis
aacacactgctgaaaaggactagg

SEQ ID NO: 123 - DNA, 24 bp, Elaeis guineensis
aaactcatggtgtcaagggacgtg

SEQ ID NO: 124 - DNA, 24 bp, Elaeis guineensis
gctacacaggcacaatctcgattt

SEQ ID NO: 125 - DNA, 19 bp, Artificial Sequence
  synthetic
ctttccgacaccaagacca

SEQ ID NO: 126 - DNA, 24 bp, Artificial Sequence
  synthetic
caagtagcggatagagaggcttac

SEQ ID NO: 127 - DNA, 23 bp, Artificial Sequence
  synthetic
gttcgtcacagaaaataccatgt

SEQ ID NO: 128 - DNA, 21 bp, Artificial Sequence
  synthetic
tcttctgatcgccttgctaga

SEQ ID NO: 129 - DNA, 21 bp, Artificial Sequence
  synthetic
accggatcaaagaccgtaaag

SEQ ID NO: 130 - DNA, 24 bp, Elaeis guineensis
aaattcttacttctgagcatactt

SEQ ID NO: 131 - DNA, 24 bp, Elaeis guineensis
cgaggtggtgtcaatggatagaat

SEQ ID NO: 132 - DNA, 24 bp, Elaeis guineensis
ctctttgttatacaatcacggtgt

SEQ ID NO: 133 - DNA, 24 bp, Elaeis guineensis
caaggcgatcagaagattatcgaa

SEQ ID NO: 134 - DNA, 24 bp, Elaeis guineensis
gtgccatatgtcatagtcaactgt

SEQ ID NO: 135 - DNA, 24 bp, Elaeis guineensis
aatctgatattggcatccacatga

SEQ ID NO: 136 - DNA, 24 bp, Elaeis guineensis
cctgactttcggttggctgtctct

SEQ ID NO: 137 - DNA, 24 bp, Elaeis guineensis
aatcctacttgtttctctgacctt

SEQ ID NO: 138 - DNA, 24 bp, Elaeis guineensis
ctctagcaaggcgatcagaagatt

SEQ ID NO: 139 - DNA, 24 bp, Elaeis guineensis
aaatggcatactctggcaattcga

SEQ ID NO: 140 - DNA, 24 bp, Elaeis guineensis
tctatctcatccctctcaaccaat

SEQ ID NO: 141 - DNA, 24 bp, Elaeis guineensis
gtagcccatgtctttgttttccct

SEQ ID NO: 142 - DNA, 24 bp, Elaeis guineensis
tgtggatggctaacgatatggact

SEQ ID NO: 143 - DNA, 24 bp, Elaeis guineensis
actagcaccatgtgtcgttatggg

SEQ ID NO: 144 - DNA, 24 bp, Elaeis guineensis
ttcagtcagagacttcaggccaat

SEQ ID NO: 145 - DNA, 24 bp, Elaeis guineensis
aggctctcacagaaaatgaatttg

SEQ ID NO: 146 - DNA, 24 bp, Elaeis guineensis
ttatacagctaaattctcagtcct

SEQ ID NO: 147 - DNA, 24 bp, Elaeis guineensis
tatacagctaaattctcagtcctt

SEQ ID NO: 148 - DNA, 24 bp, Elaeis guineensis
acagctaaattctcagtccttatt

SEQ ID NO: 149 - DNA, 24 bp, Elaeis guineensis
gctaaattctcagtccttattaat

SEQ ID NO: 150 - DNA, 24 bp, Elaeis guineensis
cattctaaactgaggaaaacttat

SEQ ID NO: 151 - DNA, 24 bp, Elaeis guineensis
aggttcagaagaaattgatcgggt

SEQ ID NO: 152 - DNA, 24 bp, Elaeis guineensis
attgatcgggtagaaaggtaaact

SEQ ID NO: 153 - DNA, 24 bp, Elaeis guineensis
tgcagtgcttacagggatcccact

SEQ ID NO: 154 - DNA, 24 bp, Elaeis guineensis
acgaggagtataactaagggcact

SEQ ID NO: 155 - DNA, 24 bp, Elaeis guineensis
aagggcactctagaatatgttggt

SEQ ID NO: 156 - DNA, 24 bp, Elaeis guineensis
aagggcactttagaatatgttggt

SEQ ID NO: 157 - DNA, 24 bp, Elaeis guineensis
tggtttacagcacacatgaaatat

SEQ ID NO: 158 - DNA, 24 bp, Elaeis guineensis
ggcatgaaggatctactattttct

SEQ ID NO: 159 - DNA, 24 bp, Elaeis guineensis
ggcatgaaggatctactattttct

SEQ ID NO: 160 - DNA, 24 bp, Elaeis guineensis
acttttatgcatgcttaacaccct

SEQ ID NO: 161 - DNA, 24 bp, Elaeis guineensis
atgcatgcttaacaccctatggga